European Patent Specification EP 3 870 297 B1, published August 30, 2023. Title: Oncolytic Virotherapy and Immunotherapy. Applicant: Baylor College of Medicine (All states) Clegg , Richard I (LS only). The sequence listing filed with the application follows.

SEQUENCE LISTING (131 sequences)

SEQ ID NO: 1 - protein, 446 aa, Artificial Sequence
  HER2(C5)-CD28TM,ICD-CD3Z CAR
QVQLQESGPGLVKPSETLSLTCTVSGGSISSSSYYWGWIRQPPGKGLEWIGSIYYSGSTYYNPSLKSRVTISVDTSKNQFSLKLSSVTAADTAVYYCARYAPDSSGYLVAFDIWGQGTMVTVSSGGGGSGGGGSGGGGSQTVVTQEPSFSVSPGGTVTLTCGLSSGSVSTGYYPSWYQQTPGQAPRTLIYSTNSRSSGVPDRFSGSILGNKAALTITGAQADDESDYYCVLYMGSGISVFGGGTKLTVLGSEPKSCDKTHTCPTRFWVLVVVGGVLACYSLLVTVAFIIFWVRSKRSRLLHSDYMNMTPRRPGPTRKHYQPYAPPRDFAAYRSRVKFSRSADAPAYQQGQNQLYNELNLGRREEYDVLDKRRGRDPEMGGKPQRRKNPQEGLYNELQKDKMAEAYSEIGMKGERRRGKGHDGLYQGLSTATKDTYDALHMQALPPR

SEQ ID NO: 2 - protein, 444 aa, Artificial Sequence
  HER2(E4)-CD28TM,ICD-CD3Z CAR
QVQLQQWGAGLLKPSETLSLTCAVYGGSFSGYYWSWIRQPPGKGLEWIGEINHSGSTNYNPSLKSRVTISVDTSKNQFSLKLSSVTTADTAVYYCARMGINSGGYLYGMDVWGQGTTVTVSSGGGGSGGGGSGGGGSQTVVTQEPSFSVSPGGTVTLTCGLSSGSVSTSYYPSWYQQIPGQAPRTLIYTTNIRSSGVPDRFGGSILGNKAALTITGAQAEDESDYYCMLYMGSGIWVFGGGTKLTVLGSEPKSCDKTHTCPTRFWVLVVVGGVLACYSLLVTVAFIIFWVRSKRSRLLHSDYMNMTPRRPGPTRKHYQPYAPPRDFAAYRSRVKFSRSADAPAYQQGQNQLYNELNLGRREEYDVLDKRRGRDPEMGGKPQRRKNPQEGLYNELQKDKMAEAYSEIGMKGERRRGKGHDGLYQGLSTATKDTYDALHMQALPPR

SEQ ID NO: 3 - protein, 445 aa, Artificial Sequence
  HER2(F1)-CD28TM,ICD-CD3Z CAR
QVQLVESGPGLVKPSGTLSLTCAVSGGSISSSNWWSWVRQPPGKGLEWIGEIYHSGSTNYNPSLKSRVTISVDTSKNQFSLKLSSVTAADTAVYYCARMGANSGGYLYGMDVWGQGTTVTVSSGGGGSGGGGSGGGGSQTVVTQEPSFSVSPGGTVTLTCGLSSGSVSTSYYPSWYQQTPGQAPRTLIYSTNTRSSGVPDRFSGSILGNKAALTITGAQADDESDYYCVLYMGSGIWVFGGGTKLTVLGSEPKSCDKTHTCPTRFWVLVVVGGVLACYSLLVTVAFIIFWVRSKRSRLLHSDYMNMTPRRPGPTRKHYQPYAPPRDFAAYRSRVKFSRSADAPAYQQGQNQLYNELNLGRREEYDVLDKRRGRDPEMGGKPQRRKNPQEGLYNELQKDKMAEAYSEIGMKGERRRGKGHDGLYQGLSTATKDTYDALHMQALPPR

SEQ ID NO: 4 - protein, 439 aa, Artificial Sequence
  HER2(A3)-CD28TM,ICD-CD3Z CAR
QLVQSGTEVKKPGASVRVSCKSSGYTFTSYYIHWVRQAPGQGLEWMAIINPGNGDTNYAQRFQGRVTMTRDTSTSTVYMELRSLRSDDTAVYFCAREIASYSGSYYDYWGQGTLVTVSSGGGGSGGGGSGGGGSQAVVLQEPSLSVSPGGTVTLTCGLSSGSVSTGHYASWYQQTPGQAPRTLFYNTNTRSSGVPDRFSGSIVGNKAALTITGAQADDESDYYCVLYVGDGIWVFGGGTKLTVLEPKSCDKTHTCPTRFWVLVVVGGVLACYSLLVTVAFIIFWVRSKRSRLLHSDYMNMTPRRPGPTRKHYQPYAPPRDFAAYRSRVKFSRSADAPAYQQGQNQLYNELNLGRREEYDVLDKRRGRDPEMGGKPQRRKNPQEGLYNELQKDKMAEAYSEIGMKGERRRGKGHDGLYQGLSTATKDTYDALHMQALPPR

SEQ ID NO: 5 - protein, 27 aa, Artificial Sequence
  CD28 TMD
FWVLVVVGGVLACYSLLVTVAFIIFWV

SEQ ID NO: 6 - protein, 41 aa, Artificial Sequence
  CD28 ICD
RSKRSRLLHSDYMNMTPRRPGPTRKHYQPYAPPRDFAAYRS

SEQ ID NO: 7 - protein, 113 aa, Artificial Sequence
  CD3Z ICD
RVKFSRSADAPAYQQGQNQLYNELNLGRREEYDVLDKRRGRDPEMGGKPQRRKNPQEGLYNELQKDKMAEAYSEIGMKGERRRGKGHDGLYQGLSTATKDTYDALHMQALPPR

SEQ ID NO: 8 - protein, 14 aa, Artificial Sequence
  Hinge
EPKSCDKTHTCPTR

SEQ ID NO: 9 - protein, 14 aa, Artificial Sequence
  HER2(C5) LC-CDR1
GLSSGSVSTGYYPS

SEQ ID NO: 10 - protein, 7 aa, Artificial Sequence
  HER2(C5) LC-CDR2
STNSRSS

SEQ ID NO: 11 - protein, 10 aa, Artificial Sequence
  HER2(C5) LC-CDR3
VLYMGSGISV

SEQ ID NO: 12 - protein, 7 aa, Artificial Sequence
  HER2(C5) HC-CDR1
SSSYYWG

SEQ ID NO: 13 - protein, 16 aa, Artificial Sequence
  HER2(C5) HC-CDR2
SIYYSGSTYYNPSLKS

SEQ ID NO: 14 - protein, 14 aa, Artificial Sequence
  HER2(C5) HC-CDR3
YAPDSSGYLVAFDI

SEQ ID NO: 15 - protein, 112 aa, Artificial Sequence
  HER2(C5) VL
QTVVTQEPSFSVSPGGTVTLTCGLSSGSVSTGYYPSWYQQTPGQAPRTLIYSTNSRSSGVPDRFSGSILGNKAALTITGAQADDESDYYCVLYMGSGISVFGGGTKLTVLGS

SEQ ID NO: 16 - protein, 124 aa, Artificial Sequence
  HER2(C5) VH
QVQLQESGPGLVKPSETLSLTCTVSGGSISSSSYYWGWIRQPPGKGLEWIGSIYYSGSTYYNPSLKSRVTISVDTSKNQFSLKLSSVTAADTAVYYCARYAPDSSGYLVAFDIWGQGTMVTVSS

SEQ ID NO: 17 - protein, 14 aa, Artificial Sequence
  HER2(E4) LC-CDR1
GLSSGSVSTSYYPS

SEQ ID NO: 18 - protein, 7 aa, Artificial Sequence
  HER2(E4) LC-CDR2
TTNIRSS

SEQ ID NO: 19 - protein, 10 aa, Artificial Sequence
  HER2(E4) LC-CDR3
MLYMGSGIWV

SEQ ID NO: 20 - protein, 6 aa, Artificial Sequence
  HER2(E4) HC-CDR1
SGYYWS

SEQ ID NO: 21 - protein, 16 aa, Artificial Sequence
  HER2(E4) HC-CDR2
EINHSGSTNYNPSLKS

SEQ ID NO: 22 - protein, 14 aa, Artificial Sequence
  HER2(E4) HC-CDR3
MGINSGGYLYGMDV

SEQ ID NO: 23 - protein, 112 aa, Artificial Sequence
  HER2(E4) VL
QTVVTQEPSFSVSPGGTVTLTCGLSSGSVSTSYYPSWYQQIPGQAPRTLIYTTNIRSSGVPDRFGGSILGNKAALTITGAQAEDESDYYCMLYMGSGIWVFGGGTKLTVLGS

SEQ ID NO: 24 - protein, 122 aa, Artificial Sequence
  HER2(E4) VH
QVQLQQWGAGLLKPSETLSLTCAVYGGSFSGYYWSWIRQPPGKGLEWIGEINHSGSTNYNPSLKSRVTISVDTSKNQFSLKLSSVTTADTAVYYCARMGINSGGYLYGMDVWGQGTTVTVSS

SEQ ID NO: 25 - protein, 14 aa, Artificial Sequence
  HER2(F1) LC-CDR1
GLSSGSVSTSYYPS

SEQ ID NO: 26 - protein, 7 aa, Artificial Sequence
  HER2(F1) LC-CDR2
STNTRSS

SEQ ID NO: 27 - protein, 10 aa, Artificial Sequence
  HER2(F1) LC-CDR3
VLYMGSGIWV

SEQ ID NO: 28 - protein, 6 aa, Artificial Sequence
  HER2(F1) HC-CDR1
SSNWWS

SEQ ID NO: 29 - protein, 16 aa, Artificial Sequence
  HER2(F1) HC-CDR2
EIYHSGSTNYNPSLKS

SEQ ID NO: 30 - protein, 14 aa, Artificial Sequence
  HER2(F1) HC-CDR3
MGANSGGYLYGMDV

SEQ ID NO: 31 - protein, 112 aa, Artificial Sequence
  HER2(F1) VL
QTVVTQEPSFSVSPGGTVTLTCGLSSGSVSTSYYPSWYQQTPGQAPRTLIYSTNTRSSGVPDRFSGSILGNKAALTITGAQADDESDYYCVLYMGSGIWVFGGGTKLTVLGS

SEQ ID NO: 32 - protein, 123 aa, Artificial Sequence
  HER2(F1) VH
QVQLVESGPGLVKPSGTLSLTCAVSGGSISSSNWWSWVRQPPGKGLEWIGEIYHSGSTNYNPSLKSRVTISVDTSKNQFSLKLSSVTAADTAVYYCARMGANSGGYLYGMDVWGQGTTVTVSS

SEQ ID NO: 33 - protein, 14 aa, Artificial Sequence
  HER2(A3) LC-CDR1
GLSSGSVSTGHYAS

SEQ ID NO: 34 - protein, 7 aa, Artificial Sequence
  HER2(A3) LC-CDR2
NTNTRSS

SEQ ID NO: 35 - protein, 10 aa, Artificial Sequence
  HER2(A3) LC-CDR3
VLYVGDGIWV

SEQ ID NO: 36 - protein, 10 aa, Artificial Sequence
  HER2(A3) HC-CDR1
SYYIHWVRQA

SEQ ID NO: 37 - protein, 17 aa, Artificial Sequence
  HER2(A3) HC-CDR2
IINPGNGDTNYAQRFQG

SEQ ID NO: 38 - protein, 12 aa, Artificial Sequence
  HER2(A3) HC-CDR3
EIASYSGSYYDY

SEQ ID NO: 39 - protein, 110 aa, Artificial Sequence
  HER2(A3) VL
QAVVLQEPSLSVSPGGTVTLTCGLSSGSVSTGHYASWYQQTPGQAPRTLFYNTNTRSSGVPDRFSGSIVGNKAALTITGAQADDESDYYCVLYVGDGIWVFGGGTKLTVL

SEQ ID NO: 40 - protein, 121 aa, Artificial Sequence
  HER2(A3) VH
EVQLVQSGTEVKKPGASVRVSCKSSGYTFTSYYIHWVRQAPGQGLEWMAIINPGNGDTNYAQRFQGRVTMTRDTSTSTVYMELRSLRSDDTAVYFCAREIASYSGSYYDYWGQGTLVTVSS

SEQ ID NO: 41 - protein, 536 aa, Artificial Sequence
  huIL-12p70
MGHQQLVISWFSLVFLASPLVAIWELKKDVYVVELDWYPDAPGEMVVLTCDTPEEDGITWTLDQSSEVLGSGKTLTIQVKEFGDAGQYTCHKGGEVLSHSLLLLHKKEDGIWSTDILKDQKEPKNKTFLRCEAKNYSGRFTCWWLTTISTDLTFSVKSSRGSSDPQGVTCGAATLSAERVRGDNKEYEYSVECQEDSACPAAEESLPIEVMVDAVHKLKYENYTSSFFIRDIIKPDPPKNLQLKPLKNSRQVEVSWEYPDTWSTPHSYFSLTFCVQVQGKSKREKKDRVFTDKTSATVICRKNASISVRAQDRYYSSSWSEWASVPCSVPGVGVPGVGARNLPVATPDPGMFPCLHHSQNLLRAVSNMLQKARQTLEFYPCTSEEIDHEDITKDKTSTVEACLPLELTKNESCLNSRETSFITNGSCLASRKTSFMMALCLSSIYEDLKMYQVEFKTMNAKLLMDPKRQIFLDQNMLAVIDELMQALNFNSETVPQKSSLEEPDFYKTKIKLCILLHAFRIRAVTIDRVMSYLNAS

SEQ ID NO: 42 - protein, 376 aa, Artificial Sequence
  HSV1 TK
MASYPGHQHASAFDQAARSRGHSNRRTALRPRRQQEATEVRPEQKMPTLLRVYIDGPHGMGKTTTTQLLVALGSRDDIVYVPEPMTYWRVLGASETIANIYTTQHRLDQGEISAGDAAVVMTSAQITMGMPYAVTDAVLAPHIGGEAGSSHAPPPALTLIFDRHPIAALLCYPAARYLMGSMTPQAVLAFVALIPPTLPGTNIVLGALPEDRHIDRLAKRQRPGERLDLAMLAAIRRVYGLLANTVRYLQGGGSWREDWGQLSGTAVPPQGAEPQSNAGPRPHIGDTLFTLFRAPELLAPNGDLYNVFAWALDVLAKRLRPMHVFILDYDQSPAGCRDALLQLTSGMIQTHVTTPGSIPTICDLARTFAREMGEAN

SEQ ID NO: 43 - protein, 481 aa, Artificial Sequence
  PD-L1(H12_gl) minibody
EVQLVQSGAEVKKPGASVKVSCKASGGTFSSYAISWVRQAPGQGLEWMGRIIPILGIANYAQKFQGRVTITADKSTSTAYMELSSLRSEDTAVYYCARSGHGYSYGAFDYWGQGTLVTVSSGGGGSGGGGSGGGGSQSVLTQPPSVSGAPGQRVTISCTGSSSNIGAGYDVHWYQQLPGTAPKLLIYGNSNRPSGVPDRFSGSKSGTSASLAITGLQAEDEADYYCQSYDSSLSGSYVVFGGGTKLTVLEAKSCDKTHTCPPCPAPELLGGPSVFLFPPKPKDTLMISRTPEVTCVVVDVSHEDPEVKFNWYVDGVEVHNAKTKPREEQYNSTYRVVSVLTVLHQDWLNGKEYKCKVSNKALPAPIEKTISKAKGQPREPQVYTLPPSRDELTKNQVSLTCLVKGFYPSDIAVEWESNGQPENNYKTTPPVLDSDGSFFLYSKLTVDKSRWQQGNVFSCSVMHEALHNHYTQKSLSLSPGK

SEQ ID NO: 44 - protein, 14 aa, Artificial Sequence
  PD-L1(H12_gl) LC-CDR1
TGSSSNIGAGYDVH

SEQ ID NO: 45 - protein, 7 aa, Artificial Sequence
  PD-L1(H12_gl) LC-CDR2
GNSNRPS

SEQ ID NO: 46 - protein, 13 aa, Artificial Sequence
  PD-L1(H12_gl) LC-CDR3
QSYDSSLSGSYVV

SEQ ID NO: 47 - protein, 5 aa, Artificial Sequence
  PD-L1(H12_gl) HC-CDR1
SYAIS

SEQ ID NO: 48 - protein, 17 aa, Artificial Sequence
  PD-L1(H12_gl) HC-CDR2
RIIPILGIANYAQKFQG

SEQ ID NO: 49 - protein, 12 aa, Artificial Sequence
  PD-L1(H12_gl) HC-CDR3
SGHGYSYGAFDY

SEQ ID NO: 50 - protein, 113 aa, Artificial Sequence
  PD-L1(H12_gl) VL
QSVLTQPPSVSGAPGQRVTISCTGSSSNIGAGYDVHWYQQLPGTAPKLLIYGNSNRPSGVPDRFSGSKSGTSASLAITGLQAEDEADYYCQSYDSSLSGSYVVFGGGTKLTVL

SEQ ID NO: 51 - protein, 121 aa, Artificial Sequence
  PD-L1(H12_gl) VH
EVQLVQSGAEVKKPGASVKVSCKASGGTFSSYAISWVRQAPGQGLEWMGRIIPILGIANYAQKFQGRVTITADKSTSTAYMELSSLRSEDTAVYYCARSGHGYSYGAFDYWGQGTLVTVSS

SEQ ID NO: 52 - protein, 473 aa, Artificial Sequence
  PD-L1 (YW243.55.S70) minibody
EVQLVESGGGLVQPGGSLRLSCAASGFTFSDSWIHWVRQAPGKGLEWVAWISPYGGSTYYADSVKGRFTISADTSKNTAYLQMNSLRAEDTAVYYCARRHWPGGFDYWGQGTLVTVSAGGGGSGGGGSGGGGSDIQMTQSPSSLSASVGDRVTITCRASQDVSTAVAWYQQKPGKAPKLLIYSASFLYSGVPSRFSGSGSGTDFTLTISSLQPEDFATYYCQQYLYHPATFGQGTKVEIKREAKSCDKTHTCPPCPAPELLGGPSVFLFPPKPKDTLMISRTPEVTCVVVDVSHEDPEVKFNWYVDGVEVHNAKTKPREEQYNSTYRVVSVLTVLHQDWLNGKEYKCKVSNKALPAPIEKTISKAKGQPREPQVYTLPPSRDELTKNQVSLTCLVKGFYPSDIAVEWESNGQPENNYKTTPPVLDSDGSFFLYSKLTVDKSRWQQGNVFSCSVMHEALHNHYTQKSLSLSPGK

SEQ ID NO: 53 - protein, 6 aa, Artificial Sequence
  PD-L1 (YW243.55.S70) LC-CDR1
QDVSTA

SEQ ID NO: 54 - protein, 3 aa, Artificial Sequence
  PD-L1 (YW243.55.S70) LC-CDR2
SAS

SEQ ID NO: 55 - protein, 9 aa, Artificial Sequence
  PD-L1 (YW243.55.S70) LC-CDR3
QQYLYHPAT

SEQ ID NO: 56 - protein, 8 aa, Artificial Sequence
  PD-L1 (YW243.55.S70) HC-CDR1
GFTFSDSW

SEQ ID NO: 57 - protein, 8 aa, Artificial Sequence
  PD-L1 (YW243.55.S70) HC-CDR2
ISPYGGST

SEQ ID NO: 58 - protein, 11 aa, Artificial Sequence
  PD-L1 (YW243.55.S70) HC-CDR3
ARRHWPGGFDY

SEQ ID NO: 59 - protein, 107 aa, Artificial Sequence [sequence omitted]

SEQ ID NO: 60 - protein, 117 aa, Artificial Sequence
  PD-L1 (YW243.55.S70) VH
EVQLVESGGGLVQPGGSLRLSCAASGFTFSDSWIHWVRQAPGKGLEWVAWISPYGGSTYYADSVKGRFTISADTSKNTAYLQMNSLRAEDTAVYYCARRHWPGGFDYWGQGTLVTVS

SEQ ID NO: 61 - protein, 10 aa, Artificial Sequence
  IgG1 hinge
KSCDKTHTCP

SEQ ID NO: 62 - protein, 113 aa, Artificial Sequence
  hIgG1 CH2
PCPAPELLGGPSVFLFPPKPKDTLMISRTPEVTCVVVDVSHEDPEVKFNWYVDGVEVHNAKTKPREEQYNSTYRVVSVLTVLHQDWLNGKEYKCKVSNKALPAPIEKTISKAK

SEQ ID NO: 63 - protein, 107 aa, Artificial Sequence
  hIgG1 CH3
GQPREPQVYTLPPSRDELTKNQVSLTCLVKGFYPSDIAVEWESNGQPENNYKTTPPVLDSDGSFFLYSKLTVDKSRWQQGNVFSCSVMHEALHNHYTQKSLSLSPGK

SEQ ID NO: 64 - protein, 487 aa, Artificial Sequence
  anti-CD44v6 BiTE
EIVLTQSPATLSLSPGERATLSCSASSSINYIYWLQQKPGQAPRILIYLTSNLASGVPARFSGSGSGTDFTLTISSLEPEDFAVYYCLQWSSNPLTFGGGTKVEIKRGGGGSGGGGSGGGGSGGGGSEVQLVESGGGLVKPGGSLRLSCAASGFTFSSYDMSWVRQAPGKGLEWVSTISSGGSYTYYLDSIKGRFTISRDNAKNSLYLQMNSLRAEDTAVYYCARQGLDYWGRGTLVTVSSGGGGGSDIKLQQSGAELARPGASVKMSCKTSGYTFTRYTMHWVKQRPGQGLEWIGYINPSRGYTNYNQKFKDKATLTTDKSSSTAYMQLSSLTSEDSAVYYCARYYDDHYCLDYWGQGTTLTVSSGGGGSGGGGSGGGGSDIQLTQSPAIMSASPGEKVTMTCRASSSVSYMNWYQQKSGTSPKRWIYDTSKVASGVPYRFSGSGSGTSYSLTISSMEAEDAATYYCQQWSSNPLTFGAGTKLELK

SEQ ID NO: 65 - protein, 241 aa, Artificial Sequence
  anti-CD44v6 (BIWA8) scFv
EIVLTQSPATLSLSPGERATLSCSASSSINYIYWLQQKPGQAPRILIYLTSNLASGVPARFSGSGSGTDFTLTISSLEPEDFAVYYCLQWSSNPLTFGGGTKVEIKRGGGGSGGGGSGGGGSGGGGSEVQLVESGGGLVKPGGSLRLSCAASGFTFSSYDMSWVRQAPGKGLEWVSTISSGGSYTYYLDSIKGRFTISRDNAKNSLYLQMNSLRAEDTAVYYCARQGLDYWGRGTLVTVSS

SEQ ID NO: 66 - protein, 5 aa, Artificial Sequence
  anti-CD44v6 (BIWA8) LC-CDR1
SSINY

SEQ ID NO: 67 - protein, 3 aa, Artificial Sequence
  anti-CD44v6 (BIWA8) LC-CDR2
LTS

SEQ ID NO: 68 - protein, 9 aa, Artificial Sequence
  anti-CD44v6 (BIWA8) LC-CDR3
LQWSSNPLT

SEQ ID NO: 69 - protein, 8 aa, Artificial Sequence
  anti-CD44v6 (BIWA8) HC-CDR1
GFTFSSYD

SEQ ID NO: 70 - protein, 8 aa, Artificial Sequence
  anti-CD44v6 (BIWA8) HC-CDR2
ISSGGSYT

SEQ ID NO: 71 - protein, 7 aa, Artificial Sequence
  anti-CD44v6 (BIWA8) HC-CDR3
ARQGLDY

SEQ ID NO: 72 - protein, 106 aa, Artificial Sequence
  anti-CD44v6 (BIWA8) VL
EIVLTQSPATLSLSPGERATLSCSASSSINYIYWLQQKPGQAPRILIYLTSNLASGVPARFSGSGSGTDFTLTISSLEPEDFAVYYCLQWSSNPLTFGGGTKVEIK

SEQ ID NO: 73 - protein, 114 aa, Artificial Sequence
  anti-CD44v6 (BIWA8) VH
EVQLVESGGGLVKPGGSLRLSCAASGFTFSSYDMSWVRQAPGKGLEWVSTISSGGSYTYYLDSIKGRFTISRDNAKNSLYLQMNSLRAEDTAVYYCARQGLDYWGRGTLVTVSS

SEQ ID NO: 74 - protein, 240 aa, Artificial Sequence
  anti-CD3 (OKT3) scFv
DIKLQQSGAELARPGASVKMSCKTSGYTFTRYTMHWVKQRPGQGLEWIGYINPSRGYTNYNQKFKDKATLTTDKSSSTAYMQLSSLTSEDSAVYYCARYYDDHYCLDYWGQGTTLTVSSGGGGSGGGGSGGGGSDIQLTQSPAIMSASPGEKVTMTCRASSSVSYMNWYQQKSGTSPKRWIYDTSKVASGVPYRFSGSGSGTSYSLTISSMEAEDAATYYCQQWSSNPLTFGAGTKLELK

SEQ ID NO: 75 - protein, 5 aa, Artificial Sequence
  anti-CD3 (OKT3) LC-CDR1
SSVSY

SEQ ID NO: 76 - protein, 3 aa, Artificial Sequence
  anti-CD3 (OKT3) LC-CDR2
DTS

SEQ ID NO: 77 - protein, 9 aa, Artificial Sequence
  anti-CD3 (OKT3) LC-CDR3
QQWSSNPLT

SEQ ID NO: 78 - protein, 8 aa, Artificial Sequence
  anti-CD3 (OKT3) HC-CDR1
GYTFTRYT

SEQ ID NO: 79 - protein, 8 aa, Artificial Sequence
  anti-CD3 (OKT3) HC-CDR2
INPSRGYT

SEQ ID NO: 80 - protein, 12 aa, Artificial Sequence
  anti-CD3 (OKT3) HC-CDR3
ARYYDDHYCLDY

SEQ ID NO: 81 - protein, 106 aa, Artificial Sequence
  anti-CD3 (OKT3) VL
DIQLTQSPAIMSASPGEKVTMTCRASSSVSYMNWYQQKSGTSPKRWIYDTSKVASGVPYRFSGSGSGTSYSLTISSMEAEDAATYYCQQWSSNPLTFGAGTKLELK

SEQ ID NO: 82 - protein, 119 aa, Artificial Sequence
  anti-CD3 (OKT3) VH
DIKLQQSGAELARPGASVKMSCKTSGYTFTRYTMHWVKQRPGQGLEWIGYINPSRGYTNYNQKFKDKATLTTDKSSSTAYMQLSSLTSEDSAVYYCARYYDDHYCLDYWGQGTTLTVSS

SEQ ID NO: 83 - protein, 488 aa, Artificial Sequence
  anti-HER2 BiTE
EVQLQQSGPELKKPGETVKISCKASGYPFTNYGMNWVKQAPGQGLKWMGWINTSTGESTFADDFKGRFDFSLETSANTAYLQINNLKSEDMATYFCARWEVYHGYVPYWGQGTTVTVSSGGGGSGGGGSGGGGSDIQLTQSHKFLSTSVGDRVSITCKASQDVYNAVAWYQQKPGQSPKLLIYSASSRYTGVPSRFTGSGSGPDFTFTISSVQAEDLAVYFCQQHFRTPFTFGSGTKLEIKALGGGGSDIKLQQSGAELARPGASVKMSCKTSGYTFTRYTMHWVKQRPGQGLEWIGYINPSRGYTNYNQKFKDKATLTTDKSSSTAYMQLSSLTSEDSAVYYCARYYDDHYCLDYWGQGTTLTVSSGGGGSGGGGSGGGGSDIQLTQSPAIMSASPGEKVTMTCRASSSVSYMNWYQQKSGTSPKRWIYDTSKVASGVPYRFSGSGSGTSYSLTISSMEAEDAATYYCQQWSSNPLTFGAGTKLELK

SEQ ID NO: 84 - protein, 241 aa, Artificial Sequence
  anti-HER2 (FRP5) scFv
EVQLQQSGPELKKPGETVKISCKASGYPFTNYGMNWVKQAPGQGLKWMGWINTSTGESTFADDFKGRFDFSLETSANTAYLQINNLKSEDMATYFCARWEVYHGYVPYWGQGTTVTVSSGGGGSGGGGSGGGGSDIQLTQSHKFLSTSVGDRVSITCKASQDVYNAVAWYQQKPGQSPKLLIYSASSRYTGVPSRFTGSGSGPDFTFTISSVQAEDLAVYFCQQHFRTPFTFGSGTKLEIK

SEQ ID NO: 85 - protein, 6 aa, Artificial Sequence
  anti-HER2 (FRP5) LC-CDR1
QDVYNA

SEQ ID NO: 86 - protein, 3 aa, Artificial Sequence
  anti-HER2 (FRP5) LC-CDR2
SAS

SEQ ID NO: 87 - protein, 9 aa, Artificial Sequence
  anti-HER2 (FRP5) LC-CDR3
QQHFRTPFT

SEQ ID NO: 88 - protein, 8 aa, Artificial Sequence
  anti-HER2 (FRP5) HC-CDR1
GYPFTNYG

SEQ ID NO: 89 - protein, 8 aa, Artificial Sequence
  anti-HER2 (FRP5) HC-CDR2
INTSTGES

SEQ ID NO: 90 - protein, 12 aa, Artificial Sequence
  anti-HER2 (FRP5) HC-CDR3
ARWEVYHGYVPY

SEQ ID NO: 91 - protein, 107 aa, Artificial Sequence
  anti-HER2 (FRP5) VL
DIQLTQSHKFLSTSVGDRVSITCKASQDVYNAVAWYQQKPGQSPKLLIYSASSRYTGVPSRFTGSGSGPDFTFTISSVQAEDLAVYFCQQHFRTPFTFGSGTKLEIK

SEQ ID NO: 92 - protein, 119 aa, Artificial Sequence
  anti-HER2 (FRP5) VH
EVQLQQSGPELKKPGETVKISCKASGYPFTNYGMNWVKQAPGQGLKWMGWINTSTGESTFADDFKGRFDFSLETSANTAYLQINNLKSEDMATYFCARWEVYHGYVPYWGQGTTVTVSS

SEQ ID NO: 93 - protein, 488 aa, Artificial Sequence
  anti-CD19 BiTE
DIQMTQTTSSLSASLGDRVTISCRASQDISKYLNWYQQKPDGTVKLLIYHTSRLHSGVPSRFSGSGSGTDYSLTISNLEQEDIATYFCQQGNTLPYTFGGGTKLEITGGGGSGGGGSGGGGSEVKLQESGPGLVAPSQSLSVTCTVSGVSLPDYGVSWIRQPPRKGLEWLGVIWGSETTYYNSALKSRLTIIKDNSKSQVFLKMNSLQTDDTAIYYCAKHYYYGGSYAMDYWGQGTSVTVSSGGGGGSDIKLQQSGAELARPGASVKMSCKTSGYTFTRYTMHWVKQRPGQGLEWIGYINPSRGYTNYNQKFKDKATLTTDKSSSTAYMQLSSLTSEDSAVYYCARYYDDHYCLDYWGQGTTLTVSSGGGGSGGGGSGGGGSDIQLTQSPAIMSASPGEKVTMTCRASSSVSYMNWYQQKSGTSPKRWIYDTSKVASGVPYRFSGSGSGTSYSLTISSMEAEDAATYYCQQWSSNPLTFGAGTKLELK

SEQ ID NO: 94 - protein, 242 aa, Artificial Sequence
  anti-CD19 (FMC63) scFv
DIQMTQTTSSLSASLGDRVTISCRASQDISKYLNWYQQKPDGTVKLLIYHTSRLHSGVPSRFSGSGSGTDYSLTISNLEQEDIATYFCQQGNTLPYTFGGGTKLEITGGGGSGGGGSGGGGSEVKLQESGPGLVAPSQSLSVTCTVSGVSLPDYGVSWIRQPPRKGLEWLGVIWGSETTYYNSALKSRLTIIKDNSKSQVFLKMNSLQTDDTAIYYCAKHYYYGGSYAMDYWGQGTSVTVSS

SEQ ID NO: 95 - protein, 6 aa, Artificial Sequence
  anti-CD19 (FMC63) LC-CDR1
QDISKY

SEQ ID NO: 96 - protein, 3 aa, Artificial Sequence
  anti-CD19 (FMC63) LC-CDR2
HTS

SEQ ID NO: 97 - protein, 9 aa, Artificial Sequence
  anti-CD19 (FMC63) LC-CDR3
QQGNTLPYT

SEQ ID NO: 98 - protein, 8 aa, Artificial Sequence
  anti-CD19 (FMC63) HC-CDR1
GVSLPDYG

SEQ ID NO: 99 - protein, 7 aa, Artificial Sequence
  anti-CD19 (FMC63) HC-CDR2
IWGSETT

SEQ ID NO: 100 - protein, 14 aa, Artificial Sequence
  anti-CD19 (FMC63) HC-CDR3
AKHYYYGGSYAMDY

SEQ ID NO: 101 - protein, 107 aa, Artificial Sequence
  anti-CD19 (FMC63) VL
DIQMTQTTSSLSASLGDRVTISCRASQDISKYLNWYQQKPDGTVKLLIYHTSRLHSGVPSRFSGSGSGTDYSLTISNLEQEDIATYFCQQGNTLPYTFGGGTKLEIT

SEQ ID NO: 102 - protein, 120 aa, Artificial Sequence
  anti-CD19 (FMC63) VH
EVKLQESGPGLVAPSQSLSVTCTVSGVSLPDYGVSWIRQPPRKGLEWLGVIWGSETTYYNSALKSRLTIIKDNSKSQVFLKMNSLQTDDTAIYYCAKHYYYGGSYAMDYWGQGTSVTVSS

SEQ ID NO: 103 - protein, 1014 aa, Artificial Sequence
  HER2 BiTE_CD44 v6BiTE fusion
EIVLTQSPATLSLSPGERATLSCSASSSINYIYWLQQKPGQAPRILIYLTSNLASGVPARFSGSGSGTDFTLTISSLEPEDFAVYYCLQWSSNPLTFGGGTKVEIKRGGGGSGGGGSGGGGSGGGGSEVQLVESGGGLVKPGGSLRLSCAASGFTFSSYDMSWVRQAPGKGLEWVSTISSGGSYTYYLDSIKGRFTISRDNAKNSLYLQMNSLRAEDTAVYYCARQGLDYWGRGTLVTVSSGGGGGSDIKLQQSGAELARPGASVKMSCKTSGYTFTRYTMHWVKQRPGQGLEWIGYINPSRGYTNYNQKFKDKATLTTDKSSSTAYMQLSSLTSEDSAVYYCARYYDDHYCLDYWGQGTTLTVSSGGGGSGGGGSGGGGSDIQLTQSPAIMSASPGEKVTMTCRASSSVSYMNWYQQKSGTSPKRWIYDTSKVASGVPYRFSGSGSGTSYSLTISSMEAEDAATYYCQQWSSNPLTFGAGTKLELKSEGRGSLLTCGDVEENPGPSMDWIWRILFLVGAATGAHSEVQLQQSGPELKKPGETVKISCKASGYPFTNYGMNWVKQAPGQGLKWMGWINTSTGESTFADDFKGRFDFSLETSANTAYLQINNLKSEDMATYFCARWEVYHGYVPYWGQGTTVTVSSGGGGSGGGGSGGGGSDIQLTQSHKFLSTSVGDRVSITCKASQDVYNAVAWYQQKPGQSPKLLIYSASSRYTGVPSRFTGSGSGPDFTFTISSVQAEDLAVYFCQQHFRTPFTFGSGTKLEIKALGGGGSDIKLQQSGAELARPGASVKMSCKTSGYTFTRYTMHWVKQRPGQGLEWIGYINPSRGYTNYNQKFKDKATLTTDKSSSTAYMQLSSLTSEDSAVYYCARYYDDHYCLDYWGQGTTLTVSSGGGGSGGGGSGGGGSDIQLTQSPAIMSASPGEKVTMTCRASSSVSYMNWYQQKSGTSPKRWIYDTSKVASGVPYRFSGSGSGTSYSLTISSMEAEDAATYYCQQWSSNPLTFGAGTKLELK

SEQ ID NO: 104 - protein, 281 aa, Artificial Sequence
  Ad2 E1Adelta24
MRHIICHGGVITEEMAASLLDQLIEEVLADNLPPPSHFEPPTLHELYDLDVTAPEDPNEEAVSQIFPESVMLAVQEGIDLFTFPPAPGSPEPPHLSRQPEQPEQRALGPVSMPNLVPEVIDPPSDDEDEEGEEFVLDYVEHPGHGCRSCHYHRRNTGDPDIMCSLCYMRTCGMFVYSPVSEPEPEPEPEPEPARPTRRPKLVPAILRRPTSPVSRECNSSTDSCDSGPSNTPPEIHPVVPLCPIKPVAVRVGGRRQAVECIEDLLNESGQPLDLSCKRPRP

SEQ ID NO: 105 - protein, 8 aa, Artificial Sequence
  Amino acids 121-128 of Ad E1A protein
LTCHEACF

SEQ ID NO: 106 - protein, 19 aa, Artificial Sequence
  SignalP 1
MDWIWRILFLVGAATGAHS

SEQ ID NO: 107 - protein, 20 aa, Artificial Sequence
  SignalP 2
MEAPAQLLFLLLLWLPDTTG

SEQ ID NO: 108 - protein, 22 aa, Artificial Sequence
  SignalP 3
MGHQQLVISWFSLVFLASPLVA

SEQ ID NO: 109 - protein, 5 aa, Artificial Sequence
  G4S linker
GGGGS

SEQ ID NO: 110 - protein, 10 aa, Artificial Sequence
  (G4S)2 linker
GGGGSGGGGS

SEQ ID NO: 111 - protein, 15 aa, Artificial Sequence
  (G4S)3 linker
GGGGSGGGGSGGGGS

SEQ ID NO: 112 - protein, 20 aa, Artificial Sequence
  (G4S)4 linker
GGGGSGGGGSGGGGSGGGGS

SEQ ID NO: 113 - protein, 9 aa, Artificial Sequence
  HA tag
YPYDVPDYA

SEQ ID NO: 114 - protein, 29 aa, Artificial Sequence
  3xHA tag
YPYDVPDYAGYPYDVPDYAGYPYDVPDYA

SEQ ID NO: 115 - protein, 18 aa, Artificial Sequence
  T2A peptide
EGRGSLLTCGDVEENPGP

SEQ ID NO: 116 - protein, 7 aa, Artificial Sequence
  2A cleavage sequence consensus
  MISC_FEATURE (1)..(1): Xaa = V or I
  MISC_FEATURE (3)..(3): Xaa = S or E
XEXNPGP

SEQ ID NO: 117 - DNA, 3750 bp, Artificial Sequence
  HER2(C5)-CD28TM,ICD-CD3Z CAR
aagttcagatcaaggtcaggaacagatggaacagctgaatatgggccaaacaggatatctgtggtaagcagttcctgccccggctcagggccaagaacagatggaacagctgaatatgggccaaacaggatatctgtggtaagcagttcctgccccggctcagggccaagaacagatggtccccagatgcggtccagccctcagcagtttctagagaaccatcagatgtttccagggtgccccaaggacctgaaatgaccctgtgccttatttgaactaaccaatcagttcgcttctcgcttctgttcgcgcgcttctgctccccgagctcaataaaagagcccacaacccctcactcggcgcgccagtcctccgattgactgagtcgcccgggtacccgtgtatccaataaaccctcttgcagttgcatccgacttgtggtctcgctgttccttgggagggtctcctctgagtgattgactacccgtcagcgggggtctttcatttgggggctcgtccgggatcgggagacccctgcccagggaccaccgacccaccaccgggaggtaagctggccagcaacttatctgtgtctgtccgattgtctagtgtctatgactgattttatgcgcctgcgtcggtactagttagctaactagctctgtatctggcggacccgtggtggaactgacgagttcggaacacccggccgcaaccctgggagacgtcccagggacttcgggggccgtttttgtggcccgacctgagtcctaaaatcccgatcgtttaggactctttggtgcaccccccttagaggagggatatgtggttctggtaggagacgagaacctaaaacagttcccgcctccgtctgaatttttgctttcggtttgggaccgaagccgcgccgcgcgtcttgtctgctgcagcatcgttctgtgttgtctctgtctgactgtgtttctgtatttgtctgaaaatatgggcccgggctagcctgttaccactcccttaagtttgaccttaggtcactggaaagatgtcgagcggatcgctcacaaccagtcggtagatgtcaagaagagacgttgggttaccttctgctctgcagaatggccaacctttaacgtcggatggccgcgagacggcacctttaaccgagacctcatcacccaggttaagatcaaggtcttttcacctggcccgcatggacacccagaccaggtcccctacatcgtgacctgggaagccttggcttttgacccccctccctgggtcaagccctttgtacaccctaagcctccgcctcctcttcctccatccgccccgtctctcccccttgaacctcctcgttcgaccccgcctcgatcctccctttatccagccctcactccttctctaggcgcccccatatggccatatgagatcttatatggggcacccccgccccttgtaaacttccctgaccctgacatgacaagagttactaacagcccctctctccaagctcacttacaggctctctacttagtccagcacgaagtctggagacctctggcggcagcctaccaagaacaactggaccgaccggtggtacctcacccttaccgagtcggcgacacagtgtgggtccgccgacaccagactaagaacctagaacctcgctggaaaggaccttacacagtcctgctgaccacccccaccgccctcaaagtagacggcatcgcagcttggatacacgccgcccacgtgaaggctgccgaccccgggggtggaccatgactcgagccatggattggatctggcgcatcctgtttctcgtgggagctgccacaggcgcccattctcaggttcagctgcaagagtctggccctggcctggtcaagcctagcgaaacactgagcctgacctgtaccgtgtctggcggcagcatcagcagcagctcttactactggggctggatcagacagcctcctggcaaaggcctggaatggatcggctccatctactacagcggcagcacctactacaaccccagcctgaagtccagagtgaccatcagcgtggacaccagcaagaaccagttctccctgaagctgagcagcgtgacagccgccgatacagccgtgtactactgtgccagatacgcccctgatagcagcggctacctggtggcctttgatatctggggccagggcacaatggtcaccgtttctagcggaggcggaggttctggtggcggaggaagtggcggcggaggatctcagacagtggtcacacaagagcccagcttctccgtgtctcctggcggaacagtgaccctgacatgtggccttagctctggctctgtgtccaccggctactaccccagctggtatcagcagacacctggacaggcccctcggacactgatctacagcaccaacagcagatccagcggcgtgcccgatagattcagcggctctatcctgggcaacaaggccgcactgacaatcacaggcgctcaggccgatgacgagagcgactactactgcgtgctgtacatgggcagcggcatctccgtttttggcggaggcacaaagctgaccgtgctgggatccgaaccaaagagttgcgacaaaacacacacctgccctacgcgtttttgggtgctcgtggtggtgggtggcgtgctcgcttgctactcacttctggtgaccgtagcgtttatcattttttgggtcaggagcaagcgatcccgcctattgcacagcgactacatgaacatgaccccccggcgccccgggccaacccggaagcactaccagccatatgcgcctccccgcgatttcgcagcgtatcggtcccgggtcaaattttcacggtccgctgacgccccggcctatcaacagggccagaatcagctgtataatgaattaaacctcggtagacgcgaggagtacgacgtcctcgacaagagaagggggcgcgacccagagatgggaggcaaaccgcagcgcaggaagaatccacaggagggcctgtacaacgaattacagaaggacaagatggcagaggcctacagcgagataggaatgaagggtgaaaggcgtcgtggaaagggccacgatgggctttaccagggcctaagtactgccacaaaagatacgtatgacgcgctgcatatgcaagccctcccccccaggtaagcatgcaacctcgatccggattagtccaatttgttaaagacaggatatcagtggtccaggctctagttttgactcaacaatatcaccagctgaagcctatagagtacgagccatagataaaataaaagattttatttagtctccagaaaaaggggggaatgaaagaccccacctgtaggtttggcaagctagcttaagtaacgccattttgcaaggcatggaaaaatacataactgagaatagagaagttcagatcaaggtcaggaacagatggaacagctgaatatgggccaaacaggatatctgtggtaagcagttcctgccccggctcagggccaagaacagatggaacagctgaatatgggccaaacaggatatctgtggtaagcagttcctgccccggctcagggccaagaacagatggtccccagatgcggtccagccctcagcagtttctagagaaccatcagatgtttccagggtgccccaaggacctgaaatgaccctgtgccttatttgaactaaccaatcagttcgcttctcgcttctgttcgcgcgcttc

SEQ ID NO: 118 - DNA, 3744 bp, Artificial Sequence
  HER2(E4)-CD28TM,ICD-CD3Z CAR
aagttcagatcaaggtcaggaacagatggaacagctgaatatgggccaaacaggatatctgtggtaagcagttcctgccccggctcagggccaagaacagatggaacagctgaatatgggccaaacaggatatctgtggtaagcagttcctgccccggctcagggccaagaacagatggtccccagatgcggtccagccctcagcagtttctagagaaccatcagatgtttccagggtgccccaaggacctgaaatgaccctgtgccttatttgaactaaccaatcagttcgcttctcgcttctgttcgcgcgcttctgctccccgagctcaataaaagagcccacaacccctcactcggcgcgccagtcctccgattgactgagtcgcccgggtacccgtgtatccaataaaccctcttgcagttgcatccgacttgtggtctcgctgttccttgggagggtctcctctgagtgattgactacccgtcagcgggggtctttcatttgggggctcgtccgggatcgggagacccctgcccagggaccaccgacccaccaccgggaggtaagctggccagcaacttatctgtgtctgtccgattgtctagtgtctatgactgattttatgcgcctgcgtcggtactagttagctaactagctctgtatctggcggacccgtggtggaactgacgagttcggaacacccggccgcaaccctgggagacgtcccagggacttcgggggccgtttttgtggcccgacctgagtcctaaaatcccgatcgtttaggactctttggtgcaccccccttagaggagggatatgtggttctggtaggagacgagaacctaaaacagttcccgcctccgtctgaatttttgctttcggtttgggaccgaagccgcgccgcgcgtcttgtctgctgcagcatcgttctgtgttgtctctgtctgactgtgtttctgtatttgtctgaaaatatgggcccgggctagcctgttaccactcccttaagtttgaccttaggtcactggaaagatgtcgagcggatcgctcacaaccagtcggtagatgtcaagaagagacgttgggttaccttctgctctgcagaatggccaacctttaacgtcggatggccgcgagacggcacctttaaccgagacctcatcacccaggttaagatcaaggtcttttcacctggcccgcatggacacccagaccaggtcccctacatcgtgacctgggaagccttggcttttgacccccctccctgggtcaagccctttgtacaccctaagcctccgcctcctcttcctccatccgccccgtctctcccccttgaacctcctcgttcgaccccgcctcgatcctccctttatccagccctcactccttctctaggcgcccccatatggccatatgagatcttatatggggcacccccgccccttgtaaacttccctgaccctgacatgacaagagttactaacagcccctctctccaagctcacttacaggctctctacttagtccagcacgaagtctggagacctctggcggcagcctaccaagaacaactggaccgaccggtggtacctcacccttaccgagtcggcgacacagtgtgggtccgccgacaccagactaagaacctagaacctcgctggaaaggaccttacacagtcctgctgaccacccccaccgccctcaaagtagacggcatcgcagcttggatacacgccgcccacgtgaaggctgccgaccccgggggtggaccatgactcgagccatggattggatctggcgcatcctgtttctcgtgggagctgccacaggcgcccattctcaggttcagctgcaacagtggggagccggactgctgaagcctagcgaaacactgagcctgacctgtgccgtgtacggcggcagctttagcggctactactggtcctggatcagacagcctcctggcaaaggcctggaatggatcggcgagatcaatcacagcggcagcaccaactacaaccccagcctgaagtccagagtgaccatcagcgtggacaccagcaagaaccagttctccctgaagctgagcagcgtgaccacagccgataccgccgtgtactactgtgcccggatgggcatcaatagcggcggctacctgtacggcatggatgtgtggggacagggcaccaccgtgacagtttctagcggaggcggaggttctggtggcggaggaagtggcggcggaggatctcagacagtggtcacacaagagcccagcttctccgtgtctcctggcggaacagtgaccctgacatgtggccttagcagcggctctgtgtccaccagctactaccctagctggtatcagcagatccccggacaggcccctcggacactgatctacaccaccaacatcagatccagcggcgtgcccgatagattcggcggatctatcctgggcaacaaggccgcactgacaatcacaggtgcccaggccgaggacgagtccgactactactgcatgctgtacatgggcagcggcatctgggttttcggcggaggcacaaagctgaccgttctgggatccgaaccaaagagttgcgacaaaacacacacctgccctacgcgtttttgggtgctcgtggtggtgggtggcgtgctcgcttgctactcacttctggtgaccgtagcgtttatcattttttgggtcaggagcaagcgatcccgcctattgcacagcgactacatgaacatgaccccccggcgccccgggccaacccggaagcactaccagccatatgcgcctccccgcgatttcgcagcgtatcggtcccgggtcaaattttcacggtccgctgacgccccggcctatcaacagggccagaatcagctgtataatgaattaaacctcggtagacgcgaggagtacgacgtcctcgacaagagaagggggcgcgacccagagatgggaggcaaaccgcagcgcaggaagaatccacaggagggcctgtacaacgaattacagaaggacaagatggcagaggcctacagcgagataggaatgaagggtgaaaggcgtcgtggaaagggccacgatgggctttaccagggcctaagtactgccacaaaagatacgtatgacgcgctgcatatgcaagccctcccccccaggtaagcatgcaacctcgatccggattagtccaatttgttaaagacaggatatcagtggtccaggctctagttttgactcaacaatatcaccagctgaagcctatagagtacgagccatagataaaataaaagattttatttagtctccagaaaaaggggggaatgaaagaccccacctgtaggtttggcaagctagcttaagtaacgccattttgcaaggcatggaaaaatacataactgagaatagagaagttcagatcaaggtcaggaacagatggaacagctgaatatgggccaaacaggatatctgtggtaagcagttcctgccccggctcagggccaagaacagatggaacagctgaatatgggccaaacaggatatctgtggtaagcagttcctgccccggctcagggccaagaacagatggtccccagatgcggtccagccctcagcagtttctagagaaccatcagatgtttccagggtgccccaaggacctgaaatgaccctgtgccttatttgaactaaccaatcagttcgcttctcgcttctgttcgcgcgcttc

SEQ ID NO: 119 - DNA, 3747 bp, Artificial Sequence
  HER2(F1)-CD28TM,ICD-CD3Z CAR
aagttcagatcaaggtcaggaacagatggaacagctgaatatgggccaaacaggatatctgtggtaagcagttcctgccccggctcagggccaagaacagatggaacagctgaatatgggccaaacaggatatctgtggtaagcagttcctgccccggctcagggccaagaacagatggtccccagatgcggtccagccctcagcagtttctagagaaccatcagatgtttccagggtgccccaaggacctgaaatgaccctgtgccttatttgaactaaccaatcagttcgcttctcgcttctgttcgcgcgcttctgctccccgagctcaataaaagagcccacaacccctcactcggcgcgccagtcctccgattgactgagtcgcccgggtacccgtgtatccaataaaccctcttgcagttgcatccgacttgtggtctcgctgttccttgggagggtctcctctgagtgattgactacccgtcagcgggggtctttcatttgggggctcgtccgggatcgggagacccctgcccagggaccaccgacccaccaccgggaggtaagctggccagcaacttatctgtgtctgtccgattgtctagtgtctatgactgattttatgcgcctgcgtcggtactagttagctaactagctctgtatctggcggacccgtggtggaactgacgagttcggaacacccggccgcaaccctgggagacgtcccagggacttcgggggccgtttttgtggcccgacctgagtcctaaaatcccgatcgtttaggactctttggtgcaccccccttagaggagggatatgtggttctggtaggagacgagaacctaaaacagttcccgcctccgtctgaatttttgctttcggtttgggaccgaagccgcgccgcgcgtcttgtctgctgcagcatcgttctgtgttgtctctgtctgactgtgtttctgtatttgtctgaaaatatgggcccgggctagcctgttaccactcccttaagtttgaccttaggtcactggaaagatgtcgagcggatcgctcacaaccagtcggtagatgtcaagaagagacgttgggttaccttctgctctgcagaatggccaacctttaacgtcggatggccgcgagacggcacctttaaccgagacctcatcacccaggttaagatcaaggtcttttcacctggcccgcatggacacccagaccaggtcccctacatcgtgacctgggaagccttggcttttgacccccctccctgggtcaagccctttgtacaccctaagcctccgcctcctcttcctccatccgccccgtctctcccccttgaacctcctcgttcgaccccgcctcgatcctccctttatccagccctcactccttctctaggcgcccccatatggccatatgagatcttatatggggcacccccgccccttgtaaacttccctgaccctgacatgacaagagttactaacagcccctctctccaagctcacttacaggctctctacttagtccagcacgaagtctggagacctctggcggcagcctaccaagaacaactggaccgaccggtggtacctcacccttaccgagtcggcgacacagtgtgggtccgccgacaccagactaagaacctagaacctcgctggaaaggaccttacacagtcctgctgaccacccccaccgccctcaaagtagacggcatcgcagcttggatacacgccgcccacgtgaaggctgccgaccccgggggtggaccatgactcgagccatggattggatctggcgcatcctgtttctcgtgggagctgccacaggcgcccattctcaggttcagctggtggaatctggccctggcctggttaagcctagcggcacactgtctctgacctgtgctgtgtctggcggcagcatcagcagcagcaattggtggtcttgggtccgacagcctcctggcaaaggcctggaatggatcggcgagatctaccacagcggcagcaccaactacaaccccagcctgaagtccagagtgaccatcagcgtggacaccagcaagaaccagttctccctgaagctgagcagcgtgacagccgccgatacagccgtgtactactgtgccagaatgggagccaatagcggcggctacctgtacggcatggatgtgtggggacagggcaccaccgtgacagtttctagcggaggcggaggttctggtggcggaggaagtggcggcggaggatctcagacagtggtcacacaagagcccagcttctccgtgtctcctggcggaacagtgaccctgacatgtggccttagcagcggctctgtgtctaccagctactacccctcctggtatcagcagacccctggacaggctccccggacactgatctactccaccaacaccagatccagcggcgtgcccgatagattctccggctctatcctgggcaacaaggccgcactgacaatcacaggcgctcaggccgatgacgagagcgactactactgcgtgctgtacatgggcagcggcatctgggttttcggcggaggcacaaagctgaccgttctgggatccgaaccaaagagttgcgacaaaacacacacctgccctacgcgtttttgggtgctcgtggtggtgggtggcgtgctcgcttgctactcacttctggtgaccgtagcgtttatcattttttgggtcaggagcaagcgatcccgcctattgcacagcgactacatgaacatgaccccccggcgccccgggccaacccggaagcactaccagccatatgcgcctccccgcgatttcgcagcgtatcggtcccgggtcaaattttcacggtccgctgacgccccggcctatcaacagggccagaatcagctgtataatgaattaaacctcggtagacgcgaggagtacgacgtcctcgacaagagaagggggcgcgacccagagatgggaggcaaaccgcagcgcaggaagaatccacaggagggcctgtacaacgaattacagaaggacaagatggcagaggcctacagcgagataggaatgaagggtgaaaggcgtcgtggaaagggccacgatgggctttaccagggcctaagtactgccacaaaagatacgtatgacgcgctgcatatgcaagccctcccccccaggtaagcatgcaacctcgatccggattagtccaatttgttaaagacaggatatcagtggtccaggctctagttttgactcaacaatatcaccagctgaagcctatagagtacgagccatagataaaataaaagattttatttagtctccagaaaaaggggggaatgaaagaccccacctgtaggtttggcaagctagcttaagtaacgccattttgcaaggcatggaaaaatacataactgagaatagagaagttcagatcaaggtcaggaacagatggaacagctgaatatgggccaaacaggatatctgtggtaagcagttcctgccccggctcagggccaagaacagatggaacagctgaatatgggccaaacaggatatctgtggtaagcagttcctgccccggctcagggccaagaacagatggtccccagatgcggtccagccctcagcagtttctagagaaccatcagatgtttccagggtgccccaaggacctgaaatgaccctgtgccttatttgaactaaccaatcagttcgcttctcgcttctgttcgcgcgcttc

SEQ ID NO: 120 - DNA, 30590 bp, Artificial Sequence
  HDAdIL-12_TK_PD-L1
aaacatcatcaataatataccttattttggattgaagccaatatgataatgagggggtggagtttgtgacgtggcgcggggcgtgggaacggggcgggtgacgtagtagtgtggcggaagtgtgatgttgcaagtgtggcggaacacatgtaagcgacggatgtggcaaaagtgacgtttttggtgtgcgccggtgtacacaggaagtgacaattttcgcgcggttttaggcggatgttgtagtaaatttgggcgtaaccgagtaagatttggccattttcgcgggaaaactgaataagaggaagtgaaatctgaataattttgtgttactcatagcgcgtaatatttgtctagggccgcggggactttgaccgtttacgtggagactcgcccaggtgtttttctcaggtgttttccgcgttccgggtcaaagttggcgttttgatatcaagcttatcgataccgtaaacaagtctttaattcaagcaagactttaacaagttaaaaggagcttatgggtaggaagtagtgttatgatgtatgggcataaagggttttaatgggatagtgaaaatgtctataataatacttaaatggctgcccaatcacctacaggattgatgtaaacatggaaaaggtcaaaaacttgggtcactaaaatagatgattaatggagaggatgaggttgatagttaaatgtagataagtggtcttattctcaataaaaatgtgaacataaggcgagtttctacaaagatggacaggactcattcatgaaacagcaaaaactggacatttgttctaatctttgaagagtatgaaaaattcctattttaaaggtaaaacagtaactcacaggaaataccaacccaacataaaatcagaaacaatagtctaaagtaataaaaatcaaacgtttgcacgatcaaattatgaatgaaattcactactaaaattcacactgattttgtttcatccacagtgtcaatgttgtgatgcatttcaattgtgtgacacaggcagactgtggatcaaaagtggtttctggtgcgacttactctcttgagtatacctgcagtcccctttcttaagtgtgttaaaaaaaaagggggatttcttcaattcgccaatactctagctctccatgtgctttctaggaaacaagtgttaacccaccttatttgtcaaacctagctccaaaggacttttgactccccacaaaccgatgtagctcaagagagggtatctgtcaccagtatgtatagtgaaaaaagtatcccaagtcccaacagcaattcctaaaaggagtttatttaaaaaaccacacacacctgtaaaataagtatatatcctccaaggtgactagttttaaaaaaacagtattggctttgatgtaaagtactagtgaatatgttagaaaaatctcactgtaaccaagtgaaatgaaagcaagtatggtttgcagagattcaaagaaaatataagaaaacctactgttgccactaaaaagaatcatatattaaatatactcacacaatagctcttcagtctgataaaatctacagtcataggaatggatctatcactatttctattcagtgctttgatgtaatccagcaggtcagcaaagaatttatagccccccttgagcacacagagggctacaatgtgatggcctcccatctccttcatcacatctcgagcaagacgttcagtcctacagaaataaaatcaggaatttaatagaaagtttcatacattaaactttataacaaacacctcttagtcattaaacttccacaccaacctgggcaatatagtgagaccccatgcctgcaaaaaaaaaaaaattagccaggcatggtagcatgtacctgtagtcccagctacttgagaggtgaggtgggaaaatcactttagtgcaggatgttgaggctggagtgaactgtgattgtgccactgcactccagcctggacaatagagcaagaccttgtctcaaaaaaatgcattaaaaattttttttaaatcttccacgtatcacatcctttgccctcatgtttcataaggtaaaaaatttgataccttcaaaaaaaccaagcataccactatcataattttttttaaatgcaaataaaaacaagataccattttcacctatcagactggcaggttctgattaaatgaaattttctggataatatacaatattaagagagactgtagaaactgggccagtggctcatgcctgtaatcccagcactttgggaggctgggtaacatggcgaaccctgtttctacaaaataaaaatattagctgggagtggtggcgcacacctatagtcccagctactcaggaggctgaggtggaaggatcgcttgaacccaggaggttgagactgcagtgaactgtgatcattctgctgcactgcaccccagcctgggcaacagagaccttgtctcaaaaaaaaaaaaaaaagagacaaattgtgaagagaaaggtactctcatataacatcaggagtataaaatgattcaacttcttagaggaaaatttggcaataccaaaatattcaataaactctttccccttgacccagaaattccacttgaataaagctgaacaagtaccaaacatgtaaaagaatgtttcttctagtacagtcggtaagaacaaaatagtgtctatcaatagtggactggttaaatcagttatggtatctccataagacagaatgctatgcaacctttaaaatatattagatagctctagacacactaatattaaaagtgtccaataacatttaaaactatactcatacgttaaaatataaatgtatatatgtacttttgcatatagtatacatgcataggccagtgcttgagaagaaatgtgtacagaaggctgaaaggagagaactttagtcttcttgtttatggcctccatagttagaatattttataacacaaatattttgatattataattttaaaataaaaacacagaatagccagacatacaatgcaagcattcaataccaggtaaggtttttcactgtaattgacttaacagaaaattttcaagctagatgtgcataataataaaaatctgaccttgccttcatgtgattcagccccagtccattaccctgtttaggactgagaaatgcaagactctggctagagttccttcttccatctcccttcaatgtttactttgttctggtccctacagagtcccactataccacaactgatactaagtaattagtaaggccctcctcttttatttttaataaagaagattttagaaagcatcagttatttaataagttggcctagtttatgttcaaatagcaagtactcagaacagctgctgatgtttgaaattaacacaagaaaaagtaaaaaacctcattttaagatcttacttacctgtccataattagtccatgaggaataaacaccctttccaaatcctcagcataatgattaggtatgcaaaataaatcaaggtcataacctggttcatcatcactaatctgaaaaagaaatatagctgtttcaatgagagcattacaggatacaaacatttgattggattaagatgttaaaaaataaccttagtctatcagagaaatttaggtgtaagatgatattagtaactgttaactttgtaggtatgataatgaattatgtaagaaaacaacaggccgggcgggttggttcacacgtgtaatcccagcactttgggaggctgaggcaggcagactgcctgagctcaggagttcgagaccagcctgggcaacacggtgaaatcccgtctctactaaaaatacaaaaaaattagccgggtgtggtgacacatgcctgtagtcccagctacttgggaggctgaggcaggagaatcacttgaacctgggaggtgaaggttgcagtgagccaagatggcaccacttcactccagcctgggaaacagagcaagactctgtctctgagctgagatggcaccacttcactccagcctgggaaacagagcaagactctgtctcaaaaaaaacaaaacacacaaacaaaaaaacaggctgggcgcggtggctcacgcctgtaatcccagcactttgggaggccgaggcgggtggatcacctgaggtcaggagttccagaccagccttgtcaacatggtgaaacctccccccgccgtctctactaaaaatacaaaaattagccaggcgtggtggcaggagcctgtaatcccagctacttgggaggctgaggcaggagaatcgcttgtacccagaaggcagaggttgcactgagctgagatggcaccattgcactccagcctgggggacaagagcgagatttcgtctttaaaaaacaaaaacaaaacaaaaaaccatgtaactatatgtcttagtcatcttagtcaagaatgtagaagtaaagtgataagatatggaatttcctttaggtcacaaagagaaaaagaaaaattttaaagagctaagacaaacgcagcaaaatctttatatttaataatattctaaacatgggtgatgaacatacgggtattcattatactattctctccacttttgagtatgtttgaaaatttagtaaaacaagttttaacacactgtagtctaacaagataaaatatcacactgaacaggaaaaactggcatggtgtggtggctcacacttgtaatcccagtgctttgggaggctgagacaggagagttgcttgaggccaggagttcaagaccgacatggggaatgtagcaagaccccgtccctacaaaaaactttgtaaaaatttgccaggtatggtggtgcatacctgtagtcccagctactcgggaggcggaggcagaaggaatcacttgagcccaggagtttgaggctgcagtgagctacgatcataccacagcactccagcgtggacaacagagtaagaccctatctcaaaaacaaaacaaaacaaaacaaacaaaaaaaaccacaagaaaaactgctggctgatgcagcggctcatgcctgtaatcccagtattttgggaggcccaggtgggcgtatcacctgaggtcaggagttagagaccagcctggccaacatggtgaaaccccatctctactaaaaatacaaaattagccaggcatgtggcacgcgcctgtagtcccagttactgggaggctgaagcaggaggatcacctgagcccgggaggtggaggttgcagtgagccgagatcacaccactgcactccagcctgggtgacacagcaataccctacctcaaaataaaaaagaaaaagaaaagaaaagttgctgtccccgctaccccaatcccaaatccaaacagcctctctcatctcacagtaagggggaaaaatcacccaaaaaagctaagtgatcttttgaaaacccaaactcttagaagtctaagattattatagtcaactcatgaagtgtcatcataaaagatactctaatattatttaagtagaaccacatattggttgtcttggtatgtctagcccctggcatacaaaatatttaataacactgatatggtacctgtgatgtgaaaatgtactatgagtacagctttataaatactatatatgtacctatatacagaaaaaaatacaacaaaatcataaaagcacttatctttgaaagaggagttacagcaattttatttagttctttattgctttgctatatattctaaatttttttcaatgaatatatatcacttttaaaaaaattcaatggtctttcttataaattatctttggcagcatgcgtttttatatatacatataaaatgtatgggaaatttttaaaggatacattaaattaaagcaaaatatacaaacaaaaaatcagaatacaaaaagataaaaagattgggaagggagggagggagtaaggaggaagggtgggtgggtatagagaaatataccaaataatggtaagaagtggggtcttgacactttctacactttttttaaataaaaaaaatttttttctctctcttttttttttttagagacgaagtctcgctatgttgcccaggctggtcttgaactcctgggatcaagagatcctcctgcctcagcctcccaaggtgcttggattacaggtgtgagccaccacgcctggtcactttctacactttaatatatatattttttcattttcaatgtcatttttattagttaatttataatacccattcaccattatattcaaagtctatttgaagaaataaaccagaaagaatgaaatactctagctcacatgctattcaatactaaattacctttcaaatcacattcaagaagctgatgatttaagctttggcggtttccaataaatattggtcaaaccataattaaatctcaatatatcagttagtacctattgagcatctccttttacaacctaagcattgtattaggtgcttaaatacaagcagcttgacttttaatacatttaaaaatacatatttaagacttaaaatcttatttatggaattcagttatattttgaggtttccagtgctgagaaatttgaggtttgtgctgtctttcagtccccaaagctcagttctgagttctcagactttggtggaacttcatgtattgtcaggttggcccgtaatacctgtgggacaacttcagcccctgtgcacatggccaggaggctggttgcaaacattttcaggtaggtggaccaggacatgcccctggtcatggccaggtggaggcatagtgctatacagcaggcagaagtcaatattgatttgtttttaaagaaacatgtactactttcataagcagaaaaaatttctattcttgggggaaaagattatgccagatcctctaggattaaatgctgatgcatctgctaaaccttcacatatcagaacatatttactatagaaagaatgaaaatgggacatttgtgtgtcacctatgtgaacattccaaaaatattttacaacaactaagtattttataaattttatgaactgaaatttagttcaagttctaggaaaatacaaaccttgctagatattataaaaatgatacaatatatattcatttcaggctcatcagaatatatctgttatcacttgacaagaatgaaaatgcaccattttgtagtgctttaaaatcaggaagatccagagtactaaaaatgacttcttccttgaagcttactcaccaacttcctcccagttactcactgcttctgccacaagcataaactaggacccagccagaactcccttgaaatatacacttgcaacgattactgcatctatcaaaatggttcagtgcctggctacaggttctgcagatcgactaagaatttgaaaagtcttgtttatttcaaaggaagcccatgtgaattctgcccagagttcatcccagatatgcagtctaagaatacagacagatcagcagagatgtattctaaaacaggaattctggcaatataacaaattgatttccaatcaaaacagatttacataccatacttatgtcaagaagttgttttgttttattgcatcctagattttatttttttgatttatggtttactttaagcataaaaaatttgtcaatacaactcttcccaaaaggcataaacaaaaattcataaaacttgcatcacttgagatacttcaggtatgaattcacaactttgttacaacttactatatatatgcacacatatatatatatttgggtatattgggggggttctaatttaagaaatgcataattggctatagacagacagttgtctggaatgaaaatcaatacttttgctataatcgattactgaaataattttactttccagtaaaactggcattataattttttttaatttttaaaacttcataattttttgccagactgacccatgtaaacatacaaattactaataattatgcacgtcacatctgtaataatggccttcatgtaaacatttttgtggtttacacataaaatctctaattacaaagctatattatctaaaattacagtaagcaagaaaattaatccaagctaagacaatacttgcaacatcaattcatcatctgtgacaaggactgcttaagtctctttgtggttaaaaaggaaaaaaaaaaaaaagacatgttggccagatgcggtggctcacacctgtaatcccagcactttgggaggctgaggtgggcggatcacccctggcctgcccaacatggtgaaaccccgtctctactaaaaacacaaaaattagctgggcgtggtggcgggcgcctgtaattccagctactcgggaggctgaggcaggagaattgctagaacccaggaggcagagattgcagtgagctgagattgcaccattgcactacagtctgggcaacaaaagtgaaactccatcttaaaaaaaaaaagacaatgttcgtgggtccaaacaagacttaatggaagtgagtctaaaaatgagctatgtgggccaggcgtagtggctcccacctgtaatcccagcactttgggaggccgaagcaggcagatcatgaggtcaggagatggagaccatcctggccaacacggtgaaatcctgtctctacaaaaattagctgggcgtggtggtgcctgcctgtaatcccagctactcagaaggctcaggcaggagaatcgcttgaaccagggagtcggtggctagagtgagccgagatttgcatcactgcactcctgcctggtgacagagcaagactccatctcaaaaaaaacaaacaaaaataaaagataaaaatgagctatgtgaattaaaagaggtataacaatagataaaccatattttatttaattcctagtaatgagtaatatttccaaacttctggaatgggcagaaattgctagttggcatatttttaccttttatattcagatacattaaaattctcaaaaaaaaacacctcaaagcagatgatccgccatctccttggataatttgtgttaactcaggataacagaaaaccaaaattatgagttactgatgcaatattcctaaatgtaaaaataattaaagctaatagtagattcatcttccaatttcatatcagtcttacaaataaactacatatataacttgcttgccttcccttctgagggataaagctgttagaagaattaaaatcagcattcttgactattcaaccaagggagggataaattattactcattctagggacatgggctcataactactacatgtgtaaggacatgaatttacccaatattacaatttttccttttattagtgtgtacagtggaagaatagacatgttcactctggacaaaaaaaaaattatacttatcagttatcagaagcacaatgctgaagacagtagttccataacaatttgaagtatgtgatcgaactagtagattatcttagtagtagtgaattattgtaaatgttagtaatttggcagccactgggcagaaaaataagaattgaggctcaatattgatattaatggtggtgattgacacataaattttatcaagtctacacaatataaaattacagaaaggtagaagagtataccagtacaacttcaacatatcttcactacaagggagtaaaatgacatggcctagttactatctaatgaactgcagaaaactaaaagaaaactccaaggcaactcttctctgctgatctggttggtccttttcctaccttttgcaatacccagatacaaacaatggatagaaaacaaagtagacttgtagtatgcaggtcacagtgctaaattcacagaaagaaacccctgaactgaactgctctatttcctggtggtcacaaagagtaattctggtttacacctacagattgatgtcaatctacaccctgttgataacagtgtggccaaggacaaaaaaaaggtgctccgttttaccaattctgtaaaaaattattggcagggtaagctcggctagggcaggattacatttctaggactaccatccccgaaatttagaagatattatatccacataaagcatatctttcacattaatttgcaaaaatctaaaagctttttcttagctcaagtgtgtccaagtttaccctggcagtttaaaacgatagttacaagcagcatgggttgtatcagacacatttgagggccaatttcatgtaagtgatattgggcaagttacttcaactatctgtgcctccaaggtcatactagtgtttatttacctaaagggtacctgttatgtaactttagggtgtttacattagataatgcctgcaaaatatttacttcaacgcctaaaacatagttaagtattcaataaatacctactattgtcactactaacttaaaagtttagagattaagagcagaatctggggtgagacaaacttaggttcaaatcctagtattgttgggtaatcttgggcaagttacttaacctctctgatttgtgtaatttaaaaaattagttaatatacataacagggcttagaagagtatctagcacatagcaccatttaagcatttgttattgctaacatgcaaacaatttaagggaaagaaattttttaaaaaggaagagggatttgcaaactaaaaacaatgagtatcttatgttcaaagaaaactaacaaacagccagctctagcaataattaaattcactatatactggggcaggcatcacaccccaaagctaaaagcgtctacctaggccaggcacggtggctcatgcctgtaatcccagcactttgggaagcagaggcgggcagatcgcttgagctcaggagttcaagaccagcctggacaacatggcaaaacaccatctctacaaaaaatacaaatattaggccgggcgcagtggctcacgcctgtaatcccagcactttgggaggccaaggcgggtggatcacctgagatcaggagttcgagagtagcctggccaacatggtgaaacctcgtctctattaaaaatacaaaaaattagccaggcatggtggcaggcgcctgtaatcccagctactcagggggatgaggtaggagaatcgcttgaacccgggaggcagaggttgcactgagccgagatcatgccactgtactccagcccgggcaacaagagcgaaactccatctcaaaaaataaataaataaataaataaaataaagtacaaatattagccagggatggtggtgcgcacctgtagtcccagctacttgggaggctgaagtgggagaatcccctgagcctggggagaatcacccgagcccgggaagtcgaggctgcagtgagcagtgattgtgccactgcactccatcctaggtgacagagtgagaccctgtctcaaaaaaaagaaattggcagaattaagtaagttgatgtttagagatgaaaaatcaacattttttcctcagcaactgaataaaaacaacagccactaccatttttttgagtacctatttgtagcctattttttaactggtattactcgagagagagagagctaggttcgagacagagctccttctcttaataactgtatgacctagggtatgtctgttagcctctctgaggcttcaaaggttcctcatctgtaaaatggtaataatcataccattgctacagggctgttttgaagactaattaggactatgtaagtaaacatgatgatggctattattactgttccccgccaggggccatgcaagggttgctgattcacatagactgtcttataatcctctcaataactccaagaggtagccagcacctcagatatacataaaatgacttaagcccagagaggtgaagtaagttgcccacagccacacaactagtaaatagcccaaacaagctggattcccagttagactccgttaatagcactgctctttaccttaagtcattacaatgcctaatatgaaatagaatcgcttctttcttagggttcaagtggttaattatttaatgtattcattcaacaaaccatcatcgaggacctcttacaagccaagtactgtgctaagtgctagagttacggcggtgattcctgcccttaaaaagttttagtgggagaaacaacaggtaaccaggtcattgccaaaacaacaaaaataatcataataaagcaggctaaagcatatttaactggccggggttttgactattttagcaagcatgatcagaacggttgaggagggaggccagcagcttggccggttcaacaaacaagaaaaaaccagtgagggtggagctaagataccagaggctgattacggttaagaatgttcttgaaggtaaggaccagattctcattttctatatcctggggcatcggtcagcatggaatctggattctagcacatgtgaatttcggcttgaaatgacctaatgccttttccctagttccttcgtgtgtcaaatacgcatggttaccgctaccagagctgtagtggggcttcaatgaggccatgagcatctccataaagatgaactacagtgtgtgcaaaactaaaggcaaaacctggtccccacacgccctcccaggtggtcgctttccgtgccgaggcccctccagaggtgccccgagaacctcaccatcgcaccccaaacttccagggaagggcctctcccgagaaagcccccacgcccccaccccgcgccatcattcccgaatctgccctcggcccctccccgcagcacgctcgcaggcggcacatgtcaaccaaaacgccatttccaccttctcttcccacacgcagtcctcttttcccagggctcccccgaggagggacccaccccaaaccccgccattccgtcctccctgccgccctcgcgtgacgtaaagccgaacccgggaaactggccgcccccgcctgcggggttccctgggcccggccgctctagaactagtggatcccaattgaaggcctggtctaaatgactccaaaatcaccacttaattcaagagactgatttccctgagtcaggccccttaaagcagctatttcaatgggacagggaaacaaccctaggatctggattagaatcacttgggggctgccacacccccagggctctgatcctgcccttctcccacacgcacattcacatactgctgcagtgaccttccatttctaatgggttcctgggccatctgtcaggtatagggaatggaaaaggggttggggaggctctgcttcagaaagtttgtgtcaggggctcccagagcctccacagatagatagcaggggtccccaccctaccatggcagctataaatgtgatcaacatttattggcctaggatacagcagttagcaaaatgcctgatgtagttcccactccgtggaggttgcaggctagctctttcctaatgagctttacagcagaagctgttttatcgttaagtgccccacagagacactttaccaggaggctgggagagttctccagatttgggagaggcgcagagacagtgtgtgagccgagccctgtctcagcaatccacctggaggagctagagtatcctcctccctttaccattcagaccgagagaaaaagcccagcttgtgtgcaccctcgtggggttaaggcgagctgttcctggtttaaagcctttcagtatttgttttgatgtaaggctctgtggtttgggggggaacatctgtaaacattattagttgatttggggtttgtctttgatggtttctatctgcaattatcgtcatgtatatttaagtgtctgttatagaaaacccacacccactgtcctgtaaacttttctcagtgtccagactttctgtaatcacattttaattgccacctcgtatttcacctctacatttgaaatctggcgtctgtttcaagccagtgtgttttttcttcgttctgtaataaacagccaggagaaaagtgcctctatgtttttatttttcaagggagtattcagtacctacaaacccaagtcaggaagcctgctagtggctttggttctttcagaggctgctcgatgccttgtgtgtcagaaagaaagattcagcagttttgcatcatggcaaagaagcctgttattttggggctcagcccctcattttatagaggatgaaacagagggggatgggaggtcacaaagacaactgccccgggagcaggtgtgggggagacttgccctgagggtctagacgctctgcaccaccgtcctgtctcccttgctgaagaccacacatgcccttctttgaccagaccctgccacctgataggccaggacctggtaggcgggtacccaggtttcatggatggaaccacatctccccaaaagtggggaggtagctactgggatgcacgcctcccgccatgtgctataggagagcagctgaagcaacagttgggatcagatgtagtcacaattgaatgcatcatcacatttatccctctaagtggctgggagagttgatatcctcatccctaaggtacaaaatgttccaatttgatcagtggctttcaggagctgagaaaggcatgtgctctgaggcagagctgttatgtcccgcagagcctaaaaatgctctaagaacatgctccctgccaaaattctcaatggctgtgacaagggacaacgatcgaccaatgggggtggaagcagacctccgcagtccaggggccagagctaggacagaggggtcggagaaagagtcattttcccaacactccagctcttggccagtcctcacacagtcccctcctgcttcctgctgagagagatatcctcataggtctgggtaaagtccttcagtcagctttcattccctgtcaccaactttgtctctgttctccctgcccgtctcaggcagcactcctcaggaaacctctccaagagccagcctcactgcagcgcccactattgtccctctgcctcaagtgtcccatccatgccaggccccaggcaggctgcagctttccctcagggccacaccaaagcacttgggctcagctgtgctgtccccctccatcactgagctcaggggcagcaggggtggggtgccaggaggcccattcacccttctctggctctgtgttggacccacctgcccagccactgctgcttagaacctacccgctgggaaaatgaagccctcccggaggggccacctcaacctgagagcctcacggatcacagttgtccccactcagctctgccagccctcagagacccatagataaaagctgagcttggctcgcagagctggttccatcttccattcccagagggttcaacttcctaccccaaccacacagggaacctcaaggctgagccagtgtgggctgcagtgcagaccagcttcctggacacgtcctgccacctgaccccaggctggcctcactgcccctggcactcctgaccctatcctcattcctcctggcagtgcgtgttctgccattccgctttcccttagctgtcctctcactgtactgtcagcttctccttttccaggtgccccccaggggctttccacatgaccctgtcaccccacagcccatccagcaccaattccagctctctgccacccttcaaaggagtgacagtgccctgcttcacctcccactcacccctcaacccagagcaatctggctccagtcttgcctccttccccctaagtactctagtcacagttccaaattcctcctggtcataaagccaaatgaagcttcctggtcctcagcggacttgccacttcagcagtactggactctctcctcccagaaacctgtttccccttggctcctggagcccacactctgctggaatccttctgcctctctggcctgtagcctggccctctctcccaacctgaggtccattctctcctgctcctccacaagatgttgctccttccattacttcctccctctcaaccaaagctccttcattagctctttatcttctggtttcttcccctgggcagacgaatggattcaagagcctgtggcccagcagcccagcactccaggatctcagcacttcagcatcccagtaccctagcatctcaataccccagcaccccagcaccatagtattccagcaccccattgtccaagcatctcagcactccagcatcccagcaccccaacactccagcagcccagaatctcagcaccctagcactgcagcatctcaggaccccagcacttcagcatcccagcacactagtactccagcatctcggcaccccagcacctaggcatcccaacacccagcaccccagcacttaagcatcccaccactacagtatctcaacactccagcaccccagcaccatagtgttccagcaccccagcatcccaacaccccagcacttaagcatcccaacacctcggcatcccaacaccccagcactgcagcatctcagcaccttagcatcccagtgccctagcatctcaatgctccagcacaccagtactacagtattccagcaccccagcactccagcatctcagcactgcagcactgcagcactccagcatcccaaaatcccagcatcccaacaccccagcagaccagcagaccagcatctcagcaccgcagcatccaaggactatcccagcatcccagcaacccagcacctcagcatcccaacaccccagcatttcagcatggcaacaccccagtaccccagcacttcagcaccccagtatcccagcatctcagcgacccagtatcacaaaacctcagcatcctagcaccccagcaccccagcaccttagcaccttagcatcccagcatctcagcgcctcagcatcttgatattctggctgaggtcagcgtggtgtatctagtcagggtcctaactttcacttcgcagggaaatgctgctggactgggtctcatgttgggctgaagctctctagaccccttgaagacagcataaaagagcttggagacgctgggtgtcccccatggaagagttcactctcatcctgctttgacaacagccttctctggggtccctcacgggcccctctttcttactgcaagtttgtctctgagaagactgtgatgcagaagtcactcagctgcctgtggctcctgaagagctgaaggtggaggcctgtaggcctccctatgagaggcgcagaaaaaaccatgattgctagtggggaggtgctccctctacaacccactccataatctgcccccgcccagctctgaggccagccccaggggaaaatgccagatccccagggaggtgtgtgagacctcaggggctccctcctcccttacagcaggctcaggcccctgggggcctcagggccaaggtctgtgggtaagctactatctctcacttgtcctctagccacaaaagccagggagatctggcaatggacatgaggttctgaagaagcacatatgactggcttcctaatgcgtggttgttcagtgattcaataaacacgcatgggccaggcatggggaaatagacaaacatgatccccaacctctcccagagtgaactgggagggaggagtgttcatccctcaggattacaccagagaaacaaaccagcaggagatatatatggttttggggggtcaagaaagaggaaaaacctggcaaggcaagtccaaaatcataggacaggctgtcaggaagggcagcctggaacctctcaagcaggagctgatgctgcagtccacaggcagaatttcttcttcctcggggaaatctcagctttgttcttaaggcctttcaactgattggctgaggtctgccccttcccccacattctccaggataatcttccttacttaaagtcaactattaatcacagctacaaaatcccttcacagctacacatagatcagtgtttgattgacgaacagcccctacagcctagccaagttgacacataaaactaaccatcacagggggacaaatgatgtaaacacatcaacaaataaaacagtaacaagttaaggtctatggaaaaaacacagaaggggcagagagaaagaaagcaagaaggagagtcccagtttgctagggcttgtgggaagtggggagcagttctctttagctaggatatttgggaaaggcatatctgaaggagtgatatttgagcttagattaaaagatgggaaggagcaagccatgcaaagagctaggatgttccaagcagagacggaacagcaagtgcaaatgtcaggaggaatagaaggaggctggtgggtggggtccagtgagcaagaggagggcaggcaggagaggggatggggaggtgggcaggcccagaccacccagggccctggagactatcctgatccaacaagggaagccttgagtcacttcagtgtccatgtggagaatggacctcagactgaatgagggaggcagtaaggagggcctctacctccagggcttcgccctgtggactgcgcatagacatctccaactcagaaagtctgaaccaaactttccatagttcccccaagtctgggcatcctcctactcagtgaaaggcagccatcacacctccctgccctgctcccggatgccccaaatcctcttggtctccaagtccagaacctgagacttgtccttgatgtttgtctttccctcaccctttctgtattctgggaagatgggtttttttcccccagatgaatctgtaaaacttctgtgatcacaataaaaattctggcagtattattttctggaacatgacaaagtgattcaaaattatttatctggaagactacaaaacaagaatagccaggaaatttctaaaaagaaagaagaaggaggaggagaaagaaggaggaggaaaaggaggagaagaagaaaagaaaaagaaccaagaaagggttctagctctaccaaatattaaaacatatcatgaagctatttaaaacaatatggttgtggatactgaaaaagatgtgaataaagtggaaggaaaataaatagaaatgcacatggggattgagactgtgaaaaaggcagcatctcacatcagtgagggatgttcaacacctggtgttgggaaaactggctagtcatttaaaccaaacaactgggtcctctacctcactcctgacattaagatacatttagatgattcaaagagtaagacagaaaaaataacacgtgaaaacactatcagaaaacaacgtgggccaggtgtggtgggtcacgcctgtaatcccagcactttgggaggccgaggcagacagatcacctgaggtggggagttcaagaccagcctgaccaacatggtgaaatcctgtctctactaaaaatacaaaattagctgagcgtggtggcgcatgcctgtaatcccagctactcaggaggccgaggcaggagaatcacttgaacctgggaggcagaggttgtggtgagccgagatcacgccattgcactccagcctgggcaacaagagtgaaaatccatctaaaaaaaaaaaaaaaagccaaggtggatatttttatagtatcagggtagatcaagcttctccaatcatgacatgaaacccagaaaccataaaagaaaagaatgataaaattgcccacgtaaagtaaaaagcttgcacacagaaaaacaccatacaggttacaagatgagcagcaaaatcagagaaaaaacattgcaattcaggacacacagaggctattgttcctaatatttaaaaataaaagtagtggattgtctacaaaaagatgaagacaagaatttcagaaaaccaaatactgcatgttttcacttacaagtggaagctaaacactgagtacacgtgtacacaaagaatggaaccataggccaggcaccgtggctcacgcctgtaatcccagtactttgcgaggccgaagcgggcggatcacctgaggtgaggagttcgagaccatcctggccaacatggtgaaacccagtctctactaaaaatacaaaaattagccgggcgtggtggtgggtgcctgtaatcccagctactcgggaggctgcggcagtagaatcgcttgaaccctggaggtggaccttgcagtgagccgagatcgcaccactgcactccagcctgggcaacagagtgagactccatctcaaaaaaaaaaaaaaggaatagaacaatagacactggggcctacttgagggaggagggtgaggatcaaaaacctgcctatcaggtactatgcttattacctgggtggtgaaataatctgtacaccaaaccccagtgacatgcaatttaccgatgtaacaaacctgcccatgtacccgctgaacctaaaataaaagttggaaaaaaatatagaaattttctttgtaatagccaaaaactgcaaacagcccaggtgtctattagtagaatgcataaacaaactcgggcatgttcatacaatgtaaaactactcatcaataaaaagtgatacttctcagcaatgaaaagaaactagctactgataccagctacaacatggatggatttcaagtgctttatgatgagagcaagaagccagacacaaaagtgtctatatatatatacagtatatatacgtatatatacacatatatacagtatatatatacatatacatgtatatatatactgtatatatactgtatatatatacacagtatatatatacatatatacagtgtatatatactgtgtatatatacatgtatatatactgtgtatatatacatgtatatatactgtgtatatatacatgtatatatactgtgtatatatacatgtatatatatgtatactgtatatatactgtatatatatatacacatatatacagtatatatatacagtatatactgtatatatacagtatatacgtgtatatatacatatatacagtatatatgtaaatatacatatatacagtatatatgtaaatatacatatatacatgtatatatatacactatatatatacatatatagtgtatatatacatatatacatgtatatatttactatatgattccatttatataaagtgccaaaacagtcaaaaataatctatgtggaaaaaatcaacaaagggatcccccgggctgcaggaattcgatggcgcgccgacgtcgcatgcagttagggataacagggtaatacgaccatggcatgtcctctagactcgagcggccgcaataaaatatctttattttcattacatctgtgtgttggttttttgtgtgaatcgtaactaacatacgctctccatcaaaacaaaacgaaacaaaacaaactagcaaaataggctgtccccagtgcaagtgcaggtgccagaacatttctctatcgaaggatctgcgatcgctccggtgcccgtcagtgggcagagcgcacatcgcccacagtccccgagaagttggggggaggggtcggcaattgaaccggtgcctagagaaggtggcgcggggtaaactgggaaagtgatgtcgtgtactggctccgcctttttcccgagggtgggggagaaccgtatataagtgcagtagtcgccgtgaacgttctttttcgcaacgggtttgccgccagaacacagctgaagcttcgaggggctcgcatctctccttcacgcgcccgccgccctacctgaggccgccatccacgccggttgagtcgcgttctgccgcctcccgcctgtggtgcctcctgaactgcgtccgccgtctaggtaagtttaaagctcaggtcgagaccgggcctttgtccggcgctcccttggagcctacctagactcagccggctctccacgctttgcctgaccctgcttgctcaactctacgtctttgtttcgttttctgttctgcgccgttacagatccaagctgtgaccggcgcctacgtaagtgatatctactagatttatcaaaaagagtgttgacttgtgagcgctcacaattgatacttagattcatcgagagggacacgtcgactactaaccttcttctctttcctacagctgagatcaccggcgaaggagggccaccatgggtcaccagcagttggtcatctcttggttttccctggtttttctggcatctcccctcgtggccatatgggaactgaagaaagatgtttatgtcgtagaattggattggtatccggatgcccctggagaaatggtggtcctcacctgtgacacccctgaagaagatggtatcacctggaccttggaccagagcagtgaggtcttaggctctggcaaaaccctgaccatccaagtcaaagagtttggagatgctggccagtacacctgtcacaaaggaggcgaggttctaagccattcgctcctgctgcttcacaaaaaggaagatggaatttggtccactgatattttaaaggaccagaaagaacccaaaaataagacctttctaagatgcgaggccaagaattattctggacgtttcacctgctggtggctgacgacaatcagtactgatttgacattcagtgtcaaaagcagcagaggctcttctgacccccaaggggtgacgtgcggagctgctacactctctgcagagagagtcagaggggacaacaaggagtatgagtactcagtggagtgccaggaggacagtgcctgcccagctgctgaggagagtctgcccattgaggtcatggtggatgccgttcacaagctcaagtatgaaaactacaccagcagcttcttcatcagggacatcatcaaacctgacccacccaagaacttgcagctgaagccattaaagaattctcggcaggtggaggtcagctgggagtaccctgacacctggagtactccacattcctacttctccctgacattctgcgttcaggtccagggcaagagcaagagagaaaagaaagatagagtcttcacggacaagacctcagccacggtcatctgccgcaaaaatgccagcattagcgtgcgggcccaggaccgctactatagctcatcttggagcgaatgggcatctgtgccctgcagtgttcctggagtaggggtacctggggtgggcgccagaaacctccccgtggccactccagacccaggaatgttcccatgccttcaccactcccaaaacctgctgagggccgtcagcaacatgctccagaaggccagacaaactctagaattttacccttgcacttctgaagagattgatcatgaagatatcacaaaagataaaaccagcacagtggaggcctgtttaccattggaattaaccaagaatgagagttgcctaaattccagagagacctctttcataactaatgggagttgcctggcctccagaaagacctcttttatgatggccctgtgccttagtagtatttatgaagacttgaagatgtaccaggtggagttcaagaccatgaatgcaaagctgctgatggatcctaagaggcagatctttctagatcaaaacatgctggcagttattgatgagctgatgcaggccctgaatttcaacagtgagactgtgccacaaaaatcctcccttgaagaaccggatttttataaaactaaaatcaagctctgcatacttcttcatgctttcagaattcgggcagtgactattgatagagtgatgagctatctgaatgcttcctaaaaagcgaggtccctccaaaccgttgtcatttttataaaactttgaaatgaggaaactttgataggatgtggattaagaactagggaggggctagctcgacatgataagatacattgatgagtttggacaaaccacaactagaatgcagtgaaaaaaatgctttatttgtgaaatttgtgatgctattgctttatttgtgaaatttgtgatgctattgctttatttgtaaccattataagctgcaataaacaagttaacaacaacaattgcattcattttatgtttcaggttcagggggaggtgtgggaggttttttaaagcaagtaaaacctctacaaatgtggtagatccatttattagctaggagtttcagaaaagggggcctgagtggccccttttttcaacttaattaacctgcagggcctgaaataacctctgaaagaggaacttggttaggtaccttctgaggctgaaagaaccagctgtggaatgtgtgtcagttagggtgtggaaagtccccaggctccccagcaggcagaagtatgcaaagcatgcatctcaattagtcagcaaccaggtgtggaaagtccccaggctccccagcaggcagaagtatgcaaagcatgcatctcaattagtcagcaaccatagtcccactagtttcatcaccaccgccacccccccgcccccccgccatctgaaagggttctaggggatttgcaacctctctcgtgtgtttcttctttccgagaagcgccgccacacgagaaagctggccgcgaaagtcgtgctggaatcacttccaacgaaaccccaggcatagatgggaaagggtgaagaacacgttgtcatggctaccgtttccccggtcacggaataaacgctctctaggatccggaagtagttccgccgcgacctctctaaaaggatggatgtgttctctgcttacattcattggacgttttcccttagaggccaaggccgcccaggcaaaggggcggtcccacgcgtgaggggcccgcggagccatttgattggagaaaagctgcaaaccctgaccaatcggaaggagccacgcttcgggcatcggtcaccgcacctggacagctccgattggtggacttccgccccccctcacgaatcctcattgggtgccgtgggtgcgtggtgcggcgcgattggtgggttcatgtttcccgtcccccgcccgcgagaagtgggggtgaaaagcggcccgacctgcttggggtgtagtgggcggaccgcgcggctggaggtgtgaggatccgaacccaggggtggggggtggaggcggctcctgcgatcgaaggggacttgagactcaccggtcgcacgtcatgaatctagaaccatggcttcgtaccccggccatcagcacgcgtctgcgttcgaccaggctgcgcgttctcgcggccatagcaaccgacgtacggcgttgcgccctcgccggcagcaagaagccacggaagtccgcccggagcagaaaatgcccacgctactgcgggtttatatagacggtccccacgggatggggaaaaccaccaccacgcaactgctggtggccctgggttcgcgcgacgatatcgtctacgtacccgagccgatgacttactggcgggtgctgggggcttccgagacaatcgcgaacatctacaccacacaacaccgccttgaccagggtgagatatcggccggggacgcggcggtggtaatgacaagcgcccagataacaatgggcatgccttatgccgtgaccgacgccgttctggctcctcatatcgggggggaggctgggagctcacatgccccgcccccggccctcaccctcatcttcgaccgccatcccatcgccgccctcctgtgctacccggccgcgcgataccttatgggcagcatgaccccccaggccgtgctggcgttcgtggccctcatcccgccgaccttgcccggcacaaacatcgtgttgggggcccttccggaggacagacacatcgaccgcctggccaaacgccagcgccccggcgagcggcttgacctggctatgctggccgcgattcgccgcgtttacgggctgcttgccaatacggtgcggtatctgcagggcggcgggtcgtggcgggaggattggggacagctttcggggacggccgtgccgccccagggtgccgagccccagagcaacgcgggcccacgaccccatatcggggacacgttatttaccctgtttcgggcccccgagttgctggcccccaacggcgacctgtacaacgtgtttgcctgggccttggacgtcttggccaaacgcctccgtcccatgcacgtctttatcctggattacgaccaatcgcccgccggctgccgggacgccctgctgcaacttacctccgggatgatccagacccacgtcaccaccccaggctccataccgacgatctgcgacctggcgcgcacgtttgcccgggagatgggggaggctaactgagtataccctaggattatccctaatacctgccaccccactcttaatcagtggtggaagaacggtctcagaactgtttgtttcaattggccatttaagtttagtagtaaaagactggttaatgataacaatgcatcgtaaaaccttcagaaggaaaggagaatgttttgtggaccactttggttttcttttttgcgtgtggcagttttaagttattagtttttaaaatcagtactttttaatggaaacaacttgaccaaaaatttgtcacagaattttgagacccattaaaaaagttaaatgagaaacctgtgtgttcctttggtcaacaccgagacatttaggtgaaagacatctaattctggttttacgaatctggaaacttcttgaaaatgtaattcttgagttaacacttctgggtggagaatagggttgttttccccccacataattggaaggggaaggaatatcatttaaagctatgggagggtttctttgattacaacactggagagaaatgcagcatgttgctgattgcctgtcactaaaacaggccaaaaactgagtccttgggttgcatagaaagctgcctgcaggcgttacataacttacggtaaatggcccgcctggctgaccgcccaacgacccccgcccattgacgtcaataatgacgtatgttcccatagtaacgccaatagggactttccattgacgtcaatgggtggagtatttacggtaaactgcccacttggcagtacatcaagtgtatcatatgccaagtacgccccctattgacgtcaatgacggtaaatggcccgcctggcattatgcccagtacatgaccttatgggactttcctacttggcagtacatctacgtattagtcatcgctattaccatgatgatgcggttttggcagtacatcaatgggcgtggatagcggtttgactcacggggatttccaagtctccaccccattgacgtcaatgggagtttgttttgactagttaccggcggaaacggtctcgggttgagaggtcacccgagggacaggcagctgctgaaccaataggaccggcgcacagggcggatgctgcccctcattggcggccgttgagagtgaccaagagccaatgagtcagcccggggggcgtagcagtgacgtaagttgcggaggaggccgcttcgaatcggcagcggccagcttggtggcatggaccaatcagcgtcctccaacgaggagcgccttcgccaatcggaggcctccacgacggggctggggggagggtatataagccgagtcggcggcggcgcgctccacacgggccgagaccacagcgacgggagcgtctgcctctgcggggccgagaggtaagcgccgcggcctgccctttccaggccaactcggagcccgtctcgtggctccgcctgatcgggggctcctgtcgccctcagatcggtcggaacgccgtcgcgctccgggactacaagcctgttgctgggcccggagactgccgaaggaccgctgagcactgtcctcagcgccggcaccatggattggatctggcggatcctgttccttgtgggagctgccacaggcgcccattctgaagttcagctggttcagtctggcgccgaagtgaagaaacctggcgcctctgtgaaggtgtcctgcaaagcttctggcggcaccttcagcagctacgccatctcttgggttcgacaggcccctggacaaggcctggaatggatgggcagaatcatccccatcctgggaatcgccaactacgcccagaaattccagggcagagtgaccatcaccgccgacaagagcacaagcaccgcctacatggaactgagcagcctgagaagcgaggacaccgccgtgtactactgtgccagaagcggccacggctacagctacggcgcctttgattattggggccagggcaccctggtcaccgtttctagcggaggcggaggtagtggtggcggaggttcaggcggcggaggatctcaatctgtgctgacacagcctccaagcgtgtcaggtgctcctggccagagagtgacaatcagctgtacaggcagcagcagcaacatcggagccggctatgacgtgcactggtatcagcagctgcctggcacagcccctaaactgctgatctacggcaacagcaacagacccagcggcgtgcccgatagattttccggctctaagagcggcacaagcgccagcctggctattactggactgcaggccgaggacgaggccgactactactgtcagagctacgacagcagcctgtccggcagctacgttgtgtttggcggcggaacaaagctgaccgtgctggaagccaagagctgcgacaagacccacacctgtcctccatgtcctgctccagaactgctcggcggaccttccgtgttcctgtttcctccaaagcctaaggacaccctgatgatcagcagaacccctgaagtgacctgcgtggtggtggatgtgtcccacgaggacccagaagtgaagttcaattggtacgtggacggcgtggaagtgcacaacgccaagaccaagcctagagaggaacagtacaacagcacctacagagtggtgtccgtgctgacagtgctgcaccaggattggctgaacggcaaagagtacaagtgcaaggtgtccaacaaggccctgcctgctcctatcgagaaaaccatcagcaaggccaagggccagcctagggaaccccaggtttacacactgccacctagcagggacgagctgaccaagaatcaggtgtccctgacctgcctggtcaagggcttctacccttccgatatcgccgtggaatgggagagcaatggccagccagagaacaactacaagacaacccctcctgtgctggacagcgacggctcattcttcctgtactccaagctgactgtggacaagagccggtggcagcagggcaatgtgttcagctgtagcgtgatgcacgaggccctgcacaaccactacacacagaagtccctgtctctgagccccggaaaaggtggcggtggctcttacccttacgacgtgccagattacgccggctatccctacgatgtgcctgactatgctggctacccctatgacgtccccgactacgcttaactagctacggaattccggctagctggccagacatgataagatacattgatgagtttggacaaaccacaactagaatgcagtgaaaaaaatgctttatttgtgaaatttgtgatgctattgctttatttgtaaccattataagctgcaataaacaagttaacaacaacaattgcattcattttatgtttcaggttcagggggaggtgtgggaggttttttaaagcaagtaaaacctctacaaatgtggtatggaaatgttaattaactagccatgaccaaaatcccttaacgtgagttttcgttccactgagcgtcagaccccgtagaaaagatcaaaggatcttcttgagatcctttttttctgcgcgtaatctgctgcttgcaaacaaaaaaaccaccgctaccagcggtggtttgtttgccggatcaagagctaccaactctttttccgaaggtaactggcttcagcagagcgcagataccaaatactgttcttctagtgtagccgtagttaggccaccacttcaagaactctgtagcaccgcctacatacctcgctctgctaatcctgttaccagtggctgctgccagtggcgataagtcgtgtcttaccgggttggactcaagacgatagttaccggataaggcgcagcggtcgggctgaacggggggttcgtgcacacagcccagcttggagcgaacgacctacaccgaactgagatacctacagcgtgagctatgagaaagcgccacgcttcccgaagggagaaaggcggacaggtatccggtaagcggcagggtcggaacaggagagcgcacgagggagcttccagggggaaacgcctggtatctttatagtcctgtcgggtttcgccacctctgacttgagcgtcgatttttgtgatgctcgtcaggggggcggagcctatggaaaaacgccagcaacgcggcctttttacggttcctggccttttgctggccttttgctcagggttcgaaatcgataagcttggatccggagagctcccaacgcgtcggctagctagtagggataacagggtaataagcgtcgacggcgcgcccctaggggccggccttaattaaatcaagcttatcgataccgtcgaacctcgagggggggcatcactccgccctaaaacctacgtcacccgccccgttcccacgccccgcgccacgtcacaaactccaccccctcattatcatattggcttcaatccaaaataaggtatattattgatgatgttt

SEQ ID NO: 121 - DNA, 30881 bp, Artificial Sequence
  HDAdCD44v6BiTE
aaacatcatcaataatataccttattttggattgaagccaatatgataatgagggggtggagtttgtgacgtggcgcggggcgtgggaacggggcgggtgacgtaggttttagggcggagtaacttgtatgtgttgggaattgtagttttcttaaaatgggaagtgacgtaacgtgggaaaacggaagtgacgatttgaggaagttgtgggttttttggctttcgtttctgggcgtaggttcgcgtgcggttttctgggtgttttttgtggactttaaccgttacgtcattttttagtcctatatatactcgctctgcacttggcccttttttacactgtgactgattgagctggtgccgtgtcgagtggtgtttttttaataggttttcttttttactggtaggcgcgccgtcgacgcttattaccctgttatccctactagctagccgacgcgttgggagctctccggatccaagcttatcgatttcgaacccaaatggatctaccacatttgtagaggttttacttgctttaaaaaacctcccacacctccccctgaacctgaaacataaaatgaatgcaattgttgttgttaacttgtttattgcagcttataatggttacaaataaagcaatagcatcacaaatttcacaaataaagcaatagcatcacaaatttcacaaataaagcatttttttcactgcattctagttgtggtttgtccaaactcatcaatgtatcttatcatgtcgagctagctagtcaggacttcagttccagctttgtgccggctccgaaggtcagcgggttgctagaccattgctgacagtaatatgtggcggcatcctcggcttccatagagctgattgtcaggctgtagctggtgccagatccagatccgctgaatctgtagggcacgccggaggccactttgcttgtgtcgtagatccaccgcttggggcttgtgccagacttctgctgataccagttcatgtaggacacgctgctgctggctctgcatgtcatggtcactttctcgcctggggaagcgctcatgatggcggggctttgtgtcagctgaatatcggagccaccaccaccgcttccaccaccacctgaaccgcctccgccactagaaactgtcagggttgtgccctggccccagtaatccagacagtagtggtcgtcgtagtaccgggcacaatagtacacagcgctatcttcagaggtcaggctggacagctgcatgtaggcggtagagctgctcttgtcggtggtcagtgtggccttgtccttgaacttctggttgtaattggtgtagccccggctggggttgatgtagccgatccattccagtccttggccaggcctctgcttgacccagtgcatggtgtaccgggtgaatgtgtagccgctggtcttgcaggacatcttcacagaggcgccaggtctagccagttcggcgccagactgttgcagcttgatatcggatccgccacctccgccagatgacactgtgaccagtgttcctctgccccagtagtcgaggccctgtctggcgcaataatacacggcggtgtcctcggctctcagggagttcatctgcaggtacaggctgttcttggcgttgtcccggctgatggtgaatctgcccttgatgctgtccaggtagtaggtgtagctgccgccgctgctgattgtggacacccattcaaggcctttgccaggagcctgtcggacccagctcatatcgtagctgctgaaggtgaagccggaagcggcacagctcagtctcagagagccgccaggtttcacaagtccgccgcctgattccaccagctgcacttcagatccaccaccgccactacctccgcctccgcttcctccgccgccagatcctccgccacctctcttgatttccaccttggtgcctccgccaaatgtcaggggattgctggaccactgcaggcagtagtacacggcgaagtcctcaggttccaggctgcttatggtcagggtgaaatcggtgccgctgccagagccagaaaatctggcaggcactccgctggccagattgctggtcaggtagatcaggattctaggggcctgtccgggcttctgctgcagccagtagatgtagttgatggagctgctggcgctacagctcagggtagctctctcgccagggctcagagacagtgtggctggagactgtgtcagcacgatctcgccggtggtatcaggcagccaaagcagcagcaggaacagcagctgagcaggggcttccatggtggccctccttcgccggtgatctcagctgtaggaaagagaagaaggttagtagtcgacgtgtccctctcgatgaatctaagtatcaattgtgagcgctcacaagtcaacactctttttgataaatctagtagatatcacttacgtaggcgccggtcacagcttggatctgtaacggcgcagaacagaaaacgaaacaaagacgtagagttgagcaagcagggtcaggcaaagcgtggagagccggctgagtctaggtaggctccaagggagcgccggacaaaggcccggtctcgacctgagctttaaacttacctagacggcggacgcagttcaggaggcaccacaggcgggaggcggcagaacgcgactcaaccggcgtggatggcggcctcaggtagggcggcgggcgcgtgaaggagagatgcgagcccctcgaagcttcagctgtgttctggcggcaaacccgttgcgaaaaagaacgttcacggcgactactgcacttatatacggttctcccccaccctcgggaaaaaggcggagccagtacacgacatcactttcccagtttaccccgcgccaccttctctaggcaccggttcaattgccgacccctccccccaacttctcggggactgtgggcgatgtgcgctctgcccactgacgggcaccggagcgatcgcagatccttcgatagagaaatgttctggcacctgcacttgcactggggacagcctattttgctagtttgttttgtttcgttttgttttgatggagagcgtatgttagttacgattcacacaaaaaaccaacacacagatgtaatgaaaataaagatattttattgcggccgctcgagtctagaggacatgccatggtcgtattaccctgttatccctaactgcatgcgacgtcggcgcgccatcgaattcctgcagcccgggggatccctttgttgattttttccacatagattatttttgactgttttggcactttatataaatggaatcatatagtaaatatatacatgtatatatgtatatatacactatatatgtatatatatagtgtatatatatacatgtatatatgtatatttacatatatactgtatatatgtatatttacatatatactgtatatatgtatatatacacgtatatactgtatatatacagtatatactgtatatatatactgtatatatgtgtatatatatatacagtatatatacagtatacatatatatacatgtatatatacacagtatatatacatgtatatatacacagtatatatacatgtatatatacacagtatatatacatgtatatatacacagtatatatacactgtatatatgtatatatatactgtgtatatatatacagtatatatacagtatatatatacatgtatatgtatatatatactgtatatatgtgtatatatacgtatatatactgtatatatatatagacacttttgtgtctggcttcttgctctcatcataaagcacttgaaatccatccatgttgtagctggtatcagtagctagtttcttttcattgctgagaagtatcactttttattgatgagtagttttacattgtatgaacatgcccgagtttgtttatgcattctactaatagacacctgggctgtttgcagtttttggctattacaaagaaaatttctatatttttttccaacttttattttaggttcagcgggtacatgggcaggtttgttacatcggtaaattgcatgtcactggggtttggtgtacagattatttcaccacccaggtaataagcatagtacctgataggcaggtttttgatcctcaccctcctccctcaagtaggccccagtgtctattgttctattccttttttttttttttgagatggagtctcactctgttgcccaggctggagtgcagtggtgcgatctcggctcactgcaaggtccacctccagggttcaagcgattctactgccgcagcctcccgagtagctgggattacaggcacccaccaccacgcccggctaatttttgtatttttagtagagactgggtttcaccatgttggccaggatggtctcgaactcctcacctcaggtgatccgcccgcttcggcctcgcaaagtactgggattacaggcgtgagccacggtgcctggcctatggttccattctttgtgtacacgtgtactcagtgtttagcttccacttgtaagtgaaaacatgcagtatttggttttctgaaattcttgtcttcatctttttgtagacaatccactacttttatttttaaatattaggaacaatagcctctgtgtgtcctgaattgcaatgttttttctctgattttgctgctcatcttgtaacctgtatggtgtttttctgtgtgcaagctttttactttacgtgggcaattttatcattcttttcttttatggtttctgggtttcatgtcatgattggagaagcttgatctaccctgatactataaaaatatccaccttggcttttttttttttttttagatggattttcactcttgttgcccaggctggagtgcaatggcgtgatctcggctcaccacaacctctgcctcccaggttcaagtgattctcctgcctcggcctcctgagtagctgggattacaggcatgcgccaccacgctcagctaattttgtatttttagtagagacaggatttcaccatgttggtcaggctggtcttgaactccccacctcaggtgatctgtctgcctcggcctcccaaagtgctgggattacaggcgtgacccaccacacctggcccacgttgttttctgatagtgttttcacgtgttattttttctgtcttactctttgaatcatctaaatgtatcttaatgtcaggagtgaggtagaggacccagttgtttggtttaaatgactagccagttttcccaacaccaggtgttgaacatccctcactgatgtgagatgctgcctttttcacagtctcaatccccatgtgcatttctatttattttccttccactttattcacatctttttcagtatccacaaccatattgttttaaatagcttcatgatatgttttaatatttggtagagctagaaccctttcttggttctttttcttttcttcttctcctccttttcctcctccttctttctcctcctccttcttctttctttttagaaatttcctggctattcttgttttgtagtcttccagataaataattttgaatcactttgtcatgttccagaaaataatactgccagaatttttattgtgatcacagaagttttacagattcatctgggggaaaaaaacccatcttcccagaatacagaaagggtgagggaaagacaaacatcaaggacaagtctcaggttctggacttggagaccaagaggatttggggcatccgggagcagggcagggaggtgtgatggctgcctttcactgagtaggaggatgcccagacttgggggaactatggaaagtttggttcagactttctgagttggagatgtctatgcgcagtccacagggcgaagccctggaggtagaggccctccttactgcctccctcattcagtctgaggtccattctccacatggacactgaagtgactcaaggcttcccttgttggatcaggatagtctccagggccctgggtggtctgggcctgcccacctccccatcccctctcctgcctgccctcctcttgctcactggaccccacccaccagcctccttctattcctcctgacatttgcacttgctgttccgtctctgcttggaacatcctagctctttgcatggcttgctccttcccatcttttaatctaagctcaaatatcactccttcagatatgcctttcccaaatatcctagctaaagagaactgctccccacttcccacaagccctagcaaactgggactctccttcttgctttctttctctctgccccttctgtgttttttccatagaccttaacttgttactgttttatttgttgatgtgtttacatcatttgtccccctgtgatggttagttttatgtgtcaacttggctaggctgtaggggctgttcgtcaatcaaacactgatctatgtgtagctgtgaagggattttgtagctgtgattaatagttgactttaagtaaggaagattatcctggagaatgtgggggaaggggcagacctcagccaatcagttgaaaggccttaagaacaaagctgagatttccccgaggaagaagaaattctgcctgtggactgcagcatcagctcctgcttgagaggttccaggctgcccttcctgacagcctgtcctatgattttggacttgccttgccaggtttttcctctttcttgaccccccaaaaccatatatatctcctgctggtttgtttctctggtgtaatcctgagggatgaacactcctccctcccagttcactctgggagaggttggggatcatgtttgtctatttccccatgcctggcccatgcgtgtttattgaatcactgaacaaccacgcattaggaagccagtcatatgtgcttcttcagaacctcatgtccattgccagatctccctggcttttgtggctagaggacaagtgagagatagtagcttacccacagaccttggccctgaggcccccaggggcctgagcctgctgtaagggaggagggagcccctgaggtctcacacacctccctggggatctggcattttcccctggggctggcctcagagctgggcgggggcagattatggagtgggttgtagagggagcacctccccactagcaatcatggttttttctgcgcctctcatagggaggcctacaggcctccaccttcagctcttcaggagccacaggcagctgagtgacttctgcatcacagtcttctcagagacaaacttgcagtaagaaagaggggcccgtgagggaccccagagaaggctgttgtcaaagcaggatgagagtgaactcttccatgggggacacccagcgtctccaagctcttttatgctgtcttcaaggggtctagagagcttcagcccaacatgagacccagtccagcagcatttccctgcgaagtgaaagttaggaccctgactagatacaccacgctgacctcagccagaatatcaagatgctgaggcgctgagatgctgggatgctaaggtgctaaggtgctggggtgctggggtgctaggatgctgaggttttgtgatactgggtcgctgagatgctgggatactggggtgctgaagtgctggggtactggggtgttgccatgctgaaatgctggggtgttgggatgctgaggtgctgggttgctgggatgctgggatagtccttggatgctgcggtgctgagatgctggtctgctggtctgctggggtgttgggatgctgggattttgggatgctggagtgctgcagtgctgcagtgctgagatgctggagtgctggggtgctggaatactgtagtactggtgtgctggagcattgagatgctagggcactgggatgctaaggtgctgagatgctgcagtgctggggtgttgggatgccgaggtgttgggatgcttaagtgctggggtgttgggatgctggggtgctggaacactatggtgctggggtgctggagtgttgagatactgtagtggtgggatgcttaagtgctggggtgctgggtgttgggatgcctaggtgctggggtgccgagatgctggagtactagtgtgctgggatgctgaagtgctggggtcctgagatgctgcagtgctagggtgctgagattctgggctgctggagtgttggggtgctgggatgctggagtgctgagatgcttggacaatggggtgctggaatactatggtgctggggtgctggggtattgagatgctagggtactgggatgctgaagtgctgagatcctggagtgctgggctgctgggccacaggctcttgaatccattcgtctgcccaggggaagaaaccagaagataaagagctaatgaaggagctttggttgagagggaggaagtaatggaaggagcaacatcttgtggaggagcaggagagaatggacctcaggttgggagagagggccaggctacaggccagagaggcagaaggattccagcagagtgtgggctccaggagccaaggggaaacaggtttctgggaggagagagtccagtactgctgaagtggcaagtccgctgaggaccaggaagcttcatttggctttatgaccaggaggaatttggaactgtgactagagtacttagggggaaggaggcaagactggagccagattgctctgggttgaggggtgagtgggaggtgaagcagggcactgtcactcctttgaagggtggcagagagctggaattggtgctggatgggctgtggggtgacagggtcatgtggaaagcccctggggggcacctggaaaaggagaagctgacagtacagtgagaggacagctaagggaaagcggaatggcagaacacgcactgccaggaggaatgaggatagggtcaggagtgccaggggcagtgaggccagcctggggtcaggtggcaggacgtgtccaggaagctggtctgcactgcagcccacactggctcagccttgaggttccctgtgtggttggggtaggaagttgaaccctctgggaatggaagatggaaccagctctgcgagccaagctcagcttttatctatgggtctctgagggctggcagagctgagtggggacaactgtgatccgtgaggctctcaggttgaggtggcccctccgggagggcttcattttcccagcgggtaggttctaagcagcagtggctgggcaggtgggtccaacacagagccagagaagggtgaatgggcctcctggcaccccacccctgctgcccctgagctcagtgatggagggggacagcacagctgagcccaagtgctttggtgtggccctgagggaaagctgcagcctgcctggggcctggcatggatgggacacttgaggcagagggacaatagtgggcgctgcagtgaggctggctcttggagaggtttcctgaggagtgctgcctgagacgggcagggagaacagagacaaagttggtgacagggaatgaaagctgactgaaggactttacccagacctatgaggatatctctctcagcaggaagcaggaggggactgtgtgaggactggccaagagctggagtgttgggaaaatgactctttctccgacccctctgtcctagctctggcccctggactgcggaggtctgcttccacccccattggtcgatcgttgtcccttgtcacagccattgagaattttggcagggagcatgttcttagagcatttttaggctctgcgggacataacagctctgcctcagagcacatgcctttctcagctcctgaaagccactgatcaaattggaacattttgtaccttagggatgaggatatcaactctcccagccacttagagggataaatgtgatgatgcattcaattgtgactacatctgatcccaactgttgcttcagctgctctcctatagcacatggcgggaggcgtgcatcccagtagctacctccccacttttggggagatgtggttccatccatgaaacctgggtacccgcctaccaggtcctggcctatcaggtggcagggtctggtcaaagaagggcatgtgtggtcttcagcaagggagacaggacggtggtgcagagcgtctagaccctcagggcaagtctcccccacacctgctcccggggcagttgtctttgtgacctcccatccccctctgtttcatcctctataaaatgaggggctgagccccaaaataacaggcttctttgccatgatgcaaaactgctgaatctttctttctgacacacaaggcatcgagcagcctctgaaagaaccaaagccactagcaggcttcctgacttgggtttgtaggtactgaatactcccttgaaaaataaaaacatagaggcacttttctcctggctgtttattacagaacgaagaaaaaacacactggcttgaaacagacgccagatttcaaatgtagaggtgaaatacgaggtggcaattaaaatgtgattacagaaagtctggacactgagaaaagtttacaggacagtgggtgtgggttttctataacagacacttaaatatacatgacgataattgcagatagaaaccatcaaagacaaaccccaaatcaactaataatgtttacagatgttcccccccaaaccacagagccttacatcaaaacaaatactgaaaggctttaaaccaggaacagctcgccttaaccccacgagggtgcacacaagctgggctttttctctcggtctgaatggtaaagggaggaggatactctagctcctccaggtggattgctgagacagggctcggctcacacactgtctctgcgcctctcccaaatctggagaactctcccagcctcctggtaaagtgtctctgtggggcacttaacgataaaacagcttctgctgtaaagctcattaggaaagagctagcggagactgaaaggttcgcaaaagagattaagaatcacacaaggcaataggatttttagtgaacatagaaataaatggccaagtggttttctatttggcatttgtcaacttgcacaacaactcttggtcatatccacattgctcattgcattaaaaccataagcgactcagccacctagcttaacaaggtatcactggagcaaacaacacggtctgcatatttgtaacattgtataataaacacaaaacaatgcatagtaaacacaactctactgaaacaaaagccgtcgctttatttacaaagtcacaaaatgaagtataaatacttctgtcattaatgtttaggaaaaccatttacaaaattttcaaatatgtacacgtagcttgaaaaatcaccagctttccattttgtcacaggtagagagagggataagcatgggctgacaacaccactcaaattgtaacgggagacaactgcgggtatggatcgacaccacttcctagagtgatgtcaccatgggggtttctatgggcatcctgctcagatttaaagtgccccagcatcctgggtgacttgcccagaattctgggctgtggcattttgagcagcagcatgctgttccaaaatgtcgtcgatcagcctcaagttgcacacccagtcttcatctgggctcacacaggagcctttcaagagagcttcaatgaaatctacctcattgcagtcaggtgacgaaatcagatcatttagtgggggttggggctggcgcaaaaagtcggcaggtggcagctcagggggaatatccgttctgtcgaacggacctgggaactggctggcagcaacggcagaagcagcagcagcggtggcagcagcagccacatagcttggtggctcgatgccctgtatggggctcaggggactaaagctggccataccctgctggaggaacttggtggtgtttgctacaggcaccgggccctgtaccgggctctgcctgaggctctggctgcccagcaggctgaagctggggttgttggccaggggcacttgtgttcccatcgcagcgggcacttgtgcctcccaatcagatggcctctgaaggcaggcctggccagaaggtgagtgctgctgaacgctattatccacttggctgaggggtgttttccccgaaactgctgtggtcacagctgctgccgctgtgacccatgcagcattgttgaacgcagtgggcattcttggcacactaggccgtctgagctggtggggactcaaggactgggtgcccagggagctgggacagaacccaggcaggggcacttctggtggggtggccttggggctctgcatatgctggcagacagagtcaagtctgcccaggggagtctggcctgagtgtgagaggatgggacactgggggctggaggtgaaaattccttgccgcttccccagagttggtgagatcactcccatgccctcgcagctctggtgcctggtgagtgggatcattcctggactcagattgttctgaagaagcccagttctgggtggcatcaagtgcttgctagatggggggcttgccttgatccggctacacttggaggtgacttgttcttggacggctacatacagaaagagagaagtggggatgagttccaaaggcatcctcgacttcggctgtggccaccggagggtagctcctggcccaacacggacttctcacctcccgcccttggctctctactgagctcccccctgctccccaattcctcgccattcccctcatttctctgccctcagcctggactgcagttcttctgggaagctgccccaactccctaggtctgtgctcaccaagagcagatcacactggactgaaatgccagctgatttgtctcttcaagaaaattggaagctcctggaggtcagggtccatgtctgcttttacactcagtgctctgtatgcaggcctggcactgcccaccctttgacaggtggtgcatattttgtagaaggaaggaaggggccaggtggggtgggctgggctggtggcgggagctagctcagcctcttagattctctacccgatggatgtgacctgggacagcaagtgagtgtggtgagtgagtgcagacggtgctttgttcccctcttgtctcatagcctagatggcctctgagcccagatctggggctcagacaacatttgttcaactgaacggtaatgggtttcctttctgaaggctgaaatctgggagctgacattctggactccctgagttctgaagagcctggggatggagagacacggagcagaagatggaaggtagagtcccaggtgcctaagatggggaatacatctcccctcattgtcatgagagtccactctagctgatatctactgtggccaatatctaccggtacttttttggggtggacactgagtcatgcagcagtcttatggtttacccaaggtcaggtaggggagacagtgcagtcagagcacaagcccagtgtgtctgacccacccaagaatccatgctcgtatctacaaaaatgattttttctcttgtaatggtgcctaggttcttttattatcatggcatgtgtatgtttttcaactaggttacaatctggccttataaggttaacctcctggaggccaccagccttcctgaaacttgtctgtgctgtccctgcaactggagtgtgcctgatgtggcactccagcctggacaagtgggacacagactccgctgttatcaggcccaaagatgtcttccataagaccagaagagcaatggtgtagaggtgtcatgggctacaataaagatgctgacctcctgtctgagggcaagcagcctcttctggccctcagacaaatgctgagtgttcccaagactaccctcggcctggtccaatctcatcccactggtgcgtaagggttgctgaactcatgacttcttggctagcctgcaacctccacggagtgggaactacatcaggcattttgctaactgctgtatcctaggccaataaatgttgatcacatttatagctgccatggtagggtggggacccctgctatctatctgtggaggctctgggagcccctgacacaaactttctgaagcagagcctccccaaccccttttccattccctatacctgacagatggcccaggaacccattagaaatggaaggtcactgcagcagtatgtgaatgtgcgtgtgggagaagggcaggatcagagccctgggggtgtggcagcccccaagtgattctaatccagatcctagggttgtttccctgtcccattgaaatagctgctttaaggggcctgactcagggaaatcagtctcttgaattaagtggtgattttggagtcatttagaccaggccttcaattgggatccactagttctagagcggccgggcccagggaaccccgcaggcgggggcggccagtttcccgggttcggctttacgtcacgcgagggcggcagggaggacggaatggcggggtttggggtgggtccctcctcgggggagccctgggaaaagaggactgcgtgtgggaagagaaggtggaaatggcgttttggttgacatgtgccgcctgcgagcgtgctgcggggaggggccgagggcagattcgggaatgatggcgcggggtgggggcgtgggggctttctcgggagaggcccttccctggaagtttggggtgcgatggtgaggttctcggggcacctctggaggggcctcggcacggaaagcgaccacctgggagggcgtgtggggaccaggttttgcctttagttttgcacacactgtagttcatctttatggagatgctcatggcctcattgaagccccactacagctctggtagcggtaaccatgcgtatttgacacacgaaggaactagggaaaaggcattaggtcatttcaagccgaaattcacatgtgctagaatccagattccatgctgaccgatgccccaggatatagaaaatgagaatctggtccttaccttcaagaacattcttaaccgtaatcagcctctggtatcttagctccaccctcactggttttttcttgtttgttgaaccggccaagctgctggcctccctcctcaaccgttctgatcatgcttgctaaaatagtcaaaaccccggccagttaaatatgctttagcctgctttattatgattatttttgttgttttggcaatgacctggttacctgttgtttctcccactaaaactttttaagggcaggaatcaccgccgtaactctagcacttagcacagtacttggcttgtaagaggtcctcgatgatggtttgttgaatgaatacattaaataattaaccacttgaaccctaagaaagaagcgattctatttcatattaggcattgtaatgacttaaggtaaagagcagtgctattaacggagtctaactgggaatccagcttgtttgggctatttactagttgtgtggctgtgggcaacttacttcacctctctgggcttaagtcattttatgtatatctgaggtgctggctacctcttggagttattgagaggattataagacagtctatgtgaatcagcaacccttgcatggcccctggcggggaacagtaataatagccatcatcatgtttacttacatagtcctaattagtcttcaaaacagccctgtagcaatggtatgattattaccattttacagatgaggaacctttgaagcctcagagaggctaacagacataccctaggtcatacagttattaagagaaggagctctgtctcgaacctagctctctctctctcgagtaataccagttaaaaaataggctacaaataggtactcaaaaaaatggtagtggctgttgtttttattcagttgctgaggaaaaaatgttgatttttcatctctaaacatcaacttacttaattctgccaatttcttttttttgagacagggtctcactctgtcacctaggatggagtgcagtggcacaatcactgctcactgcagcctcgacttcccgggctcgggtgattctccccaggctcaggggattctcccacttcagcctcccaagtagctgggactacaggtgcgcaccaccatccctggctaatatttgtactttattttatttatttatttatttattttttgagatggagtttcgctcttgttgcccgggctggagtacagtggcatgatctcggctcagtgcaacctctgcctcccgggttcaagcgattctcctacctcatccccctgagtagctgggattacaggcgcctgccaccatgcctggctaattttttgtatttttaatagagacgaggtttcaccatgttggccaggctactctcgaactcctgatctcaggtgatccacccgccttggcctcccaaagtgctgggattacaggcgtgagccactgcgcccggcctaatatttgtattttttgtagagatggtgttttgccatgttgtccaggctggtcttgaactcctgagctcaagcgatctgcccgcctctgcttcccaaagtgctgggattacaggcatgagccaccgtgcctggcctaggtagacgcttttagctttggggtgtgatgcctgccccagtatatagtgaatttaattattgctagagctggctgtttgttagttttctttgaacataagatactcattgtttttagtttgcaaatccctcttcctttttaaaaaatttctttcccttaaattgtttgcatgttagcaataacaaatgcttaaatggtgctatgtgctagatactcttctaagccctgttatgtatattaactaattttttaaattacacaaatcagagaggttaagtaacttgcccaagattacccaacaatactaggatttgaacctaagtttgtctcaccccagattctgctcttaatctctaaacttttaagttagtagtgacaatagtaggtatttattgaatacttaactatgttttaggcgttgaagtaaatattttgcaggcattatctaatgtaaacaccctaaagttacataacaggtaccctttaggtaaataaacactagtatgaccttggaggcacagatagttgaagtaacttgcccaatatcacttacatgaaattggccctcaaatgtgtctgatacaacccatgctgcttgtaactatcgttttaaactgccagggtaaacttggacacacttgagctaagaaaaagcttttagatttttgcaaattaatgtgaaagatatgctttatgtggatataatatcttctaaatttcggggatggtagtcctagaaatgtaatcctgccctagccgagcttaccctgccaataattttttacagaattggtaaaacggagcaccttttttttgtccttggccacactgttatcaacagggtgtagattgacatcaatctgtaggtgtaaaccagaattactctttgtgaccaccaggaaatagagcagttcagttcaggggtttctttctgtgaatttagcactgtgacctgcatactacaagtctactttgttttctatccattgtttgtatctgggtattgcaaaaggtaggaaaaggaccaaccagatcagcagagaagagttgccttggagttttcttttagttttctgcagttcattagatagtaactaggccatgtcattttactcccttgtagtgaagatatgttgaagttgtactggtatactcttctacctttctgtaattttatattgtgtagacttgataaaatttatgtgtcaatcaccaccattaatatcaatattgagcctcaattcttatttttctgcccagtggctgccaaattactaacatttacaataattcactactactaagataatctactagttcgatcacatacttcaaattgttatggaactactgtcttcagcattgtgcttctgataactgataagtataattttttttttgtccagagtgaacatgtctattcttccactgtacacactaataaaaggaaaaattgtaatattgggtaaattcatgtccttacacatgtagtagttatgagcccatgtccctagaatgagtaataatttatccctcccttggttgaatagtcaagaatgctgattttaattcttctaacagctttatccctcagaagggaaggcaagcaagttatatatgtagtttatttgtaagactgatatgaaattggaagatgaatctactattagctttaattatttttacatttaggaatattgcatcagtaactcataattttggttttctgttatcctgagttaacacaaattatccaaggagatggcggatcatctgctttgaggtgtttttttttgagaattttaatgtatctgaatataaaaggtaaaaatatgccaactagcaatttctgcccattccagaagtttggaaatattactcattactaggaattaaataaaatatggtttatctattgttatacctcttttaattcacatagctcatttttatcttttatttttgtttgttttttttgagatggagtcttgctctgtcaccaggcaggagtgcagtgatgcaaatctcggctcactctagccaccgactccctggttcaagcgattctcctgcctgagccttctgagtagctgggattacaggcaggcaccaccacgcccagctaatttttgtagagacaggatttcaccgtgttggccaggatggtctccatctcctgacctcatgatctgcctgcttcggcctcccaaagtgctgggattacaggtgggagccactacgcctggcccacatagctcatttttagactcacttccattaagtcttgtttggacccacgaacattgtctttttttttttaagatggagtttcacttttgttgcccagactgtagtgcaatggtgcaatctcagctcactgcaatctctgcctcctgggttctagcaattctcctgcctcagcctcccgagtagctggaattacaggcgcccgccaccacgcccagctaatttttgtgtttttagtagagacggggtttcaccatgttgggcaggccaggggtgatccgcccacctcagcctcccaaagtgctgggattacaggtgtgagccaccgcatctggccaacatgtcttttttttttttttcctttttaaccacaaagagacttaagcagtccttgtcacagatgatgaattgatgttgcaagtattgtcttagcttggattaattttcttgcttactgtaattttagataatatagctttgtaattagagattttatgtgtaaaccacaaaaatgtttacatgaaggccattattacagatgtgacgtgcataattattagtaatttgtatgtttacatgggtcagtctggcaaaaaattatgaagttttaaaaattaaaaaaaattataatgccagttttactggaaagtaaaattatttcagtaatcgattatagcaaaagtattgattttcattccagacaaaagtcagaatgaaaggtaatttctcaatactctttcagattaataaaagtacctgtagcgatttttatcattcacaagtatatcacaagtaagttagaatttgagaactgtgttctagatctctgaggagatgcagtcagatttctgaactgtctcagcaaatggtaagtaacttagagctagtaattaataacctgtcctttgatttctgattcagccaagaatggccatatttgggaaaggcagatctggagagtaaccacgttttcattcatttaccacttctaggcccctccagagctctcagatattttggggttgagcccttccccaaagccatacaggaccttttttttgtgatctgttctagccatttttatgttgggtgcttgttatggactgagcatttatgtcctcccacaccccccccataccttttttgaagtcctaacccccagtgtgatggtatttggagacagggcctttggaaggtaattacagttagaagaagtcgggagggttgggcccaggtctgattggattagtgcccttatatgaaaagacaccaggacgggcgcagtggctcacacctgtaatcccagcactttgggaggccaaggtgggtggatcacgaggtcaggagtttgagaccagcctggccaatgtagtgaaacaccatctctactaaaaatacaaaaattagctgggtgtggtagcgggctcctgtcatccaagctactcgggagggtgaggcatgagaatcacttgaacccgggagttggaggttgcagtgagcccagattgtgccactgtactccagcctgggtgacagagtgagactctgtctcaaaaaagaaaaaaaaaaaaaaagagacaccagagagcttgttagaagaggtcatgtgagcacacagttagaagaccttcaagccaaagaagaggcctgagattgaaacctaccttgcaggtaccttaattttggacttcccagcctccaaaactgtgagaaataagtttctgttaagtcactcagtctgtggtattttgttatggcagcctgagcaggtagttgttctttcagaaggtgttgataataaccacatgcaacaccaagtcacaaataataaaacagatgtaacttatattcatacagaaagttgggcactgccattgccttgttggtttacacggctgtgctagttcagtagcagaaaggtgctggtctcctttactcagtttacaatctaggcagtagaatgtaatcactgctttaaacttgatactgcttagggagagaatcattggtgctgggtaactttgggttctaggtttactttttgtgtatatataactgtttttggtaaatcacaagtttctgggcttgtcgaattagattttgttacagattatgagctttattatgctatacagttagttgtatgtatatatgcctttcccactagattttaagctttttttttttttttttttttgtgacggagtcttgctcttgtcgcccaggctgaagtggagtgcagtggcacaatctcggctcactgcagcctccacctcctaggttcaagcgattctcctgcctcggcctcccaagtaactgggactacaggcacgtgccaccacacccggctaatttttgtattttttgtagagacagggtttcgccatgttggctaggctggtcttgaacttctggcctcaggtgatccacccgcctcagcctcccaaagtgctgggatttacaggcatgagccaccacgcccagctatagctctttaagggttgtaaatttataatcattcttttactctcctgcaaattctgttgcacactgccttaatcaaggtagatgctgaatgcatttttgtataattgaatatgttgcaatccccaactctctccaactgttcctgtcaaagcagccactggattgttaactaatccatattagatggggttaattaatatcagatgggacaagtaagggctaataagattataggccaccaagtagatttctgtctagctcttatagagattgagtttattggacctgtttgataggaagttttggtgtttgggatgattaaaactgaagttcctatttattgaattatacctatttatattatttcatatcagtggtccacatgcaagtgaggcttctgagacagagtttgagttctctcttcaactaccataacacttaacctgtatctttttttttttttttttttttagacaggagtctcgctctgtcactcaggctggagtgtagtggtatgatctcggctcactgtaacctctgcctcctggattcaagcagttctccatgtctcagcctccctagtagctgggattacaggcctgtgccaccatgcctggctaattttttttttgtatttttagtagagacggggttttaccacgttggccaggctggtctcgaactcttgacctcgagcgatcaacttgccttggcctcccaaagtgctgggattacaggcatgagccacagcgcccagccgtctttttttttaaatagcaatttaacactgttcacagttactcatgtacatgtcatgccatctattacactgtaagttctgtgagggtagctgtatcaaatttatctaactctctctagtatgcatgacatagtaagtattcaataaatatttgcatattagtgataaggatacaggttctgaatagtgggtccttaccatttaagaattagtatttgatggccgggcggggtggctcacgcctgtaatcccagcactttgggaggctgaggcgggcggatcatgagatcaggagatcgagaccatcctggctaacatggtgaaatcccgtctttacaaaaaaaatacaaaagaattaaccaagtgtggtggtgggtgcctgtagtcccagctactgctttgtgaggctgaggcaggcagatcacctgaggtgggaaattcaagaccagcctgaccaacatggagaaaccccatctctactaaaaatacaaaattagccgggcgtggtggcgcatgtctgtaatcccagctactcgggaggctgaggcaggagaatggcgtgaacccgggaggcggagcttgcagtgagccaggatcgcgccactgcactccagcctgggcgacagagcgagactccgtctcaaaaaaaaaaaaaaaaaaaaaattagtatttgatatttgatcattaaatatgaattaagaggacttagactttttgttaaatgtcaagctgggaaaagttgtcatttaaatgaattgcctcttatttaatttcgtctgatgatacattttgtttttattttgtaaaaaattattttttttctttttggagacagggtcttgctctgttgcccaggctggtcacaaactcctgacctcaagcaatcctcctgccttagcctcccaaaatgctgggattacaggcgtgacgacctcgcccggccttgtattatgatacattttgaacaactacaagtagacttggtataatgaacctgcacgtacccattgccaagttctgacaactgtctgtctatagccaattatgcatttcttaaattagaacccccccaatatacccaaatatatatatatgtgtgcatatatatagtaagttgtaacaaagttgtgaattcatacctgaagtatctcaagtgatgcaagttttatgaatttttgtttatgccttttgggaagagttgtattgacaaattttttatgcttaaagtaaaccataaatcaaaaaaataaaatctaggatgcaataaaacaaaacaacttcttgacataagtatggtatgtaaatctgttttgattggaaatcaatttgttatattgccagaattcctgttttagaatacatctctgctgatctgtctgtattcttagactgcatatctgggatgaactctgggcagaattcacatgggcttcctttgaaataaacaagacttttcaaattcttagtcgatctgcagaacctgtagccaggcactgaaccattttgatagatgcagtaatcgttgcaagtgtatatttcaagggagttctggctgggtcctagtttatgcttgtggcagaagcagtgagtaactgggaggaagttggtgagtaagcttcaaggaagaagtcatttttagtactctggatcttcctgattttaaagcactacaaaatggtgcattttcattcttgtcaagtgataacagatatattctgatgagcctgaaatgaatatatattgtatcatttttataatatctagcaaggtttgtattttcctagaacttgaactaaatttcagttcataaaatttataaaatacttagttgttgtaaaatatttttggaatgttcacataggtgacacacaaatgtcccattttcattctttctatagtaaatatgttctgatatgtgaaggtttagcagatgcatcagcatttaatcctagaggatctggcataatcttttcccccaagaatagaaattttttctgcttatgaaagtagtacatgtttctttaaaaacaaatcaatattgacttctgcctgctgtatagcactatgcctccacctggccatgaccaggggcatgtcctggtccacctacctgaaaatgtttgcaaccagcctcctggccatgtgcacaggggctgaagttgtcccacaggtattacgggccaacctgacaatacatgaagttccaccaaagtctgagaactcagaactgagctttggggactgaaagacagcacaaacctcaaatttctcagcactggaaacctcaaaatataactgaattccataaataagattttaagtcttaaatatgtatttttaaatgtattaaaagtcaagctgcttgtatttaagcacctaatacaatgcttaggttgtaaaaggagatgctcaataggtactaactgatatattgagatttaattatggtttgaccaatatttattggaaaccgccaaagcttaaatcatcagcttcttgaatgtgatttgaaaggtaatttagtattgaatagcatgtgagctagagtatttcattctttctggtttatttcttcaaatagactttgaatataatggtgaatgggtattataaattaactaataaaaatgacattgaaaatgaaaaaatatatatattaaagtgtagaaagtgaccaggcgtggtggctcacacctgtaatccaagcaccttgggaggctgaggcaggaggatctcttgatcccaggagttcaagaccagcctgggcaacatagcgagacttcgtctctaaaaaaaaaaaagagagagaaaaaaattttttttatttaaaaaaagtgtagaaagtgtcaagaccccacttcttaccattatttggtatatttctctatacccacccacccttcctccttactccctccctcccttcccaatctttttatctttttgtattctgattttttgtttgtatattttgctttaatttaatgtatcctttaaaaatttcccatacattttatatgtatatataaaaacgcatgctgccaaagataatttataagaaagaccattgaatttttttaaaagtgatatatattcattgaaaaaaatttagaatatatagcaaagcaataaagaactaaataaaattgctgtaactcctctttcaaagataagtgcttttatgattttgttgtatttttttctgtatataggtacatatatagtatttataaagctgtactcatagtacattttcacatcacaggtaccatatcagtgttattaaatattttgtatgccaggggctagacataccaagacaaccaatatgtggttctacttaaataatattagagtatcttttatgatgacacttcatgagttgactataataatcttagacttctaagagtttgggttttcaaaagatcacttagcttttttgggtgatttttcccccttactgtgagatgagagaggctgtttggatttgggattggggtagcggggacagcaacttttcttttctttttcttttttattttgaggtagggtattgctgtgtcacccaggctggagtgcagtggtgtgatctcggctcactgcaacctccacctcccgggctcaggtgatcctcctgcttcagcctcccagtaactgggactacaggcgcgtgccacatgcctggctaattttgtatttttagtagagatggggtttcaccatgttggccaggctggtctctaactcctgacctcaggtgatacgcccacctgggcctcccaaaatactgggattacaggcatgagccgctgcatcagccagcagtttttcttgtggttttttttgtttgttttgttttgttttgtttttgagatagggtcttactctgttgtccacgctggagtgctgtggtatgatcgtagctcactgcagcctcaaactcctgggctcaagtgattccttctgcctccgcctcccgagtagctgggactacaggtatgcaccaccatacctggcaaatttttacaaagttttttgtagggacggggtcttgctacattccccatgtcggtcttgaactcctggcctcaagcaactctcctgtctcagcctcccaaagcactgggattacaagtgtgagccaccacaccatgccagtttttcctgttcagtgtgatattttatcttgttagactacagtgtgttaaaacttgttttactaaattttcaaacatactcaaaagtggagagaatagtataatgaatacccgtatgttcatcacccatgtttagaatattattaaatataaagattttgctgcgtttgtcttagctctttaaaatttttctttttctctttgtgacctaaaggaaattccatatcttatcactttacttctacattcttgactaagatgactaagacatatagttacatggttttttgttttgtttttgttttttaaagacgaaatctcgctcttgtcccccaggctggagtgcaatggtgccatctcagctcagtgcaacctctgccttctgggtacaagcgattctcctgcctcagcctcccaagtagctgggattacaggctcctgccaccacgcctggctaatttttgtatttttagtagagacggcggggggaggtttcaccatgttgacaaggctggtctggaactcctgacctcaggtgatccacccgcctcggcctcccaaagtgctgggattacaggcgtgagccaccgcgcccagcctgtttttttgtttgtgtgttttgttttttttgagacagagtcttgctctgtttcccaggctggagtgaagtggtgccatctcagctcagagacagagtcttgctctgtttcccaggctggagtgaagtggtgccatcttggctcactgcaaccttcacctcccaggttcaagtgattctcctgcctcagcctcccaagtagctgggactacaggcatgtgtcaccacacccggctaatttttttgtatttttagtagagacgggatttcaccgtgttgcccaggctggtctcgaactcctgagctcaggcagtctgcctgcctcagcctcccaaagtgctgggattacacgtgtgaaccaacccgcccggcctgttgttttcttacataattcattatcatacctacaaagttaacagttactaatatcatcttacacctaaatttctctgatagactaaggttattttttaacatcttaatccaatcaaatgtttgtatcctgtaatgctctcattgaaacagctatatttctttttcagattagtgatgatgaaccaggttatgaccttgatttattttgcatacctaatcattatgctgaggatttggaaagggtgtttattcctcatggactaattatggacaggtaagtaagatcttaaaatgaggttttttactttttcttgtgttaatttcaaacatcagcagctgttctgagtacttgctatttgaacataaactaggccaacttattaaataactgatgctttctaaaatcttctttattaaaaataaaagaggagggccttactaattacttagtatcagttgtggtatagtgggactctgtagggaccagaacaaagtaaacattgaagggagatggaagaaggaactctagccagagtcttgcatttctcagtcctaaacagggtaatggactggggctgaatcacatgaaggcaaggtcagatttttattattatgcacatctagcttgaaaattttctgttaagtcaattacagtgaaaaaccttacctggtattgaatgcttgcattgtatgtctggctattctgtgtttttattttaaaattataatatcaaaatatttgtgttataaaatattctaactatggaggccataaacaagaagactaaagttctctcctttcagccttctgtacacatttcttctcaagcactggcctatgcatgtatactatatgcaaaagtacatatatacatttatattttaacgtatgagtatagttttaaatgttattggacacttttaatattagtgtgtctagagctatctaatatattttaaaggttgcatagcattctgtcttatggagataccataactgatttaaccagtccactattgatagacactattttgttcttaccgactgtactagaagaaacattcttttacatgtttggtacttgttcagctttattcaagtggaatttctgggtcaaggggaaagagtttattgaatattttggtattgccaaattttcctctaagaagttgaatcattttatactcctgatgttatatgagagtacctttctcttcacaatttgtctcttttttttttttttttgagacaaggtctctgttgcccaggctggggtgcagtgcagcagaatgatcacagttcactgcagtctcaacctcctgggttcaagcgatccttccacctcagcctcctgagtagctgggactataggtgtgcgccaccactcccagctaatatttttattttgtagaaacagggttcgccatgttacccagcctcccaaagtgctgggattacaggcatgagccactggcccagtttctacagtctctcttaatattgtatattatccagaaaatttcatttaatcagaacctgccagtctgataggtgaaaatggtatcttgtttttatttgcatttaaaaaaaattatgatagtggtatgcttggtttttttgaaggtatcaaattttttaccttatgaaacatgagggcaaaggatgtgatacgtggaagatttaaaaaaaatttttaatgcatttttttgagacaaggtcttgctctattgtccaggctggagtgcagtggcacaatcacagttcactccagcctcaacatcctgcactaaagtgattttcccacctcacctctcaagtagctgggactacaggtacatgctaccatgcctggctaatttttttttttttgcaggcatggggtctcactatattgcccaggttggtgtggaagtttaatgactaagaggtgtttgttataaagtttaatgtatgaaactttctattaaattcctgattttatttctgtaggactgaacgtcttgctcgagatgtgatgaaggagatgggaggccatcacattgtagccctctgtgtgctcaaggggggctataaattctttgctgacctgctggattacatcaaagcactgaatagaaatagtgatagatccattcctatgactgtagattttatcagactgaagagctattgtgtgagtatatttaatatatgattctttttagtggcaacagtaggttttcttatattttctttgaatctctgcaaaccatacttgctttcatttcacttggttacagtgagatttttctaacatattcactagtactttacatcaaagccaatactgtttttttaaaactagtcaccttggaggatatatacttattttacaggtgtgtgtggttttttaaataaactccttttaggaattgctgttgggacttgggatacttttttcactatacatactggtgacagataccctctcttgagctacatcggtttgtggggagtcaaaagtcctttggagctaggtttgacaaataaggtgggttaacacttgtttcctagaaagcacatggagagctagagtattggcgaattgaagaaatccccctttttttttaacacacttaagaaaggggactgcaggtatactcaagagagtaagtcgcaccagaaaccacttttgatccacagtctgcctgtgtcacacaattgaaatgcatcacaacattgacactgtggatgaaacaaaatcagtgtgaattttagtagtgaatttcattcataatttgatcgtgcaaacgtttgatttttattactttagactattgtttctgattttatgttgggttggtatttcctgtgagttactgttttacctttaaaataggaatttttcatactcttcaaagattagaacaaatgtccagtttttgctgtttcatgaatgagtcctgtccatctttgtagaaactcgccttatgttcacatttttattgagaataagaccacttatctacatttaactatcaacctcatcctctccattaatcatctattttagtgacccaagtttttgaccttttccatgtttacatcaatcctgtaggtgattgggcagccatttaagtattattatagacattttcactatcccattaaaaccctttatgcccatacatcataacactacttcctacccataagctccttttaacttgttaaagtcttgcttgaattaaagacttgtttacggtatcgataagcttgatatcaaaacgccaactttgacccggaacgcggaaaacacctgagaaaaacacctgggcgagtctccacgtaaacggtcaaagtccccgcggccctagacaaatattacgcgctatgagtaacacaaaattattcagatttcacttcctcttattcagttttcccgcgaaaatggccaaatcttactcggttacgcccaaatttactacaacatccgcctaaaaccgcgcgaaaattgtcacttcctgtgtacaccggcgcacaccaaaaacgtcacttttgccacatccgtcgcttacatgtgttccgccacacttgcaacatcacacttccgccacactactacgtcacccgccccgttcccacgccccgcgccacgtcacaaactccaccccctcattatcatattggcttcaatccaaaataaggtatattattgatgatgttt

SEQ ID NO: 122 - DNA, 30924 bp, Artificial Sequence
  HDAdHER2BiTE
aaacatcatcaataatataccttattttggattgaagccaatatgataatgagggggtggagtttgtgacgtggcgcggggcgtgggaacggggcgggtgacgtaggttttagggcggagtaacttgtatgtgttgggaattgtagttttcttaaaatgggaagtgacgtaacgtgggaaaacggaagtgacgatttgaggaagttgtgggttttttggctttcgtttctgggcgtaggttcgcgtgcggttttctgggtgttttttgtggactttaaccgttacgtcattttttagtcctatatatactcgctctgcacttggcccttttttacactgtgactgattgagctggtgccgtgtcgagtggtgtttttttaataggttttcttttttactggtaggcgcgccgtcgacgcgacaactgtcttattaccctgttatccctaccttaattaagctagccgacgcgttggccaggagctcagatctccggatccaagcttatcgatttcgaacccaaatggatctaccacatttgtagaggttttacttgctttaaaaaacctcccacacctccccctgaacctgaaacataaaatgaatgcaattgttgttgttaacttgtttattgcagcttataatggttacaaataaagcaatagcatcacaaatttcacaaataaagcaatagcatcacaaatttcacaaataaagcatttttttcactgcattctagttgtggtttgtccaaactcatcaatgtatcttatcatgtcgagctagctagtcaggacttcagttccagctttgtgccggctccgaaggtcagcgggttgctagaccattgctgacagtaatatgtggcggcatcctcggcttccatagagctgattgtcaggctgtagctggtgccagatccagatccgctgaatctgtagggcacgccggaggccactttgcttgtgtcgtagatccaccgcttggggcttgtgccagacttctgctgataccagttcatgtaggacacgctgctgctggctctgcatgtcatggtcactttctcgcctggggaagcgctcatgatggcggggctttgtgtcagctgaatatcggagccaccaccaccgcttccaccaccacctgaaccgcctccgccactagaaactgtcagggttgtgccctggccccagtaatccagacagtagtggtcgtcgtagtaccgggcacaatagtacacagcgctatcttcagaggtcaggctggacagctgcatgtaggcggtagagctgctcttgtcggtggtcagtgtggccttgtccttgaacttctggttgtaattggtgtagccccggctggggttgatgtagccgatccattccagtccttggccaggcctctgcttgacccagtgcatggtgtaccgggtgaatgtgtagccgctggtcttgcaggacatcttcacagaggcgccaggtctagccagttcggcgccagactgttgcagcttgatatcggatccaccgccaccaagggctttgatttccagcttggtgccgctgccgaaggtgaaaggggttctgaagtgctgctgacaaaagtacacggccagatcctcggcctgcacgctgctgatggtaaaggtgaagtcagggccagagccagagccggtgaatctagagggcacgcctgtgtatctgctgctggcgctgtagatcagcagcttaggagactggccaggcttctgctgataccaggccacggcgttgtacacgtcctggctggctttacaggtgatggacactctgtcgcccacgctggtgctcagaaacttgtggctctgggtcagctgaatatcagatcctccgccgcctgaacctccgcctccgcttcctccgccaccagaagagactgtcacggttgtgccctggccccaatatggcacgtagccgtggtacacttcccatctggcacaaaagtaggtggccatgtcctcggacttcaggttgttgatctgcaggtaggcggtgttggcgctggtttccaggctgaagtcgaatctgcccttgaaatcgtcggcgaaggtgctctcgccggtgctggtattgatccagcccatccatttcaggccctgtccaggggcctgcttgacccagttcatgccgtagttggtgaaggggtagccgctggccttgcaggagatcttcactgtctcgccaggtttcttcagctcggggccagactgctgcagctgaacttcagaatgggcgcctgtggcggctcccacaagaaacaggatgcgccagatccagtccatggtggccctccttcgccggtgatctcagctgtaggaaagagaagaaggttagtagtcgacgtgtccctctcgatgaatctaagtatcaattgtgagcgctcacaagtcaacactctttttgataaatctagtagatatcacttacgtaggcgccggtcacagcttggatctgtaacggcgcagaacagaaaacgaaacaaagacgtagagttgagcaagcagggtcaggcaaagcgtggagagccggctgagtctaggtaggctccaagggagcgccggacaaaggcccggtctcgacctgagctttaaacttacctagacggcggacgcagttcaggaggcaccacaggcgggaggcggcagaacgcgactcaaccggcgtggatggcggcctcaggtagggcggcgggcgcgtgaaggagagatgcgagcccctcgaagcttcagctgtgttctggcggcaaacccgttgcgaaaaagaacgttcacggcgactactgcacttatatacggttctcccccaccctcgggaaaaaggcggagccagtacacgacatcactttcccagtttaccccgcgccaccttctctaggcaccggttcaattgccgacccctccccccaacttctcggggactgtgggcgatgtgcgctctgcccactgacgggcaccggagcgatcgcagatccttcgatagagaaatgttctggcacctgcacttgcactggggacagcctattttgctagtttgttttgtttcgttttgttttgatggagagcgtatgttagttacgattcacacaaaaaaccaacacacagatgtaatgaaaataaagatattttattgcggccgctcgagtctagaggtatacatgccatggtccgcggtattaccctgttatccctaagacaactgtcctgcatgcgacgtcggcgcgccatcgaattcctgcagcccgggggatccctttgttgattttttccacatagattatttttgactgttttggcactttatataaatggaatcatatagtaaatatatacatgtatatatgtatatatacactatatatgtatatatatagtgtatatatatacatgtatatatgtatatttacatatatactgtatatatgtatatttacatatatactgtatatatgtatatatacacgtatatactgtatatatacagtatatactgtatatatatactgtatatatgtgtatatatatatacagtatatatacagtatacatatatatacatgtatatatacacagtatatatacatgtatatatacacagtatatatacatgtatatatacacagtatatatacatgtatatatacacagtatatatacactgtatatatgtatatatatactgtgtatatatatacagtatatatacagtatatatatacatgtatatgtatatatatactgtatatatgtgtatatatacgtatatatactgtatatatatatagacacttttgtgtctggcttcttgctctcatcataaagcacttgaaatccatccatgttgtagctggtatcagtagctagtttcttttcattgctgagaagtatcactttttattgatgagtagttttacattgtatgaacatgcccgagtttgtttatgcattctactaatagacacctgggctgtttgcagtttttggctattacaaagaaaatttctatatttttttccaacttttattttaggttcagcgggtacatgggcaggtttgttacatcggtaaattgcatgtcactggggtttggtgtacagattatttcaccacccaggtaataagcatagtacctgataggcaggtttttgatcctcaccctcctccctcaagtaggccccagtgtctattgttctattccttttttttttttttgagatggagtctcactctgttgcccaggctggagtgcagtggtgcgatctcggctcactgcaaggtccacctccagggttcaagcgattctactgccgcagcctcccgagtagctgggattacaggcacccaccaccacgcccggctaatttttgtatttttagtagagactgggtttcaccatgttggccaggatggtctcgaactcctcacctcaggtgatccgcccgcttcggcctcgcaaagtactgggattacaggcgtgagccacggtgcctggcctatggttccattctttgtgtacacgtgtactcagtgtttagcttccacttgtaagtgaaaacatgcagtatttggttttctgaaattcttgtcttcatctttttgtagacaatccactacttttatttttaaatattaggaacaatagcctctgtgtgtcctgaattgcaatgttttttctctgattttgctgctcatcttgtaacctgtatggtgtttttctgtgtgcaagctttttactttacgtgggcaattttatcattcttttcttttatggtttctgggtttcatgtcatgattggagaagcttgatctaccctgatactataaaaatatccaccttggcttttttttttttttttagatggattttcactcttgttgcccaggctggagtgcaatggcgtgatctcggctcaccacaacctctgcctcccaggttcaagtgattctcctgcctcggcctcctgagtagctgggattacaggcatgcgccaccacgctcagctaattttgtatttttagtagagacaggatttcaccatgttggtcaggctggtcttgaactccccacctcaggtgatctgtctgcctcggcctcccaaagtgctgggattacaggcgtgacccaccacacctggcccacgttgttttctgatagtgttttcacgtgttattttttctgtcttactctttgaatcatctaaatgtatcttaatgtcaggagtgaggtagaggacccagttgtttggtttaaatgactagccagttttcccaacaccaggtgttgaacatccctcactgatgtgagatgctgcctttttcacagtctcaatccccatgtgcatttctatttattttccttccactttattcacatctttttcagtatccacaaccatattgttttaaatagcttcatgatatgttttaatatttggtagagctagaaccctttcttggttctttttcttttcttcttctcctccttttcctcctccttctttctcctcctccttcttctttctttttagaaatttcctggctattcttgttttgtagtcttccagataaataattttgaatcactttgtcatgttccagaaaataatactgccagaatttttattgtgatcacagaagttttacagattcatctgggggaaaaaaacccatcttcccagaatacagaaagggtgagggaaagacaaacatcaaggacaagtctcaggttctggacttggagaccaagaggatttggggcatccgggagcagggcagggaggtgtgatggctgcctttcactgagtaggaggatgcccagacttgggggaactatggaaagtttggttcagactttctgagttggagatgtctatgcgcagtccacagggcgaagccctggaggtagaggccctccttactgcctccctcattcagtctgaggtccattctccacatggacactgaagtgactcaaggcttcccttgttggatcaggatagtctccagggccctgggtggtctgggcctgcccacctccccatcccctctcctgcctgccctcctcttgctcactggaccccacccaccagcctccttctattcctcctgacatttgcacttgctgttccgtctctgcttggaacatcctagctctttgcatggcttgctccttcccatcttttaatctaagctcaaatatcactccttcagatatgcctttcccaaatatcctagctaaagagaactgctccccacttcccacaagccctagcaaactgggactctccttcttgctttctttctctctgccccttctgtgttttttccatagaccttaacttgttactgttttatttgttgatgtgtttacatcatttgtccccctgtgatggttagttttatgtgtcaacttggctaggctgtaggggctgttcgtcaatcaaacactgatctatgtgtagctgtgaagggattttgtagctgtgattaatagttgactttaagtaaggaagattatcctggagaatgtgggggaaggggcagacctcagccaatcagttgaaaggccttaagaacaaagctgagatttccccgaggaagaagaaattctgcctgtggactgcagcatcagctcctgcttgagaggttccaggctgcccttcctgacagcctgtcctatgattttggacttgccttgccaggtttttcctctttcttgaccccccaaaaccatatatatctcctgctggtttgtttctctggtgtaatcctgagggatgaacactcctccctcccagttcactctgggagaggttggggatcatgtttgtctatttccccatgcctggcccatgcgtgtttattgaatcactgaacaaccacgcattaggaagccagtcatatgtgcttcttcagaacctcatgtccattgccagatctccctggcttttgtggctagaggacaagtgagagatagtagcttacccacagaccttggccctgaggcccccaggggcctgagcctgctgtaagggaggagggagcccctgaggtctcacacacctccctggggatctggcattttcccctggggctggcctcagagctgggcgggggcagattatggagtgggttgtagagggagcacctccccactagcaatcatggttttttctgcgcctctcatagggaggcctacaggcctccaccttcagctcttcaggagccacaggcagctgagtgacttctgcatcacagtcttctcagagacaaacttgcagtaagaaagaggggcccgtgagggaccccagagaaggctgttgtcaaagcaggatgagagtgaactcttccatgggggacacccagcgtctccaagctcttttatgctgtcttcaaggggtctagagagcttcagcccaacatgagacccagtccagcagcatttccctgcgaagtgaaagttaggaccctgactagatacaccacgctgacctcagccagaatatcaagatgctgaggcgctgagatgctgggatgctaaggtgctaaggtgctggggtgctggggtgctaggatgctgaggttttgtgatactgggtcgctgagatgctgggatactggggtgctgaagtgctggggtactggggtgttgccatgctgaaatgctggggtgttgggatgctgaggtgctgggttgctgggatgctgggatagtccttggatgctgcggtgctgagatgctggtctgctggtctgctggggtgttgggatgctgggattttgggatgctggagtgctgcagtgctgcagtgctgagatgctggagtgctggggtgctggaatactgtagtactggtgtgctggagcattgagatgctagggcactgggatgctaaggtgctgagatgctgcagtgctggggtgttgggatgccgaggtgttgggatgcttaagtgctggggtgttgggatgctggggtgctggaacactatggtgctggggtgctggagtgttgagatactgtagtggtgggatgcttaagtgctggggtgctgggtgttgggatgcctaggtgctggggtgccgagatgctggagtactagtgtgctgggatgctgaagtgctggggtcctgagatgctgcagtgctagggtgctgagattctgggctgctggagtgttggggtgctgggatgctggagtgctgagatgcttggacaatggggtgctggaatactatggtgctggggtgctggggtattgagatgctagggtactgggatgctgaagtgctgagatcctggagtgctgggctgctgggccacaggctcttgaatccattcgtctgcccaggggaagaaaccagaagataaagagctaatgaaggagctttggttgagagggaggaagtaatggaaggagcaacatcttgtggaggagcaggagagaatggacctcaggttgggagagagggccaggctacaggccagagaggcagaaggattccagcagagtgtgggctccaggagccaaggggaaacaggtttctgggaggagagagtccagtactgctgaagtggcaagtccgctgaggaccaggaagcttcatttggctttatgaccaggaggaatttggaactgtgactagagtacttagggggaaggaggcaagactggagccagattgctctgggttgaggggtgagtgggaggtgaagcagggcactgtcactcctttgaagggtggcagagagctggaattggtgctggatgggctgtggggtgacagggtcatgtggaaagcccctggggggcacctggaaaaggagaagctgacagtacagtgagaggacagctaagggaaagcggaatggcagaacacgcactgccaggaggaatgaggatagggtcaggagtgccaggggcagtgaggccagcctggggtcaggtggcaggacgtgtccaggaagctggtctgcactgcagcccacactggctcagccttgaggttccctgtgtggttggggtaggaagttgaaccctctgggaatggaagatggaaccagctctgcgagccaagctcagcttttatctatgggtctctgagggctggcagagctgagtggggacaactgtgatccgtgaggctctcaggttgaggtggcccctccgggagggcttcattttcccagcgggtaggttctaagcagcagtggctgggcaggtgggtccaacacagagccagagaagggtgaatgggcctcctggcaccccacccctgctgcccctgagctcagtgatggagggggacagcacagctgagcccaagtgctttggtgtggccctgagggaaagctgcagcctgcctggggcctggcatggatgggacacttgaggcagagggacaatagtgggcgctgcagtgaggctggctcttggagaggtttcctgaggagtgctgcctgagacgggcagggagaacagagacaaagttggtgacagggaatgaaagctgactgaaggactttacccagacctatgaggatatctctctcagcaggaagcaggaggggactgtgtgaggactggccaagagctggagtgttgggaaaatgactctttctccgacccctctgtcctagctctggcccctggactgcggaggtctgcttccacccccattggtcgatcgttgtcccttgtcacagccattgagaattttggcagggagcatgttcttagagcatttttaggctctgcgggacataacagctctgcctcagagcacatgcctttctcagctcctgaaagccactgatcaaattggaacattttgtaccttagggatgaggatatcaactctcccagccacttagagggataaatgtgatgatgcattcaattgtgactacatctgatcccaactgttgcttcagctgctctcctatagcacatggcgggaggcgtgcatcccagtagctacctccccacttttggggagatgtggttccatccatgaaacctgggtacccgcctaccaggtcctggcctatcaggtggcagggtctggtcaaagaagggcatgtgtggtcttcagcaagggagacaggacggtggtgcagagcgtctagaccctcagggcaagtctcccccacacctgctcccggggcagttgtctttgtgacctcccatccccctctgtttcatcctctataaaatgaggggctgagccccaaaataacaggcttctttgccatgatgcaaaactgctgaatctttctttctgacacacaaggcatcgagcagcctctgaaagaaccaaagccactagcaggcttcctgacttgggtttgtaggtactgaatactcccttgaaaaataaaaacatagaggcacttttctcctggctgtttattacagaacgaagaaaaaacacactggcttgaaacagacgccagatttcaaatgtagaggtgaaatacgaggtggcaattaaaatgtgattacagaaagtctggacactgagaaaagtttacaggacagtgggtgtgggttttctataacagacacttaaatatacatgacgataattgcagatagaaaccatcaaagacaaaccccaaatcaactaataatgtttacagatgttcccccccaaaccacagagccttacatcaaaacaaatactgaaaggctttaaaccaggaacagctcgccttaaccccacgagggtgcacacaagctgggctttttctctcggtctgaatggtaaagggaggaggatactctagctcctccaggtggattgctgagacagggctcggctcacacactgtctctgcgcctctcccaaatctggagaactctcccagcctcctggtaaagtgtctctgtggggcacttaacgataaaacagcttctgctgtaaagctcattaggaaagagctagcggagactgaaaggttcgcaaaagagattaagaatcacacaaggcaataggatttttagtgaacatagaaataaatggccaagtggttttctatttggcatttgtcaacttgcacaacaactcttggtcatatccacattgctcattgcattaaaaccataagcgactcagccacctagcttaacaaggtatcactggagcaaacaacacggtctgcatatttgtaacattgtataataaacacaaaacaatgcatagtaaacacaactctactgaaacaaaagccgtcgctttatttacaaagtcacaaaatgaagtataaatacttctgtcattaatgtttaggaaaaccatttacaaaattttcaaatatgtacacgtagcttgaaaaatcaccagctttccattttgtcacaggtagagagagggataagcatgggctgacaacaccactcaaattgtaacgggagacaactgcgggtatggatcgacaccacttcctagagtgatgtcaccatgggggtttctatgggcatcctgctcagatttaaagtgccccagcatcctgggtgacttgcccagaattctgggctgtggcattttgagcagcagcatgctgttccaaaatgtcgtcgatcagcctcaagttgcacacccagtcttcatctgggctcacacaggagcctttcaagagagcttcaatgaaatctacctcattgcagtcaggtgacgaaatcagatcatttagtgggggttggggctggcgcaaaaagtcggcaggtggcagctcagggggaatatccgttctgtcgaacggacctgggaactggctggcagcaacggcagaagcagcagcagcggtggcagcagcagccacatagcttggtggctcgatgccctgtatggggctcaggggactaaagctggccataccctgctggaggaacttggtggtgtttgctacaggcaccgggccctgtaccgggctctgcctgaggctctggctgcccagcaggctgaagctggggttgttggccaggggcacttgtgttcccatcgcagcgggcacttgtgcctcccaatcagatggcctctgaaggcaggcctggccagaaggtgagtgctgctgaacgctattatccacttggctgaggggtgttttccccgaaactgctgtggtcacagctgctgccgctgtgacccatgcagcattgttgaacgcagtgggcattcttggcacactaggccgtctgagctggtggggactcaaggactgggtgcccagggagctgggacagaacccaggcaggggcacttctggtggggtggccttggggctctgcatatgctggcagacagagtcaagtctgcccaggggagtctggcctgagtgtgagaggatgggacactgggggctggaggtgaaaattccttgccgcttccccagagttggtgagatcactcccatgccctcgcagctctggtgcctggtgagtgggatcattcctggactcagattgttctgaagaagcccagttctgggtggcatcaagtgcttgctagatggggggcttgccttgatccggctacacttggaggtgacttgttcttggacggctacatacagaaagagagaagtggggatgagttccaaaggcatcctcgacttcggctgtggccaccggagggtagctcctggcccaacacggacttctcacctcccgcccttggctctctactgagctcccccctgctccccaattcctcgccattcccctcatttctctgccctcagcctggactgcagttcttctgggaagctgccccaactccctaggtctgtgctcaccaagagcagatcacactggactgaaatgccagctgatttgtctcttcaagaaaattggaagctcctggaggtcagggtccatgtctgcttttacactcagtgctctgtatgcaggcctggcactgcccaccctttgacaggtggtgcatattttgtagaaggaaggaaggggccaggtggggtgggctgggctggtggcgggagctagctcagcctcttagattctctacccgatggatgtgacctgggacagcaagtgagtgtggtgagtgagtgcagacggtgctttgttcccctcttgtctcatagcctagatggcctctgagcccagatctggggctcagacaacatttgttcaactgaacggtaatgggtttcctttctgaaggctgaaatctgggagctgacattctggactccctgagttctgaagagcctggggatggagagacacggagcagaagatggaaggtagagtcccaggtgcctaagatggggaatacatctcccctcattgtcatgagagtccactctagctgatatctactgtggccaatatctaccggtacttttttggggtggacactgagtcatgcagcagtcttatggtttacccaaggtcaggtaggggagacagtgcagtcagagcacaagcccagtgtgtctgacccacccaagaatccatgctcgtatctacaaaaatgattttttctcttgtaatggtgcctaggttcttttattatcatggcatgtgtatgtttttcaactaggttacaatctggccttataaggttaacctcctggaggccaccagccttcctgaaacttgtctgtgctgtccctgcaactggagtgtgcctgatgtggcactccagcctggacaagtgggacacagactccgctgttatcaggcccaaagatgtcttccataagaccagaagagcaatggtgtagaggtgtcatgggctacaataaagatgctgacctcctgtctgagggcaagcagcctcttctggccctcagacaaatgctgagtgttcccaagactaccctcggcctggtccaatctcatcccactggtgcgtaagggttgctgaactcatgacttcttggctagcctgcaacctccacggagtgggaactacatcaggcattttgctaactgctgtatcctaggccaataaatgttgatcacatttatagctgccatggtagggtggggacccctgctatctatctgtggaggctctgggagcccctgacacaaactttctgaagcagagcctccccaaccccttttccattccctatacctgacagatggcccaggaacccattagaaatggaaggtcactgcagcagtatgtgaatgtgcgtgtgggagaagggcaggatcagagccctgggggtgtggcagcccccaagtgattctaatccagatcctagggttgtttccctgtcccattgaaatagctgctttaaggggcctgactcagggaaatcagtctcttgaattaagtggtgattttggagtcatttagaccaggccttcaattgggatccactagttctagagcggccgggcccagggaaccccgcaggcgggggcggccagtttcccgggttcggctttacgtcacgcgagggcggcagggaggacggaatggcggggtttggggtgggtccctcctcgggggagccctgggaaaagaggactgcgtgtgggaagagaaggtggaaatggcgttttggttgacatgtgccgcctgcgagcgtgctgcggggaggggccgagggcagattcgggaatgatggcgcggggtgggggcgtgggggctttctcgggagaggcccttccctggaagtttggggtgcgatggtgaggttctcggggcacctctggaggggcctcggcacggaaagcgaccacctgggagggcgtgtggggaccaggttttgcctttagttttgcacacactgtagttcatctttatggagatgctcatggcctcattgaagccccactacagctctggtagcggtaaccatgcgtatttgacacacgaaggaactagggaaaaggcattaggtcatttcaagccgaaattcacatgtgctagaatccagattccatgctgaccgatgccccaggatatagaaaatgagaatctggtccttaccttcaagaacattcttaaccgtaatcagcctctggtatcttagctccaccctcactggttttttcttgtttgttgaaccggccaagctgctggcctccctcctcaaccgttctgatcatgcttgctaaaatagtcaaaaccccggccagttaaatatgctttagcctgctttattatgattatttttgttgttttggcaatgacctggttacctgttgtttctcccactaaaactttttaagggcaggaatcaccgccgtaactctagcacttagcacagtacttggcttgtaagaggtcctcgatgatggtttgttgaatgaatacattaaataattaaccacttgaaccctaagaaagaagcgattctatttcatattaggcattgtaatgacttaaggtaaagagcagtgctattaacggagtctaactgggaatccagcttgtttgggctatttactagttgtgtggctgtgggcaacttacttcacctctctgggcttaagtcattttatgtatatctgaggtgctggctacctcttggagttattgagaggattataagacagtctatgtgaatcagcaacccttgcatggcccctggcggggaacagtaataatagccatcatcatgtttacttacatagtcctaattagtcttcaaaacagccctgtagcaatggtatgattattaccattttacagatgaggaacctttgaagcctcagagaggctaacagacataccctaggtcatacagttattaagagaaggagctctgtctcgaacctagctctctctctctcgagtaataccagttaaaaaataggctacaaataggtactcaaaaaaatggtagtggctgttgtttttattcagttgctgaggaaaaaatgttgatttttcatctctaaacatcaacttacttaattctgccaatttcttttttttgagacagggtctcactctgtcacctaggatggagtgcagtggcacaatcactgctcactgcagcctcgacttcccgggctcgggtgattctccccaggctcaggggattctcccacttcagcctcccaagtagctgggactacaggtgcgcaccaccatccctggctaatatttgtactttattttatttatttatttatttattttttgagatggagtttcgctcttgttgcccgggctggagtacagtggcatgatctcggctcagtgcaacctctgcctcccgggttcaagcgattctcctacctcatccccctgagtagctgggattacaggcgcctgccaccatgcctggctaattttttgtatttttaatagagacgaggtttcaccatgttggccaggctactctcgaactcctgatctcaggtgatccacccgccttggcctcccaaagtgctgggattacaggcgtgagccactgcgcccggcctaatatttgtattttttgtagagatggtgttttgccatgttgtccaggctggtcttgaactcctgagctcaagcgatctgcccgcctctgcttcccaaagtgctgggattacaggcatgagccaccgtgcctggcctaggtagacgcttttagctttggggtgtgatgcctgccccagtatatagtgaatttaattattgctagagctggctgtttgttagttttctttgaacataagatactcattgtttttagtttgcaaatccctcttcctttttaaaaaatttctttcccttaaattgtttgcatgttagcaataacaaatgcttaaatggtgctatgtgctagatactcttctaagccctgttatgtatattaactaattttttaaattacacaaatcagagaggttaagtaacttgcccaagattacccaacaatactaggatttgaacctaagtttgtctcaccccagattctgctcttaatctctaaacttttaagttagtagtgacaatagtaggtatttattgaatacttaactatgttttaggcgttgaagtaaatattttgcaggcattatctaatgtaaacaccctaaagttacataacaggtaccctttaggtaaataaacactagtatgaccttggaggcacagatagttgaagtaacttgcccaatatcacttacatgaaattggccctcaaatgtgtctgatacaacccatgctgcttgtaactatcgttttaaactgccagggtaaacttggacacacttgagctaagaaaaagcttttagatttttgcaaattaatgtgaaagatatgctttatgtggatataatatcttctaaatttcggggatggtagtcctagaaatgtaatcctgccctagccgagcttaccctgccaataattttttacagaattggtaaaacggagcaccttttttttgtccttggccacactgttatcaacagggtgtagattgacatcaatctgtaggtgtaaaccagaattactctttgtgaccaccaggaaatagagcagttcagttcaggggtttctttctgtgaatttagcactgtgacctgcatactacaagtctactttgttttctatccattgtttgtatctgggtattgcaaaaggtaggaaaaggaccaaccagatcagcagagaagagttgccttggagttttcttttagttttctgcagttcattagatagtaactaggccatgtcattttactcccttgtagtgaagatatgttgaagttgtactggtatactcttctacctttctgtaattttatattgtgtagacttgataaaatttatgtgtcaatcaccaccattaatatcaatattgagcctcaattcttatttttctgcccagtggctgccaaattactaacatttacaataattcactactactaagataatctactagttcgatcacatacttcaaattgttatggaactactgtcttcagcattgtgcttctgataactgataagtataattttttttttgtccagagtgaacatgtctattcttccactgtacacactaataaaaggaaaaattgtaatattgggtaaattcatgtccttacacatgtagtagttatgagcccatgtccctagaatgagtaataatttatccctcccttggttgaatagtcaagaatgctgattttaattcttctaacagctttatccctcagaagggaaggcaagcaagttatatatgtagtttatttgtaagactgatatgaaattggaagatgaatctactattagctttaattatttttacatttaggaatattgcatcagtaactcataattttggttttctgttatcctgagttaacacaaattatccaaggagatggcggatcatctgctttgaggtgtttttttttgagaattttaatgtatctgaatataaaaggtaaaaatatgccaactagcaatttctgcccattccagaagtttggaaatattactcattactaggaattaaataaaatatggtttatctattgttatacctcttttaattcacatagctcatttttatcttttatttttgtttgttttttttgagatggagtcttgctctgtcaccaggcaggagtgcagtgatgcaaatctcggctcactctagccaccgactccctggttcaagcgattctcctgcctgagccttctgagtagctgggattacaggcaggcaccaccacgcccagctaatttttgtagagacaggatttcaccgtgttggccaggatggtctccatctcctgacctcatgatctgcctgcttcggcctcccaaagtgctgggattacaggtgggagccactacgcctggcccacatagctcatttttagactcacttccattaagtcttgtttggacccacgaacattgtctttttttttttaagatggagtttcacttttgttgcccagactgtagtgcaatggtgcaatctcagctcactgcaatctctgcctcctgggttctagcaattctcctgcctcagcctcccgagtagctggaattacaggcgcccgccaccacgcccagctaatttttgtgtttttagtagagacggggtttcaccatgttgggcaggccaggggtgatccgcccacctcagcctcccaaagtgctgggattacaggtgtgagccaccgcatctggccaacatgtcttttttttttttttcctttttaaccacaaagagacttaagcagtccttgtcacagatgatgaattgatgttgcaagtattgtcttagcttggattaattttcttgcttactgtaattttagataatatagctttgtaattagagattttatgtgtaaaccacaaaaatgtttacatgaaggccattattacagatgtgacgtgcataattattagtaatttgtatgtttacatgggtcagtctggcaaaaaattatgaagttttaaaaattaaaaaaaattataatgccagttttactggaaagtaaaattatttcagtaatcgattatagcaaaagtattgattttcattccagacaaaagtcagaatgaaaggtaatttctcaatactctttcagattaataaaagtacctgtagcgatttttatcattcacaagtatatcacaagtaagttagaatttgagaactgtgttctagatctctgaggagatgcagtcagatttctgaactgtctcagcaaatggtaagtaacttagagctagtaattaataacctgtcctttgatttctgattcagccaagaatggccatatttgggaaaggcagatctggagagtaaccacgttttcattcatttaccacttctaggcccctccagagctctcagatattttggggttgagcccttccccaaagccatacaggaccttttttttgtgatctgttctagccatttttatgttgggtgcttgttatggactgagcatttatgtcctcccacaccccccccataccttttttgaagtcctaacccccagtgtgatggtatttggagacagggcctttggaaggtaattacagttagaagaagtcgggagggttgggcccaggtctgattggattagtgcccttatatgaaaagacaccaggacgggcgcagtggctcacacctgtaatcccagcactttgggaggccaaggtgggtggatcacgaggtcaggagtttgagaccagcctggccaatgtagtgaaacaccatctctactaaaaatacaaaaattagctgggtgtggtagcgggctcctgtcatccaagctactcgggagggtgaggcatgagaatcacttgaacccgggagttggaggttgcagtgagcccagattgtgccactgtactccagcctgggtgacagagtgagactctgtctcaaaaaagaaaaaaaaaaaaaaagagacaccagagagcttgttagaagaggtcatgtgagcacacagttagaagaccttcaagccaaagaagaggcctgagattgaaacctaccttgcaggtaccttaattttggacttcccagcctccaaaactgtgagaaataagtttctgttaagtcactcagtctgtggtattttgttatggcagcctgagcaggtagttgttctttcagaaggtgttgataataaccacatgcaacaccaagtcacaaataataaaacagatgtaacttatattcatacagaaagttgggcactgccattgccttgttggtttacacggctgtgctagttcagtagcagaaaggtgctggtctcctttactcagtttacaatctaggcagtagaatgtaatcactgctttaaacttgatactgcttagggagagaatcattggtgctgggtaactttgggttctaggtttactttttgtgtatatataactgtttttggtaaatcacaagtttctgggcttgtcgaattagattttgttacagattatgagctttattatgctatacagttagttgtatgtatatatgcctttcccactagattttaagctttttttttttttttttttttgtgacggagtcttgctcttgtcgcccaggctgaagtggagtgcagtggcacaatctcggctcactgcagcctccacctcctaggttcaagcgattctcctgcctcggcctcccaagtaactgggactacaggcacgtgccaccacacccggctaatttttgtattttttgtagagacagggtttcgccatgttggctaggctggtcttgaacttctggcctcaggtgatccacccgcctcagcctcccaaagtgctgggatttacaggcatgagccaccacgcccagctatagctctttaagggttgtaaatttataatcattcttttactctcctgcaaattctgttgcacactgccttaatcaaggtagatgctgaatgcatttttgtataattgaatatgttgcaatccccaactctctccaactgttcctgtcaaagcagccactggattgttaactaatccatattagatggggttaattaatatcagatgggacaagtaagggctaataagattataggccaccaagtagatttctgtctagctcttatagagattgagtttattggacctgtttgataggaagttttggtgtttgggatgattaaaactgaagttcctatttattgaattatacctatttatattatttcatatcagtggtccacatgcaagtgaggcttctgagacagagtttgagttctctcttcaactaccataacacttaacctgtatctttttttttttttttttttttagacaggagtctcgctctgtcactcaggctggagtgtagtggtatgatctcggctcactgtaacctctgcctcctggattcaagcagttctccatgtctcagcctccctagtagctgggattacaggcctgtgccaccatgcctggctaattttttttttgtatttttagtagagacggggttttaccacgttggccaggctggtctcgaactcttgacctcgagcgatcaacttgccttggcctcccaaagtgctgggattacaggcatgagccacagcgcccagccgtctttttttttaaatagcaatttaacactgttcacagttactcatgtacatgtcatgccatctattacactgtaagttctgtgagggtagctgtatcaaatttatctaactctctctagtatgcatgacatagtaagtattcaataaatatttgcatattagtgataaggatacaggttctgaatagtgggtccttaccatttaagaattagtatttgatggccgggcggggtggctcacgcctgtaatcccagcactttgggaggctgaggcgggcggatcatgagatcaggagatcgagaccatcctggctaacatggtgaaatcccgtctttacaaaaaaaatacaaaagaattaaccaagtgtggtggtgggtgcctgtagtcccagctactgctttgtgaggctgaggcaggcagatcacctgaggtgggaaattcaagaccagcctgaccaacatggagaaaccccatctctactaaaaatacaaaattagccgggcgtggtggcgcatgtctgtaatcccagctactcgggaggctgaggcaggagaatggcgtgaacccgggaggcggagcttgcagtgagccaggatcgcgccactgcactccagcctgggcgacagagcgagactccgtctcaaaaaaaaaaaaaaaaaaaaaattagtatttgatatttgatcattaaatatgaattaagaggacttagactttttgttaaatgtcaagctgggaaaagttgtcatttaaatgaattgcctcttatttaatttcgtctgatgatacattttgtttttattttgtaaaaaattattttttttctttttggagacagggtcttgctctgttgcccaggctggtcacaaactcctgacctcaagcaatcctcctgccttagcctcccaaaatgctgggattacaggcgtgacgacctcgcccggccttgtattatgatacattttgaacaactacaagtagacttggtataatgaacctgcacgtacccattgccaagttctgacaactgtctgtctatagccaattatgcatttcttaaattagaacccccccaatatacccaaatatatatatatgtgtgcatatatatagtaagttgtaacaaagttgtgaattcatacctgaagtatctcaagtgatgcaagttttatgaatttttgtttatgccttttgggaagagttgtattgacaaattttttatgcttaaagtaaaccataaatcaaaaaaataaaatctaggatgcaataaaacaaaacaacttcttgacataagtatggtatgtaaatctgttttgattggaaatcaatttgttatattgccagaattcctgttttagaatacatctctgctgatctgtctgtattcttagactgcatatctgggatgaactctgggcagaattcacatgggcttcctttgaaataaacaagacttttcaaattcttagtcgatctgcagaacctgtagccaggcactgaaccattttgatagatgcagtaatcgttgcaagtgtatatttcaagggagttctggctgggtcctagtttatgcttgtggcagaagcagtgagtaactgggaggaagttggtgagtaagcttcaaggaagaagtcatttttagtactctggatcttcctgattttaaagcactacaaaatggtgcattttcattcttgtcaagtgataacagatatattctgatgagcctgaaatgaatatatattgtatcatttttataatatctagcaaggtttgtattttcctagaacttgaactaaatttcagttcataaaatttataaaatacttagttgttgtaaaatatttttggaatgttcacataggtgacacacaaatgtcccattttcattctttctatagtaaatatgttctgatatgtgaaggtttagcagatgcatcagcatttaatcctagaggatctggcataatcttttcccccaagaatagaaattttttctgcttatgaaagtagtacatgtttctttaaaaacaaatcaatattgacttctgcctgctgtatagcactatgcctccacctggccatgaccaggggcatgtcctggtccacctacctgaaaatgtttgcaaccagcctcctggccatgtgcacaggggctgaagttgtcccacaggtattacgggccaacctgacaatacatgaagttccaccaaagtctgagaactcagaactgagctttggggactgaaagacagcacaaacctcaaatttctcagcactggaaacctcaaaatataactgaattccataaataagattttaagtcttaaatatgtatttttaaatgtattaaaagtcaagctgcttgtatttaagcacctaatacaatgcttaggttgtaaaaggagatgctcaataggtactaactgatatattgagatttaattatggtttgaccaatatttattggaaaccgccaaagcttaaatcatcagcttcttgaatgtgatttgaaaggtaatttagtattgaatagcatgtgagctagagtatttcattctttctggtttatttcttcaaatagactttgaatataatggtgaatgggtattataaattaactaataaaaatgacattgaaaatgaaaaaatatatatattaaagtgtagaaagtgaccaggcgtggtggctcacacctgtaatccaagcaccttgggaggctgaggcaggaggatctcttgatcccaggagttcaagaccagcctgggcaacatagcgagacttcgtctctaaaaaaaaaaaagagagagaaaaaaattttttttatttaaaaaaagtgtagaaagtgtcaagaccccacttcttaccattatttggtatatttctctatacccacccacccttcctccttactccctccctcccttcccaatctttttatctttttgtattctgattttttgtttgtatattttgctttaatttaatgtatcctttaaaaatttcccatacattttatatgtatatataaaaacgcatgctgccaaagataatttataagaaagaccattgaatttttttaaaagtgatatatattcattgaaaaaaatttagaatatatagcaaagcaataaagaactaaataaaattgctgtaactcctctttcaaagataagtgcttttatgattttgttgtatttttttctgtatataggtacatatatagtatttataaagctgtactcatagtacattttcacatcacaggtaccatatcagtgttattaaatattttgtatgccaggggctagacataccaagacaaccaatatgtggttctacttaaataatattagagtatcttttatgatgacacttcatgagttgactataataatcttagacttctaagagtttgggttttcaaaagatcacttagcttttttgggtgatttttcccccttactgtgagatgagagaggctgtttggatttgggattggggtagcggggacagcaacttttcttttctttttcttttttattttgaggtagggtattgctgtgtcacccaggctggagtgcagtggtgtgatctcggctcactgcaacctccacctcccgggctcaggtgatcctcctgcttcagcctcccagtaactgggactacaggcgcgtgccacatgcctggctaattttgtatttttagtagagatggggtttcaccatgttggccaggctggtctctaactcctgacctcaggtgatacgcccacctgggcctcccaaaatactgggattacaggcatgagccgctgcatcagccagcagtttttcttgtggttttttttgtttgttttgttttgttttgtttttgagatagggtcttactctgttgtccacgctggagtgctgtggtatgatcgtagctcactgcagcctcaaactcctgggctcaagtgattccttctgcctccgcctcccgagtagctgggactacaggtatgcaccaccatacctggcaaatttttacaaagttttttgtagggacggggtcttgctacattccccatgtcggtcttgaactcctggcctcaagcaactctcctgtctcagcctcccaaagcactgggattacaagtgtgagccaccacaccatgccagtttttcctgttcagtgtgatattttatcttgttagactacagtgtgttaaaacttgttttactaaattttcaaacatactcaaaagtggagagaatagtataatgaatacccgtatgttcatcacccatgtttagaatattattaaatataaagattttgctgcgtttgtcttagctctttaaaatttttctttttctctttgtgacctaaaggaaattccatatcttatcactttacttctacattcttgactaagatgactaagacatatagttacatggttttttgttttgtttttgttttttaaagacgaaatctcgctcttgtcccccaggctggagtgcaatggtgccatctcagctcagtgcaacctctgccttctgggtacaagcgattctcctgcctcagcctcccaagtagctgggattacaggctcctgccaccacgcctggctaatttttgtatttttagtagagacggcggggggaggtttcaccatgttgacaaggctggtctggaactcctgacctcaggtgatccacccgcctcggcctcccaaagtgctgggattacaggcgtgagccaccgcgcccagcctgtttttttgtttgtgtgttttgttttttttgagacagagtcttgctctgtttcccaggctggagtgaagtggtgccatctcagctcagagacagagtcttgctctgtttcccaggctggagtgaagtggtgccatcttggctcactgcaaccttcacctcccaggttcaagtgattctcctgcctcagcctcccaagtagctgggactacaggcatgtgtcaccacacccggctaatttttttgtatttttagtagagacgggatttcaccgtgttgcccaggctggtctcgaactcctgagctcaggcagtctgcctgcctcagcctcccaaagtgctgggattacacgtgtgaaccaacccgcccggcctgttgttttcttacataattcattatcatacctacaaagttaacagttactaatatcatcttacacctaaatttctctgatagactaaggttattttttaacatcttaatccaatcaaatgtttgtatcctgtaatgctctcattgaaacagctatatttctttttcagattagtgatgatgaaccaggttatgaccttgatttattttgcatacctaatcattatgctgaggatttggaaagggtgtttattcctcatggactaattatggacaggtaagtaagatcttaaaatgaggttttttactttttcttgtgttaatttcaaacatcagcagctgttctgagtacttgctatttgaacataaactaggccaacttattaaataactgatgctttctaaaatcttctttattaaaaataaaagaggagggccttactaattacttagtatcagttgtggtatagtgggactctgtagggaccagaacaaagtaaacattgaagggagatggaagaaggaactctagccagagtcttgcatttctcagtcctaaacagggtaatggactggggctgaatcacatgaaggcaaggtcagatttttattattatgcacatctagcttgaaaattttctgttaagtcaattacagtgaaaaaccttacctggtattgaatgcttgcattgtatgtctggctattctgtgtttttattttaaaattataatatcaaaatatttgtgttataaaatattctaactatggaggccataaacaagaagactaaagttctctcctttcagccttctgtacacatttcttctcaagcactggcctatgcatgtatactatatgcaaaagtacatatatacatttatattttaacgtatgagtatagttttaaatgttattggacacttttaatattagtgtgtctagagctatctaatatattttaaaggttgcatagcattctgtcttatggagataccataactgatttaaccagtccactattgatagacactattttgttcttaccgactgtactagaagaaacattcttttacatgtttggtacttgttcagctttattcaagtggaatttctgggtcaaggggaaagagtttattgaatattttggtattgccaaattttcctctaagaagttgaatcattttatactcctgatgttatatgagagtacctttctcttcacaatttgtctcttttttttttttttttgagacaaggtctctgttgcccaggctggggtgcagtgcagcagaatgatcacagttcactgcagtctcaacctcctgggttcaagcgatccttccacctcagcctcctgagtagctgggactataggtgtgcgccaccactcccagctaatatttttattttgtagaaacagggttcgccatgttacccagcctcccaaagtgctgggattacaggcatgagccactggcccagtttctacagtctctcttaatattgtatattatccagaaaatttcatttaatcagaacctgccagtctgataggtgaaaatggtatcttgtttttatttgcatttaaaaaaaattatgatagtggtatgcttggtttttttgaaggtatcaaattttttaccttatgaaacatgagggcaaaggatgtgatacgtggaagatttaaaaaaaatttttaatgcatttttttgagacaaggtcttgctctattgtccaggctggagtgcagtggcacaatcacagttcactccagcctcaacatcctgcactaaagtgattttcccacctcacctctcaagtagctgggactacaggtacatgctaccatgcctggctaatttttttttttttgcaggcatggggtctcactatattgcccaggttggtgtggaagtttaatgactaagaggtgtttgttataaagtttaatgtatgaaactttctattaaattcctgattttatttctgtaggactgaacgtcttgctcgagatgtgatgaaggagatgggaggccatcacattgtagccctctgtgtgctcaaggggggctataaattctttgctgacctgctggattacatcaaagcactgaatagaaatagtgatagatccattcctatgactgtagattttatcagactgaagagctattgtgtgagtatatttaatatatgattctttttagtggcaacagtaggttttcttatattttctttgaatctctgcaaaccatacttgctttcatttcacttggttacagtgagatttttctaacatattcactagtactttacatcaaagccaatactgtttttttaaaactagtcaccttggaggatatatacttattttacaggtgtgtgtggttttttaaataaactccttttaggaattgctgttgggacttgggatacttttttcactatacatactggtgacagataccctctcttgagctacatcggtttgtggggagtcaaaagtcctttggagctaggtttgacaaataaggtgggttaacacttgtttcctagaaagcacatggagagctagagtattggcgaattgaagaaatccccctttttttttaacacacttaagaaaggggactgcaggtatactcaagagagtaagtcgcaccagaaaccacttttgatccacagtctgcctgtgtcacacaattgaaatgcatcacaacattgacactgtggatgaaacaaaatcagtgtgaattttagtagtgaatttcattcataatttgatcgtgcaaacgtttgatttttattactttagactattgtttctgattttatgttgggttggtatttcctgtgagttactgttttacctttaaaataggaatttttcatactcttcaaagattagaacaaatgtccagtttttgctgtttcatgaatgagtcctgtccatctttgtagaaactcgccttatgttcacatttttattgagaataagaccacttatctacatttaactatcaacctcatcctctccattaatcatctattttagtgacccaagtttttgaccttttccatgtttacatcaatcctgtaggtgattgggcagccatttaagtattattatagacattttcactatcccattaaaaccctttatgcccatacatcataacactacttcctacccataagctccttttaacttgttaaagtcttgcttgaattaaagacttgtttacggtatcgataagcttgatatcaaaacgccaactttgacccggaacgcggaaaacacctgagaaaaacacctgggcgagtctccacgtaaacggtcaaagtccccgcggccctagacaaatattacgcgctatgagtaacacaaaattattcagatttcacttcctcttattcagttttcccgcgaaaatggccaaatcttactcggttacgcccaaatttactacaacatccgcctaaaaccgcgcgaaaattgtcacttcctgtgtacaccggcgcacaccaaaaacgtcacttttgccacatccgtcgcttacatgtgttccgccacacttgcaacatcacacttccgccacactactacgtcacccgccccgttcccacgccccgcgccacgtcacaaactccaccccctcattatcatattggcttcaatccaaaataaggtatattattgatgatgttt

SEQ ID NO: 123 - DNA, 30881 bp, Artificial Sequence
  HDAdCD19BiTE
aaacatcatcaataatataccttattttggattgaagccaatatgataatgagggggtggagtttgtgacgtggcgcggggcgtgggaacggggcgggtgacgtaggttttagggcggagtaacttgtatgtgttgggaattgtagttttcttaaaatgggaagtgacgtaacgtgggaaaacggaagtgacgatttgaggaagttgtgggttttttggctttcgtttctgggcgtaggttcgcgtgcggttttctgggtgttttttgtggactttaaccgttacgtcattttttagtcctatatatactcgctctgcacttggcccttttttacactgtgactgattgagctggtgccgtgtcgagtggtgtttttttaataggttttcttttttactggtaggcgcgccgtcgacgcttattaccctgttatccctactagctagccgacgcgttgggagctctccggatccaagcttatcgatttcgaacccaaatggatctaccacatttgtagaggttttacttgctttaaaaaacctcccacacctccccctgaacctgaaacataaaatgaatgcaattgttgttgttaacttgtttattgcagcttataatggttacaaataaagcaatagcatcacaaatttcacaaataaagcaatagcatcacaaatttcacaaataaagcatttttttcactgcattctagttgtggtttgtccaaactcatcaatgtatcttatcatgtcgagctagctagtcaggacttcagttccagctttgtgccggctccgaaggtcagcgggttgctagaccattgctgacagtaatatgtggcggcatcctcggcttccatagagctgattgtcaggctgtagctggtgccagatccagatccgctgaatctgtagggcacgccggaggccactttgcttgtgtcgtagatccaccgcttggggcttgtgccagacttctgctgataccagttcatgtaggacacgctgctgctggctctgcatgtcatggtcactttctcgcctggggaagcgctcatgatggcggggctttgtgtcagctgaatatcggagccaccaccaccgcttccaccaccacctgaaccgcctccgccactagaaactgtcagggttgtgccctggccccagtaatccagacagtagtggtcgtcgtagtaccgggcacaatagtacacagcgctatcttcagaggtcaggctggacagctgcatgtaggcggtagagctgctcttgtcggtggtcagtgtggccttgtccttgaacttctggttgtaattggtgtagccccggctggggttgatgtagccgatccattccagtccttggccaggcctctgcttgacccagtgcatggtgtaccgggtgaatgtgtagccgctggtcttgcaggacatcttcacagaggcgccaggtctagccagttcggcgccagactgttgcagcttgatatcggatccaccacctccgccagaagaaactgtcacgctggtgccctggccccaatagtccatagcgtagctgccgccgtagtagtagtgcttggcgcaatagtagatggcggtgtcgtcggtctgcaggctgttcatcttcaggaacacctggctcttggagttgtccttgatgatggtcagccgggacttcagggcgctgttgtagtaggttgtctcgctgccccagatcactcccagccattccaggcctttccgaggaggctgtctgatccaggacacgccataatcaggcagggacactccgctgacggtacaggtcacgctcagagattgagatggggccaccaggccagggccagactcttgcagtttcacttcagatcctccgccaccagaacctccgcctccgcttcctccgccgcctgtgatttccagcttggtgcctccgccaaaggtgtaaggcagggtgttgccttgctggcagaagtaggtagcgatatcctcttgttccaggttgctgattgtcaggctgtagtcggtgccagagccgctgccagaaaatctgcttggcacgccgctgtgcagtctgctggtgtggtagatcagcagcttcacggtgccgtcgggtttctgctgataccagttcaggtacttgctgatgtcctggctggctctacagctgatggtcactctatcgcccagagaggcagacaggctgctggtggtctgggtcatctgaatatcgctgtgggcgcctgtggcagctcccacaaggaacaggatgcgccagatccaatccatggtggccctccttcgccggtgatctcagctgtaggaaagagaagaaggttagtagtcgacgtgtccctctcgatgaatctaagtatcaattgtgagcgctcacaagtcaacactctttttgataaatctagtagatatcacttacgtaggcgccggtcacagcttggatctgtaacggcgcagaacagaaaacgaaacaaagacgtagagttgagcaagcagggtcaggcaaagcgtggagagccggctgagtctaggtaggctccaagggagcgccggacaaaggcccggtctcgacctgagctttaaacttacctagacggcggacgcagttcaggaggcaccacaggcgggaggcggcagaacgcgactcaaccggcgtggatggcggcctcaggtagggcggcgggcgcgtgaaggagagatgcgagcccctcgaagcttcagctgtgttctggcggcaaacccgttgcgaaaaagaacgttcacggcgactactgcacttatatacggttctcccccaccctcgggaaaaaggcggagccagtacacgacatcactttcccagtttaccccgcgccaccttctctaggcaccggttcaattgccgacccctccccccaacttctcggggactgtgggcgatgtgcgctctgcccactgacgggcaccggagcgatcgcagatccttcgatagagaaatgttctggcacctgcacttgcactggggacagcctattttgctagtttgttttgtttcgttttgttttgatggagagcgtatgttagttacgattcacacaaaaaaccaacacacagatgtaatgaaaataaagatattttattgcggccgctcgagtctagaggacatgccatggtcgtattaccctgttatccctaactgcatgcgacgtcggcgcgccatcgaattcctgcagcccgggggatccctttgttgattttttccacatagattatttttgactgttttggcactttatataaatggaatcatatagtaaatatatacatgtatatatgtatatatacactatatatgtatatatatagtgtatatatatacatgtatatatgtatatttacatatatactgtatatatgtatatttacatatatactgtatatatgtatatatacacgtatatactgtatatatacagtatatactgtatatatatactgtatatatgtgtatatatatatacagtatatatacagtatacatatatatacatgtatatatacacagtatatatacatgtatatatacacagtatatatacatgtatatatacacagtatatatacatgtatatatacacagtatatatacactgtatatatgtatatatatactgtgtatatatatacagtatatatacagtatatatatacatgtatatgtatatatatactgtatatatgtgtatatatacgtatatatactgtatatatatatagacacttttgtgtctggcttcttgctctcatcataaagcacttgaaatccatccatgttgtagctggtatcagtagctagtttcttttcattgctgagaagtatcactttttattgatgagtagttttacattgtatgaacatgcccgagtttgtttatgcattctactaatagacacctgggctgtttgcagtttttggctattacaaagaaaatttctatatttttttccaacttttattttaggttcagcgggtacatgggcaggtttgttacatcggtaaattgcatgtcactggggtttggtgtacagattatttcaccacccaggtaataagcatagtacctgataggcaggtttttgatcctcaccctcctccctcaagtaggccccagtgtctattgttctattccttttttttttttttgagatggagtctcactctgttgcccaggctggagtgcagtggtgcgatctcggctcactgcaaggtccacctccagggttcaagcgattctactgccgcagcctcccgagtagctgggattacaggcacccaccaccacgcccggctaatttttgtatttttagtagagactgggtttcaccatgttggccaggatggtctcgaactcctcacctcaggtgatccgcccgcttcggcctcgcaaagtactgggattacaggcgtgagccacggtgcctggcctatggttccattctttgtgtacacgtgtactcagtgtttagcttccacttgtaagtgaaaacatgcagtatttggttttctgaaattcttgtcttcatctttttgtagacaatccactacttttatttttaaatattaggaacaatagcctctgtgtgtcctgaattgcaatgttttttctctgattttgctgctcatcttgtaacctgtatggtgtttttctgtgtgcaagctttttactttacgtgggcaattttatcattcttttcttttatggtttctgggtttcatgtcatgattggagaagcttgatctaccctgatactataaaaatatccaccttggcttttttttttttttttagatggattttcactcttgttgcccaggctggagtgcaatggcgtgatctcggctcaccacaacctctgcctcccaggttcaagtgattctcctgcctcggcctcctgagtagctgggattacaggcatgcgccaccacgctcagctaattttgtatttttagtagagacaggatttcaccatgttggtcaggctggtcttgaactccccacctcaggtgatctgtctgcctcggcctcccaaagtgctgggattacaggcgtgacccaccacacctggcccacgttgttttctgatagtgttttcacgtgttattttttctgtcttactctttgaatcatctaaatgtatcttaatgtcaggagtgaggtagaggacccagttgtttggtttaaatgactagccagttttcccaacaccaggtgttgaacatccctcactgatgtgagatgctgcctttttcacagtctcaatccccatgtgcatttctatttattttccttccactttattcacatctttttcagtatccacaaccatattgttttaaatagcttcatgatatgttttaatatttggtagagctagaaccctttcttggttctttttcttttcttcttctcctccttttcctcctccttctttctcctcctccttcttctttctttttagaaatttcctggctattcttgttttgtagtcttccagataaataattttgaatcactttgtcatgttccagaaaataatactgccagaatttttattgtgatcacagaagttttacagattcatctgggggaaaaaaacccatcttcccagaatacagaaagggtgagggaaagacaaacatcaaggacaagtctcaggttctggacttggagaccaagaggatttggggcatccgggagcagggcagggaggtgtgatggctgcctttcactgagtaggaggatgcccagacttgggggaactatggaaagtttggttcagactttctgagttggagatgtctatgcgcagtccacagggcgaagccctggaggtagaggccctccttactgcctccctcattcagtctgaggtccattctccacatggacactgaagtgactcaaggcttcccttgttggatcaggatagtctccagggccctgggtggtctgggcctgcccacctccccatcccctctcctgcctgccctcctcttgctcactggaccccacccaccagcctccttctattcctcctgacatttgcacttgctgttccgtctctgcttggaacatcctagctctttgcatggcttgctccttcccatcttttaatctaagctcaaatatcactccttcagatatgcctttcccaaatatcctagctaaagagaactgctccccacttcccacaagccctagcaaactgggactctccttcttgctttctttctctctgccccttctgtgttttttccatagaccttaacttgttactgttttatttgttgatgtgtttacatcatttgtccccctgtgatggttagttttatgtgtcaacttggctaggctgtaggggctgttcgtcaatcaaacactgatctatgtgtagctgtgaagggattttgtagctgtgattaatagttgactttaagtaaggaagattatcctggagaatgtgggggaaggggcagacctcagccaatcagttgaaaggccttaagaacaaagctgagatttccccgaggaagaagaaattctgcctgtggactgcagcatcagctcctgcttgagaggttccaggctgcccttcctgacagcctgtcctatgattttggacttgccttgccaggtttttcctctttcttgaccccccaaaaccatatatatctcctgctggtttgtttctctggtgtaatcctgagggatgaacactcctccctcccagttcactctgggagaggttggggatcatgtttgtctatttccccatgcctggcccatgcgtgtttattgaatcactgaacaaccacgcattaggaagccagtcatatgtgcttcttcagaacctcatgtccattgccagatctccctggcttttgtggctagaggacaagtgagagatagtagcttacccacagaccttggccctgaggcccccaggggcctgagcctgctgtaagggaggagggagcccctgaggtctcacacacctccctggggatctggcattttcccctggggctggcctcagagctgggcgggggcagattatggagtgggttgtagagggagcacctccccactagcaatcatggttttttctgcgcctctcatagggaggcctacaggcctccaccttcagctcttcaggagccacaggcagctgagtgacttctgcatcacagtcttctcagagacaaacttgcagtaagaaagaggggcccgtgagggaccccagagaaggctgttgtcaaagcaggatgagagtgaactcttccatgggggacacccagcgtctccaagctcttttatgctgtcttcaaggggtctagagagcttcagcccaacatgagacccagtccagcagcatttccctgcgaagtgaaagttaggaccctgactagatacaccacgctgacctcagccagaatatcaagatgctgaggcgctgagatgctgggatgctaaggtgctaaggtgctggggtgctggggtgctaggatgctgaggttttgtgatactgggtcgctgagatgctgggatactggggtgctgaagtgctggggtactggggtgttgccatgctgaaatgctggggtgttgggatgctgaggtgctgggttgctgggatgctgggatagtccttggatgctgcggtgctgagatgctggtctgctggtctgctggggtgttgggatgctgggattttgggatgctggagtgctgcagtgctgcagtgctgagatgctggagtgctggggtgctggaatactgtagtactggtgtgctggagcattgagatgctagggcactgggatgctaaggtgctgagatgctgcagtgctggggtgttgggatgccgaggtgttgggatgcttaagtgctggggtgttgggatgctggggtgctggaacactatggtgctggggtgctggagtgttgagatactgtagtggtgggatgcttaagtgctggggtgctgggtgttgggatgcctaggtgctggggtgccgagatgctggagtactagtgtgctgggatgctgaagtgctggggtcctgagatgctgcagtgctagggtgctgagattctgggctgctggagtgttggggtgctgggatgctggagtgctgagatgcttggacaatggggtgctggaatactatggtgctggggtgctggggtattgagatgctagggtactgggatgctgaagtgctgagatcctggagtgctgggctgctgggccacaggctcttgaatccattcgtctgcccaggggaagaaaccagaagataaagagctaatgaaggagctttggttgagagggaggaagtaatggaaggagcaacatcttgtggaggagcaggagagaatggacctcaggttgggagagagggccaggctacaggccagagaggcagaaggattccagcagagtgtgggctccaggagccaaggggaaacaggtttctgggaggagagagtccagtactgctgaagtggcaagtccgctgaggaccaggaagcttcatttggctttatgaccaggaggaatttggaactgtgactagagtacttagggggaaggaggcaagactggagccagattgctctgggttgaggggtgagtgggaggtgaagcagggcactgtcactcctttgaagggtggcagagagctggaattggtgctggatgggctgtggggtgacagggtcatgtggaaagcccctggggggcacctggaaaaggagaagctgacagtacagtgagaggacagctaagggaaagcggaatggcagaacacgcactgccaggaggaatgaggatagggtcaggagtgccaggggcagtgaggccagcctggggtcaggtggcaggacgtgtccaggaagctggtctgcactgcagcccacactggctcagccttgaggttccctgtgtggttggggtaggaagttgaaccctctgggaatggaagatggaaccagctctgcgagccaagctcagcttttatctatgggtctctgagggctggcagagctgagtggggacaactgtgatccgtgaggctctcaggttgaggtggcccctccgggagggcttcattttcccagcgggtaggttctaagcagcagtggctgggcaggtgggtccaacacagagccagagaagggtgaatgggcctcctggcaccccacccctgctgcccctgagctcagtgatggagggggacagcacagctgagcccaagtgctttggtgtggccctgagggaaagctgcagcctgcctggggcctggcatggatgggacacttgaggcagagggacaatagtgggcgctgcagtgaggctggctcttggagaggtttcctgaggagtgctgcctgagacgggcagggagaacagagacaaagttggtgacagggaatgaaagctgactgaaggactttacccagacctatgaggatatctctctcagcaggaagcaggaggggactgtgtgaggactggccaagagctggagtgttgggaaaatgactctttctccgacccctctgtcctagctctggcccctggactgcggaggtctgcttccacccccattggtcgatcgttgtcccttgtcacagccattgagaattttggcagggagcatgttcttagagcatttttaggctctgcgggacataacagctctgcctcagagcacatgcctttctcagctcctgaaagccactgatcaaattggaacattttgtaccttagggatgaggatatcaactctcccagccacttagagggataaatgtgatgatgcattcaattgtgactacatctgatcccaactgttgcttcagctgctctcctatagcacatggcgggaggcgtgcatcccagtagctacctccccacttttggggagatgtggttccatccatgaaacctgggtacccgcctaccaggtcctggcctatcaggtggcagggtctggtcaaagaagggcatgtgtggtcttcagcaagggagacaggacggtggtgcagagcgtctagaccctcagggcaagtctcccccacacctgctcccggggcagttgtctttgtgacctcccatccccctctgtttcatcctctataaaatgaggggctgagccccaaaataacaggcttctttgccatgatgcaaaactgctgaatctttctttctgacacacaaggcatcgagcagcctctgaaagaaccaaagccactagcaggcttcctgacttgggtttgtaggtactgaatactcccttgaaaaataaaaacatagaggcacttttctcctggctgtttattacagaacgaagaaaaaacacactggcttgaaacagacgccagatttcaaatgtagaggtgaaatacgaggtggcaattaaaatgtgattacagaaagtctggacactgagaaaagtttacaggacagtgggtgtgggttttctataacagacacttaaatatacatgacgataattgcagatagaaaccatcaaagacaaaccccaaatcaactaataatgtttacagatgttcccccccaaaccacagagccttacatcaaaacaaatactgaaaggctttaaaccaggaacagctcgccttaaccccacgagggtgcacacaagctgggctttttctctcggtctgaatggtaaagggaggaggatactctagctcctccaggtggattgctgagacagggctcggctcacacactgtctctgcgcctctcccaaatctggagaactctcccagcctcctggtaaagtgtctctgtggggcacttaacgataaaacagcttctgctgtaaagctcattaggaaagagctagcggagactgaaaggttcgcaaaagagattaagaatcacacaaggcaataggatttttagtgaacatagaaataaatggccaagtggttttctatttggcatttgtcaacttgcacaacaactcttggtcatatccacattgctcattgcattaaaaccataagcgactcagccacctagcttaacaaggtatcactggagcaaacaacacggtctgcatatttgtaacattgtataataaacacaaaacaatgcatagtaaacacaactctactgaaacaaaagccgtcgctttatttacaaagtcacaaaatgaagtataaatacttctgtcattaatgtttaggaaaaccatttacaaaattttcaaatatgtacacgtagcttgaaaaatcaccagctttccattttgtcacaggtagagagagggataagcatgggctgacaacaccactcaaattgtaacgggagacaactgcgggtatggatcgacaccacttcctagagtgatgtcaccatgggggtttctatgggcatcctgctcagatttaaagtgccccagcatcctgggtgacttgcccagaattctgggctgtggcattttgagcagcagcatgctgttccaaaatgtcgtcgatcagcctcaagttgcacacccagtcttcatctgggctcacacaggagcctttcaagagagcttcaatgaaatctacctcattgcagtcaggtgacgaaatcagatcatttagtgggggttggggctggcgcaaaaagtcggcaggtggcagctcagggggaatatccgttctgtcgaacggacctgggaactggctggcagcaacggcagaagcagcagcagcggtggcagcagcagccacatagcttggtggctcgatgccctgtatggggctcaggggactaaagctggccataccctgctggaggaacttggtggtgtttgctacaggcaccgggccctgtaccgggctctgcctgaggctctggctgcccagcaggctgaagctggggttgttggccaggggcacttgtgttcccatcgcagcgggcacttgtgcctcccaatcagatggcctctgaaggcaggcctggccagaaggtgagtgctgctgaacgctattatccacttggctgaggggtgttttccccgaaactgctgtggtcacagctgctgccgctgtgacccatgcagcattgttgaacgcagtgggcattcttggcacactaggccgtctgagctggtggggactcaaggactgggtgcccagggagctgggacagaacccaggcaggggcacttctggtggggtggccttggggctctgcatatgctggcagacagagtcaagtctgcccaggggagtctggcctgagtgtgagaggatgggacactgggggctggaggtgaaaattccttgccgcttccccagagttggtgagatcactcccatgccctcgcagctctggtgcctggtgagtgggatcattcctggactcagattgttctgaagaagcccagttctgggtggcatcaagtgcttgctagatggggggcttgccttgatccggctacacttggaggtgacttgttcttggacggctacatacagaaagagagaagtggggatgagttccaaaggcatcctcgacttcggctgtggccaccggagggtagctcctggcccaacacggacttctcacctcccgcccttggctctctactgagctcccccctgctccccaattcctcgccattcccctcatttctctgccctcagcctggactgcagttcttctgggaagctgccccaactccctaggtctgtgctcaccaagagcagatcacactggactgaaatgccagctgatttgtctcttcaagaaaattggaagctcctggaggtcagggtccatgtctgcttttacactcagtgctctgtatgcaggcctggcactgcccaccctttgacaggtggtgcatattttgtagaaggaaggaaggggccaggtggggtgggctgggctggtggcgggagctagctcagcctcttagattctctacccgatggatgtgacctgggacagcaagtgagtgtggtgagtgagtgcagacggtgctttgttcccctcttgtctcatagcctagatggcctctgagcccagatctggggctcagacaacatttgttcaactgaacggtaatgggtttcctttctgaaggctgaaatctgggagctgacattctggactccctgagttctgaagagcctggggatggagagacacggagcagaagatggaaggtagagtcccaggtgcctaagatggggaatacatctcccctcattgtcatgagagtccactctagctgatatctactgtggccaatatctaccggtacttttttggggtggacactgagtcatgcagcagtcttatggtttacccaaggtcaggtaggggagacagtgcagtcagagcacaagcccagtgtgtctgacccacccaagaatccatgctcgtatctacaaaaatgattttttctcttgtaatggtgcctaggttcttttattatcatggcatgtgtatgtttttcaactaggttacaatctggccttataaggttaacctcctggaggccaccagccttcctgaaacttgtctgtgctgtccctgcaactggagtgtgcctgatgtggcactccagcctggacaagtgggacacagactccgctgttatcaggcccaaagatgtcttccataagaccagaagagcaatggtgtagaggtgtcatgggctacaataaagatgctgacctcctgtctgagggcaagcagcctcttctggccctcagacaaatgctgagtgttcccaagactaccctcggcctggtccaatctcatcccactggtgcgtaagggttgctgaactcatgacttcttggctagcctgcaacctccacggagtgggaactacatcaggcattttgctaactgctgtatcctaggccaataaatgttgatcacatttatagctgccatggtagggtggggacccctgctatctatctgtggaggctctgggagcccctgacacaaactttctgaagcagagcctccccaaccccttttccattccctatacctgacagatggcccaggaacccattagaaatggaaggtcactgcagcagtatgtgaatgtgcgtgtgggagaagggcaggatcagagccctgggggtgtggcagcccccaagtgattctaatccagatcctagggttgtttccctgtcccattgaaatagctgctttaaggggcctgactcagggaaatcagtctcttgaattaagtggtgattttggagtcatttagaccaggccttcaattgggatccactagttctagagcggccgggcccagggaaccccgcaggcgggggcggccagtttcccgggttcggctttacgtcacgcgagggcggcagggaggacggaatggcggggtttggggtgggtccctcctcgggggagccctgggaaaagaggactgcgtgtgggaagagaaggtggaaatggcgttttggttgacatgtgccgcctgcgagcgtgctgcggggaggggccgagggcagattcgggaatgatggcgcggggtgggggcgtgggggctttctcgggagaggcccttccctggaagtttggggtgcgatggtgaggttctcggggcacctctggaggggcctcggcacggaaagcgaccacctgggagggcgtgtggggaccaggttttgcctttagttttgcacacactgtagttcatctttatggagatgctcatggcctcattgaagccccactacagctctggtagcggtaaccatgcgtatttgacacacgaaggaactagggaaaaggcattaggtcatttcaagccgaaattcacatgtgctagaatccagattccatgctgaccgatgccccaggatatagaaaatgagaatctggtccttaccttcaagaacattcttaaccgtaatcagcctctggtatcttagctccaccctcactggttttttcttgtttgttgaaccggccaagctgctggcctccctcctcaaccgttctgatcatgcttgctaaaatagtcaaaaccccggccagttaaatatgctttagcctgctttattatgattatttttgttgttttggcaatgacctggttacctgttgtttctcccactaaaactttttaagggcaggaatcaccgccgtaactctagcacttagcacagtacttggcttgtaagaggtcctcgatgatggtttgttgaatgaatacattaaataattaaccacttgaaccctaagaaagaagcgattctatttcatattaggcattgtaatgacttaaggtaaagagcagtgctattaacggagtctaactgggaatccagcttgtttgggctatttactagttgtgtggctgtgggcaacttacttcacctctctgggcttaagtcattttatgtatatctgaggtgctggctacctcttggagttattgagaggattataagacagtctatgtgaatcagcaacccttgcatggcccctggcggggaacagtaataatagccatcatcatgtttacttacatagtcctaattagtcttcaaaacagccctgtagcaatggtatgattattaccattttacagatgaggaacctttgaagcctcagagaggctaacagacataccctaggtcatacagttattaagagaaggagctctgtctcgaacctagctctctctctctcgagtaataccagttaaaaaataggctacaaataggtactcaaaaaaatggtagtggctgttgtttttattcagttgctgaggaaaaaatgttgatttttcatctctaaacatcaacttacttaattctgccaatttcttttttttgagacagggtctcactctgtcacctaggatggagtgcagtggcacaatcactgctcactgcagcctcgacttcccgggctcgggtgattctccccaggctcaggggattctcccacttcagcctcccaagtagctgggactacaggtgcgcaccaccatccctggctaatatttgtactttattttatttatttatttatttattttttgagatggagtttcgctcttgttgcccgggctggagtacagtggcatgatctcggctcagtgcaacctctgcctcccgggttcaagcgattctcctacctcatccccctgagtagctgggattacaggcgcctgccaccatgcctggctaattttttgtatttttaatagagacgaggtttcaccatgttggccaggctactctcgaactcctgatctcaggtgatccacccgccttggcctcccaaagtgctgggattacaggcgtgagccactgcgcccggcctaatatttgtattttttgtagagatggtgttttgccatgttgtccaggctggtcttgaactcctgagctcaagcgatctgcccgcctctgcttcccaaagtgctgggattacaggcatgagccaccgtgcctggcctaggtagacgcttttagctttggggtgtgatgcctgccccagtatatagtgaatttaattattgctagagctggctgtttgttagttttctttgaacataagatactcattgtttttagtttgcaaatccctcttcctttttaaaaaatttctttcccttaaattgtttgcatgttagcaataacaaatgcttaaatggtgctatgtgctagatactcttctaagccctgttatgtatattaactaattttttaaattacacaaatcagagaggttaagtaacttgcccaagattacccaacaatactaggatttgaacctaagtttgtctcaccccagattctgctcttaatctctaaacttttaagttagtagtgacaatagtaggtatttattgaatacttaactatgttttaggcgttgaagtaaatattttgcaggcattatctaatgtaaacaccctaaagttacataacaggtaccctttaggtaaataaacactagtatgaccttggaggcacagatagttgaagtaacttgcccaatatcacttacatgaaattggccctcaaatgtgtctgatacaacccatgctgcttgtaactatcgttttaaactgccagggtaaacttggacacacttgagctaagaaaaagcttttagatttttgcaaattaatgtgaaagatatgctttatgtggatataatatcttctaaatttcggggatggtagtcctagaaatgtaatcctgccctagccgagcttaccctgccaataattttttacagaattggtaaaacggagcaccttttttttgtccttggccacactgttatcaacagggtgtagattgacatcaatctgtaggtgtaaaccagaattactctttgtgaccaccaggaaatagagcagttcagttcaggggtttctttctgtgaatttagcactgtgacctgcatactacaagtctactttgttttctatccattgtttgtatctgggtattgcaaaaggtaggaaaaggaccaaccagatcagcagagaagagttgccttggagttttcttttagttttctgcagttcattagatagtaactaggccatgtcattttactcccttgtagtgaagatatgttgaagttgtactggtatactcttctacctttctgtaattttatattgtgtagacttgataaaatttatgtgtcaatcaccaccattaatatcaatattgagcctcaattcttatttttctgcccagtggctgccaaattactaacatttacaataattcactactactaagataatctactagttcgatcacatacttcaaattgttatggaactactgtcttcagcattgtgcttctgataactgataagtataattttttttttgtccagagtgaacatgtctattcttccactgtacacactaataaaaggaaaaattgtaatattgggtaaattcatgtccttacacatgtagtagttatgagcccatgtccctagaatgagtaataatttatccctcccttggttgaatagtcaagaatgctgattttaattcttctaacagctttatccctcagaagggaaggcaagcaagttatatatgtagtttatttgtaagactgatatgaaattggaagatgaatctactattagctttaattatttttacatttaggaatattgcatcagtaactcataattttggttttctgttatcctgagttaacacaaattatccaaggagatggcggatcatctgctttgaggtgtttttttttgagaattttaatgtatctgaatataaaaggtaaaaatatgccaactagcaatttctgcccattccagaagtttggaaatattactcattactaggaattaaataaaatatggtttatctattgttatacctcttttaattcacatagctcatttttatcttttatttttgtttgttttttttgagatggagtcttgctctgtcaccaggcaggagtgcagtgatgcaaatctcggctcactctagccaccgactccctggttcaagcgattctcctgcctgagccttctgagtagctgggattacaggcaggcaccaccacgcccagctaatttttgtagagacaggatttcaccgtgttggccaggatggtctccatctcctgacctcatgatctgcctgcttcggcctcccaaagtgctgggattacaggtgggagccactacgcctggcccacatagctcatttttagactcacttccattaagtcttgtttggacccacgaacattgtctttttttttttaagatggagtttcacttttgttgcccagactgtagtgcaatggtgcaatctcagctcactgcaatctctgcctcctgggttctagcaattctcctgcctcagcctcccgagtagctggaattacaggcgcccgccaccacgcccagctaatttttgtgtttttagtagagacggggtttcaccatgttgggcaggccaggggtgatccgcccacctcagcctcccaaagtgctgggattacaggtgtgagccaccgcatctggccaacatgtcttttttttttttttcctttttaaccacaaagagacttaagcagtccttgtcacagatgatgaattgatgttgcaagtattgtcttagcttggattaattttcttgcttactgtaattttagataatatagctttgtaattagagattttatgtgtaaaccacaaaaatgtttacatgaaggccattattacagatgtgacgtgcataattattagtaatttgtatgtttacatgggtcagtctggcaaaaaattatgaagttttaaaaattaaaaaaaattataatgccagttttactggaaagtaaaattatttcagtaatcgattatagcaaaagtattgattttcattccagacaaaagtcagaatgaaaggtaatttctcaatactctttcagattaataaaagtacctgtagcgatttttatcattcacaagtatatcacaagtaagttagaatttgagaactgtgttctagatctctgaggagatgcagtcagatttctgaactgtctcagcaaatggtaagtaacttagagctagtaattaataacctgtcctttgatttctgattcagccaagaatggccatatttgggaaaggcagatctggagagtaaccacgttttcattcatttaccacttctaggcccctccagagctctcagatattttggggttgagcccttccccaaagccatacaggaccttttttttgtgatctgttctagccatttttatgttgggtgcttgttatggactgagcatttatgtcctcccacaccccccccataccttttttgaagtcctaacccccagtgtgatggtatttggagacagggcctttggaaggtaattacagttagaagaagtcgggagggttgggcccaggtctgattggattagtgcccttatatgaaaagacaccaggacgggcgcagtggctcacacctgtaatcccagcactttgggaggccaaggtgggtggatcacgaggtcaggagtttgagaccagcctggccaatgtagtgaaacaccatctctactaaaaatacaaaaattagctgggtgtggtagcgggctcctgtcatccaagctactcgggagggtgaggcatgagaatcacttgaacccgggagttggaggttgcagtgagcccagattgtgccactgtactccagcctgggtgacagagtgagactctgtctcaaaaaagaaaaaaaaaaaaaaagagacaccagagagcttgttagaagaggtcatgtgagcacacagttagaagaccttcaagccaaagaagaggcctgagattgaaacctaccttgcaggtaccttaattttggacttcccagcctccaaaactgtgagaaataagtttctgttaagtcactcagtctgtggtattttgttatggcagcctgagcaggtagttgttctttcagaaggtgttgataataaccacatgcaacaccaagtcacaaataataaaacagatgtaacttatattcatacagaaagttgggcactgccattgccttgttggtttacacggctgtgctagttcagtagcagaaaggtgctggtctcctttactcagtttacaatctaggcagtagaatgtaatcactgctttaaacttgatactgcttagggagagaatcattggtgctgggtaactttgggttctaggtttactttttgtgtatatataactgtttttggtaaatcacaagtttctgggcttgtcgaattagattttgttacagattatgagctttattatgctatacagttagttgtatgtatatatgcctttcccactagattttaagctttttttttttttttttttttgtgacggagtcttgctcttgtcgcccaggctgaagtggagtgcagtggcacaatctcggctcactgcagcctccacctcctaggttcaagcgattctcctgcctcggcctcccaagtaactgggactacaggcacgtgccaccacacccggctaatttttgtattttttgtagagacagggtttcgccatgttggctaggctggtcttgaacttctggcctcaggtgatccacccgcctcagcctcccaaagtgctgggatttacaggcatgagccaccacgcccagctatagctctttaagggttgtaaatttataatcattcttttactctcctgcaaattctgttgcacactgccttaatcaaggtagatgctgaatgcatttttgtataattgaatatgttgcaatccccaactctctccaactgttcctgtcaaagcagccactggattgttaactaatccatattagatggggttaattaatatcagatgggacaagtaagggctaataagattataggccaccaagtagatttctgtctagctcttatagagattgagtttattggacctgtttgataggaagttttggtgtttgggatgattaaaactgaagttcctatttattgaattatacctatttatattatttcatatcagtggtccacatgcaagtgaggcttctgagacagagtttgagttctctcttcaactaccataacacttaacctgtatctttttttttttttttttttttagacaggagtctcgctctgtcactcaggctggagtgtagtggtatgatctcggctcactgtaacctctgcctcctggattcaagcagttctccatgtctcagcctccctagtagctgggattacaggcctgtgccaccatgcctggctaattttttttttgtatttttagtagagacggggttttaccacgttggccaggctggtctcgaactcttgacctcgagcgatcaacttgccttggcctcccaaagtgctgggattacaggcatgagccacagcgcccagccgtctttttttttaaatagcaatttaacactgttcacagttactcatgtacatgtcatgccatctattacactgtaagttctgtgagggtagctgtatcaaatttatctaactctctctagtatgcatgacatagtaagtattcaataaatatttgcatattagtgataaggatacaggttctgaatagtgggtccttaccatttaagaattagtatttgatggccgggcggggtggctcacgcctgtaatcccagcactttgggaggctgaggcgggcggatcatgagatcaggagatcgagaccatcctggctaacatggtgaaatcccgtctttacaaaaaaaatacaaaagaattaaccaagtgtggtggtgggtgcctgtagtcccagctactgctttgtgaggctgaggcaggcagatcacctgaggtgggaaattcaagaccagcctgaccaacatggagaaaccccatctctactaaaaatacaaaattagccgggcgtggtggcgcatgtctgtaatcccagctactcgggaggctgaggcaggagaatggcgtgaacccgggaggcggagcttgcagtgagccaggatcgcgccactgcactccagcctgggcgacagagcgagactccgtctcaaaaaaaaaaaaaaaaaaaaaattagtatttgatatttgatcattaaatatgaattaagaggacttagactttttgttaaatgtcaagctgggaaaagttgtcatttaaatgaattgcctcttatttaatttcgtctgatgatacattttgtttttattttgtaaaaaattattttttttctttttggagacagggtcttgctctgttgcccaggctggtcacaaactcctgacctcaagcaatcctcctgccttagcctcccaaaatgctgggattacaggcgtgacgacctcgcccggccttgtattatgatacattttgaacaactacaagtagacttggtataatgaacctgcacgtacccattgccaagttctgacaactgtctgtctatagccaattatgcatttcttaaattagaacccccccaatatacccaaatatatatatatgtgtgcatatatatagtaagttgtaacaaagttgtgaattcatacctgaagtatctcaagtgatgcaagttttatgaatttttgtttatgccttttgggaagagttgtattgacaaattttttatgcttaaagtaaaccataaatcaaaaaaataaaatctaggatgcaataaaacaaaacaacttcttgacataagtatggtatgtaaatctgttttgattggaaatcaatttgttatattgccagaattcctgttttagaatacatctctgctgatctgtctgtattcttagactgcatatctgggatgaactctgggcagaattcacatgggcttcctttgaaataaacaagacttttcaaattcttagtcgatctgcagaacctgtagccaggcactgaaccattttgatagatgcagtaatcgttgcaagtgtatatttcaagggagttctggctgggtcctagtttatgcttgtggcagaagcagtgagtaactgggaggaagttggtgagtaagcttcaaggaagaagtcatttttagtactctggatcttcctgattttaaagcactacaaaatggtgcattttcattcttgtcaagtgataacagatatattctgatgagcctgaaatgaatatatattgtatcatttttataatatctagcaaggtttgtattttcctagaacttgaactaaatttcagttcataaaatttataaaatacttagttgttgtaaaatatttttggaatgttcacataggtgacacacaaatgtcccattttcattctttctatagtaaatatgttctgatatgtgaaggtttagcagatgcatcagcatttaatcctagaggatctggcataatcttttcccccaagaatagaaattttttctgcttatgaaagtagtacatgtttctttaaaaacaaatcaatattgacttctgcctgctgtatagcactatgcctccacctggccatgaccaggggcatgtcctggtccacctacctgaaaatgtttgcaaccagcctcctggccatgtgcacaggggctgaagttgtcccacaggtattacgggccaacctgacaatacatgaagttccaccaaagtctgagaactcagaactgagctttggggactgaaagacagcacaaacctcaaatttctcagcactggaaacctcaaaatataactgaattccataaataagattttaagtcttaaatatgtatttttaaatgtattaaaagtcaagctgcttgtatttaagcacctaatacaatgcttaggttgtaaaaggagatgctcaataggtactaactgatatattgagatttaattatggtttgaccaatatttattggaaaccgccaaagcttaaatcatcagcttcttgaatgtgatttgaaaggtaatttagtattgaatagcatgtgagctagagtatttcattctttctggtttatttcttcaaatagactttgaatataatggtgaatgggtattataaattaactaataaaaatgacattgaaaatgaaaaaatatatatattaaagtgtagaaagtgaccaggcgtggtggctcacacctgtaatccaagcaccttgggaggctgaggcaggaggatctcttgatcccaggagttcaagaccagcctgggcaacatagcgagacttcgtctctaaaaaaaaaaaagagagagaaaaaaattttttttatttaaaaaaagtgtagaaagtgtcaagaccccacttcttaccattatttggtatatttctctatacccacccacccttcctccttactccctccctcccttcccaatctttttatctttttgtattctgattttttgtttgtatattttgctttaatttaatgtatcctttaaaaatttcccatacattttatatgtatatataaaaacgcatgctgccaaagataatttataagaaagaccattgaatttttttaaaagtgatatatattcattgaaaaaaatttagaatatatagcaaagcaataaagaactaaataaaattgctgtaactcctctttcaaagataagtgcttttatgattttgttgtatttttttctgtatataggtacatatatagtatttataaagctgtactcatagtacattttcacatcacaggtaccatatcagtgttattaaatattttgtatgccaggggctagacataccaagacaaccaatatgtggttctacttaaataatattagagtatcttttatgatgacacttcatgagttgactataataatcttagacttctaagagtttgggttttcaaaagatcacttagcttttttgggtgatttttcccccttactgtgagatgagagaggctgtttggatttgggattggggtagcggggacagcaacttttcttttctttttcttttttattttgaggtagggtattgctgtgtcacccaggctggagtgcagtggtgtgatctcggctcactgcaacctccacctcccgggctcaggtgatcctcctgcttcagcctcccagtaactgggactacaggcgcgtgccacatgcctggctaattttgtatttttagtagagatggggtttcaccatgttggccaggctggtctctaactcctgacctcaggtgatacgcccacctgggcctcccaaaatactgggattacaggcatgagccgctgcatcagccagcagtttttcttgtggttttttttgtttgttttgttttgttttgtttttgagatagggtcttactctgttgtccacgctggagtgctgtggtatgatcgtagctcactgcagcctcaaactcctgggctcaagtgattccttctgcctccgcctcccgagtagctgggactacaggtatgcaccaccatacctggcaaatttttacaaagttttttgtagggacggggtcttgctacattccccatgtcggtcttgaactcctggcctcaagcaactctcctgtctcagcctcccaaagcactgggattacaagtgtgagccaccacaccatgccagtttttcctgttcagtgtgatattttatcttgttagactacagtgtgttaaaacttgttttactaaattttcaaacatactcaaaagtggagagaatagtataatgaatacccgtatgttcatcacccatgtttagaatattattaaatataaagattttgctgcgtttgtcttagctctttaaaatttttctttttctctttgtgacctaaaggaaattccatatcttatcactttacttctacattcttgactaagatgactaagacatatagttacatggttttttgttttgtttttgttttttaaagacgaaatctcgctcttgtcccccaggctggagtgcaatggtgccatctcagctcagtgcaacctctgccttctgggtacaagcgattctcctgcctcagcctcccaagtagctgggattacaggctcctgccaccacgcctggctaatttttgtatttttagtagagacggcggggggaggtttcaccatgttgacaaggctggtctggaactcctgacctcaggtgatccacccgcctcggcctcccaaagtgctgggattacaggcgtgagccaccgcgcccagcctgtttttttgtttgtgtgttttgttttttttgagacagagtcttgctctgtttcccaggctggagtgaagtggtgccatctcagctcagagacagagtcttgctctgtttcccaggctggagtgaagtggtgccatcttggctcactgcaaccttcacctcccaggttcaagtgattctcctgcctcagcctcccaagtagctgggactacaggcatgtgtcaccacacccggctaatttttttgtatttttagtagagacgggatttcaccgtgttgcccaggctggtctcgaactcctgagctcaggcagtctgcctgcctcagcctcccaaagtgctgggattacacgtgtgaaccaacccgcccggcctgttgttttcttacataattcattatcatacctacaaagttaacagttactaatatcatcttacacctaaatttctctgatagactaaggttattttttaacatcttaatccaatcaaatgtttgtatcctgtaatgctctcattgaaacagctatatttctttttcagattagtgatgatgaaccaggttatgaccttgatttattttgcatacctaatcattatgctgaggatttggaaagggtgtttattcctcatggactaattatggacaggtaagtaagatcttaaaatgaggttttttactttttcttgtgttaatttcaaacatcagcagctgttctgagtacttgctatttgaacataaactaggccaacttattaaataactgatgctttctaaaatcttctttattaaaaataaaagaggagggccttactaattacttagtatcagttgtggtatagtgggactctgtagggaccagaacaaagtaaacattgaagggagatggaagaaggaactctagccagagtcttgcatttctcagtcctaaacagggtaatggactggggctgaatcacatgaaggcaaggtcagatttttattattatgcacatctagcttgaaaattttctgttaagtcaattacagtgaaaaaccttacctggtattgaatgcttgcattgtatgtctggctattctgtgtttttattttaaaattataatatcaaaatatttgtgttataaaatattctaactatggaggccataaacaagaagactaaagttctctcctttcagccttctgtacacatttcttctcaagcactggcctatgcatgtatactatatgcaaaagtacatatatacatttatattttaacgtatgagtatagttttaaatgttattggacacttttaatattagtgtgtctagagctatctaatatattttaaaggttgcatagcattctgtcttatggagataccataactgatttaaccagtccactattgatagacactattttgttcttaccgactgtactagaagaaacattcttttacatgtttggtacttgttcagctttattcaagtggaatttctgggtcaaggggaaagagtttattgaatattttggtattgccaaattttcctctaagaagttgaatcattttatactcctgatgttatatgagagtacctttctcttcacaatttgtctcttttttttttttttttgagacaaggtctctgttgcccaggctggggtgcagtgcagcagaatgatcacagttcactgcagtctcaacctcctgggttcaagcgatccttccacctcagcctcctgagtagctgggactataggtgtgcgccaccactcccagctaatatttttattttgtagaaacagggttcgccatgttacccagcctcccaaagtgctgggattacaggcatgagccactggcccagtttctacagtctctcttaatattgtatattatccagaaaatttcatttaatcagaacctgccagtctgataggtgaaaatggtatcttgtttttatttgcatttaaaaaaaattatgatagtggtatgcttggtttttttgaaggtatcaaattttttaccttatgaaacatgagggcaaaggatgtgatacgtggaagatttaaaaaaaatttttaatgcatttttttgagacaaggtcttgctctattgtccaggctggagtgcagtggcacaatcacagttcactccagcctcaacatcctgcactaaagtgattttcccacctcacctctcaagtagctgggactacaggtacatgctaccatgcctggctaatttttttttttttgcaggcatggggtctcactatattgcccaggttggtgtggaagtttaatgactaagaggtgtttgttataaagtttaatgtatgaaactttctattaaattcctgattttatttctgtaggactgaacgtcttgctcgagatgtgatgaaggagatgggaggccatcacattgtagccctctgtgtgctcaaggggggctataaattctttgctgacctgctggattacatcaaagcactgaatagaaatagtgatagatccattcctatgactgtagattttatcagactgaagagctattgtgtgagtatatttaatatatgattctttttagtggcaacagtaggttttcttatattttctttgaatctctgcaaaccatacttgctttcatttcacttggttacagtgagatttttctaacatattcactagtactttacatcaaagccaatactgtttttttaaaactagtcaccttggaggatatatacttattttacaggtgtgtgtggttttttaaataaactccttttaggaattgctgttgggacttgggatacttttttcactatacatactggtgacagataccctctcttgagctacatcggtttgtggggagtcaaaagtcctttggagctaggtttgacaaataaggtgggttaacacttgtttcctagaaagcacatggagagctagagtattggcgaattgaagaaatccccctttttttttaacacacttaagaaaggggactgcaggtatactcaagagagtaagtcgcaccagaaaccacttttgatccacagtctgcctgtgtcacacaattgaaatgcatcacaacattgacactgtggatgaaacaaaatcagtgtgaattttagtagtgaatttcattcataatttgatcgtgcaaacgtttgatttttattactttagactattgtttctgattttatgttgggttggtatttcctgtgagttactgttttacctttaaaataggaatttttcatactcttcaaagattagaacaaatgtccagtttttgctgtttcatgaatgagtcctgtccatctttgtagaaactcgccttatgttcacatttttattgagaataagaccacttatctacatttaactatcaacctcatcctctccattaatcatctattttagtgacccaagtttttgaccttttccatgtttacatcaatcctgtaggtgattgggcagccatttaagtattattatagacattttcactatcccattaaaaccctttatgcccatacatcataacactacttcctacccataagctccttttaacttgttaaagtcttgcttgaattaaagacttgtttacggtatcgataagcttgatatcaaaacgccaactttgacccggaacgcggaaaacacctgagaaaaacacctgggcgagtctccacgtaaacggtcaaagtccccgcggccctagacaaatattacgcgctatgagtaacacaaaattattcagatttcacttcctcttattcagttttcccgcgaaaatggccaaatcttactcggttacgcccaaatttactacaacatccgcctaaaaccgcgcgaaaattgtcacttcctgtgtacaccggcgcacaccaaaaacgtcacttttgccacatccgtcgcttacatgtgttccgccacacttgcaacatcacacttccgccacactactacgtcacccgccccgttcccacgccccgcgccacgtcacaaactccaccccctcattatcatattggcttcaatccaaaataaggtatattattgatgatgttt

SEQ ID NO: 124 - DNA, 29539 bp, Artificial Sequence
  HDAd2xBITEs
aaacatcatcaataatataccttattttggattgaagccaatatgataatgagggggtggagtttgtgacgtggcgcggggcgtgggaacggggcgggtgacgtaggttttagggcggagtaacttgtatgtgttgggaattgtagttttcttaaaatgggaagtgacgtaacgtgggaaaacggaagtgacgatttgaggaagttgtgggttttttggctttcgtttctgggcgtaggttcgcgtgcggttttctgggtgttttttgtggactttaaccgttacgtcattttttagtcctatatatactcgctctgcacttggcccttttttacactgtgactgattgagctggtgccgtgtcgagtggtgtttttttaataggttttcttttttactggtaggcgcgccgtcgacgcgacaactgtcttattaccctgttatccctaccttaattaagctagccgacgcgttggccaggagctcagatctccggatccaagcttatcgatttcgaacccaaatggatctaccacatttgtagaggttttacttgctttaaaaaacctcccacacctccccctgaacctgaaacataaaatgaatgcaattgttgttgttaacttgtttattgcagcttataatggttacaaataaagcaatagcatcacaaatttcacaaataaagcaatagcatcacaaatttcacaaataaagcatttttttcactgcattctagttgtggtttgtccaaactcatcaatgtatcttatcatgtcgagctagctagtcaggacttcagttccagctttgtgccggctccgaaggtcagcgggttgctagaccattgctgacagtaatatgtggcggcatcctcggcttccatagagctgattgtcaggctgtagctggtgccagatccagatccgctgaatctgtagggcacgccggaggccactttgcttgtgtcgtagatccaccgcttggggcttgtgccagacttctgctgataccagttcatgtaggacacgctgctgctggctctgcatgtcatggtcactttctcgcctggggaagcgctcatgatggcggggctttgtgtcagctgaatatcggagccaccaccaccgcttccaccaccacctgaaccgcctccgccactagaaactgtcagggttgtgccctggccccagtaatccagacagtagtggtcgtcgtagtaccgggcacaatagtacacagcgctatcttcagaggtcaggctggacagctgcatgtaggcggtagagctgctcttgtcggtggtcagtgtggccttgtccttgaacttctggttgtaattggtgtagccccggctggggttgatgtagccgatccattccagtccttggccaggcctctgcttgacccagtgcatggtgtaccgggtgaatgtgtagccgctggtcttgcaggacatcttcacagaggcgccaggtctagccagttcggcgccagactgttgcagcttgatatcggatccaccgccaccaagggctttgatttccagcttggtgccgctgccgaaggtgaaaggggttctgaagtgctgctgacaaaagtacacggccagatcctcggcctgcacgctgctgatggtaaaggtgaagtcagggccagagccagagccggtgaatctagagggcacgcctgtgtatctgctgctggcgctgtagatcagcagcttaggagactggccaggcttctgctgataccaggccacggcgttgtacacgtcctggctggctttacaggtgatggacactctgtcgcccacgctggtgctcagaaacttgtggctctgggtcagctgaatatcagatcctccgccgcctgaacctccgcctccgcttcctccgccaccagaagagactgtcacggttgtgccctggccccaatatggcacgtagccgtggtacacttcccatctggcacaaaagtaggtggccatgtcctcggacttcaggttgttgatctgcaggtaggcggtgttggcgctggtttccaggctgaagtcgaatctgcccttgaaatcgtcggcgaaggtgctctcgccggtgctggtattgatccagcccatccatttcaggccctgtccaggggcctgcttgacccagttcatgccgtagttggtgaaggggtagccgctggccttgcaggagatcttcactgtctcgccaggtttcttcagctcggggccagactgctgcagctgaacttcagaatgggcgcctgtggcggctcccacaagaaacaggatgcgccagatccagtccatggaaggtccggggttctcttccacgtcgccacatgtcagcaggctgcctctgccttcggacttcagttccagctttgtgccggctccgaaggtcagcgggttgctagaccattgctgacagtaatatgtggcggcatcctcggcttccatgctggagattgtcaggctgtagctggttccgctgccgcttccggaaaatctgtagggcacgccggaggccactttgcttgtgtcgtagatccaccgcttggggcttgtgccagacttctgctgataccagttcatgtaggacacgctggagctggctctacaggtcatggtcactttctcgcctgggctagcgctcatgatggcaggagactgggtcagctgaatatcagaaccgccaccaccgcttccgccgccacctgaaccaccaccacctgaagaaactgtcagtgtggtgccctggccccagtaatccagacagtagtggtcgtcgtagtaccgggcacaatagtacacagcgctatcttcagaggtcaggctgctcagctgcatgtaggcggtagagctgctcttgtcggtggtcagagtggccttgtccttgaacttctggttgtaattggtgtagccccggctggggttgatgtagccgatccattccagtccttggccaggcctctgcttgacccagtgcatggtgtaccgggtgaatgtgtatccgctggtcttgcagctcatcttcacagaagcgccaggtctagccagctcggcgccagactgttgcagcttaatatcgctgcctccgcctccgccactagacactgtgaccagtgttcctctgccccagtagtcgaggccctgtctggcgcaataatacacggcggtgtcctcggctctcagggagttcatctgcaggtacaggctgttcttggcgttgtcccggctgatggtgaatctgcccttgatgctgtccaggtagtaggtgtagctgccgccgctgctgattgtggacacccattcaaggcctttgccaggagcctgtcggacccagctcatatcgtagctgctgaaggtgaagccgctggcggcacaagacagtctcagagatccgccaggcttaaccaggcctccgcctgattccaccagctgaacttcagatccaccaccgccggatccgccgcctccgcttcctccgccgccagatcctccgccacctctcttgatttccaccttggtgcctccgccaaatgtcaggggattgctggaccactgcaggcagtagtacacggcgaagtcctcaggttccaggctgcttatggtcagggtgaaatcggtgccgctgccagagccagaaaatctggcaggcactccgctggccagattgctggtcaggtagatcaggattctaggggcctgtccgggcttctgctgcagccagtagatgtagttgatggagctgctggcgctacagctcagtgtggctctttcgccagggctaagagacagtgtggcagggctctgtgtcagcacaatctcgccggtggtatcaggcagccacagcagcagcagaaacagcagttgagctggagcctccatggtggccctccttcgccggtgatctcagctgtaggaaagagaagaaggttagtagtcgacgtgtccctctcgatgaatctaagtatcaattgtgagcgctcacaagtcaacactctttttgataaatctagtagatatcacttacgtaggcgccggtcacagcttggatctgtaacggcgcagaacagaaaacgaaacaaagacgtagagttgagcaagcagggtcaggcaaagcgtggagagccggctgagtctaggtaggctccaagggagcgccggacaaaggcccggtctcgacctgagctttaaacttacctagacggcggacgcagttcaggaggcaccacaggcgggaggcggcagaacgcgactcaaccggcgtggatggcggcctcaggtagggcggcgggcgcgtgaaggagagatgcgagcccctcgaagcttcagctgtgttctggcggcaaacccgttgcgaaaaagaacgttcacggcgactactgcacttatatacggttctcccccaccctcgggaaaaaggcggagccagtacacgacatcactttcccagtttaccccgcgccaccttctctaggcaccggttcaattgccgacccctccccccaacttctcggggactgtgggcgatgtgcgctctgcccactgacgggcaccggagcgatcgcagatccttcgatagagaaatgttctggcacctgcacttgcactggggacagcctattttgctagtttgttttgtttcgttttgttttgatggagagcgtatgttagttacgattcacacaaaaaaccaacacacagatgtaatgaaaataaagatattttattgcggccgctcgagtctagaggtatacatgccatggtccgcggtattaccctgttatccctaagacaactgtcctgcatgcgacgtcggcgcgccatcgaattcctgcagcccgggggatccctttgttgattttttccacatagattatttttgactgttttggcactttatataaatggaatcatatagtaaatatatacatgtatatatgtatatatacactatatatgtatatatatagtgtatatatatacatgtatatatgtatatttacatatatactgtatatatgtatatttacatatatactgtatatatgtatatatacacgtatatactgtatatatacagtatatactgtatatatatactgtatatatgtgtatatatatatacagtatatatacagtatacatatatatacatgtatatatacacagtatatatacatgtatatatacacagtatatatacatgtatatatacacagtatatatacatgtatatatacacagtatatatacactgtatatatgtatatatatactgtgtatatatatacagtatatatacagtatatatatacatgtatatgtatatatatactgtatatatgtgtatatatacgtatatatactgtatatatatatagacacttttgtgtctggcttcttgctctcatcataaagcacttgaaatccatccatgttgtagctggtatcagtagctagtttcttttcattgctgagaagtatcactttttattgatgagtagttttacattgtatgaacatgcccgagtttgtttatgcattctactaatagacacctgggctgtttgcagtttttggctattacaaagaaaatttctatatttttttccaacttttattttaggttcagcgggtacatgggcaggtttgttacatcggtaaattgcatgtcactggggtttggtgtacagattatttcaccacccaggtaataagcatagtacctgataggcaggtttttgatcctcaccctcctccctcaagtaggccccagtgtctattgttctattccttttttttttttttgagatggagtctcactctgttgcccaggctggagtgcagtggtgcgatctcggctcactgcaaggtccacctccagggttcaagcgattctactgccgcagcctcccgagtagctgggattacaggcacccaccaccacgcccggctaatttttgtatttttagtagagactgggtttcaccatgttggccaggatggtctcgaactcctcacctcaggtgatccgcccgcttcggcctcgcaaagtactgggattacaggcgtgagccacggtgcctggcctatggttccattctttgtgtacacgtgtactcagtgtttagcttccacttgtaagtgaaaacatgcagtatttggttttctgaaattcttgtcttcatctttttgtagacaatccactacttttatttttaaatattaggaacaatagcctctgtgtgtcctgaattgcaatgttttttctctgattttgctgctcatcttgtaacctgtatggtgtttttctgtgtgcaagctttttactttacgtgggcaattttatcattcttttcttttatggtttctgggtttcatgtcatgattggagaagcttgatctaccctgatactataaaaatatccaccttggcttttttttttttttttagatggattttcactcttgttgcccaggctggagtgcaatggcgtgatctcggctcaccacaacctctgcctcccaggttcaagtgattctcctgcctcggcctcctgagtagctgggattacaggcatgcgccaccacgctcagctaattttgtatttttagtagagacaggatttcaccatgttggtcaggctggtcttgaactccccacctcaggtgatctgtctgcctcggcctcccaaagtgctgggattacaggcgtgacccaccacacctggcccacgttgttttctgatagtgttttcacgtgttattttttctgtcttactctttgaatcatctaaatgtatcttaatgtcaggagtgaggtagaggacccagttgtttggtttaaatgactagccagttttcccaacaccaggtgttgaacatccctcactgatgtgagatgctgcctttttcacagtctcaatccccatgtgcatttctatttattttccttccactttattcacatctttttcagtatccacaaccatattgttttaaatagcttcatgatatgttttaatatttggtagagctagaaccctttcttggttctttttcttttcttcttctcctccttttcctcctccttctttctcctcctccttcttctttctttttagaaatttcctggctattcttgttttgtagtcttccagataaataattttgaatcactttgtcatgttccagaaaataatactgccagaatttttattgtgatcacagaagttttacagattcatctgggggaaaaaaacccatcttcccagaatacagaaagggtgagggaaagacaaacatcaaggacaagtctcaggttctggacttggagaccaagaggatttggggcatccgggagcagggcagggaggtgtgatggctgcctttcactgagtaggaggatgcccagacttgggggaactatggaaagtttggttcagactttctgagttggagatgtctatgcgcagtccacagggcgaagccctggaggtagaggccctccttactgcctccctcattcagtctgaggtccattctccacatggacactgaagtgactcaaggcttcccttgttggatcaggatagtctccagggccctgggtggtctgggcctgcccacctccccatcccctctcctgcctgccctcctcttgctcactggaccccacccaccagcctccttctattcctcctgacatttgcacttgctgttccgtctctgcttggaacatcctagctctttgcatggcttgctccttcccatcttttaatctaagctcaaatatcactccttcagatatgcctttcccaaatatcctagctaaagagaactgctccccacttcccacaagccctagcaaactgggactctccttcttgctttctttctctctgccccttctgtgttttttccatagaccttaacttgttactgttttatttgttgatgtgtttacatcatttgtccccctgtgatggttagttttatgtgtcaacttggctaggctgtaggggctgttcgtcaatcaaacactgatctatgtgtagctgtgaagggattttgtagctgtgattaatagttgactttaagtaaggaagattatcctggagaatgtgggggaaggggcagacctcagccaatcagttgaaaggccttaagaacaaagctgagatttccccgaggaagaagaaattctgcctgtggactgcagcatcagctcctgcttgagaggttccaggctgcccttcctgacagcctgtcctatgattttggacttgccttgccaggtttttcctctttcttgaccccccaaaaccatatatatctcctgctggtttgtttctctggtgtaatcctgagggatgaacactcctccctcccagttcactctgggagaggttggggatcatgtttgtctatttccccatgcctggcccatgcgtgtttattgaatcactgaacaaccacgcattaggaagccagtcatatgtgcttcttcagaacctcatgtccattgccagatctccctggcttttgtggctagaggacaagtgagagatagtagcttacccacagaccttggccctgaggcccccaggggcctgagcctgctgtaagggaggagggagcccctgaggtctcacacacctccctggggatctggcattttcccctggggctggcctcagagctgggcgggggcagattatggagtgggttgtagagggagcacctccccactagcaatcatggttttttctgcgcctctcatagggaggcctacaggcctccaccttcagctcttcaggagccacaggcagctgagtgacttctgcatcacagtcttctcagagacaaacttgcagtaagaaagaggggcccgtgagggaccccagagaaggctgttgtcaaagcaggatgagagtgaactcttccatgggggacacccagcgtctccaagctcttttatgctgtcttcaaggggtctagagagcttcagcccaacatgagacccagtccagcagcatttccctgcgaagtgaaagttaggaccctgactagatacaccacgctgacctcagccagaatatcaagatgctgaggcgctgagatgctgggatgctaaggtgctaaggtgctggggtgctggggtgctaggatgctgaggttttgtgatactgggtcgctgagatgctgggatactggggtgctgaagtgctggggtactggggtgttgccatgctgaaatgctggggtgttgggatgctgaggtgctgggttgctgggatgctgggatagtccttggatgctgcggtgctgagatgctggtctgctggtctgctggggtgttgggatgctgggattttgggatgctggagtgctgcagtgctgcagtgctgagatgctggagtgctggggtgctggaatactgtagtactggtgtgctggagcattgagatgctagggcactgggatgctaaggtgctgagatgctgcagtgctggggtgttgggatgccgaggtgttgggatgcttaagtgctggggtgttgggatgctggggtgctggaacactatggtgctggggtgctggagtgttgagatactgtagtggtgggatgcttaagtgctggggtgctgggtgttgggatgcctaggtgctggggtgccgagatgctggagtactagtgtgctgggatgctgaagtgctggggtcctgagatgctgcagtgctagggtgctgagattctgggctgctggagtgttggggtgctgggatgctggagtgctgagatgcttggacaatggggtgctggaatactatggtgctggggtgctggggtattgagatgctagggtactgggatgctgaagtgctgagatcctggagtgctgggctgctgggccacaggctcttgaatccattcgtctgcccaggggaagaaaccagaagataaagagctaatgaaggagctttggttgagagggaggaagtaatggaaggagcaacatcttgtggaggagcaggagagaatggacctcaggttgggagagagggccaggctacaggccagagaggcagaaggattccagcagagtgtgggctccaggagccaaggggaaacaggtttctgggaggagagagtccagtactgctgaagtggcaagtccgctgaggaccaggaagcttcatttggctttatgaccaggaggaatttggaactgtgactagagtacttagggggaaggaggcaagactggagccagattgctctgggttgaggggtgagtgggaggtgaagcagggcactgtcactcctttgaagggtggcagagagctggaattggtgctggatgggctgtggggtgacagggtcatgtggaaagcccctggggggcacctggaaaaggagaagctgacagtacagtgagaggacagctaagggaaagcggaatggcagaacacgcactgccaggaggaatgaggatagggtcaggagtgccaggggcagtgaggccagcctggggtcaggtggcaggacgtgtccaggaagctggtctgcactgcagcccacactggctcagccttgaggttccctgtgtggttggggtaggaagttgaaccctctgggaatggaagatggaaccagctctgcgagccaagctcagcttttatctatgggtctctgagggctggcagagctgagtggggacaactgtgatccgtgaggctctcaggttgaggtggcccctccgggagggcttcattttcccagcgggtaggttctaagcagcagtggctgggcaggtgggtccaacacagagccagagaagggtgaatgggcctcctggcaccccacccctgctgcccctgagctcagtgatggagggggacagcacagctgagcccaagtgctttggtgtggccctgagggaaagctgcagcctgcctggggcctggcatggatgggacacttgaggcagagggacaatagtgggcgctgcagtgaggctggctcttggagaggtttcctgaggagtgctgcctgagacgggcagggagaacagagacaaagttggtgacagggaatgaaagctgactgaaggactttacccagacctatgaggatatctctctcagcaggaagcaggaggggactgtgtgaggactggccaagagctggagtgttgggaaaatgactctttctccgacccctctgtcctagctctggcccctggactgcggaggtctgcttccacccccattggtcgatcgttgtcccttgtcacagccattgagaattttggcagggagcatgttcttagagcatttttaggctctgcgggacataacagctctgcctcagagcacatgcctttctcagctcctgaaagccactgatcaaattggaacattttgtaccttagggatgaggatatcaactctcccagccacttagagggataaatgtgatgatgcattcaattgtgactacatctgatcccaactgttgcttcagctgctctcctatagcacatggcgggaggcgtgcatcccagtagctacctccccacttttggggagatgtggttccatccatgaaacctgggtacccgcctaccaggtcctggcctatcaggtggcagggtctggtcaaagaagggcatgtgtggtcttcagcaagggagacaggacggtggtgcagagcgtctagaccctcagggcaagtctcccccacacctgctcccggggcagttgtctttgtgacctcccatccccctctgtttcatcctctataaaatgaggggctgagccccaaaataacaggcttctttgccatgatgcaaaactgctgaatctttctttctgacacacaaggcatcgagcagcctctgaaagaaccaaagccactagcaggcttcctgacttgggtttgtaggtactgaatactcccttgaaaaataaaaacatagaggcacttttctcctggctgtttattacagaacgaagaaaaaacacactggcttgaaacagacgccagatttcaaatgtagaggtgaaatacgaggtggcaattaaaatgtgattacagaaagtctggacactgagaaaagtttacaggacagtgggtgtgggttttctataacagacacttaaatatacatgacgataattgcagatagaaaccatcaaagacaaaccccaaatcaactaataatgtttacagatgttcccccccaaaccacagagccttacatcaaaacaaatactgaaaggctttaaaccaggaacagctcgccttaaccccacgagggtgcacacaagctgggctttttctctcggtctgaatggtaaagggaggaggatactctagctcctccaggtggattgctgagacagggctcggctcacacactgtctctgcgcctctcccaaatctggagaactctcccagcctcctggtaaagtgtctctgtggggcacttaacgataaaacagcttctgctgtaaagctcattaggaaagagctagcctgcaacctccacggagtgggaactacatcaggcattttgctaactgctgtatcctaggccaataaatgttgatcacatttatagctgccatggtagggtggggacccctgctatctatctgtggaggctctgggagcccctgacacaaactttctgaagcagagcctccccaaccccttttccattccctatacctgacagatggcccaggaacccattagaaatggaaggtcactgcagcagtatgtgaatgtgcgtgtgggagaagggcaggatcagagccctgggggtgtggcagcccccaagtgattctaatccagatcctagggttgtttccctgtcccattgaaatagctgctttaaggggcctgactcagggaaatcagtctcttgaattaagtggtgattttggagtcatttagaccaggccttcaattgggatccactagttctagagcggccgggcccagggaaccccgcaggcgggggcggccagtttcccgggttcggctttacgtcacgcgagggcggcagggaggacggaatggcggggtttggggtgggtccctcctcgggggagccctgggaaaagaggactgcgtgtgggaagagaaggtggaaatggcgttttggttgacatgtgccgcctgcgagcgtgctgcggggaggggccgagggcagattcgggaatgatggcgcggggtgggggcgtgggggctttctcgggagaggcccttccctggaagtttggggtgcgatggtgaggttctcggggcacctctggaggggcctcggcacggaaagcgaccacctgggagggcgtgtggggaccaggttttgcctttagttttgcacacactgtagttcatctttatggagatgctcatggcctcattgaagccccactacagctctggtagcggtaaccatgcgtatttgacacacgaaggaactagggaaaaggcattaggtcatttcaagccgaaattcacatgtgctagaatccagattccatgctgaccgatgccccaggatatagaaaatgagaatctggtccttaccttcaagaacattcttaaccgtaatcagcctctggtatcttagctccaccctcactggttttttcttgtttgttgaaccggccaagctgctggcctccctcctcaaccgttctgatcatgcttgctaaaatagtcaaaaccccggccagttaaatatgctttagcctgctttattatgattatttttgttgttttggcaatgacctggttacctgttgtttctcccactaaaactttttaagggcaggaatcaccgccgtaactctagcacttagcacagtacttggcttgtaagaggtcctcgatgatggtttgttgaatgaatacattaaataattaaccacttgaaccctaagaaagaagcgattctatttcatattaggcattgtaatgacttaaggtaaagagcagtgctattaacggagtctaactgggaatccagcttgtttgggctatttactagttgtgtggctgtgggcaacttacttcacctctctgggcttaagtcattttatgtatatctgaggtgctggctacctcttggagttattgagaggattataagacagtctatgtgaatcagcaacccttgcatggcccctggcggggaacagtaataatagccatcatcatgtttacttacatagtcctaattagtcttcaaaacagccctgtagcaatggtatgattattaccattttacagatgaggaacctttgaagcctcagagaggctaacagacataccctaggtcatacagttattaagagaaggagctctgtctcgaacctagctctctctctctcgagtaataccagttaaaaaataggctacaaataggtactcaaaaaaatggtagtggctgttgtttttattcagttgctgaggaaaaaatgttgatttttcatctctaaacatcaacttacttaattctgccaatttcttttttttgagacagggtctcactctgtcacctaggatggagtgcagtggcacaatcactgctcactgcagcctcgacttcccgggctcgggtgattctccccaggctcaggggattctcccacttcagcctcccaagtagctgggactacaggtgcgcaccaccatccctggctaatatttgtactttattttatttatttatttatttattttttgagatggagtttcgctcttgttgcccgggctggagtacagtggcatgatctcggctcagtgcaacctctgcctcccgggttcaagcgattctcctacctcatccccctgagtagctgggattacaggcgcctgccaccatgcctggctaattttttgtatttttaatagagacgaggtttcaccatgttggccaggctactctcgaactcctgatctcaggtgatccacccgccttggcctcccaaagtgctgggattacaggcgtgagccactgcgcccggcctaatatttgtattttttgtagagatggtgttttgccatgttgtccaggctggtcttgaactcctgagctcaagcgatctgcccgcctctgcttcccaaagtgctgggattacaggcatgagccaccgtgcctggcctaggtagacgcttttagctttggggtgtgatgcctgccccagtatatagtgaatttaattattgctagagctggctgtttgttagttttctttgaacataagatactcattgtttttagtttgcaaatccctcttcctttttaaaaaatttctttcccttaaattgtttgcatgttagcaataacaaatgcttaaatggtgctatgtgctagatactcttctaagccctgttatgtatattaactaattttttaaattacacaaatcagagaggttaagtaacttgcccaagattacccaacaatactaggatttgaacctaagtttgtctcaccccagattctgctcttaatctctaaacttttaagttagtagtgacaatagtaggtatttattgaatacttaactatgttttaggcgttgaagtaaatattttgcaggcattatctaatgtaaacaccctaaagttacataacaggtaccctttaggtaaataaacactagtatgaccttggaggcacagatagttgaagtaacttgcccaatatcacttacatgaaattggccctcaaatgtgtctgatacaacccatgctgcttgtaactatcgttttaaactgccagggtaaacttggacacacttgagctaagaaaaagcttttagatttttgcaaattaatgtgaaagatatgctttatgtggatataatatcttctaaatttcggggatggtagtcctagaaatgtaatcctgccctagccgagcttaccctgccaataattttttacagaattggtaaaacggagcaccttttttttgtccttggccacactgttatcaacagggtgtagattgacatcaatctgtaggtgtaaaccagaattactctttgtgaccaccaggaaatagagcagttcagttcaggggtttctttctgtgaatttagcactgtgacctgcatactacaagtctactttgttttctatccattgtttgtatctgggtattgcaaaaggtaggaaaaggaccaaccagatcagcagagaagagttgccttggagttttcttttagttttctgcagttcattagatagtaactaggccatgtcattttactcccttgtagtgaagatatgttgaagttgtactggtatactcttctacctttctgtaattttatattgtgtagacttgataaaatttatgtgtcaatcaccaccattaatatcaatattgagcctcaattcttatttttctgcccagtggctgccaaattactaacatttacaataattcactactactaagataatctactagttcgatcacatacttcaaattgttatggaactactgtcttcagcattgtgcttctgataactgataagtataattttttttttgtccagagtgaacatgtctattcttccactgtacacactaataaaaggaaaaattgtaatattgggtaaattcatgtccttacacatgtagtagttatgagcccatgtccctagaatgagtaataatttatccctcccttggttgaatagtcaagaatgctgattttaattcttctaacagctttatccctcagaagggaaggcaagcaagttatatatgtagtttatttgtaagactgatatgaaattggaagatgaatctactattagctttaattatttttacatttaggaatattgcatcagtaactcataattttggttttctgttatcctgagttaacacaaattatccaaggagatggcggatcatctgctttgaggtgtttttttttgagaattttaatgtatctgaatataaaaggtaaaaatatgccaactagcaatttctgcccattccagaagtttggaaatattactcattactaggaattaaataaaatatggtttatctattgttatacctcttttaattcacatagctcatttttatcttttatttttgtttgttttttttgagatggagtcttgctctgtcaccaggcaggagtgcagtgatgcaaatctcggctcactctagccaccgactccctggttcaagcgattctcctgcctgagccttctgagtagctgggattacaggcaggcaccaccacgcccagctaatttttgtagagacaggatttcaccgtgttggccaggatggtctccatctcctgacctcatgatctgcctgcttcggcctcccaaagtgctgggattacaggtgggagccactacgcctggcccacatagctcatttttagactcacttccattaagtcttgtttggacccacgaacattgtctttttttttttaagatggagtttcacttttgttgcccagactgtagtgcaatggtgcaatctcagctcactgcaatctctgcctcctgggttctagcaattctcctgcctcagcctcccgagtagctggaattacaggcgcccgccaccacgcccagctaatttttgtgtttttagtagagacggggtttcaccatgttgggcaggccaggggtgatccgcccacctcagcctcccaaagtgctgggattacaggtgtgagccaccgcatctggccaacatgtcttttttttttttttcctttttaaccacaaagagacttaagcagtccttgtcacagatgatgaattgatgttgcaagtattgtcttagcttggattaattttcttgcttactgtaattttagataatatagctttgtaattagagattttatgtgtaaaccacaaaaatgtttacatgaaggccattattacagatgtgacgtgcataattattagtaatttgtatgtttacatgggtcagtctggcaaaaaattatgaagttttaaaaattaaaaaaaattataatgccagttttactggaaagtaaaattatttcagtaatcgattatagcaaaagtattgattttcattccagacaaaagtcagaatgaaaggtaatttctcaatactctttcagattaataaaagtacctgtagcgatttttatcattcacaagtatatcacaagtaagttagaatttgagaactgtgttctagatctctgaggagatgcagtcagatttctgaactgtctcagcaaatggtaagtaacttagagctagtaattaataacctgtcctttgatttctgattcagccaagaatggccatatttgggaaaggcagatctggagagtaaccacgttttcattcatttaccacttctaggcccctccagagctctcagatattttggggttgagcccttccccaaagccatacaggaccttttttttgtgatctgttctagccatttttatgttgggtgcttgttatggactgagcatttatgtcctcccacaccccccccataccttttttgaagtcctaacccccagtgtgatggtatttggagacagggcctttggaaggtaattacagttagaagaagtcgggagggttgggcccaggtctgattggattagtgcccttatatgaaaagacaccaggacgggcgcagtggctcacacctgtaatcccagcactttgggaggccaaggtgggtggatcacgaggtcaggagtttgagaccagcctggccaatgtagtgaaacaccatctctactaaaaatacaaaaattagctgggtgtggtagcgggctcctgtcatccaagctactcgggagggtgaggcatgagaatcacttgaacccgggagttggaggttgcagtgagcccagattgtgccactgtactccagcctgggtgacagagtgagactctgtctcaaaaaagaaaaaaaaaaaaaaagagacaccagagagcttgttagaagaggtcatgtgagcacacagttagaagaccttcaagccaaagaagaggcctgagattgaaacctaccttgcaggtaccttaattttggacttcccagcctccaaaactgtgagaaataagtttctgttaagtcactcagtctgtggtattttgttatggcagcctgagcaggtagttgttctttcagaaggtgttgataataaccacatgcaacaccaagtcacaaataataaaacagatgtaacttatattcatacagaaagttgggcactgccattgccttgttggtttacacggctgtgctagttcagtagcagaaaggtgctggtctcctttactcagtttacaatctaggcagtagaatgtaatcactgctttaaacttgatactgcttagggagagaatcattggtgctgggtaactttgggttctaggtttactttttgtgtatatataactgtttttggtaaatcacaagtttctgggcttgtcgaattagattttgttacagattatgagctttattatgctatacagttagttgtatgtatatatgcctttcccactagattttaagctttttttttttttttttttttgtgacggagtcttgctcttgtcgcccaggctgaagtggagtgcagtggcacaatctcggctcactgcagcctccacctcctaggttcaagcgattctcctgcctcggcctcccaagtaactgggactacaggcacgtgccaccacacccggctaatttttgtattttttgtagagacagggtttcgccatgttggctaggctggtcttgaacttctggcctcaggtgatccacccgcctcagcctcccaaagtgctgggatttacaggcatgagccaccacgcccagctatagctctttaagggttgtaaatttataatcattcttttactctcctgcaaattctgttgcacactgccttaatcaaggtagatgctgaatgcatttttgtataattgaatatgttgcaatccccaactctctccaactgttcctgtcaaagcagccactggattgttaactaatccatattagatggggttaattaatatcagatgggacaagtaagggctaataagattataggccaccaagtagatttctgtctagctcttatagagattgagtttattggacctgtttgataggaagttttggtgtttgggatgattaaaactgaagttcctatttattgaattatacctatttatattatttcatatcagtggtccacatgcaagtgaggcttctgagacagagtttgagttctctcttcaactaccataacacttaacctgtatctttttttttttttttttttttagacaggagtctcgctctgtcactcaggctggagtgtagtggtatgatctcggctcactgtaacctctgcctcctggattcaagcagttctccatgtctcagcctccctagtagctgggattacaggcctgtgccaccatgcctggctaattttttttttgtatttttagtagagacggggttttaccacgttggccaggctggtctcgaactcttgacctcgagcgatcaacttgccttggcctcccaaagtgctgggattacaggcatgagccacagcgcccagccgtctttttttttaaatagcaatttaacactgttcacagttactcatgtacatgtcatgccatctattacactgtaagttctgtgagggtagctgtatcaaatttatctaactctctctagtatgcatgacatagtaagtattcaataaatatttgcatattagtgataaggatacaggttctgaatagtgggtccttaccatttaagaattagtatttgatggccgggcggggtggctcacgcctgtaatcccagcactttgggaggctgaggcgggcggatcatgagatcaggagatcgagaccatcctggctaacatggtgaaatcccgtctttacaaaaaaaatacaaaagaattaaccaagtgtggtggtgggtgcctgtagtcccagctactgctttgtgaggctgaggcaggcagatcacctgaggtgggaaattcaagaccagcctgaccaacatggagaaaccccatctctactaaaaatacaaaattagccgggcgtggtggcgcatgtctgtaatcccagctactcgggaggctgaggcaggagaatggcgtgaacccgggaggcggagcttgcagtgagccaggatcgcgccactgcactccagcctgggcgacagagcgagactccgtctcaaaaaaaaaaaaaaaaaaaaaattagtatttgatatttgatcattaaatatgaattaagaggacttagactttttgttaaatgtcaagctgggaaaagttgtcatttaaatgaattgcctcttatttaatttcgtctgatgatacattttgtttttattttgtaaaaaattattttttttctttttggagacagggtcttgctctgttgcccaggctggtcacaaactcctgacctcaagcaatcctcctgccttagcctcccaaaatgctgggattacaggcgtgacgacctcgcccggccttgtattatgatacattttgaacaactacaagtagacttggtataatgaacctgcacgtacccattgccaagttctgacaactgtctgtctatagccaattatgcatttcttaaattagaacccccccaatatacccaaatatatatatatgtgtgcatatatatagtaagttgtaacaaagttgtgaattcatacctgaagtatctcaagtgatgcaagttttatgaatttttgtttatgccttttgggaagagttgtattgacaaattttttatgcttaaagtaaaccataaatcaaaaaaataaaatctaggatgcaataaaacaaaacaacttcttgacataagtatggtatgtaaatctgttttgattggaaatcaatttgttatattgccagaattcctgttttagaatacatctctgctgatctgtctgtattcttagactgcatatctgggatgaactctgggcagaattcacatgggcttcctttgaaataaacaagacttttcaaattcttagtcgatctgcagaacctgtagccaggcactgaaccattttgatagatgcagtaatcgttgcaagtgtatatttcaagggagttctggctgggtcctagtttatgcttgtggcagaagcagtgagtaactgggaggaagttggtgagtaagcttcaaggaagaagtcatttttagtactctggatcttcctgattttaaagcactacaaaatggtgcattttcattcttgtcaagtgataacagatatattctgatgagcctgaaatgaatatatattgtatcatttttataatatctagcaaggtttgtattttcctagaacttgaactaaatttcagttcataaaatttataaaatacttagttgttgtaaaatatttttggaatgttcacataggtgacacacaaatgtcccattttcattctttctatagtaaatatgttctgatatgtgaaggtttagcagatgcatcagcatttaatcctagaggatctggcataatcttttcccccaagaatagaaattttttctgcttatgaaagtagtacatgtttctttaaaaacaaatcaatattgacttctgcctgctgtatagcactatgcctccacctggccatgaccaggggcatgtcctggtccacctacctgaaaatgtttgcaaccagcctcctggccatgtgcacaggggctgaagttgtcccacaggtattacgggccaacctgacaatacatgaagttccaccaaagtctgagaactcagaactgagctttggggactgaaagacagcacaaacctcaaatttctcagcactggaaacctcaaaatataactgaattccataaataagattttaagtcttaaatatgtatttttaaatgtattaaaagtcaagctgcttgtatttaagcacctaatacaatgcttaggttgtaaaaggagatgctcaataggtactaactgatatattgagatttaattatggtttgaccaatatttattggaaaccgccaaagcttaaatcatcagcttcttgaatgtgatttgaaaggtaatttagtattgaatagcatgtgagctagagtatttcattctttctggtttatttcttcaaatagactttgaatataatggtgaatgggtattataaattaactaataaaaatgacattgaaaatgaaaaaatatatatattaaagtgtagaaagtgaccaggcgtggtggctcacacctgtaatccaagcaccttgggaggctgaggcaggaggatctcttgatcccaggagttcaagaccagcctgggcaacatagcgagacttcgtctctaaaaaaaaaaaagagagagaaaaaaattttttttatttaaaaaaagtgtagaaagtgtcaagaccccacttcttaccattatttggtatatttctctatacccacccacccttcctccttactccctccctcccttcccaatctttttatctttttgtattctgattttttgtttgtatattttgctttaatttaatgtatcctttaaaaatttcccatacattttatatgtatatataaaaacgcatgctgccaaagataatttataagaaagaccattgaatttttttaaaagtgatatatattcattgaaaaaaatttagaatatatagcaaagcaataaagaactaaataaaattgctgtaactcctctttcaaagataagtgcttttatgattttgttgtatttttttctgtatataggtacatatatagtatttataaagctgtactcatagtacattttcacatcacaggtaccatatcagtgttattaaatattttgtatgccaggggctagacataccaagacaaccaatatgtggttctacttaaataatattagagtatcttttatgatgacacttcatgagttgactataataatcttagacttctaagagtttgggttttcaaaagatcacttagcttttttgggtgatttttcccccttactgtgagatgagagaggctgtttggatttgggattggggtagcggggacagcaacttttcttttctttttcttttttattttgaggtagggtattgctgtgtcacccaggctggagtgcagtggtgtgatctcggctcactgcaacctccacctcccgggctcaggtgatcctcctgcttcagcctcccagtaactgggactacaggcgcgtgccacatgcctggctaattttgtatttttagtagagatggggtttcaccatgttggccaggctggtctctaactcctgacctcaggtgatacgcccacctgggcctcccaaaatactgggattacaggcatgagccgctgcatcagccagcagtttttcttgtggttttttttgtttgttttgttttgttttgtttttgagatagggtcttactctgttgtccacgctggagtgctgtggtatgatcgtagctcactgcagcctcaaactcctgggctcaagtgattccttctgcctccgcctcccgagtagctgggactacaggtatgcaccaccatacctggcaaatttttacaaagttttttgtagggacggggtcttgctacattccccatgtcggtcttgaactcctggcctcaagcaactctcctgtctcagcctcccaaagcactgggattacaagtgtgagccaccacaccatgccagtttttcctgttcagtgtgatattttatcttgttagactacagtgtgttaaaacttgttttactaaattttcaaacatactcaaaagtggagagaatagtataatgaatacccgtatgttcatcacccatgtttagaatattattaaatataaagattttgctgcgtttgtcttagctctttaaaatttttctttttctctttgtgacctaaaggaaattccatatcttatcactttacttctacattcttgactaagatgactaagacatatagttacatggttttttgttttgtttttgttttttaaagacgaaatctcgctcttgtcccccaggctggagtgcaatggtgccatctcagctcagtgcaacctctgccttctgggtacaagcgattctcctgcctcagcctcccaagtagctgggattacaggctcctgccaccacgcctggctaatttttgtatttttagtagagacggcggggggaggtttcaccatgttgacaaggctggtctggaactcctgacctcaggtgatccacccgcctcggcctcccaaagtgctgggattacaggcgtgagccaccgcgcccagcctgtttttttgtttgtgtgttttgttttttttgagacagagtcttgctctgtttcccaggctggagtgaagtggtgccatctcagctcagagacagagtcttgctctgtttcccaggctggagtgaagtggtgccatcttggctcactgcaaccttcacctcccaggttcaagtgattctcctgcctcagcctcccaagtagctgggactacaggcatgtgtcaccacacccggctaatttttttgtatttttagtagagacgggatttcaccgtgttgcccaggctggtctcgaactcctgagctcaggcagtctgcctgcctcagcctcccaaagtgctgggattacacgtgtgaaccaacccgcccggcctgttgttttcttacataattcattatcatacctacaaagttaacagttactaatatcatcttacacctaaatttctctgatagactaaggttattttttaacatcttaatccaatcaaatgtttgtatcctgtaatgctctcattgaaacagctatatttctttttcagattagtgatgatgaaccaggttatgaccttgatttattttgcatacctaatcattatgctgaggatttggaaagggtgtttattcctcatggactaattatggacaggtaagtaagatcttaaaatgaggttttttactttttcttgtgttaatttcaaacatcagcagctgttctgagtacttgctatttgaacataaactaggccaacttattaaataactgatgctttctaaaatcttctttattaaaaataaaagaggagggccttactaattacttagtatcagttgtggtatagtgggactctgtagggaccagaacaaagtaaacattgaagggagatggaagaaggaactctagccagagtcttgcatttctcagtcctaaacagggtaatggactggggctgaatcacatgaaggcaaggtcagatttttattattatgcacatctagcttgaaaattttctgttaagtcaattacagtgaaaaaccttacctggtattgaatgcttgcattgtatgtctggctattctgtgtttttattttaaaattataatatcaaaatatttgtgttataaaatattctaactatggaggccataaacaagaagactaaagttctctcctttcagccttctgtacacatttcttctcaagcactggcctatgcatgtatactatatgcaaaagtacatatatacatttatattttaacgtatgagtatagttttaaatgttattggacacttttaatattagtgtgtctagagctatctaatatattttaaaggttgcatagcattctgtcttatggagataccataactgatttaaccagtccactattgatagacactattttgttcttaccgactgtactagaagaaacattcttttacatgtttggtacttgttcagctttattcaagtggaatttctgggtcaaggggaaagagtttattgaatattttggtattgccaaattttcctctaagaagttgaatcattttatactcctgatgttatatgagagtacctttctcttcacaatttgtctcttttttttttttttttgagacaaggtctctgttgcccaggctggggtgcagtgcagcagaatgatcacagttcactgcagtctcaacctcctgggttcaagcgatccttccacctcagcctcctgagtagctgggactataggtgtgcgccaccactcccagctaatatttttattttgtagaaacagggttcgccatgttacccagcctcccaaagtgctgggattacaggcatgagccactggcccagtttctacagtctctcttaatattgtatattatccagaaaatttcatttaatcagaacctgccagtctgataggtgaaaatggtatcttgtttttatttgcatttaaaaaaaattatgatagtggtatgcttggtttttttgaaggtatcaaattttttaccttatgaaacatgagggcaaaggatgtgatacgtggaagatttaaaaaaaatttttaatgcatttttttgagacaaggtcttgctctattgtccaggctggagtgcagtggcacaatcacagttcactccagcctcaacatcctgcactaaagtgattttcccacctcacctctcaagtagctgggactacaggtacatgctaccatgcctggctaatttttttttttttgcaggcatggggtctcactatattgcccaggttggtgtggaagtttaatgactaagaggtgtttgttataaagtttaatgtatgaaactttctattaaattcctgattttatttctgtaggactgaacgtcttgctcgagatgtgatgaaggagatgggaggccatcacattgtagccctctgtgtgctcaaggggggctataaattctttgctgacctgctggattacatcaaagcactgaatagaaatagtgatagatccattcctatgactgtagattttatcagactgaagagctattgtgtgagtatatttaatatatgattctttttagtggcaacagtaggttttcttatattttctttgaatctctgcaaaccatacttgctttcatttcacttggttacagtgagatttttctaacatattcactagtactttacatcaaagccaatactgtttttttaaaactagtcaccttggaggatatatacttattttacaggtgtgtgtggttttttaaataaactccttttaggaattgctgttgggacttgggatacttttttcactatacatactggtgacagataccctctcttgagctacatcggtttgtggggagtcaaaagtcctttggagctaggtttgacaaataaggtgggttaacacttgtttcctagaaagcacatggagagctagagtattggcgaattgaagaaatccccctttttttttaacacacttaagaaaggggactgcaggtatactcaagagagtaagtcgcaccagaaaccacttttgatccacagtctgcctgtgtcacacaattgaaatgcatcacaacattgacactgtggatgaaacaaaatcagtgtgaattttagtagtgaatttcattcataatttgatcgtgcaaacgtttgatttttattactttagactattgtttctgattttatgttgggttggtatttcctgtgagttactgttttacctttaaaataggaatttttcatactcttcaaagattagaacaaatgtccagtttttgctgtttcatgaatgagtcctgtccatctttgtagaaactcgccttatgttcacatttttattgagaataagaccacttatctacatttaactatcaacctcatcctctccattaatcatctattttagtgacccaagtttttgaccttttccatgtttacatcaatcctgtaggtgattgggcagccatttaagtattattatagacattttcactatcccattaaaaccctttatgcccatacatcataacactacttcctacccataagctccttttaacttgttaaagtcttgcttgaattaaagacttgtttacggtatcgataagcttgatatcaaaacgccaactttgacccggaacgcggaaaacacctgagaaaaacacctgggcgagtctccacgtaaacggtcaaagtccccgcggccctagacaaatattacgcgctatgagtaacacaaaattattcagatttcacttcctcttattcagttttcccgcgaaaatggccaaatcttactcggttacgcccaaatttactacaacatccgcctaaaaccgcgcgaaaattgtcacttcctgtgtacaccggcgcacaccaaaaacgtcacttttgccacatccgtcgcttacatgtgttccgccacacttgcaacatcacacttccgccacactactacgtcacccgccccgttcccacgccccgcgccacgtcacaaactccaccccctcattatcatattggcttcaatccaaaataaggtatattattgatgatgttt

SEQ ID NO: 125 - DNA, 30122 bp, Artificial Sequence
  HDAdTrio
aaacatcatcaataatataccttattttggattgaagccaatatgataatgagggggtggagtttgtgacgtggcgcggggcgtgggaacggggcgggtgacgtaggttttagggcggagtgatgccccccctcgaggttcgacggtatcgataagcttgatttaattaaggccggcccctaggggcgcgccgtcgacgcgacaactgtcttattaccctgttatccctaccttaattaacatttccataccacatttgtagaggttttacttgctttaaaaaacctcccacacctccccctgaacctgaaacataaaatgaatgcaattgttgttgttaacttgtttattgcagcttataatggttacaaataaagcaatagcatcacaaatttcacaaataaagcatttttttcactgcattctagttgtggtttgtccaaactcatcaatgtatcttatcatgtctggccagctagctagtcaagcgtaatcaggcacatcgtatggatagccggcataatctggcacgtcataagggtagccggcgtagtcgggcacatcataggggtagctgccccctccgcccttgccggggctcaggctcagggacttctgggtgtagtggttgtgcagggcctcgtgcatcacgctgcagctgaacacgttgccctgctgccaccggctcttgtccacggtcagcttggagtacaggaagaatgagccgtcgctgtccagcacagggggggtggtcttgtagttgttctcgggctggccgttgctctcccattccacggcgatatcgctggggtagaagcctttcaccaggcaggtcagggacacctggttcttggtcagctcgtcccggctggggggcagtgtgtacacctggggctcgcggggctggcccttggccttgctgatggttttctcgatgggggcaggcagagccttgttggacaccttgcacttgtactctttgccgttcagccagtcctggtgcagcacggtcagcacggacaccacccggtaggtgctgttgtactgttcctctctgggcttggtcttggcgttgtgcacttccacgccgtccacgtaccaattaaacttcacttcagggtcctcgtgggacacgtccaccaccacgcaggtcacttcgggggtccggctgatcatcagggtgtccttgggctttggggggaacaggaacacgctaggtccgcccagcagctcaggggcagggcaggggggacaggtgtgggtcttgtcgcagctcttggcctctctcttgatttccaccttggtgccctgtccgaaggtggcggggtggtacaggtactgctggcagtagtaggtggcgaagtcttcgggctgcagggagctgatggtcagggtgaagtcggtgccggagccgctgccgctgaatctgctgggcacgccgctgtacaggaagctggcgctgtagatcagcagcttgggggccttgccgggcttctgctgataccaagccacggcggtggacacgtcctggctggcccgacaggtgatggtcactctgtcgcccacgctggcgctcaggctgctggggctctgggtcatctggatgtcgctgcctccgccgcctgatcctccccctccggatccgcctccgccagcagacacagtcaccagtgtgccctggccccagtaatcgaagccgccaggccagtgccttctggcgcagtagtacacagcggtgtcctcggcccgcaggctgttcatctgcaggtaggcggtgttcttgctggtgtcggcgctgatggtgaaccggcccttcacgctgtcggcgtagtaggtgctgccgccgtaggggctgatccaggccacccattccagtcccttgccaggggcctggcgcacccagtggatccagctgtcgctgaaggtgaagccgctggcggcgcaagacagtctcaggctgccgccaggctgcaccagtccgccgccagattccaccagctgcacctcagagtgggcgcctgtggcggctccgaccaggaacaggatccgccagatccagtccatggtgccggcgctgaggacagtgctcagcggtccttcggcagtctccgggcccagcaacaggcttgtagtcccggagcgcgacggcgttccgaccgatctgagggcgacaggagcccccgatcaggcggagccacgagacgggctccgagttggcctggaaagggcaggccgcggcgcttacctctcggccccgcagaggcagacgctcccgtcgctgtggtctcggcccgtgtggagcgcgccgccgccgactcggcttatataccctccccccagccccgtcgtggaggcctccgattggcgaaggcgctcctcgttggaggacgctgattggtccatgccaccaagctggccgctgccgattcgaagcggcctcctccgcaacttacgtcactgctacgccccccgggctgactcattggctcttggtcactctcaacggccgccaatgaggggcagcatccgccctgtgcgccggtcctattggttcagcagctgcctgtccctcgggtgacctctcaacccgagaccgtttccgccggtaactagtcaaaacaaactcccattgacgtcaatggggtggagacttggaaatccccgtgagtcaaaccgctatccacgcccattgatgtactgccaaaaccgcatcatcatggtaatagcgatgactaatacgtagatgtactgccaagtaggaaagtcccataaggtcatgtactgggcataatgccaggcgggccatttaccgtcattgacgtcaatagggggcgtacttggcatatgatacacttgatgtactgccaagtgggcagtttaccgtaaatactccacccattgacgtcaatggaaagtccctattggcgttactatgggaacatacgtcattattgacgtcaatgggcgggggtcgttgggcggtcagccaggcgggccatttaccgtaagttatgtaacgcctgcaggcagctttctatgcaacccaaggactcagtttttggcctgttttagtgacaggcaatcagcaacatgctgcatttctctccagtgttgtaatcaaagaaaccctcccatagctttaaatgatattccttccccttccaattatgtggggggaaaacaaccctattctccacccagaagtgttaactcaagaattacattttcaagaagtttccagattcgtaaaaccagaattagatgtctttcacctaaatgtctcggtgttgaccaaaggaacacacaggtttctcatttaacttttttaatgggtctcaaaattctgtgacaaatttttggtcaagttgtttccattaaaaagtactgattttaaaaactaataacttaaaactgccacacgcaaaaaagaaaaccaaagtggtccacaaaacattctcctttccttctgaaggttttacgatgcattgttatcattaaccagtcttttactactaaacttaaatggccaattgaaacaaacagttctgagaccgttcttccaccactgattaagagtggggtggcaggtattagggataatcctaggttaggaagcattcagatagctcatcactctatcaatagtcactgcccgaattctgaaagcatgaagaagtatgcagagcttgattttagttttataaaaatccggttcttcaagggaggatttttgtggcacagtctcactgttgaaattcagggcctgcatcagctcatcaataactgccagcatgttttgatctagaaagatctgcctcttaggatccatcagcagctttgcattcatggtcttgaactccacctggtacatcttcaagtcttcataaatactactaaggcacagggccatcataaaagaggtctttctggaggccaggcaactcccattagttatgaaagaggtctctctggaatttaggcaactctcattcttggttaattccaatggtaaacaggcctccactgtgctggttttatcttttgtgatatcttcatgatcaatctcttcagaagtgcaagggtaaaattctagagtttgtctggccttctggagcatgttgctgacggccctcagcaggttttgggagtggtgaaggcatgggaacattcctgggtctggagtggccacggggaggtttctggcgcccaccccaggtacccctactccaggaacactgcagggcacagatgcccattcgctccaagatgagctatagtagcggtcctgggcccgcacgctaatgctggcatttttgcggcagatgaccgtggctgaggtcttgtccgtgaagactctatctttcttttctctcttgctcttgccctggacctgaacgcagaatgtcagggagaagtaggaatgtggagtactccaggtgtcagggtactcccagctgacctccacctgccgagaattctttaatggcttcagctgcaagttcttgggtgggtcaggtttgatgatgtccctgatgaagaagctgctggtgtagttttcatacttgagcttgtgaacggcatccaccatgacctcaatgggcagactctcctcagcagctgggcaggcactgtcctcctggcactccactgagtactcatactccttgttgtcccctctgactctctctgcagagagtgtagcagctccgcacgtcaccccttgggggtcagaagagcctctgctgcttttgacactgaatgtcaaatcagtactgattgtcgtcagccaccagcaggtgaaacgtccagaataattcttggcctcgcatcttagaaaggtcttatttttgggttctttctggtcctttaaaatatcagtggaccaaattccatcttcctttttgtgaagcagcaggagcgaatggcttagaacctcgcctcctttgtgacaggtgtactggccagcatctccaaactctttgacttggatggtcagggttttgccagagcctaagacctcactgctctggtccaaggtccaggtgataccatcttcttcaggggtgtcacaggtgaggaccaccatttctccaggggcatccggataccaatccaattctacgacataaacatctttcttcagttcccatatggccacgaggggagatgccagaaaaaccagggaaaaccaagagatgaccaactgctggtgacccatggtaagctttctagattcatgacgtgcgaccggtgagtctcaagtccccttcgatcgcaggagccgcctccaccccccacccctgggttcggatcctcacacctccagccgcgcggtccgcccactacaccccaagcaggtcgggccgcttttcacccccacttctcgcgggcgggggacgggaaacatgaacccaccaatcgcgccgcaccacgcacccacggcacccaatgaggattcgtgagggggggcggaagtccaccaatcggagctgtccaggtgcggtgaccgatgcccgaagcgtggctccttccgattggtcagggtttgcagcttttctccaatcaaatggctccgcgggcccctcacgcgtgggaccgcccctttgcctgggcggccttggcctctaagggaaaacgtccaatgaatgtaagcagagaacacatccatccttttagagaggtcgcggcggaactacttccggatcctagagagcgtttattccgtgaccggggaaacggtagccatgacaacgtgttcttcaccctttcccatctatgcctggggtttcgttggaagtgattccagcacgactttcgcggccagctttctcgtgtggcggcgcttctcggaaagaagaaacacacgagagaggttgcaaatcccctagaaccctttcagatggcgggggggcgggggggtggcggtggtgatgaaactagtgggactatggttgctgactaattgagatgcatgctttgcatacttctgcctgctggggagcctggggactttccacacctggttgctgactaattgagatgcatgctttgcatacttctgcctgctggggagcctggggactttccacaccctaactgacacacattccacagctggttctttcagcctcagaaggtacctaaccaagttcctctttcagaggttatttcaggccctgcaggttaattaagctagccgacgcgttggccaggagctcagatctccggatccaagcttatcgatttcgaacccaaatggatctaccacatttgtagaggttttacttgctttaaaaaacctcccacacctccccctgaacctgaaacataaaatgaatgcaattgttgttgttaacttgtttattgcagcttataatggttacaaataaagcaatagcatcacaaatttcacaaataaagcaatagcatcacaaatttcacaaataaagcatttttttcactgcattctagttgtggtttgtccaaactcatcaatgtatcttatcatgtcgagctagctagtcaggacttcagttccagctttgtgccggctccgaaggtcagcgggttgctagaccattgctgacagtaatatgtggcggcatcctcggcttccatagagctgattgtcaggctgtagctggtgccagatccagatccgctgaatctgtagggcacgccggaggccactttgcttgtgtcgtagatccaccgcttggggcttgtgccagacttctgctgataccagttcatgtaggacacgctgctgctggctctgcatgtcatggtcactttctcgcctggggaagcgctcatgatggcggggctttgtgtcagctgaatatcggagccaccaccaccgcttccaccaccacctgaaccgcctccgccactagaaactgtcagggttgtgccctggccccagtaatccagacagtagtggtcgtcgtagtaccgggcacaatagtacacagcgctatcttcagaggtcaggctggacagctgcatgtaggcggtagagctgctcttgtcggtggtcagtgtggccttgtccttgaacttctggttgtaattggtgtagccccggctggggttgatgtagccgatccattccagtccttggccaggcctctgcttgacccagtgcatggtgtaccgggtgaatgtgtagccgctggtcttgcaggacatcttcacagaggcgccaggtctagccagttcggcgccagactgttgcagcttgatatcggatccgccacctccgccagatgacactgtgaccagtgttcctctgccccagtagtcgaggccctgtctggcgcaataatacacggcggtgtcctcggctctcagggagttcatctgcaggtacaggctgttcttggcgttgtcccggctgatggtgaatctgcccttgatgctgtccaggtagtaggtgtagctgccgccgctgctgattgtggacacccattcaaggcctttgccaggagcctgtcggacccagctcatatcgtagctgctgaaggtgaagccggaagcggcacagctcagtctcagagagccgccaggtttcacaagtccgccgcctgattccaccagctgcacttcagatccaccaccgccactacctccgcctccgcttcctccgccgccagatcctccgccacctctcttgatttccaccttggtgcctccgccaaatgtcaggggattgctggaccactgcaggcagtagtacacggcgaagtcctcaggttccaggctgcttatggtcagggtgaaatcggtgccgctgccagagccagaaaatctggcaggcactccgctggccagattgctggtcaggtagatcaggattctaggggcctgtccgggcttctgctgcagccagtagatgtagttgatggagctgctggcgctacagctcagggtagctctctcgccagggctcagagacagtgtggctggagactgtgtcagcacgatctcgccggtggtatcaggcagccaaagcagcagcaggaacagcagctgagcaggggcttccatggtggccctccttcgccggtgatctcagctgtaggaaagagaagaaggttagtagtcgacgtgtccctctcgatgaatctaagtatcaattgtgagcgctcacaagtcaacactctttttgataaatctagtagatatcacttacgtaggcgccggtcacagcttggatctgtaacggcgcagaacagaaaacgaaacaaagacgtagagttgagcaagcagggtcaggcaaagcgtggagagccggctgagtctaggtaggctccaagggagcgccggacaaaggcccggtctcgacctgagctttaaacttacctagacggcggacgcagttcaggaggcaccacaggcgggaggcggcagaacgcgactcaaccggcgtggatggcggcctcaggtagggcggcgggcgcgtgaaggagagatgcgagcccctcgaagcttcagctgtgttctggcggcaaacccgttgcgaaaaagaacgttcacggcgactactgcacttatatacggttctcccccaccctcgggaaaaaggcggagccagtacacgacatcactttcccagtttaccccgcgccaccttctctaggcaccggttcaattgccgacccctccccccaacttctcggggactgtgggcgatgtgcgctctgcccactgacgggcaccggagcgatcgcagatccttcgatagagaaatgttctggcacctgcacttgcactggggacagcctattttgctagtttgttttgtttcgttttgttttgatggagagcgtatgttagttacgattcacacaaaaaaccaacacacagatgtaatgaaaataaagatattttattgcggccgctcgagtctagaggtatacatgccatggtccgcggtattaccctgttatccctaagacaactgtcctgcatgcgacgtcggcgcgccatcgaattcctgcagcccgggggatccctttgttgattttttccacatagattatttttgactgttttggcactttatataaatggaatcatatagtaaatatatacatgtatatatgtatatatacactatatatgtatatatatagtgtatatatatacatgtatatatgtatatttacatatatactgtatatatgtatatttacatatatactgtatatatgtatatatacacgtatatactgtatatatacagtatatactgtatatatatactgtatatatgtgtatatatatatacagtatatatacagtatacatatatatacatgtatatatacacagtatatatacatgtatatatacacagtatatatacatgtatatatacacagtatatatacatgtatatatacacagtatatatacactgtatatatgtatatatatactgtgtatatatatacagtatatatacagtatatatatacatgtatatgtatatatatactgtatatatgtgtatatatacgtatatatactgtatatatatatagacacttttgtgtctggcttcttgctctcatcataaagcacttgaaatccatccatgttgtagctggtatcagtagctagtttcttttcattgctgagaagtatcactttttattgatgagtagttttacattgtatgaacatgcccgagtttgtttatgcattctactaatagacacctgggctgtttgcagtttttggctattacaaagaaaatttctatatttttttccaacttttattttaggttcagcgggtacatgggcaggtttgttacatcggtaaattgcatgtcactggggtttggtgtacagattatttcaccacccaggtaataagcatagtacctgataggcaggtttttgatcctcaccctcctccctcaagtaggccccagtgtctattgttctattccttttttttttttttgagatggagtctcactctgttgcccaggctggagtgcagtggtgcgatctcggctcactgcaaggtccacctccagggttcaagcgattctactgccgcagcctcccgagtagctgggattacaggcacccaccaccacgcccggctaatttttgtatttttagtagagactgggtttcaccatgttggccaggatggtctcgaactcctcacctcaggtgatccgcccgcttcggcctcgcaaagtactgggattacaggcgtgagccacggtgcctggcctatggttccattctttgtgtacacgtgtactcagtgtttagcttccacttgtaagtgaaaacatgcagtatttggttttctgaaattcttgtcttcatctttttgtagacaatccactacttttatttttaaatattaggaacaatagcctctgtgtgtcctgaattgcaatgttttttctctgattttgctgctcatcttgtaacctgtatggtgtttttctgtgtgcaagctttttactttacgtgggcaattttatcattcttttcttttatggtttctgggtttcatgtcatgattggagaagcttgatctaccctgatactataaaaatatccaccttggcttttttttttttttttagatggattttcactcttgttgcccaggctggagtgcaatggcgtgatctcggctcaccacaacctctgcctcccaggttcaagtgattctcctgcctcggcctcctgagtagctgggattacaggcatgcgccaccacgctcagctaattttgtatttttagtagagacaggatttcaccatgttggtcaggctggtcttgaactccccacctcaggtgatctgtctgcctcggcctcccaaagtgctgggattacaggcgtgacccaccacacctggcccacgttgttttctgatagtgttttcacgtgttattttttctgtcttactctttgaatcatctaaatgtatcttaatgtcaggagtgaggtagaggacccagttgtttggtttaaatgactagccagttttcccaacaccaggtgttgaacatccctcactgatgtgagatgctgcctttttcacagtctcaatccccatgtgcatttctatttattttccttccactttattcacatctttttcagtatccacaaccatattgttttaaatagcttcatgatatgttttaatatttggtagagctagaaccctttcttggttctttttcttttcttcttctcctccttttcctcctccttctttctcctcctccttcttctttctttttagaaatttcctggctattcttgttttgtagtcttccagataaataattttgaatcactttgtcatgttccagaaaataatactgccagaatttttattgtgatcacagaagttttacagattcatctgggggaaaaaaacccatcttcccagaatacagaaagggtgagggaaagacaaacatcaaggacaagtctcaggttctggacttggagaccaagaggatttggggcatccgggagcagggcagggaggtgtgatggctgcctttcactgagtaggaggatgcccagacttgggggaactatggaaagtttggttcagactttctgagttggagatgtctatgcgcagtccacagggcgaagccctggaggtagaggccctccttactgcctccctcattcagtctgaggtccattctccacatggacactgaagtgactcaaggcttcccttgttggatcaggatagtctccagggccctgggtggtctgggcctgcccacctccccatcccctctcctgcctgccctcctcttgctcactggaccccacccaccagcctccttctattcctcctgacatttgcacttgctgttccgtctctgcttggaacatcctagctctttgcatggcttgctccttcccatcttttaatctaagctcaaatatcactccttcagatatgcctttcccaaatatcctagctaaagagaactgctccccacttcccacaagccctagcaaactgggactctccttcttgctttctttctctctgccccttctgtgttttttccatagaccttaacttgttactgttttatttgttgatgtgtttacatcatttgtccccctgtgatggttagttttatgtgtcaacttggctaggctgtaggggctgttcgtcaatcaaacactgatctatgtgtagctgtgaagggattttgtagctgtgattaatagttgactttaagtaaggaagattatcctggagaatgtgggggaaggggcagacctcagccaatcagttgaaaggccttaagaacaaagctgagatttccccgaggaagaagaaattctgcctgtggactgcagcatcagctcctgcttgagaggttccaggctgcccttcctgacagcctgtcctatgattttggacttgccttgccaggtttttcctctttcttgaccccccaaaaccatatatatctcctgctggtttgtttctctggtgtaatcctgagggatgaacactcctccctcccagttcactctgggagaggttggggatcatgtttgtctatttccccatgcctggcccatgcgtgtttattgaatcactgaacaaccacgcattaggaagccagtcatatgtgcttcttcagaacctcatgtccattgccagatctccctggcttttgtggctagaggacaagtgagagatagtagcttacccacagaccttggccctgaggcccccaggggcctgagcctgctgtaagggaggagggagcccctgaggtctcacacacctccctggggatctggcattttcccctggggctggcctcagagctgggcgggggcagattatggagtgggttgtagagggagcacctccccactagcaatcatggttttttctgcgcctctcatagggaggcctacaggcctccaccttcagctcttcaggagccacaggcagctgagtgacttctgcatcacagtcttctcagagacaaacttgcagtaagaaagaggggcccgtgagggaccccagagaaggctgttgtcaaagcaggatgagagtgaactcttccatgggggacacccagcgtctccaagctcttttatgctgtcttcaaggggtctagagagcttcagcccaacatgagacccagtccagcagcatttccctgcgaagtgaaagttaggaccctgactagatacaccacgctgacctcagccagaatatcaagatgctgaggcgctgagatgctgggatgctaaggtgctaaggtgctggggtgctggggtgctaggatgctgaggttttgtgatactgggtcgctgagatgctgggatactggggtgctgaagtgctggggtactggggtgttgccatgctgaaatgctggggtgttgggatgctgaggtgctgggttgctgggatgctgggatagtccttggatgctgcggtgctgagatgctggtctgctggtctgctggggtgttgggatgctgggattttgggatgctggagtgctgcagtgctgcagtgctgagatgctggagtgctggggtgctggaatactgtagtactggtgtgctggagcattgagatgctagggcactgggatgctaaggtgctgagatgctgcagtgctggggtgttgggatgccgaggtgttgggatgcttaagtgctggggtgttgggatgctggggtgctggaacactatggtgctggggtgctggagtgttgagatactgtagtggtgggatgcttaagtgctggggtgctgggtgttgggatgcctaggtgctggggtgccgagatgctggagtactagtgtgctgggatgctgaagtgctggggtcctgagatgctgcagtgctagggtgctgagattctgggctgctggagtgttggggtgctgggatgctggagtgctgagatgcttggacaatggggtgctggaatactatggtgctggggtgctggggtattgagatgctagggtactgggatgctgaagtgctgagatcctggagtgctgggctgctgggccacaggctcttgaatccattcgtctgcccaggggaagaaaccagaagataaagagctaatgaaggagctttggttgagagggaggaagtaatggaaggagcaacatcttgtggaggagcaggagagaatggacctcaggttgggagagagggccaggctacaggccagagaggcagaaggattccagcagagtgtgggctccaggagccaaggggaaacaggtttctgggaggagagagtccagtactgctgaagtggcaagtccgctgaggaccaggaagcttcatttggctttatgaccaggaggaatttggaactgtgactagagtacttagggggaaggaggcaagactggagccagattgctctgggttgaggggtgagtgggaggtgaagcagggcactgtcactcctttgaagggtggcagagagctggaattggtgctggatgggctgtggggtgacagggtcatgtggaaagcccctggggggcacctggaaaaggagaagctgacagtacagtgagaggacagctaagggaaagcggaatggcagaacacgcactgccaggaggaatgaggatagggtcaggagtgccaggggcagtgaggccagcctggggtcaggtggcaggacgtgtccaggaagctggtctgcactgcagcccacactggctcagccttgaggttccctgtgtggttggggtaggaagttgaaccctctgggaatggaagatggaaccagctctgcgagccaagctcagcttttatctatgggtctctgagggctggcagagctgagtggggacaactgtgatccgtgaggctctcaggttgaggtggcccctccgggagggcttcattttcccagcgggtaggttctaagcagcagtggctgggcaggtgggtccaacacagagccagagaagggtgaatgggcctcctggcaccccacccctgctgcccctgagctcagtgatggagggggacagcacagctgagcccaagtgctttggtgtggccctgagggaaagctgcagcctgcctggggcctggcatggatgggacacttgaggcagagggacaatagtgggcgctgcagtgaggctggctcttggagaggtttcctgaggagtgctgcctgagacgggcagggagaacagagacaaagttggtgacagggaatgaaagctgactgaaggactttacccagacctatgaggatatctctctcagcaggaagcaggaggggactgtgtgaggactggccaagagctggagtgttgggaaaatgactctttctccgacccctctgtcctagctctggcccctggactgcggaggtctgcttccacccccattggtcgatcgttgtcccttgtcacagccattgagaattttggcagggagcatgttcttagagcatttttaggctctgcgggacataacagctctgcctcagagcacatgcctttctcagctcctgaaagccactgatcaaattggaacattttgtaccttagggatgaggatatcaactctcccagccacttagagggataaatgtgatgatgcattcaattgtgactacatctgatcccaactgttgcttcagctgctctcctatagcacatggcgggaggcgtgcatcccagtagctacctccccacttttggggagatgtggttccatccatgaaacctgggtacccgcctaccaggtcctggcctatcaggtggcagggtctggtcaaagaagggcatgtgtggtcttcagcaagggagacaggacggtggtgcagagcgtctagaccctcagggcaagtctcccccacacctgctcccggggcagttgtctttgtgacctcccatccccctctgtttcatcctctataaaatgaggggctgagccccaaaataacaggcttctttgccatgatgcaaaactgctgaatctttctttctgacacacaaggcatcgagcagcctctgaaagaaccaaagccactagcaggcttcctgacttgggtttgtaggtactgaatactcccttgaaaaataaaaacatagaggcacttttctcctggctgtttattacagaacgaagaaaaaacacactggcttgaaacagacgccagatttcaaatgtagaggtgaaatacgaggtggcaattaaaatgtgattacagaaagtctggacactgagaaaagtttacaggacagtgggtgtgggttttctataacagacacttaaatatacatgacgataattgcagatagaaaccatcaaagacaaaccccaaatcaactaataatgtttacagatgttcccccccaaaccacagagccttacatcaaaacaaatactgaaaggctttaaaccaggaacagctcgccttaaccccacgagggtgcacacaagctgggctttttctctcggtctgaatggtaaagggaggaggatactctagctcctccaggtggattgctgagacagggctcggctcacacactgtctctgcgcctctcccaaatctggagaactctcccagcctcctggtaaagtgtctctgtggggcacttaacgataaaacagcttctgctgtaaagctcattaggaaagagctagcctgcaacctccacggagtgggaactacatcaggcattttgctaactgctgtatcctaggccaataaatgttgatcacatttatagctgccatggtagggtggggacccctgctatctatctgtggaggctctgggagcccctgacacaaactttctgaagcagagcctccccaaccccttttccattccctatacctgacagatggcccaggaacccattagaaatggaaggtcactgcagcagtatgtgaatgtgcgtgtgggagaagggcaggatcagagccctgggggtgtggcagcccccaagtgattctaatccagatcctagggttgtttccctgtcccattgaaatagctgctttaaggggcctgactcagggaaatcagtctcttgaattaagtggtgattttggagtcatttagaccaggccttcaattgggatccactagttctagagcggccgggcccagggaaccccgcaggcgggggcggccagtttcccgggttcggctttacgtcacgcgagggcggcagggaggacggaatggcggggtttggggtgggtccctcctcgggggagccctgggaaaagaggactgcgtgtgggaagagaaggtggaaatggcgttttggttgacatgtgccgcctgcgagcgtgctgcggggaggggccgagggcagattcgggaatgatggcgcggggtgggggcgtgggggctttctcgggagaggcccttccctggaagtttggggtgcgatggtgaggttctcggggcacctctggaggggcctcggcacggaaagcgaccacctgggagggcgtgtggggaccaggttttgcctttagttttgcacacactgtagttcatctttatggagatgctcatggcctcattgaagccccactacagctctggtagcggtaaccatgcgtatttgacacacgaaggaactagggaaaaggcattaggtcatttcaagccgaaattcacatgtgctagaatccagattccatgctgaccgatgccccaggatatagaaaatgagaatctggtccttaccttcaagaacattcttaaccgtaatcagcctctggtatcttagctccaccctcactggttttttcttgtttgttgaaccggccaagctgctggcctccctcctcaaccgttctgatcatgcttgctaaaatagtcaaaaccccggccagttaaatatgctttagcctgctttattatgattatttttgttgttttggcaatgacctggttacctgttgtttctcccactaaaactttttaagggcaggaatcaccgccgtaactctagcacttagcacagtacttggcttgtaagaggtcctcgatgatggtttgttgaatgaatacattaaataattaaccacttgaaccctaagaaagaagcgattctatttcatattaggcattgtaatgacttaaggtaaagagcagtgctattaacggagtctaactgggaatccagcttgtttgggctatttactagttgtgtggctgtgggcaacttacttcacctctctgggcttaagtcattttatgtatatctgaggtgctggctacctcttggagttattgagaggattataagacagtctatgtgaatcagcaacccttgcatggcccctggcggggaacagtaataatagccatcatcatgtttacttacatagtcctaattagtcttcaaaacagccctgtagcaatggtatgattattaccattttacagatgaggaacctttgaagcctcagagaggctaacagacataccctaggtcatacagttattaagagaaggagctctgtctcgaacctagctctctctctctcgagtaataccagttaaaaaataggctacaaataggtactcaaaaaaatggtagtggctgttgtttttattcagttgctgaggaaaaaatgttgatttttcatctctaaacatcaacttacttaattctgccaatttcttttttttgagacagggtctcactctgtcacctaggatggagtgcagtggcacaatcactgctcactgcagcctcgacttcccgggctcgggtgattctccccaggctcaggggattctcccacttcagcctcccaagtagctgggactacaggtgcgcaccaccatccctggctaatatttgtactttattttatttatttatttatttattttttgagatggagtttcgctcttgttgcccgggctggagtacagtggcatgatctcggctcagtgcaacctctgcctcccgggttcaagcgattctcctacctcatccccctgagtagctgggattacaggcgcctgccaccatgcctggctaattttttgtatttttaatagagacgaggtttcaccatgttggccaggctactctcgaactcctgatctcaggtgatccacccgccttggcctcccaaagtgctgggattacaggcgtgagccactgcgcccggcctaatatttgtattttttgtagagatggtgttttgccatgttgtccaggctggtcttgaactcctgagctcaagcgatctgcccgcctctgcttcccaaagtgctgggattacaggcatgagccaccgtgcctggcctaggtagacgcttttagctttggggtgtgatgcctgccccagtatatagtgaatttaattattgctagagctggctgtttgttagttttctttgaacataagatactcattgtttttagtttgcaaatccctcttcctttttaaaaaatttctttcccttaaattgtttgcatgttagcaataacaaatgcttaaatggtgctatgtgctagatactcttctaagccctgttatgtatattaactaattttttaaattacacaaatcagagaggttaagtaacttgcccaagattacccaacaatactaggatttgaacctaagtttgtctcaccccagattctgctcttaatctctaaacttttaagttagtagtgacaatagtaggtatttattgaatacttaactatgttttaggcgttgaagtaaatattttgcaggcattatctaatgtaaacaccctaaagttacataacaggtaccctttaggtaaataaacactagtatgaccttggaggcacagatagttgaagtaacttgcccaatatcacttacatgaaattggccctcaaatgtgtctgatacaacccatgctgcttgtaactatcgttttaaactgccagggtaaacttggacacacttgagctaagaaaaagcttttagatttttgcaaattaatgtgaaagatatgctttatgtggatataatatcttctaaatttcggggatggtagtcctagaaatgtaatcctgccctagccgagcttaccctgccaataattttttacagaattggtaaaacggagcaccttttttttgtccttggccacactgttatcaacagggtgtagattgacatcaatctgtaggtgtaaaccagaattactctttgtgaccaccaggaaatagagcagttcagttcaggggtttctttctgtgaatttagcactgtgacctgcatactacaagtctactttgttttctatccattgtttgtatctgggtattgcaaaaggtaggaaaaggaccaaccagatcagcagagaagagttgccttggagttttcttttagttttctgcagttcattagatagtaactaggccatgtcattttactcccttgtagtgaagatatgttgaagttgtactggtatactcttctacctttctgtaattttatattgtgtagacttgataaaatttatgtgtcaatcaccaccattaatatcaatattgagcctcaattcttatttttctgcccagtggctgccaaattactaacatttacaataattcactactactaagataatctactagttcgatcacatacttcaaattgttatggaactactgtcttcagcattgtgcttctgataactgataagtataattttttttttgtccagagtgaacatgtctattcttccactgtacacactaataaaaggaaaaattgtaatattgggtaaattcatgtccttacacatgtagtagttatgagcccatgtccctagaatgagtaataatttatccctcccttggttgaatagtcaagaatgctgattttaattcttctaacagctttatccctcagaagggaaggcaagcaagttatatatgtagtttatttgtaagactgatatgaaattggaagatgaatctactattagctttaattatttttacatttaggaatattgcatcagtaactcataattttggttttctgttatcctgagttaacacaaattatccaaggagatggcggatcatctgctttgaggtgtttttttttgagaattttaatgtatctgaatataaaaggtaaaaatatgccaactagcaatttctgcccattccagaagtttggaaatattactcattactaggaattaaataaaatatggtttatctattgttatacctcttttaattcacatagctcatttttatcttttatttttgtttgttttttttgagatggagtcttgctctgtcaccaggcaggagtgcagtgatgcaaatctcggctcactctagccaccgactccctggttcaagcgattctcctgcctgagccttctgagtagctgggattacaggcaggcaccaccacgcccagctaatttttgtagagacaggatttcaccgtgttggccaggatggtctccatctcctgacctcatgatctgcctgcttcggcctcccaaagtgctgggattacaggtgggagccactacgcctggcccacatagctcatttttagactcacttccattaagtcttgtttggacccacgaacattgtctttttttttttaagatggagtttcacttttgttgcccagactgtagtgcaatggtgcaatctcagctcactgcaatctctgcctcctgggttctagcaattctcctgcctcagcctcccgagtagctggaattacaggcgcccgccaccacgcccagctaatttttgtgtttttagtagagacggggtttcaccatgttgggcaggccaggggtgatccgcccacctcagcctcccaaagtgctgggattacaggtgtgagccaccgcatctggccaacatgtcttttttttttttttcctttttaaccacaaagagacttaagcagtccttgtcacagatgatgaattgatgttgcaagtattgtcttagcttggattaattttcttgcttactgtaattttagataatatagctttgtaattagagattttatgtgtaaaccacaaaaatgtttacatgaaggccattattacagatgtgacgtgcataattattagtaatttgtatgtttacatgggtcagtctggcaaaaaattatgaagttttaaaaattaaaaaaaattataatgccagttttactggaaagtaaaattatttcagtaatcgattatagcaaaagtattgattttcattccagacaactgtctgtctatagccaattatgcatttcttaaattagaacccccccaatatacccaaatatatatatatgtgtgcatatatatagtaagttgtaacaaagttgtgaattcatacctgaagtatctcaagtgatgcaagttttatgaatttttgtttatgccttttgggaagagttgtattgacaaattttttatgcttaaagtaaaccataaatcaaaaaaataaaatctaggatgcaataaaacaaaacaacttcttgacataagtatggtatgtaaatctgttttgattggaaatcaatttgttatattgccagaattcctgttttagaatacatctctgctgatctgtctgtattcttagactgcatatctgggatgaactctgggcagaattcacatgggcttcctttgaaataaacaagacttttcaaattcttagtcgatctgcagaacctgtagccaggcactgaaccattttgatagatgcagtaatcgttgcaagtgtatatttcaagggagttctggctgggtcctagtttatgcttgtggcagaagcagtgagtaactgggaggaagttggtgagtaagcttcaaggaagaagtcatttttagtactctggatcttcctgattttaaagcactacaaaatggtgcattttcattcttgtcaagtgataacagatatattctgatgagcctgaaatgaatatatattgtatcatttttataatatctagcaaggtttgtattttcctagaacttgaactaaatttcagttcataaaatttataaaatacttagttgttgtaaaatatttttggaatgttcacataggtgacacacaaatgtcccattttcattctttctatagtaaatatgttctgatatgtgaaggtttagcagatgcatcagcatttaatcctagaggatctggcataatcttttcccccaagaatagaaattttttctgcttatgaaagtagtacatgtttctttaaaaacaaatcaatattgacttctgcctgctgtatagcactatgcctccacctggccatgaccaggggcatgtcctggtccacctacctgaaaatgtttgcaaccagcctcctggccatgtgcacaggggctgaagttgtcccacaggtattacgggccaacctgacaatacatgaagttccaccaaagtctgagaactcagaactgagctttggggactgaaagacagcacaaacctcaaatttctcagcactggaaacctcaaaatataactgaattccataaataagattttaagtcttaaatatgtatttttaaatgtattaaaagtcaagctgcttgtatttaagcacctaatacaatgcttaggttgtaaaaggagatgctcaataggtactaactgatatattgagatttaattatggtttgaccaatatttattggaaaccgccaaagcttaaatcatcagcttcttgaatgtgatttgaaaggtaatttagtattgaatagcatgtgagctagagtatttcattctttctggtttatttcttcaaatagactttgaatataatggtgaatgggtattataaattaactaataaaaatgacattgaaaatgaaaaaatatatatattaaagtgtagaaagtgaccaggcgtggtggctcacacctgtaatccaagcaccttgggaggctgaggcaggaggatctcttgatcccaggagttcaagaccagcctgggcaacatagcgagacttcgtctctaaaaaaaaaaaagagagagaaaaaaattttttttatttaaaaaaagtgtagaaagtgtcaagaccccacttcttaccattatttggtatatttctctatacccacccacccttcctccttactccctccctcccttcccaatctttttatctttttgtattctgattttttgtttgtatattttgctttaatttaatgtatcctttaaaaatttcccatacattttatatgtatatataaaaacgcatgctgccaaagataatttataagaaagaccattgaatttttttaaaagtgatatatattcattgaaaaaaatttagaatatatagcaaagcaataaagaactaaataaaattgctgtaactcctctttcaaagataagtgcttttatgattttgttgtatttttttctgtatataggtacatatatagtatttataaagctgtactcatagtacattttcacatcacaggtaccatatcagtgttattaaatattttgtatgccaggggctagacataccaagacaaccaatatgtggttctacttaaataatattagagtatcttttatgatgacacttcatgagttgactataataatcttagacttctaagagtttgggttttcaaaagatcacttagcttttttgggtgatttttcccccttactgtgagatgagagaggctgtttggatttgggattggggtagcggggacagcaacttttcttttctttttcttttttattttgaggtagggtattgctgtgtcacccaggctggagtgcagtggtgtgatctcggctcactgcaacctccacctcccgggctcaggtgatcctcctgcttcagcctcccagtaactgggactacaggcgcgtgccacatgcctggctaattttgtatttttagtagagatggggtttcaccatgttggccaggctggtctctaactcctgacctcaggtgatacgcccacctgggcctcccaaaatactgggattacaggcatgagccgctgcatcagccagcagtttttcttgtggttttttttgtttgttttgttttgttttgtttttgagatagggtcttactctgttgtccacgctggagtgctgtggtatgatcgtagctcactgcagcctcaaactcctgggctcaagtgattccttctgcctccgcctcccgagtagctgggactacaggtatgcaccaccatacctggcaaatttttacaaagttttttgtagggacggggtcttgctacattccccatgtcggtcttgaactcctggcctcaagcaactctcctgtctcagcctcccaaagcactgggattacaagtgtgagccaccacaccatgccagtttttcctgttcagtgtgatattttatcttgttagactacagtgtgttaaaacttgttttactaaattttcaaacatactcaaaagtggagagaatagtataatgaatacccgtatgttcatcacccatgtttagaatattattaaatataaagattttgctgcgtttgtcttagctctttaaaatttttctttttctctttgtgacctaaaggaaattccatatcttatcactttacttctacattcttgactaagatgactaagacatatagttacatggttttttgttttgtttttgttttttaaagacgaaatctcgctcttgtcccccaggctggagtgcaatggtgccatctcagctcagtgcaacctctgccttctgggtacaagcgattctcctgcctcagcctcccaagtagctgggattacaggctcctgccaccacgcctggctaatttttgtatttttagtagagacggcggggggaggtttcaccatgttgacaaggctggtctggaactcctgacctcaggtgatccacccgcctcggcctcccaaagtgctgggattacaggcgtgagccaccgcgcccagcctgtttttttgtttgtgtgttttgttttttttgagacagagtcttgctctgtttcccaggctggagtgaagtggtgccatctcagctcagagacagagtcttgctctgtttcccaggctggagtgaagtggtgccatcttggctcactgcaaccttcacctcccaggttcaagtgattctcctgcctcagcctcccaagtagctgggactacaggcatgtgtcaccacacccggctaatttttttgtatttttagtagagacgggatttcaccgtgttgcccaggctggtctcgaactcctgagctcaggcagtctgcctgcctcagcctcccaaagtgctgggattacacgtgtgaaccaacccgcccggcctgttgttttcttacataattcattatcatacctacaaagttaacagttactaatatcatcttacacctaaatttctctgatagactaaggttattttttaacatcttaatccaatcaaatgtttgtatcctgtaatgctctcattgaaacagctatatttctttttcagattagtgatgatgaaccaggttatgaccttgatttattttgcatacctaatcattatgctgaggatttggaaagggtgtttattcctcatggactaattatggacaggtaagtaagatcttaaaatgaggttttttactttttcttgtgttaatttcaaacatcagcagctgttctgagtacttgctatttgaacataaactaggccaacttattaaataactgatgctttctaaaatcttctttattaaaaataaaagaggagggccttactaattacttagtatcagttgtggtatagtgggactctgtagggaccagaacaaagtaaacattgaagggagatggaagaaggaactctagccagagtcttgcatttctcagtcctaaacagggtaatggactggggctgaatcacatgaaggcaaggtcagatttttattattatgcacatctagcttgaaaattttctgttaagtcaattacagtgaaaaaccttacctggtattgaatgcttgcattgtatgtctggctattctgtgtttttattttaaaattataatatcaaaatatttgtgttataaaatattctaactatggaggccataaacaagaagactaaagttctctcctttcagccttctgtacacatttcttctcaagcactggcctatgcatgtatactatatgcaaaagtacatatatacatttatattttaacgtatgagtatagttttaaatgttattggacacttttaatattagtgtgtctagagctatctaatatattttaaaggttgcatagcattctgtcttatggagataccataactgatttaaccagtccactattgatagacactattttgttcttaccgactgtactagaagaaacattcttttacatgtttggtacttgttcagctttattcaagtggaatttctgggtcaaggggaaagagtttattgaatattttggtattgccaaattttcctctaagaagttgaatcattttatactcctgatgttatatgagagtacctttctcttcacaatttgtctcttttttttttttttttgagacaaggtctctgttgcccaggctggggtgcagtgcagcagaatgatcacagttcactgcagtctcaacctcctgggttcaagcgatccttccacctcagcctcctgagtagctgggactataggtgtgcgccaccactcccagctaatatttttattttgtagaaacagggttcgccatgttacccagcctcccaaagtgctgggattacaggcatgagccactggcccagtttctacagtctctcttaatattgtatattatccagaaaatttcatttaatcagaacctgccagtctgataggtgaaaatggtatcttgtttttatttgcatttaaaaaaaattatgatagtggtatgcttggtttttttgaaggtatcaaattttttaccttatgaaacatgagggcaaaggatgtgatacgtggaagatttaaaaaaaatttttaatgcatttttttgagacaaggtcttgctctattgtccaggctggagtgcagtggcacaatcacagttcactccagcctcaacatcctgcactaaagtgattttcccacctcacctctcaagtagctgggactacaggtacatgctaccatgcctggctaatttttttttttttgcaggcatggggtctcactatattgcccaggttggtgtggaagtttaatgactaagaggtgtttgttataaagtttaatgtatgaaactttctattaaattcctgattttatttctgtaggactgaacgtcttgctcgagatgtgatgaaggagatgggaggccatcacattgtagccctctgtgtgctcaaggggggctataaattctttgctgacctgctggattacatcaaagcactgaatagaaatagtgatagatccattcctatgactgtagattttatcagactgaagagctattgtgtgagtatatttaatatatgattctttttagtggcaacagtaggttttcttatattttctttgaatctctgcaaaccatacttgctttcatttcacttggttacagtgagatttttctaacatattcactagtactttacatcaaagccaatactgtttttttaaaactagtcaccttggaggatatatacttattttacaggtgtgtgtggttttttaaataaactccttttaggaattgctgttgggacttgggatacttttttcactatacatactggtgacagataccctctcttgagctacatcggtttgtggggagtcaaaagtcctttggagctaggtttgacaaataaggtgggttaacacttgtttcctagaaagcacatggagagctagagtattggcgaattgaagaaatccccctttttttttaacacacttaagaaaggggactgcaggtatactcaagagagtaagtcgcaccagaaaccacttttgatccacagtctgcctgtgtcacacaattgaaatgcatcacaacattgacactgtggatgaaacaaaatcagtgtgaattttagtagtgaatttcattcataatttgatcgtgcaaacgtttgatttttattactttagactattgtttctgattttatgttgggttggtatttcctgtgagttactgttttacctttaaaataggaatttttcatactcttcaaagattagaacaaatgtccagtttttgctgtttcatgaatgagtcctgtccatctttgtagaaactcgccttatgttcacatttttattgagaataagaccacttatctacatttaactatcaacctcatcctctccattaatcatctattttagtgacccaagtttttgaccttttccatgtttacatcaatcctgtaggtgattgggcagccatttaagtattattatagacattttcactatcccattaaaaccctttatgcccatacatcataacactacttcctacccataagctccttttaacttgttaaagtcttgcttgaattaaagacttgtttacggtatcgataagcttgatatcaaaacgccaactttgacccggaacgcggaaaacacctgagaaaaacacctgggcgagtctccacgtaaacggtcaaagtccccgcggccctagacaaatattacgcgctatgagtaacacaaaattattcagatttcacttcctcttattcagttttcccgcgaaaatggccaaatcttactcggttacgcccaaatttactacaacatccgcctaaaaccgcgcgaaaattgtcacttcctgtgtacaccggcgcacaccaaaaacgtcacttttgccacatccgtcgcttacatgtgttccgccacacttgcaacatcacacttccgccacactactacgtcacccgccccgttcccacgccccgcgccacgtcacaaactccaccccctcattatcatattggcttcaatccaaaataaggtatattattgatgatgttt

SEQ ID NO: 126 - DNA, 35010 bp, Artificial Sequence
  Ad5/3Ad2E1Adelta24
taacatcatcaataatataccttattttggattgaagccaatatgataatgagggggtggagtttgtgacgtggcgcggggcgtgggaacggggcgggtgacgtagtagtgtggcggaagtgtgatgttgcaagtgtggcggaacacatgtaagcgacggatgtggcaaaagtgacgtttttggtgtgcgccggtgtacacaggaagtgacaattttcgcgcggttttaggcggatgttgtagtaaatttgggcgtaaccgagtaagatttggccattttcgcgggaaaactgaataagaggaagtgaaatctgaataattttgtgttactcatagcgcgtaatatttgtctagggccgcggggactttgaccgtttacgtggagactcgcccaggtgtttttctcaggtgttttccgcgttccgggtcaaagttggcgttttattattatagtcagctgacgtgtagtgtatttatacccggtgagttcctcaagaggccactcttgagtgccagcgagtagagttttctcctccgagccgctccgacaccgggactgaaaatgagacatattatctgccacggaggtgttattaccgaagaaatggccgccagtcttttggaccagctgatcgaagaggtactggctgataatcttccacctcctagccattttgaaccacctacccttcacgaactgtatgatttagacgtgacggcccccgaagatcccaacgaggaggcggtttcgcagatttttcccgagtctgtaatgttggcggtgcaggaagggattgacttattcacttttccgccggcgcccggttctccggagccgcctcacctttcccggcagcccgagcagccggagcagagagccttgggtccggtttctatgccaaaccttgtgccggaggtgatcgatccacccagtgacgacgaggatgaagagggtgaggagtttgtgttagattatgtggagcaccccgggcacggttgcaggtcttgtcattatcaccggaggaatacgggggacccagatattatgtgttcgctttgctatatgaggacctgtggcatgtttgtctacagtaagtgaaaattatgggcagtcggtgatagagtggtgggtttggtgtggtaatttttttttaatttttacagttttgtggtttaaagaattttgtattgtgattttttaaaaggtcctgtgtctgaacctgagcctgagcccgagccagaaccggagcctgcaagacctacccggcgtcctaaattggtgcctgctatcctgagacgcccgacatcacctgtgtctagagaatgcaatagtagtacggatagctgtgactccggtccttctaacacacctcctgagatacacccggtggtcccgctgtgccccattaaaccagttgccgtgagagttggtgggcgtcgccaggctgtggaatgtatcgaggacttgcttaacgagtctgggcaacctttggacttgagctgtaaacgccccaggccataaggtgtaaacctgtgattgcgtgtgtggttaacgcctttgtttgctgaatgagttgatgtaagtttaataaagggtgagataatgtttaacttgcatggcgtgttaaatggggcggggcttaaagggtatataatgcgccgtgggctaatcttggttacatctgacctcatggaggcttgggagtgtttggaagatttttctgctgtgcgtaacttgctggaacagagctctaacagtacctcttggttttggaggtttctgtggggctcatcccaggcaaagttagtctgcagaattaaggaggattacaagtgggaatttgaagagcttttgaaatcctgtggtgagctgtttgattctttgaatctgggtcaccaggcgcttttccaagagaaggtcatcaagactttggatttttccacaccggggcgcgctgcggctgctgttgcttttttgagttttataaaggataaatggagcgaagaaacccatctgagcggggggtacctgctggattttctggccatgcatctgtggagagcggttgtgagacacaagaatcgcctgctactgttgtcttccgtccgcccggcgataataccgacggaggagcagcagcagcagcaggaggaagccaggcggcggcggcaggagcagagcccatggaacccgagagccggcctggaccctcgggaatgaatgttgttcaggtggctgaactgtatccagaactgagacgcattttgacaattacagaggatgggcaggggctaaagggggtaaagagggagcggggggcttgtgaggctacagaggaggctaggaatctagcttttagcttaatgaccagacaccgtcctgagtgtattacttttcaacagatcaaggataattgcgctaatgagcttgatctgctggcgcagaagtattccatagagcagctgaccacttactggctgcagccaggggatgattttgaggaggctattagggtatatgcaaaggtggcacttaggccagattgcaagtacaagatcagcaaacttgtaaatatcaggaattgttgctacatttctgggaacggggccgaggtggagatagatacggaggatagggtggcctttagatgtagcatgataaatatgtggccgggggtgcttggcatggacggggtggttattatgaatgtaaggtttactggccccaattttagcggtacggttttcctggccaataccaaccttatcctacacggtgtaagcttctatgggtttaacaatacctgtgtggaagcctggaccgatgtaagggttcggggctgtgccttttactgctgctggaagggggtggtgtgtcgccccaaaagcagggcttcaattaagaaatgcctctttgaaaggtgtaccttgggtatcctgtctgagggtaactccagggtgcgccacaatgtggcctccgactgtggttgcttcatgctagtgaaaagcgtggctgtgattaagcataacatggtatgtggcaactgcgaggacagggcctctcagatgctgacctgctcggacggcaactgtcaccttctgaagaccattcacgtagccagccactctcgcaaggcctggccagtgtttgagcataacatactgacccgctgttccttgcatttgggtaacaggaggggggtgttcctaccttaccaatgcaatttgagtcacactaagatattgcttgagcccgagagcatgtccaaggtgaacctgaacggggtgtttgacatgaccatgaagatctggaaggtgctgaggtacgatgagacccgcaccaggtgcagaccctgcgagtgtggcggtaaacatattaggaaccagcctgtgatgctggatgtgaccgaggagctgaggcccgatcacttggtgctggcctgcacccgcgctgagtttggctctagcgatgaagatacagattgaggtactgaaatgtgtgggcgtggcttaagggtgggaaagaatatataaggtgggggtcttatgtagttttgtatctgttttgcagcagccgccgccgccatgagcaccaactcgtttgatggaagcattgtgagctcatatttgacaacgcgcatgcccccatgggccggggtgcgtcagaatgtgatgggctccagcattgatggtcgccccgtcctgcccgcaaactctactaccttgacctacgagaccgtgtctggaacgccgttggagactgcagcctccgccgccgcttcagccgctgcagccaccgcccgcgggattgtgactgactttgctttcctgagcccgcttgcaagcagtgcagcttcccgttcatccgcccgcgatgacaagttgacggctcttttggcacaattggattctttgacccgggaacttaatgtcgtttctcagcagctgttggatctgcgccagcaggtttctgccctgaaggcttcctcccctcccaatgcggtttaaaacataaataaaaaaccagactctgtttggatttggatcaagcaagtgtcttgctgtctttatttaggggttttgcgcgcgcggtaggcccgggaccagcggtctcggtcgttgagggtcctgtgtattttttccaggacgtggtaaaggtgactctggatgttcagatacatgggcataagcccgtctctggggtggaggtagcaccactgcagagcttcatgctgcggggtggtgttgtagatgatccagtcgtagcaggagcgctgggcgtggtgcctaaaaatgtctttcagtagcaagctgattgccaggggcaggcccttggtgtaagtgtttacaaagcggttaagctgggatgggtgcatacgtggggatatgagatgcatcttggactgtatttttaggttggctatgttcccagccatatccctccggggattcatgttgtgcagaaccaccagcacagtgtatccggtgcacttgggaaatttgtcatgtagcttagaaggaaatgcgtggaagaacttggagacgcccttgtgacctccaagattttccatgcattcgtccataatgatggcaatgggcccacgggcggcggcctgggcgaagatatttctgggatcactaacgtcatagttgtgttccaggatgagatcgtcataggccatttttacaaagcgcgggcggagggtgccagactgcggtataatggttccatccggcccaggggcgtagttaccctcacagatttgcatttcccacgctttgagttcagatggggggatcatgtctacctgcggggcgatgaagaaaacggtttccggggtaggggagatcagctgggaagaaagcaggttcctgagcagctgcgacttaccgcagccggtgggcccgtaaatcacacctattaccgggtgcaactggtagttaagagagctgcagctgccgtcatccctgagcaggggggccacttcgttaagcatgtccctgactcgcatgttttccctgaccaaatccgccagaaggcgctcgccgcccagcgatagcagttcttgcaaggaagcaaagtttttcaacggtttgagaccgtccgccgtaggcatgcttttgagcgtttgaccaagcagttccaggcggtcccacagctcggttacctgctctacggcatctcgatccagcatatctcctcgtttcgcgggttggggcggctttcgctgtacggcagtagtcggtgctcgtccagacgggccagggtcatgtctttccacgggcgcagggtcctcgtcagcgtagtctgggtcacggtgaaggggtgcgctccgggctgcgcgctggccagggtgcgcttgaggctggtcctgctggtgctgaagcgctgccggtcttcgccctgcgcgtcggccaggtagcatttgaccatggtgtcatagtccagcccctccgcggcgtggcccttggcgcgcagcttgcccttggaggaggcgccgcacgaggggcagtgcagacttttgagggcgtagagcttgggcgcgagaaataccgattccggggagtaggcatccgcgccgcaggccccgcagacggtctcgcattccacgagccaggtgagctctggccgttcggggtcaaaaaccaggtttcccccatgctttttgatgcgtttcttacctctggtttccatgagccggtgtccacgctcggtgacgaaaaggctgtccgtgtccccgtatacagacttgagaggcctgtcctcgagcggtgttccgcggtcctcctcgtatagaaactcggaccactctgagacaaaggctcgcgtccaggccagcacgaaggaggctaagtgggaggggtagcggtcgttgtccactagggggtccactcgctccagggtgtgaagacacatgtcgccctcttcggcatcaaggaaggtgattggtttgtaggtgtaggccacgtgaccgggtgttcctgaaggggggctataaaagggggtgggggcgcgttcgtcctcactctcttccgcatcgctgtctgcgagggccagctgttggggtgagtactccctctgaaaagcgggcatgacttctgcgctaagattgtcagtttccaaaaacgaggaggatttgatattcacctggcccgcggtgatgcctttgagggtggccgcatccatctggtcagaaaagacaatctttttgttgtcaagcttggtggcaaacgacccgtagagggcgttggacagcaacttggcgatggagcgcagggtttggtttttgtcgcgatcggcgcgctccttggccgcgatgtttagctgcacgtattcgcgcgcaacgcaccgccattcgggaaagacggtggtgcgctcgtcgggcaccaggtgcacgcgccaaccgcggttgtgcagggtgacaaggtcaacgctggtggctacctctccgcgtaggcgctcgttggtccagcagaggcggccgcccttgcgcgagcagaatggcggtagggggtctagctgcgtctcgtccggggggtctgcgtccacggtaaagaccccgggcagcaggcgcgcgtcgaagtagtctatcttgcatccttgcaagtctagcgcctgctgccatgcgcgggcggcaagcgcgcgctcgtatgggttgagtgggggaccccatggcatggggtgggtgagcgcggaggcgtacatgccgcaaatgtcgtaaacgtagaggggctctctgagtattccaagatatgtagggtagcatcttccaccgcggatgctggcgcgcacgtaatcgtatagttcgtgcgagggagcgaggaggtcgggaccgaggttgctacgggcgggctgctctgctcggaagactatctgcctgaagatggcatgtgagttggatgatatggttggacgctggaagacgttgaagctggcgtctgtgagacctaccgcgtcacgcacgaaggaggcgtaggagtcgcgcagcttgttgaccagctcggcggtgacctgcacgtctagggcgcagtagtccagggtttccttgatgatgtcatacttatcctgtcccttttttttccacagctcgcggttgaggacaaactcttcgcggtctttccagtactcttggatcggaaacccgtcggcctccgaacggtaagagcctagcatgtagaactggttgacggcctggtaggcgcagcatcccttttctacgggtagcgcgtatgcctgcgcggccttccggagcgaggtgtgggtgagcgcaaaggtgtccctgaccatgactttgaggtactggtatttgaagtcagtgtcgtcgcatccgccctgctcccagagcaaaaagtccgtgcgctttttggaacgcggatttggcagggcgaaggtgacatcgttgaagagtatctttcccgcgcgaggcataaagttgcgtgtgatgcggaagggtcccggcacctcggaacggttgttaattacctgggcggcgagcacgatctcgtcaaagccgttgatgttgtggcccacaatgtaaagttccaagaagcgcgggatgcccttgatggaaggcaattttttaagttcctcgtaggtgagctcttcaggggagctgagcccgtgctctgaaagggcccagtctgcaagatgagggttggaagcgacgaatgagctccacaggtcacgggccattagcatttgcaggtggtcgcgaaaggtcctaaactggcgacctatggccattttttctggggtgatgcagtagaaggtaagcgggtcttgttcccagcggtcccatccaaggttcgcggctaggtctcgcgcggcagtcactagaggctcatctccgccgaacttcatgaccagcatgaagggcacgagctgcttcccaaaggcccccatccaagtataggtctctacatcgtaggtgacaaagagacgctcggtgcgaggatgcgagccgatcgggaagaactggatctcccgccaccaattggaggagtggctattgatgtggtgaaagtagaagtccctgcgacgggccgaacactcgtgctggcttttgtaaaaacgtgcgcagtactggcagcggtgcacgggctgtacatcctgcacgaggttgacctgacgaccgcgcacaaggaagcagagtgggaatttgagcccctcgcctggcgggtttggctggtggtcttctacttcggctgcttgtccttgaccgtctggctgctcgaggggagttacggtggatcggaccaccacgccgcgcgagcccaaagtccagatgtccgcgcgcggcggtcggagcttgatgacaacatcgcgcagatgggagctgtccatggtctggagctcccgcggcgtcaggtcaggcgggagctcctgcaggtttacctcgcatagacgggtcagggcgcgggctagatccaggtgatacctaatttccaggggctggttggtggcggcgtcgatggcttgcaagaggccgcatccccgcggcgcgactacggtaccgcgcggcgggcggtgggccgcgggggtgtccttggatgatgcatctaaaagcggtgacgcgggcgagcccccggaggtagggggggctccggacccgccgggagagggggcaggggcacgtcggcgccgcgcgcgggcaggagctggtgctgcgcgcgtaggttgctggcgaacgcgacgacgcggcggttgatctcctgaatctggcgcctctgcgtgaagacgacgggcccggtgagcttgagcctgaaagagagttcgacagaatcaatttcggtgtcgttgacggcggcctggcgcaaaatctcctgcacgtctcctgagttgtcttgataggcgatctcggccatgaactgctcgatctcttcctcctggagatctccgcgtccggctcgctccacggtggcggcgaggtcgttggaaatgcgggccatgagctgcgagaaggcgttgaggcctccctcgttccagacgcggctgtagaccacgcccccttcggcatcgcgggcgcgcatgaccacctgcgcgagattgagctccacgtgccgggcgaagacggcgtagtttcgcaggcgctgaaagaggtagttgagggtggtggcggtgtgttctgccacgaagaagtacataacccagcgtcgcaacgtggattcgttgatatcccccaaggcctcaaggcgctccatggcctcgtagaagtccacggcgaagttgaaaaactgggagttgcgcgccgacacggttaactcctcctccagaagacggatgagctcggcgacagtgtcgcgcacctcgcgctcaaaggctacaggggcctcttcttcttcttcaatctcctcttccataagggcctccccttcttcttcttctggcggcggtgggggaggggggacacggcggcgacgacggcgcaccgggaggcggtcgacaaagcgctcgatcatctccccgcggcgacggcgcatggtctcggtgacggcgcggccgttctcgcgggggcgcagttggaagacgccgcccgtcatgtcccggttatgggttggcggggggctgccatgcggcagggatacggcgctaacgatgcatctcaacaattgttgtgtaggtactccgccgccgagggacctgagcgagtccgcatcgaccggatcggaaaacctctcgagaaaggcgtctaaccagtcacagtcgcaaggtaggctgagcaccgtggcgggcggcagcgggcggcggtcggggttgtttctggcggaggtgctgctgatgatgtaattaaagtaggcggtcttgagacggcggatggtcgacagaagcaccatgtccttgggtccggcctgctgaatgcgcaggcggtcggccatgccccaggcttcgttttgacatcggcgcaggtctttgtagtagtcttgcatgagcctttctaccggcacttcttcttctccttcctcttgtcctgcatctcttgcatctatcgctgcggcggcggcggagtttggccgtaggtggcgccctcttcctcccatgcgtgtgaccccgaagcccctcatcggctgaagcagggctaggtcggcgacaacgcgctcggctaatatggcctgctgcacctgcgtgagggtagactggaagtcatccatgtccacaaagcggtggtatgcgcccgtgttgatggtgtaagtgcagttggccataacggaccagttaacggtctggtgacccggctgcgagagctcggtgtacctgagacgcgagtaagccctcgagtcaaatacgtagtcgttgcaagtccgcaccaggtactggtatcccaccaaaaagtgcggcggcggctggcggtagaggggccagcgtagggtggccggggctccgggggcgagatcttccaacataaggcgatgatatccgtagatgtacctggacatccaggtgatgccggcggcggtggtggaggcgcgcggaaagtcgcggacgcggttccagatgttgcgcagcggcaaaaagtgctccatggtcgggacgctctggccggtcaggcgcgcgcaatcgttgacgctctagaccgtgcaaaaggagagcctgtaagcgggcactcttccgtggtctggtggataaattcgcaagggtatcatggcggacgaccggggttcgagccccgtatccggccgtccgccgtgatccatgcggttaccgcccgcgtgtcgaacccaggtgtgcgacgtcagacaacgggggagtgctccttttggcttccttccaggcgcggcggctgctgcgctagcttttttggccactggccgcgcgcagcgtaagcggttaggctggaaagcgaaagcattaagtggctcgctccctgtagccggagggttattttccaagggttgagtcgcgggacccccggttcgagtctcggaccggccggactgcggcgaacgggggtttgcctccccgtcatgcaagaccccgcttgcaaattcctccggaaacagggacgagccccttttttgcttttcccagatgcatccggtgctgcggcagatgcgcccccctcctcagcagcggcaagagcaagagcagcggcagacatgcagggcaccctcccctcctcctaccgcgtcaggaggggcgacatccgcggttgacgcggcagcagatggtgattacgaacccccgcggcgccgggcccggcactacctggacttggaggagggcgagggcctggcgcggctaggagcgccctctcctgagcggtacccaagggtgcagctgaagcgtgatacgcgtgaggcgtacgtgccgcggcagaacctgtttcgcgaccgcgagggagaggagcccgaggagatgcgggatcgaaagttccacgcagggcgcgagctgcggcatggcctgaatcgcgagcggttgctgcgcgaggaggactttgagcccgacgcgcgaaccgggattagtcccgcgcgcgcacacgtggcggccgccgacctggtaaccgcatacgagcagacggtgaaccaggagattaactttcaaaaaagctttaacaaccacgtgcgtacgcttgtggcgcgcgaggaggtggctataggactgatgcatctgtgggactttgtaagcgcgctggagcaaaacccaaatagcaagccgctcatggcgcagctgttccttatagtgcagcacagcagggacaacgaggcattcagggatgcgctgctaaacatagtagagcccgagggccgctggctgctcgatttgataaacatcctgcagagcatagtggtgcaggagcgcagcttgagcctggctgacaaggtggccgccatcaactattccatgcttagcctgggcaagttttacgcccgcaagatataccataccccttacgttcccatagacaaggaggtaaagatcgaggggttctacatgcgcatggcgctgaaggtgcttaccttgagcgacgacctgggcgtttatcgcaacgagcgcatccacaaggccgtgagcgtgagccggcggcgcgagctcagcgaccgcgagctgatgcacagcctgcaaagggccctggctggcacgggcagcggcgatagagaggccgagtcctactttgacgcgggcgctgacctgcgctgggccccaagccgacgcgccctggaggcagctggggccggacctgggctggcggtggcacccgcgcgcgctggcaacgtcggcggcgtggaggaatatgacgaggacgatgagtacgagccagaggacggcgagtactaagcggtgatgtttctgatcagatgatgcaagacgcaacggacccggcggtgcgggcggcgctgcagagccagccgtccggccttaactccacggacgactggcgccaggtcatggaccgcatcatgtcgctgactgcgcgcaatcctgacgcgttccggcagcagccgcaggccaaccggctctccgcaattctggaagcggtggtcccggcgcgcgcaaaccccacgcacgagaaggtgctggcgatcgtaaacgcgctggccgaaaacagggccatccggcccgacgaggccggcctggtctacgacgcgctgcttcagcgcgtggctcgttacaacagcggcaacgtgcagaccaacctggaccggctggtgggggatgtgcgcgaggccgtggcgcagcgtgagcgcgcgcagcagcagggcaacctgggctccatggttgcactaaacgccttcctgagtacacagcccgccaacgtgccgcggggacaggaggactacaccaactttgtgagcgcactgcggctaatggtgactgagacaccgcaaagtgaggtgtaccagtctgggccagactattttttccagaccagtagacaaggcctgcagaccgtaaacctgagccaggctttcaaaaacttgcaggggctgtggggggtgcgggctcccacaggcgaccgcgcgaccgtgtctagcttgctgacgcccaactcgcgcctgttgctgctgctaatagcgcccttcacggacagtggcagcgtgtcccgggacacatacctaggtcacttgctgacactgtaccgcgaggccataggtcaggcgcatgtggacgagcatactttccaggagattacaagtgtcagccgcgcgctggggcaggaggacacgggcagcctggaggcaaccctaaactacctgctgaccaaccggcggcagaagatcccctcgttgcacagtttaaacagcgaggaggagcgcattttgcgctacgtgcagcagagcgtgagccttaacctgatgcgcgacggggtaacgcccagcgtggcgctggacatgaccgcgcgcaacatggaaccgggcatgtatgcctcaaaccggccgtttatcaaccgcctaatggactacttgcatcgcgcggccgccgtgaaccccgagtatttcaccaatgccatcttgaacccgcactggctaccgccccctggtttctacaccgggggattcgaggtgcccgagggtaacgatggattcctctgggacgacatagacgacagcgtgttttccccgcaaccgcagaccctgctagagttgcaacagcgcgagcaggcagaggcggcgctgcgaaaggaaagcttccgcaggccaagcagcttgtccgatctaggcgctgcggccccgcggtcagatgctagtagcccatttccaagcttgatagggtctcttaccagcactcgcaccacccgcccgcgcctgctgggcgaggaggagtacctaaacaactcgctgctgcagccgcagcgcgaaaaaaacctgcctccggcatttcccaacaacgggatagagagcctagtggacaagatgagtagatggaagacgtacgcgcaggagcacagggacgtgccaggcccgcgcccgcccacccgtcgtcaaaggcacgaccgtcagcggggtctggtgtgggaggacgatgactcggcagacgacagcagcgtcctggatttgggagggagtggcaacccgtttgcgcaccttcgccccaggctggggagaatgttttaaaaaaaaaaaagcatgatgcaaaataaaaaactcaccaaggccatggcaccgagcgttggttttcttgtattccccttagtatgcggcgcgcggcgatgtatgaggaaggtcctcctccctcctacgagagtgtggtgagcgcggcgccagtggcggcggcgctgggttctcccttcgatgctcccctggacccgccgtttgtgcctccgcggtacctgcggcctaccggggggagaaacagcatccgttactctgagttggcacccctattcgacaccacccgtgtgtacctggtggacaacaagtcaacggatgtggcatccctgaactaccagaacgaccacagcaactttctgaccacggtcattcaaaacaatgactacagcccgggggaggcaagcacacagaccatcaatcttgacgaccggtcgcactggggcggcgacctgaaaaccatcctgcataccaacatgccaaatgtgaacgagttcatgtttaccaataagtttaaggcgcgggtgatggtgtcgcgcttgcctactaaggacaatcaggtggagctgaaatacgagtgggtggagttcacgctgcccgagggcaactactccgagaccatgaccatagaccttatgaacaacgcgatcgtggagcactacttgaaagtgggcagacagaacggggttctggaaagcgacatcggggtaaagtttgacacccgcaacttcagactggggtttgaccccgtcactggtcttgtcatgcctggggtatatacaaacgaagccttccatccagacatcattttgctgccaggatgcggggtggacttcacccacagccgcctgagcaacttgttgggcatccgcaagcggcaacccttccaggagggctttaggatcacctacgatgatctggagggtggtaacattcccgcactgttggatgtggacgcctaccaggcgagcttgaaagatgacaccgaacagggcgggggtggcgcaggcggcagcaacagcagtggcagcggcgcggaagagaactccaacgcggcagccgcggcaatgcagccggtggaggacatgaacgatcatgccattcgcggcgacacctttgccacacgggctgaggagaagcgcgctgaggccgaagcagcggccgaagctgccgcccccgctgcgcaacccgaggtcgagaagcctcagaagaaaccggtgatcaaacccctgacagaggacagcaagaaacgcagttacaacctaataagcaatgacagcaccttcacccagtaccgcagctggtaccttgcatacaactacggcgaccctcagaccggaatccgctcatggaccctgctttgcactcctgacgtaacctgcggctcggagcaggtctactggtcgttgccagacatgatgcaagaccccgtgaccttccgctccacgcgccagatcagcaactttccggtggtgggcgccgagctgttgcccgtgcactccaagagcttctacaacgaccaggccgtctactcccaactcatccgccagtttacctctctgacccacgtgttcaatcgctttcccgagaaccagattttggcgcgcccgccagcccccaccatcaccaccgtcagtgaaaacgttcctgctctcacagatcacgggacgctaccgctgcgcaacagcatcggaggagtccagcgagtgaccattactgacgccagacgccgcacctgcccctacgtttacaaggccctgggcatagtctcgccgcgcgtcctatcgagccgcactttttgagcaagcatgtccatccttatatcgcccagcaataacacaggctggggcctgcgcttcccaagcaagatgtttggcggggccaagaagcgctccgaccaacacccagtgcgcgtgcgcgggcactaccgcgcgccctggggcgcgcacaaacgcggccgcactgggcgcaccaccgtcgatgacgccatcgacgcggtggtggaggaggcgcgcaactacacgcccacgccgccaccagtgtccacagtggacgcggccattcagaccgtggtgcgcggagcccggcgctatgctaaaatgaagagacggcggaggcgcgtagcacgtcgccaccgccgccgacccggcactgccgcccaacgcgcggcggcggccctgcttaaccgcgcacgtcgcaccggccgacgggcggccatgcgggccgctcgaaggctggccgcgggtattgtcactgtgccccccaggtccaggcgacgagcggccgccgcagcagccgcggccattagtgctatgactcagggtcgcaggggcaacgtgtattgggtgcgcgactcggttagcggcctgcgcgtgcccgtgcgcacccgccccccgcgcaactagattgcaagaaaaaactacttagactcgtactgttgtatgtatccagcggcggcggcgcgcaacgaagctatgtccaagcgcaaaatcaaagaagagatgctccaggtcatcgcgccggagatctatggccccccgaagaaggaagagcaggattacaagccccgaaagctaaagcgggtcaaaaagaaaaagaaagatgatgatgatgaacttgacgacgaggtggaactgctgcacgctaccgcgcccaggcgacgggtacagtggaaaggtcgacgcgtaaaacgtgttttgcgacccggcaccaccgtagtctttacgcccggtgagcgctccacccgcacctacaagcgcgtgtatgatgaggtgtacggcgacgaggacctgcttgagcaggccaacgagcgcctcggggagtttgcctacggaaagcggcataaggacatgctggcgttgccgctggacgagggcaacccaacacctagcctaaagcccgtaacactgcagcaggtgctgcccgcgcttgcaccgtccgaagaaaagcgcggcctaaagcgcgagtctggtgacttggcacccaccgtgcagctgatggtacccaagcgccagcgactggaagatgtcttggaaaaaatgaccgtggaacctgggctggagcccgaggtccgcgtgcggccaatcaagcaggtggcgccgggactgggcgtgcagaccgtggacgttcagatacccactaccagtagcaccagtattgccaccgccacagagggcatggagacacaaacgtccccggttgcctcagcggtggcggatgccgcggtgcaggcggtcgctgcggccgcgtccaagacctctacggaggtgcaaacggacccgtggatgtttcgcgtttcagccccccggcgcccgcgcggttcgaggaagtacggcgccgccagcgcgctactgcccgaatatgccctacatccttccattgcgcctacccccggctatcgtggctacacctaccgccccagaagacgagcaactacccgacgccgaaccaccactggaacccgccgccgccgtcgccgtcgccagcccgtgctggccccgatttccgtgcgcagggtggctcgcgaaggaggcaggaccctggtgctgccaacagcgcgctaccaccccagcatcgtttaaaagccggtctttgtggttcttgcagatatggccctcacctgccgcctccgtttcccggtgccgggattccgaggaagaatgcaccgtaggaggggcatggccggccacggcctgacgggcggcatgcgtcgtgcgcaccaccggcggcggcgcgcgtcgcaccgtcgcatgcgcggcggtatcctgcccctccttattccactgatcgccgcggcgattggcgccgtgcccggaattgcatccgtggccttgcaggcgcagagacactgattaaaaacaagttgcatgtggaaaaatcaaaataaaaagtctggactctcacgctcgcttggtcctgtaactattttgtagaatggaagacatcaactttgcgtctctggccccgcgacacggctcgcgcccgttcatgggaaactggcaagatatcggcaccagcaatatgagcggtggcgccttcagctggggctcgctgtggagcggcattaaaaatttcggttccaccgttaagaactatggcagcaaggcctggaacagcagcacaggccagatgctgagggataagttgaaagagcaaaatttccaacaaaaggtggtagatggcctggcctctggcattagcggggtggtggacctggccaaccaggcagtgcaaaataagattaacagtaagcttgatccccgccctcccgtagaggagcctccaccggccgtggagacagtgtctccagaggggcgtggcgaaaagcgtccgcgccccgacagggaagaaactctggtgacgcaaatagacgagcctccctcgtacgaggaggcactaaagcaaggcctgcccaccacccgtcccatcgcgcccatggctaccggagtgctgggccagcacacacccgtaacgctggacctgcctccccccgccgacacccagcagaaacctgtgctgccaggcccgaccgccgttgttgtaacccgtcctagccgcgcgtccctgcgccgcgccgccagcggtccgcgatcgttgcggcccgtagccagtggcaactggcaaagcacactgaacagcatcgtgggtctgggggtgcaatccctgaagcgccgacgatgcttctgaatagctaacgtgtcgtatgtgtgtcatgtatgcgtccatgtcgccgccagaggagctgctgagccgccgcgcgcccgctttccaagatggctaccccttcgatgatgccgcagtggtcttacatgcacatctcgggccaggacgcctcggagtacctgagccccgggctggtgcagtttgcccgcgccaccgagacgtacttcagcctgaataacaagtttagaaaccccacggtggcgcctacgcacgacgtgaccacagaccggtcccagcgtttgacgctgcggttcatccctgtggaccgtgaggatactgcgtactcgtacaaggcgcggttcaccctagctgtgggtgataaccgtgtgctggacatggcttccacgtactttgacatccgcggcgtgctggacaggggccctacttttaagccctactctggcactgcctacaacgccctggctcccaagggtgccccaaatccttgcgaatgggatgaagctgctactgctcttgaaataaacctagaagaagaggacgatgacaacgaagacgaagtagacgagcaagctgagcagcaaaaaactcacgtatttgggcaggcgccttattctggtataaatattacaaaggagggtattcaaataggtgtcgaaggtcaaacacctaaatatgccgataaaacatttcaacctgaacctcaaataggagaatctcagtggtacgaaactgaaattaatcatgcagctgggagagtccttaaaaagactaccccaatgaaaccatgttacggttcatatgcaaaacccacaaatgaaaatggagggcaaggcattcttgtaaagcaacaaaatggaaagctagaaagtcaagtggaaatgcaatttttctcaactactgaggcgaccgcaggcaatggtgataacttgactcctaaagtggtattgtacagtgaagatgtagatatagaaaccccagacactcatatttcttacatgcccactattaaggaaggtaactcacgagaactaatgggccaacaatctatgcccaacaggcctaattacattgcttttagggacaattttattggtctaatgtattacaacagcacgggtaatatgggtgttctggcgggccaagcatcgcagttgaatgctgttgtagatttgcaagacagaaacacagagctttcataccagcttttgcttgattccattggtgatagaaccaggtacttttctatgtggaatcaggctgttgacagctatgatccagatgttagaattattgaaaatcatggaactgaagatgaacttccaaattactgctttccactgggaggtgtgattaatacagagactcttaccaaggtaaaacctaaaacaggtcaggaaaatggatgggaaaaagatgctacagaattttcagataaaaatgaaataagagttggaaataattttgccatggaaatcaatctaaatgccaacctgtggagaaatttcctgtactccaacatagcgctgtatttgcccgacaagctaaagtacagtccttccaacgtaaaaatttctgataacccaaacacctacgactacatgaacaagcgagtggtggctcccgggttagtggactgctacattaaccttggagcacgctggtcccttgactatatggacaacgtcaacccatttaaccaccaccgcaatgctggcctgcgctaccgctcaatgttgctgggcaatggtcgctatgtgcccttccacatccaggtgcctcagaagttctttgccattaaaaacctccttctcctgccgggctcatacacctacgagtggaacttcaggaaggatgttaacatggttctgcagagctccctaggaaatgacctaagggttgacggagccagcattaagtttgatagcatttgcctttacgccaccttcttccccatggcccacaacaccgcctccacgcttgaggccatgcttagaaacgacaccaacgaccagtcctttaacgactatctctccgccgccaacatgctctaccctatacccgccaacgctaccaacgtgcccatatccatcccctcccgcaactgggcggctttccgcggctgggccttcacgcgccttaagactaaggaaaccccatcactgggctcgggctacgacccttattacacctactctggctctataccctacctagatggaaccttttacctcaaccacacctttaagaaggtggccattacctttgactcttctgtcagctggcctggcaatgaccgcctgcttacccccaacgagtttgaaattaagcgctcagttgacggggagggttacaacgttgcccagtgtaacatgaccaaagactggttcctggtacaaatgctagctaactacaacattggctaccagggcttctatatcccagagagctacaaggaccgcatgtactccttctttagaaacttccagcccatgagccgtcaggtggtggatgatactaaatacaaggactaccaacaggtgggcatcctacaccaacacaacaactctggatttgttggctaccttgcccccaccatgcgcgaaggacaggcctaccctgctaacttcccctatccgcttataggcaagaccgcagttgacagcattacccagaaaaagtttctttgcgatcgcaccctttggcgcatcccattctccagtaactttatgtccatgggcgcactcacagacctgggccaaaaccttctctacgccaactccgcccacgcgctagacatgacttttgaggtggatcccatggacgagcccacccttctttatgttttgtttgaagtctttgacgtggtccgtgtgcaccggccgcaccgcggcgtcatcgaaaccgtgtacctgcgcacgcccttctcggccggcaacgccacaacataaagaagcaagcaacatcaacaacagctgccgccatgggctccagtgagcaggaactgaaagccattgtcaaagatcttggttgtgggccatattttttgggcacctatgacaagcgctttccaggctttgtttctccacacaagctcgcctgcgccatagtcaatacggccggtcgcgagactgggggcgtacactggatggcctttgcctggaacccgcactcaaaaacatgctacctctttgagccctttggcttttctgaccagcgactcaagcaggtttaccagtttgagtacgagtcactcctgcgccgtagcgccattgcttcttcccccgaccgctgtataacgctggaaaagtccacccaaagcgtacaggggcccaactcggccgcctgtggactattctgctgcatgtttctccacgcctttgccaactggccccaaactcccatggatcacaaccccaccatgaaccttattaccggggtacccaactccatgctcaacagtccccaggtacagcccaccctgcgtcgcaaccaggaacagctctacagcttcctggagcgccactcgccctacttccgcagccacagtgcgcagattaggagcgccacttctttttgtcacttgaaaaacatgtaaaaataatgtactagagacactttcaataaaggcaaatgcttttatttgtacactctcgggtgattatttacccccacccttgccgtctgcgccgtttaaaaatcaaaggggttctgccgcgcatcgctatgcgccactggcagggacacgttgcgatactggtgtttagtgctccacttaaactcaggcacaaccatccgcggcagctcggtgaagttttcactccacaggctgcgcaccatcaccaacgcgtttagcaggtcgggcgccgatatcttgaagtcgcagttggggcctccgccctgcgcgcgcgagttgcgatacacagggttgcagcactggaacactatcagcgccgggtggtgcacgctggccagcacgctcttgtcggagatcagatccgcgtccaggtcctccgcgttgctcagggcgaacggagtcaactttggtagctgccttcccaaaaagggcgcgtgcccaggctttgagttgcactcgcaccgtagtggcatcaaaaggtgaccgtgcccggtctgggcgttaggatacagcgcctgcataaaagccttgatctgcttaaaagccacctgagcctttgcgccttcagagaagaacatgccgcaagacttgccggaaaactgattggccggacaggccgcgtcgtgcacgcagcaccttgcgtcggtgttggagatctgcaccacatttcggccccaccggttcttcacgatcttggccttgctagactgctccttcagcgcgcgctgcccgttttcgctcgtcacatccatttcaatcacgtgctccttatttatcataatgcttccgtgtagacacttaagctcgccttcgatctcagcgcagcggtgcagccacaacgcgcagcccgtgggctcgtgatgcttgtaggtcacctctgcaaacgactgcaggtacgcctgcaggaatcgccccatcatcgtcacaaaggtcttgttgctggtgaaggtcagctgcaacccgcggtgctcctcgttcagccaggtcttgcatacggccgccagagcttccacttggtcaggcagtagtttgaagttcgcctttagatcgttatccacgtggtacttgtccatcagcgcgcgcgcagcctccatgcccttctcccacgcagacacgatcggcacactcagcgggttcatcaccgtaatttcactttccgcttcgctgggctcttcctcttcctcttgcgtccgcataccacgcgccactgggtcgtcttcattcagccgccgcactgtgcgcttacctcctttgccatgcttgattagcaccggtgggttgctgaaacccaccatttgtagcgccacatcttctctttcttcctcgctgtccacgattacctctggtgatggcgggcgctcgggcttgggagaagggcgcttctttttcttcttgggcgcaatggccaaatccgccgccgaggtcgatggccgcgggctgggtgtgcgcggcaccagcgcgtcttgtgatgagtcttcctcgtcctcggactcgatacgccgcctcatccgcttttttgggggcgcccggggaggcggcggcgacggggacggggacgacacgtcctccatggttgggggacgtcgcgccgcaccgcgtccgcgctcgggggtggtttcgcgctgctcctcttcccgactggccatttccttctcctataggcagaaaaagatcatggagtcagtcgagaagaaggacagcctaaccgccccctctgagttcgccaccaccgcctccaccgatgccgccaacgcgcctaccaccttccccgtcgaggcacccccgcttgaggaggaggaagtgattatcgagcaggacccaggttttgtaagcgaagacgacgaggaccgctcagtaccaacagaggataaaaagcaagaccaggacaacgcagaggcaaacgaggaacaagtcgggcggggggacgaaaggcatggcgactacctagatgtgggagacgacgtgctgttgaagcatctgcagcgccagtgcgccattatctgcgacgcgttgcaagagcgcagcgatgtgcccctcgccatagcggatgtcagccttgcctacgaacgccacctattctcaccgcgcgtaccccccaaacgccaagaaaacggcacatgcgagcccaacccgcgcctcaacttctaccccgtatttgccgtgccagaggtgcttgccacctatcacatctttttccaaaactgcaagatacccctatcctgccgtgccaaccgcagccgagcggacaagcagctggccttgcggcagggcgctgtcatacctgatatcgcctcgctcaacgaagtgccaaaaatctttgagggtcttggacgcgacgagaagcgcgcggcaaacgctctgcaacaggaaaacagcgaaaatgaaagtcactctggagtgttggtggaactcgagggtgacaacgcgcgcctagccgtactaaaacgcagcatcgaggtcacccactttgcctacccggcacttaacctaccccccaaggtcatgagcacagtcatgagtgagctgatcgtgcgccgtgcgcagcccctggagagggatgcaaatttgcaagaacaaacagaggagggcctacccgcagttggcgacgagcagctagcgcgctggcttcaaacgcgcgagcctgccgacttggaggagcgacgcaaactaatgatggccgcagtgctcgttaccgtggagcttgagtgcatgcagcggttctttgctgacccggagatgcagcgcaagctagaggaaacattgcactacacctttcgacagggctacgtacgccaggcctgcaagatctccaacgtggagctctgcaacctggtctcctaccttggaattttgcacgaaaaccgccttgggcaaaacgtgcttcattccacgctcaagggcgaggcgcgccgcgactacgtccgcgactgcgtttacttatttctatgctacacctggcagacggccatgggcgtttggcagcagtgcttggaggagtgcaacctcaaggagctgcagaaactgctaaagcaaaacttgaaggacctatggacggccttcaacgagcgctccgtggccgcgcacctggcggacatcattttccccgaacgcctgcttaaaaccctgcaacagggtctgccagacttcaccagtcaaagcatgttgcagaactttaggaactttatcctagagcgctcaggaatcttgcccgccacctgctgtgcacttcctagcgactttgtgcccattaagtaccgcgaatgccctccgccgctttggggccactgctaccttctgcagctagccaactaccttgcctaccactctgacataatggaagacgtgagcggtgacggtctactggagtgtcactgtcgctgcaacctatgcaccccgcaccgctccctggtttgcaattcgcagctgcttaacgaaagtcaaattatcggtacctttgagctgcagggtccctcgcctgacgaaaagtccgcggctccggggttgaaactcactccggggctgtggacgtcggcttaccttcgcaaatttgtacctgaggactaccacgcccacgagattaggttctacgaagaccaatcccgcccgccaaatgcggagcttaccgcctgcgtcattacccagggccacattcttggccaattgcaagccatcaacaaagcccgccaagagtttctgctacgaaagggacggggggtttacttggacccccagtccggcgaggagctcaacccaatccccccgccgccgcagccctatcagcagcagccgcgggcccttgcttcccaggatggcacccaaaaagaagctgcagctgccgccgccacccacggacgaggaggaatactgggacagtcaggcagaggaggttttggacgaggaggaggaggacatgatggaagactgggagagcctagacgaggaagcttccgaggtcgaagaggtgtcagacgaaacaccgtcaccctcggtcgcattcccctcgccggcgccccagaaatcggcaaccggttccagcatggctacaacctccgctcctcaggcgccgccggcactgcccgttcgccgacccaaccgtagatgggacaccactggaaccagggccggtaagtccaagcagccgccgccgttagcccaagagcaacaacagcgccaaggctaccgctcatggcgcgggcacaagaacgccatagttgcttgcttgcaagactgtgggggcaacatctccttcgcccgccgctttcttctctaccatcacggcgtggccttcccccgtaacatcctgcattactaccgtcatctctacagcccatactgcaccggcggcagcggcagcggcagcaacagcagcggccacacagaagcaaaggcgaccggatagcaagactctgacaaagcccaagaaatccacagcggcggcagcagcaggaggaggagcgctgcgtctggcgcccaacgaacccgtatcgacccgcgagcttagaaacaggatttttcccactctgtatgctatatttcaacagagcaggggccaagaacaagagctgaaaataaaaaacaggtctctgcgatccctcacccgcagctgcctgtatcacaaaagcgaagatcagcttcggcgcacgctggaagacgcggaggctctcttcagtaaatactgcgcgctgactcttaaggactagtttcgcgccctttctcaaatttaagcgcgaaaactacgtcatctccagcggccacacccggcgccagcacctgtcgtcagcgccattatgagcaaggaaattcccacgccctacatgtggagttaccagccacaaatgggacttgcggctggagctgcccaagactactcaacccgaataaactacatgagcgcgggaccccacatgatatcccgggtcaacggaatccgcgcccaccgaaaccgaattctcttggaacaggcggctattaccaccacacctcgtaataaccttaatccccgtagttggcccgctgccctggtgtaccaggaaagtcccgctcccaccactgtggtacttcccagagacgcccaggccgaagttcagatgactaactcaggggcgcagcttgcgggcggctttcgtcacagggtgcggtcgcccgggcagggtataactcacctgacaatcagagggcgaggtattcagctcaacgacgagtcggtgagctcctcgcttggtctccgtccggacgggacatttcagatcggcggcgccggccgctcttcattcacgcctcgtcaggcaatcctaactctgcagacctcgtcctctgagccgcgctctggaggcattggaactctgcaatttattgaggagtttgtgccatcggtctactttaaccccttctcgggacctcccggccactatccggatcaatttattcctaactttgacgcggtaaaggactcggcggatggctacgactgaatgttaagtggagaggcagagcaactgcgcctgaaacacctggtccactgtcgccgccacaagtgctttgcccgcgactccggtgagttttgctactttgaattgcccgaggatcatatcgagggcccggcgcacggcgtccggcttaccgcccagggagagcttgcccgtagcctgattcgggagtttacccagcgccccctgctagttgagcgggacaggggaccctgtgttctcactgtgatttgcaactgtcctaaccctggattacatcaagatctttgttgccatctctgtgctgagtataataaatacagaaattaaaatatactggggctcctatcgccatcctgtaaacgccaccgtcttcacccgcccaagcaaaccaaggcgaaccttacctggtacttttaacatctctccctctgtgatttacaacagtttcaacccagacggagtgagtctacgagagaacctctccgagctcagctactccatcagaaaaaacaccaccctccttacctgccgggaacgtacgacctagggataacagggtaataagcaattgactctatgtgggatatgctccagcgctacaaccttgaagtcaggcttcctggatgtcagcatctgactttggccagcacctgtcccgcggatttgttccagtccaactacagcgacccaccctaacagagatgaccaacacaaccaacgcggccgccgctaccggacttacatctaccacaaatacaccccaagtttctgcctttgtcaataactgggataacttgggcatgtggtggttctccatagcgcttatgtttgtatgccttattattatgtggctcatctgctgcctaaagcgcaaacgcgcccgaccacccatctatagtcccatcattgtgctacacccaaacaatgatggaatccatagattggacggactgaaacacatgttcttttctcttacagtatgattaaatgagacatgattcctcgagtttttatattactgacccttgttgcgcttttttgtgcgtgctccacattggctgcggtttctcacatcgaagtagactgcattccagccttcacagtctatttgctttacggatttgtcaccctcacgctcatctgcagcctcatcactgtggtcatcgcctttatccagtgcattgactgggtctgtgtgcgctttgcatatctcagacaccatccccagtacagggacaggactatagctgagcttcttagaattctttaattatgaaatttactgtgacttttctgctgattatttgcaccctatctgcgttttgttccccgacctccaagcctcaaagacatatatcatgcagattcactcgtatatggaatattccaagttgctacaatgaaaaaagcgatctttccgaagcctggttatatgcaatcatctctgttatggtgttctgcagtaccatcttagccctagctatatatccctaccttgacattggctggaaacgaatagatgccatgaaccacccaactttccccgcgcccgctatgcttccactgcaacaagttgttgccggcggctttgtcccagccaatcagcctcgccccacttctcccacccccactgaaatcagctactttaatctaacaggaggagatgactgacaccctagatctagaaatggacggaattattacagagcagcgcctgctagaaagacgcagggcagcggccgagcaacagcgcatgaatcaagagctccaagacatggttaacttgcaccagtgcaaaaggggtatcttttgtctggtaaagcaggccaaagtcacctacgacagtaataccaccggacaccgccttagctacaagttgccaaccaagcgtcagaaattggtggtcatggtgggagaaaagcccattaccataactcagcactcggtagaaaccgaaggctgcattcactcaccttgtcaaggacctgaggatctctgcacccttattaagaccctgtgcggtctcaaagatcttattccctttaactaataaaaaaaaataataaagcatcacttacttaaaatcagttagcaaatttctgtccagtttattcagcagcacctccttgccctcctcccagctctggtattgcagcttcctcctggctgcaaactttctccacaatctaaatggaatgtcagtttcctcctgttcctgtccatccgcacccactatcttcatgttgttgcagatgaagcgcgcaagaccgtctgaagataccttcaaccccgtgtatccatatgacacggaaaccggtcctccaactgtgccttttcttactcctccctttgtatcccccaatgggtttcaagagagtccccctggggtactctctttgcgcctatccgaacctctagttacctccaatggcatgcttgcgctcaaaatgggcaacggcctctctctggacgaggccggcaaccttacctcccaaaatgtaaccactgtgagcccacctctcaaaaaaaccaagtcaaacataaacctggaaatatctgcacccctcacagttacctcagaagccctaactgtggctgccgccgcacctctaatggtcgcgggcaacacactcaccatgcaatcacaggccccgctaaccgtgcacgactccaaacttagcattgccacccaaggacccctcacagtgtcagaaggaaagctagccctgcaaacatcaggccccctcaccaccaccgatagcagtacccttactatcactgcctcaccccctctaactactgccactggtagcttgggcattgacttgaaagagcccatttatacacaaaatggaaaactaggactaaagtacggggctcctttgcatgtaacagacgacctaaacactttgaccgtagcaactggtccaggtgtgactattaataatacttccttgcaaactaaagttactggagccttgggttttgattcacaaggcaatatgcaacttaatgtagcaggaggactaaggattgattctcaaaacagacgccttatacttgatgttagttatccgtttgatgctcaaaaccaactaaatctaagactaggacagggccctctttttataaactcagcccacaacttggatattaactacaacaaaggcctttacttgtttacagcttcaaacaattccaaaaagcttgaggttaacctaagcactgccaaggggttgatgtttgacgctacagccatagccattaatgcaggagatgggcttgaatttggttcacctaatgcaccaaacacaaatcccctcaaaacaaaaattggccatggcctagaatttgattcaaacaaggctatggttcctaaactaggaactggccttagttttgacagcacaggtgccattacagtaggaaacaaaaataatgataagctaaccctatggacaggtccaaaaccagaagccaactgcataattgaatacgggaaacaaaacccagatagcaaactaactttaatccttgtaaaaaatggaggaattgttaatggatatgtaacgctaatgggagcctcagactacgttaacaccttatttaaaaacaaaaatgtctccattaatgtagaactatactttgatgccactggtcatatattaccagactcatcttctcttaaaacagatctagaactaaaatacaagcaaaccgctgactttagtgcaagaggttttatgccaagtactacagcgtatccatttgtccttcctaatgcgggaacacataatgaaaattatatttttggtcaatgctactacaaagcaagcgatggtgccctttttccgttggaagttactgttatgcttaataaacgcctgccagatagtcgcacatcctatgttatgacttttttatggtccttgaatgctggtctagctccagaaactactcaggcaaccctcataacctccccatttaccttttcctatattagagaagatgactaataaactctaaagaatcgtttgtgttatgtttcaacgtgtttatttttcaattgcagaaaatttcaagtcatttttcattcagtagtatagccccaccaccacatagcttatacagatcaccgtaccttaatcaaactcacagaaccctagtattcaacctgccacctccctcccaacacacagagtacacagtcctttctccccggctggccttaaaaagcatcatatcatgggtaacagacatattcttaggtgttatattccacacggtttcctgtcgagccaaacgctcatcagtgatattaataaactccccgggcagctcacttaagttcatgtcgctgtccagctgctgagccacaggctgctgtccaacttgcggttgcttaacgggcggcgaaggagaagtccacgcctacatgggggtagagtcataatcgtgcatcaggatagggcggtggtgctgcagcagcgcgcgaataaactgctgccgccgccgctccgtcctgcaggaatacaacatggcagtggtctcctcagcgatgattcgcaccgcccgcagcataaggcgccttgtcctccgggcacagcagcgcaccctgatctcacttaaatcagcacagtaactgcagcacagcaccacaatattgttcaaaatcccacagtgcaaggcgctgtatccaaagctcatggcggggaccacagaacccacgtggccatcataccacaagcgcaggtagattaagtggcgacccctcataaacacgctggacataaacattacctcttttggcatgttgtaattcaccacctcccggtaccatataaacctctgattaaacatggcgccatccaccaccatcctaaaccagctggccaaaacctgcccgccggctatacactgcagggaaccgggactggaacaatgacagtggagagcccaggactcgtaaccatggatcatcatgctcgtcatgatatcaatgttggcacaacacaggcacacgtgcatacacttcctcaggattacaagctcctcccgcgttagaaccatatcccagggaacaacccattcctgaatcagcgtaaatcccacactgcagggaagacctcgcacgtaactcacgttgtgcattgtcaaagtgttacattcgggcagcagcggatgatcctccagtatggtagcgcgggtttctgtctcaaaaggaggtagacgatccctactgtacggagtgcgccgagacaaccgagatcgtgttggtcgtagtgtcatgccaaatggaacgccggacgtagtcatatttcctgaagcaaaaccaggtgcgggcgtgacaaacagatctgcgtctccggtctcgccgcttagatcgctctgtgtagtagttgtagtatatccactctctcaaagcatccaggcgccccctggcttcgggttctatgtaaactccttcatgcgccgctgccctgataacatccaccaccgcagaataagccacacccagccaacctacacattcgttctgcgagtcacacacgggaggagcgggaagagctggaagaaccatgtttttttttttattccaaaagattatccaaaacctcaaaatgaagatctattaagtgaacgcgctcccctccggtggcgtggtcaaactctacagccaaagaacagataatggcatttgtaagatgttgcacaatggcttccaaaaggcaaacggccctcacgtccaagtggacgtaaaggctaaacccttcagggtgaatctcctctataaacattccagcaccttcaaccatgcccaaataattctcatctcgccaccttctcaatatatctctaagcaaatcccgaatattaagtccggccattgtaaaaatctgctccagagcgccctccaccttcagcctcaagcagcgaatcatgattgcaaaaattcaggttcctcacagacctgtataagattcaaaagcggaacattaacaaaaataccgcgatcccgtaggtcccttcgcagggccagctgaacataatcgtgcaggtctgcacggaccagcgcggccacttccccgccaggaaccttgacaaaagaacccacactgattatgacacgcatactcggagctatgctaaccagcgtagccccgatgtaagctttgttgcatgggcggcgatataaaatgcaaggtgctgctcaaaaaatcaggcaaagcctcgcgcaaaaaagaaagcacatcgtagtcatgctcatgcagataaaggcaggtaagctccggaaccaccacagaaaaagacaccatttttctctcaaacatgtctgcgggtttctgcataaacacaaaataaaataacaaaaaaacatttaaacattagaagcctgtcttacaacaggaaaaacaacccttataagcataagacggactacggccatgccggcgtgaccgtaaaaaaactggtcaccgtgattaaaaagcaccaccgacagctcctcggtcatgtccggagtcataatgtaagactcggtaaacacatcaggttgattcatcggtcagtgctaaaaagcgaccgaaatagcccgggggaatacatacccgcaggcgtagagacaacattacagcccccataggaggtataacaaaattaataggagagaaaaacacataaacacctgaaaaaccctcctgcctaggcaaaatagcaccctcccgctccagaacaacatacagcgcttcacagcggcagcctaacagtcagccttaccagtaaaaaagaaaacctattaaaaaaacaccactcgacacggcaccagctcaatcagtcacagtgtaaaaaagggccaagtgcagagcgagtatatataggactaaaaaatgacgtaacggttaaagtccacaaaaaacacccagaaaaccgcacgcgaacctacgcccagaaacgaaagccaaaaaacccacaacttcctcaaatcgtcacttccgttttcccacgttacgtaacttcccattttaagaaaactacaattcccaacacatacaagttactccgccctaaaacctacgtcacccgccccgttcccacgccccgcgccacgtcacaaactccaccccctcattatcatattggcttcaatccaaaataaggtatattattgatgatgttaat

SEQ ID NO: 127 - DNA, 39752 bp, Artificial Sequence
  ICOSTAT
  misc_feature (5915)..(5917): n is a, c, g, or t
  misc_feature (32912)..(32912): n is a, c, g, or t
  misc_feature (34601)..(34601): n is a, c, g, or t
  misc_feature (38163)..(38168): n is a, c, g, or t
taacatcatcaattataccttccattttggattgaagccaatatgataatgagggggtggagtttgtgacgtggcgcggggcgtgggaacggggcgggtgacgtagtagtgtggcggaagtgtgatgttgcaagtgtggcggaacacatgtaagcgacggatgtggcaaaagtgacgtttttggtgtgcgccggtgtacacaggaagtgacaattttcgcgcggttttaggcggatgttgtagtaaatttgggcgtaaccgagtaagatttggccattttcgcgggaaaactgaataagaggaagtgaaatctgaataattttgtgttactcatagcgcgtaatatttgtctagggccgcggggactttgaccgtttacgtggagactcgcccaggtgtttttctcaggtgttttccgcgtacgtcggcggctcgtggctcttccgggaaaaggattctcggaaagtggttcgagtacgtcggcggctcgtggctcttccgggaaaaggattctcggaaagtggttcgaagtacgtcgaccacaaaccccgcccagcgtcttgtcattggcgtcgacgctgtacggggtcaaagttggcgttttattattatagtcagctgacgtgtagtgtatttatacccggtgagttcctcaagaggccactcttgagtgccagcgagtagagttttctcctccgagccgctccgacaccgggactgaaaatgagacatattatctgccacggaggtgttattaccgaagaaatggccgccagtcttttggaccagctgatcgaagaggtactggctgataatcttccacctcctagccattttgaaccacctacccttcacgaactgtatgatttagacgtgacggcccccgaagatcccaacgaggaggcggtttcgcagatttttcccgactctgtaatgttggcggtgcaggaagggattgacttactcacttttccgccggcgcccggttctccggagccgcctcacctttcccggcagcccgagcagccggagcagagagccttgggtccggtttctatgccaaaccttgtaccggaggtgatcgatccacccagtgacgacgaggatgaagagggtgaggagtttgtgttagattatgtggagcaccccgggcacggttgcaggtcttgtcattatcaccggaggaatacgggggacccagatattatgtgttcgctttgctatatgaggacctgtggcatgtttgtctacagtaagtgaaaattatgggcagtgggtgatagagtggtgggtttggtgtggtaattttttttttaatttttacagttttgtggtttaaagaattttgtattgtgatttttttaaaaggtcctgtgtctgaacctgagcctgagcccgagccagaaccggagcctgcaagacctacccgccgtcctaaaatggcgcctgctatcctgagacgcccgacatcacctgtgtctagagaatgcaatagtagtacggatagctgtgactccggtccttctaacacacctcctgagatacacccggtggtcccgctgtgccccattaaaccagttgccgtgagagttggtgggcgtcgccaggctgtggaatgtatcgaggacttgcttaacgagcctgggcaacctttggacttgagctgtaaacgccccaggccataaggtgtaaacctgtgattgcgtgtgtggttaacgcctttgtttgctgaatgagttgatgtaagtttaataaagggtgagataatgtttaacttgcatggcgtgttaaatggggcggggcttaaagggtatataatgcgccgtgggctaatcttggttacatctgacctcatggaggcttgggagtgtttggaagatttttctgctgtgcgtaacttgctggaacagagctctaacagtacctcttggttttggaggtttctgtggggctcatcccaggcaaagttagtctgcagaattaaggaggattacaagtgggaatttgaagagcttttgaaatcctgtggtgagctgtttgattctttgaatctgggtcaccaggcgcttttccaagagaaggtcatcaagactttggatttttccacaccggggcgcgctgcggctgctgttgcttttttgagttttataaaggataaatggagcgaagaaacccatctgagcggggggtacctgctggattttctggccatgcatctgtggagagcggttgtgagacacaagaatcgcctgctactgttgtcttccgtccgcccggcgataataccgacggaggagcagcagcagcagcaggaggaagccaggcggcggcggcaggagcagagcccatggaacccgagagccggcctggaccctcgggaatgaatgttgtacaggtggctgaactgtatccagaactgagacgcattttgacaattacagaggatgggcaggggctaaagggggtaaagagggagcggggggcttgtgaggctacagaggaggctaggaatctagcttttagcttaatgaccagacaccgtcctgagtgtattacttttcaacagatcaaggataattgcgctaatgagcttgatctgctggcgcagaagtattccatagagcagctgaccacttactggctgcagccaggggatgattttgaggaggctattagggtatatgcaaaggtggcacttaggccagattgcaagtacaagatcagcaaacttgtaaatatcaggaattgttgctacatttctgggaacggggccgaggtggagatagatacggaggatagggtggcctttagatgtagcatgataaatatgtggccgggggtgcttggcatggacggggtggttattatgaatgtaaggtttactggccccaattttagcggtacggttttcctggccaataccaaccttatcctacacggtgtaagcttctatgggtttaacaatacctgtgtggaagcctggaccgatgtaagggttcggggctgtgccttttactgctgctggaagggggtggtgtgtcgccccaaaagcagggcttcaattaagaaatgcctctttgaaaggtgtaccttgggtatcctgtctgagggtaactccagggtgcgccacaatgtggcctccgactgtggttgcttcatgctagtgaaaagcgtggctgtgattaagcataacatggtatgtggcaactgcgaggacagggcctctcagatgctgacctgctcggacggcaactgtcacctgctgaagaccattcacgtagccagccactctcgcaaggcctggccagtgtttgagcataacatactgacccgctgttccttgcatttgggtaacaggaggggggtgttcctaccttaccaatgcaatttgagtcacactaagatattgcttgagcccgagagcatgtccaaggtgaacctgaacggggtgtttgacatgaccatgaagatctggaaggtgctgaggtacgatgagacccgcaccaggtgcagaccctgcgagtgtggcggtaaacatattaggaaccagcctgtgatgctggatgtgaccgaggagctgaggcccgatcacttggtgctggcctgcacccgcgctgagtttggctctagcgatgaagatacagattgaggtactgaaatgtgtgggcgtggcttaagggtgggaaagaatatataaggtgggggtcttatgtagttttgtatctgttttgcagcagccgccgccgccatgagcaccaactcgtttgatggaagcattgtgagctcatatttgacaacgcgcatgcccccatgggccggggtgcgtcagaatgtgatgggctccagcattgatggtcgccccgtcctgcccgcaaactctactaccttgacctacgagaccgtgtctggaacgccgttggagactgcagcctccgccgccgcttcagccgctgcagccaccgcccgcgggattgtgactgactttgctttcctgagcccgcttgcaagcagtgcagcttcccgttcatccgcccgcgatgacaagttgacggctcttttggcacaattggattctttgacccgggaacttaatgtcgtttctcagcagctgttggatctgcgccagcaggtttctgccctgaaggcttcctcccctcccaatgcggtttaaaacataaataaaaaaccagactctgtttggatttggatcaagcaagtgtcttgctgtctttatttaggggttttgcgcgcgcggtaggcccgggaccagcggtctcggtcgttgagggtcctgtgtattttttccaggacgtggtaaaggtgactctggatgttcagatacatgggcataagcccgtctctggggtggaggtagcaccactgcagagcttcatgctgcggggtggtgttgtagatgatccagtcgtagcaggagcgctgggcgtggtgcctaaaaatgtctttcagtagcaagctgattgccaggggcaggcccttggtgtaagtgtttacaaagcggttaagctgggatgggtgcatacgtggggatatgagatgcatcttggactgtatttttaggttggctatgttcccagccatatccctccggggattcatgttgtgcagaaccaccagcacagtgtatccggtgcacttgggaaatttgtcatgtagcttagaaggaaatgcgtggaagaacttggagacgcccttgtgacctccaagattttccatgcattcgtccataatgatggcaatgggcccacgggcggcggcctgggcgaagatatttctgggatcactaacgtcatagttgtgttccaggatgagatcgtcataggccatttttacaaagcgcgggcggagggtgccagactgcggtataatggttccatccggcccaggggcgtagttaccctcacagatttgcatttcccacgctttgagttcagatggggggatcatgtctacctgcggggcgatgaagaaaacggtttccggggtaggggagatcagctgggaagaaagcaggttcctgagcagctgcgacttaccgcagccggtgggcccgtaaatcacacctattaccgggtgcaactggtagttaagagagctgcagctgccgtcatccctgagcaggggggccacttcgttaagcatgtccctgactcgcatgttttccctgaccaaatccgccagaaggcgctcgccgcccagcgatagcagttcttgcaaggaagcaaagtttttcaacggtttgagaccgtccgccgtaggcatgcttttgagcgtttgaccaagcagttccaggcggtcccacagctcggtcacctgctctacggcatctcgatccagcatatctcctcgtttcgcgggttggggcggctttcgctgtacggcagtagtcggtgctcgtccagacgggccagggtcatgtctttccacgggcgcagggtcctcgtcagcgtagtctgggtcacggtgaaggggtgcgctccgggctgcgcgctggccagggtgcgcttgaggctggtcctgctggtgctgaagcgctgccggtcttcgccctgcgcgtcggccaggtagcatttgaccatggtgtcatagtccagcccctccgcggcgtggcccttggcgcgcagcttgcccttggaggaggcgccgcacgaggggcagtgcagacttttgagggcgtagagcttgggcgcgagaaataccgattccggggagtaggcatccgcgccgcaggccccgcagacggtctcgcattccacgagccaggtgagctctggccgttcggggtcaaaaaccaggtttcccccatgctttttgatgcgtttcttacctctggtttccatgagccggtgtccacgctcggtgacgaaaaggctgtccgtgtccccgtatacagactnnngttttgagaggcctgtcctcgagcggtgttccgcggtcctcctcgtatagaaactcggaccactctgagacaaaggctcgcgtccaggccagcacgaaggaggctaagtgggaggggtagcggtcgttgtccactagggggtccactcgctccagggtgtgaagacacatgtcgccctcttcggcatcaaggaaggtgattggtttgtaggtgtaggccacgtgaccgggtgttcctgaaggggggctataaaagggggtgggggcgcgttcgtcctcactctcttccgcatcgctgtctgcgagggccagctgttggggtgagtactccctctgaaaagcgggcatgacttctgcgctaagattgtcagtttccaaaaacgaggaggatttgatattcacctggcccgcggtgatgcctttgagggtggccgcatccatctggtcagaaaagacaatctttttgttgtcaagcttggtggcaaacgacccgtagagggcgttggacagcaacttggcgatggagcgcagggtttggtttttgtcgcgatcggcgcgctccttggccgcgatgtttagctgcacgtattcgcgcgcaacgcaccgccattcgggaaagacggtggtgcgctcgtcgggcaccaggtgcacgcgccaaccgcggttgtgcagggtgacaaggtcaacgctggtggctacctctccgcgtaggcgctcgttggtccagcagaggcggccgcccttgcgcgagcagaatggcggtagggggtctagctgcgtctcgtccggggggtctgcgtccacggtaaagaccccgggcagcaggcgcgcgtcgaagtagtctatcttgcatccttgcaagtctagcgcctgctgccatgcgcgggcggcaagcgcgcgctcgtatgggttgagtgggggaccccatggcatggggtgggtgagcgcggaggcgtacatgccgcaaatgtcgtaaacgtagaggggctctctgagtattccaagatatgtagggtagcatcttccaccgcggatgctggcgcgcacgtaatcgtatagttcgtgcgagggagcgaggaggtcgggaccgaggttgctacgggcgggctgctctgctcggaagactatctgcctgaagatggcatgtgagttggatgatatggttggacgctggaagacgttgaagctggcgtctgtgagacctaccgcgtcacgcacgaaggaggcgtaggagtcgcgcagcttgttgaccagctcggcggtgacctgcacgtctagggcgcagtagtccagggtttccttgatgatgtcatacttatcctgtcccttttttttccacagctcgcggttgaggacaaactcttcgcggtctttccagtactcttggatcggaaacccgtcggcctccgaacggtaagagcctagcatgtagaactggttgacggcctggtaggcgcagcatcccttttctacgggtagcgcgtatgcctgcgcggccttccggagcgaggtgtgggtgagcgcaaaggtgtccctgaccatgactttgaggtactggtatttgaagtcagtgtcgtcgcatccgccctgctcccagagcaaaaagtccgtgcgctttttggaacgcggatttggcagggcgaaggtgacatcgttgaagagtatctttcccgcgcgaggcataaagttgcgtgtgatgcggaagggtcccggcacctcggaacggttgttaattacctgggcggcgagcacgatctcgtcaaagccgttgatgttgtggcccacaatgtaaagttccaagaagcgcgggatgcccttgatggaaggcaattttttaagttcctcgtaggtgagctcttcaggggagctgagcccgtgctctgaaagggcccagtctgcaagatgagggttggaagcgacgaatgagctccacaggtcacgggccattagcatttgcaggtggtcgcgaaaggtcctaaactggcgacctatggccattttttctggggtgatgcagtagaaggtaagcgggtcttgttcccagcggtcccatccaaggttcgcggctaggtctcgcgcggcagtcactagaggctcatctccgccgaacttcatgaccagcatgaagggcacgagctgcttcccaaaggcccccatccaagtataggtctctacatcgtaggtgacaaagagacgctcggtgcgaggatgcgagccgatcgggaagaactggatctcccgccaccaattggaggagtggctattgatgtggtgaaagtagaagtccctgcgacgggccgaacactcgtgctggcttttgtaaaaacgtgcgcagtactggcagcggtgcacgggctgtacatcctgcacgaggttgacctgacgaccgcgcacaaggaagcagagtgggaatttgagcccctcgcctggcgggtttggctggtggtcttctacttcggctgcttgtccttgaccgtctggctgctcgaggggagttacggtggatcggaccaccacgccgcgcgagcccaaagtccagatgtccgcgcgcggcggtcggagcttgatgacaacatcgcgcagatgggagctgtccatggtctggagctcccgcggcgtcaggtcaggcgggagctcctgcaggtttacctcgcatagacgggtcagggcgcgggctagatccaggtgatacctaatttccaggggctggttggtggcggcgtcgatggcttgcaagaggccgcatccccgcggcgcgactacggtaccgcgcggcgggcggtgggccgcgggggtgtccttggatgatgcatctaaaagcggtgacgcgggcgagcccccggaggtagggggggctccggacccgccgggagagggggcaggggcacgtcggcgccgcgcgcgggcaggagctggtgctgcgcgcgtaggttgctggcgaacgcgacgacgcggcggttgatctcctgaatctggcgcctctgcgtgaagacgacgggcccggtgagcttgagcctgaaagagagttcgacagaatcaatttcggtgtcgttgacggcggcctggcgcaaaatctcctgcacgtctcctgagttgtcttgataggcgatctcggccatgaactgctcgatctcttcctcctggagatctccgcgtccggctcgctccacggtggcggcgaggtcgttggaaatgcgggccatgagctgcgagaaggcgttgaggcctccctcgttccagacgcggctgtagaccacgcccccttcggcatcgcgggcgcgcatgaccacctgcgcgagattgagctccacgtgccgggcgaagacggcgtagtttcgcaggcgctgaaagaggtagttgagggtggtggcggtgtgttctgccacgaagaagtacataacccagcgtcgcaacgtggattcgttgatatcccccaaggcctcaaggcgctccatggcctcgtagaagtccacggcgaagttgaaaaactgggagttgcgcgccgacacggttaactcctcctccagaagacggatgagctcggcgacagtgtcgcgcacctcgcgctcaaaggctacaggggcctcttcttcttcttcaatctcctcttccataagggcctccccttcttcttcttctggcggcggtgggggaggggggacacggcggcgacgacggcgcaccgggaggcggtcgacaaagcgctcgatcatctccccgcggcgacggcgcatggtctcggtgacggcgcggccgttctcgcgggggcgcagttggaagacgccgcccgtcatgtcccggttatgggttggcggggggctgccatgcggcagggatacggcgctaacgatgcatctcaacaattgttgtgtaggtactccgccgccgagggacctgagcgagtccgcatcgaccggatcggaaaacctctcgagaaaggcgtctaaccagtcacagtcgcaaggtaggctgagcaccgtggcgggcggcagcgggcggcggtcggggttgtttctggcggaggtgctgctgatgatgtaattaaagtaggcggtcttgagacggcggatggtcgacagaagcaccatgtccttgggtccggcctgctgaatgcgcaggcggtcggccatgccccaggcttcgttttgacatcggcgcaggtctttgtagtagtcttgcatgagcctttctaccggcacttcttcttctccttcctcttgtcctgcatctcttgcatctatcgctgcggcggcggcggagtttggccgtaggtggcgccctcttcctcccatgcgtgtgaccccgaagcccctcatcggctgaagcagggctaggtcggcgacaacgcgctcggctaatatggcctgctgcacctgcgtgagggtagactggaagtcatccatgtccacaaagcggtggtatgcgcccgtgttgatggtgtaagtgcagttggccataacggaccagttaacggtctggtgacccggctgcgagagctcggtgtacctgagacgcgagtaagccctcgagtcaaatacgtagtcgttgcaagtccgcaccaggtactggtatcccaccaaaaagtgcggcggcggctggcggtagaggggccagcgtagggtggccggggctccgggggcgagatcttccaacataaggcgatgatatccgtagatgtacctggacatccaggtgatgccggcggcggtggtggaggcgcgcggaaagtcgcggacgcggttccagatgttgcgcagcggcaaaaagtgctccatggtcgggacgctctggccggtcaggcgcgcgcaatcgttgacgctctaccgtgcaaaaggagagcctgtaagcgggcactcttccgtggtctggtggataaattcgcaagggtatcatggcggacgaccggggttcgagccccgtatccggccgtccgccgtgatccatgcggttaccgcccgcgtgtcgaacccaggtgtgcgacgtcagacaacgggggagtgctccttttggcttccttccaggcgcggcggctgctgcgctagcttttttggccactggccgcgcgcagcgtaagcggttaggctggaaagcgaaagcattaagtggctcgctccctgtagccggagggttattttccaagggttgagtcgcgggacccccggttcgagtctcggaccggccggactgcggcgaacgggggtttgcctccccgtcatgcaagaccccgcttgcaaattcctccggaaacagggacgagccccttttttgcttttcccagatgcatccggtgctgcggcagatgcgcccccctcctcagcagcggcaagagcaagagcagcggcagacatgcagggcaccctcccctcctcctaccgcgtcaggaggggcgacatccgcggttgacgcggcagcagatggtgattacgaacccccgcggcgccgggcccggcactacctggacttggaggagggcgagggcctggcgcggctaggagcgccctctcctgagcggtacccaagggtgcagctgaagcgtgatacgcgtgaggcgtacgtgccgcggcagaacctgtttcgcgaccgcgagggagaggagcccgaggagatgcgggatcgaaagttccacgcagggcgcgagctgcggcatggcctgaatcgcgagcggttgctgcgcgaggaggactttgagcccgacgcgcgaaccgggattagtcccgcgcgcgcacacgtggcggccgccgacctggtaaccgcatacgagcagacggtgaaccaggagattaactttcaaaaaagctttaacaaccacgtgcgtacgcttgtggcgcgcgaggaggtggctataggactgatgcatctgtgggactttgtaagcgcgctggagcaaaacccaaatagcaagccgctcatggcgcagctgttccttatagtgcagcacagcagggacaacgaggcattcagggatgcgctgctaaacatagtagagcccgagggccgctggctgctcgatttgataaacatcctgcagagcatagtggtgcaggagcgcagcttgagcctggctgacaaggtggccgccatcaactattccatgcttagcctgggcaagttttacgcccgcaagatataccataccccttacgttcccatagacaaggaggtaaagatcgaggggttctacatgcgcatggcgctgaaggtgcttaccttgagcgacgacctgggcgtttatcgcaacgagcgcatccacaaggccgtgagcgtgagccggcggcgcgagctcagcgaccgcgagctgatgcacagcctgcaaagggccctggctggcacgggcagcggcgatagagaggccgagtcctactttgacgcgggcgctgacctgcgctgggccccaagccgacgcgccctggaggcagctggggccggacctgggctggcggtggcacccgcgcgcgctggcaacgtcggcggcgtggaggaatatgacgaggacgatgagtacgagccagaggacggcgagtactaagcggtgatgtttctgatcagatgatgcaagacgcaacggacccggcggtgcgggcggcgctgcagagccagccgtccggccttaactccacggacgactggcgccaggtcatggaccgcatcatgtcgctgactgcgcgcaatcctgacgcgttccggcagcagccgcaggccaaccggctctccgcaattctggaagcggtggtcccggcgcgcgcaaaccccacgcacgagaaggtgctggcgatcgtaaacgcgctggccgaaaacagggccatccggcccgacgaggccggcctggtctacgacgcgctgcttcagcgcgtggctcgttacaacagcggcaacgtgcagaccaacctggaccggctggtgggggatgtgcgcgaggccgtggcgcagcgtgagcgcgcgcagcagcagggcaacctgggctccatggttgcactaaacgccttcctgagtacacagcccgccaacgtgccgcggggacaggaggactacaccaactttgtgagcgcactgcggctaatggtgactgagacaccgcaaagtgaggtgtaccagtctgggccagactattttttccagaccagtagacaaggcctgcagaccgtaaacctgagccaggctttcaaaaacttgcaggggctgtggggggtgcgggctcccacaggcgaccgcgcgaccgtgtctagcttgctgacgcccaactcgcgcctgttgctgctgctaatagcgcccttcacggacagtggcagcgtgtcccgggacacatacctaggtcacttgctgacactgtaccgcgaggccataggtcaggcgcatgtggacgagcatactttccaggagattacaagtgtcagccgcgcgctggggcaggaggacacgggcagcctggaggcaaccctaaactacctgctgaccaaccggcggcagaagatcccctcgttgcacagtttaaacagcgaggaggagcgcattttgcgctacgtgcagcagagcgtgagccttaacctgatgcgcgacggggtaacgcccagcgtggcgctggacatgaccgcgcgcaacatggaaccgggcatgtatgcctcaaaccggccgtttatcaaccgcctaatggactacttgcatcgcgcggccgccgtgaaccccgagtatttcaccaatgccatcttgaacccgcactggctaccgccccctggtttctacaccgggggattcgaggtgcccgagggtaacgatggattcctctgggacgacatagacgacagcgtgttttccccgcaaccgcagaccctgctagagttgcaacagcgcgagcaggcagaggcggcgctgcgaaaggaaagcttccgcaggccaagcagcttgtccgatctaggcgctgcggccccgcggtcagatgctagtagcccatttccaagcttgatagggtctcttaccagcactcgcaccacccgcccgcgcctgctgggcgaggaggagtacctaaacaactcgctgctgcagccgcagcgcgaaaaaaacctgcctccggcatttcccaacaacgggatagagagcctagtggacaagatgagtagatggaagacgtacgcgcaggagcacagggacgtgccaggcccgcgcccgcccacccgtcgtcaaaggcacgaccgtcagcggggtctggtgtgggaggacgatgactcggcagacgacagcagcgtcctggatttgggagggagtggcaacccgtttgcgcaccttcgccccaggctggggagaatgttttaaaaaaaaaaaagcatgatgcaaaataaaaaactcaccaaggccatggcaccgagcgttggttttcttgtattccccttagtatgcggcgcgcggcgatgtatgaggaaggtcctcctccctcctacgagagtgtggtgagcgcggcgccagtggcggcggcgctgggttctcccttcgatgctcccctggacccgccgtttgtgcctccgcggtacctgcggcctaccggggggagaaacagcatccgttactctgagttggcacccctattcgacaccacccgtgtgtacctggtggacaacaagtcaacggatgtggcatccctgaactaccagaacgaccacagcaactttctgaccacggtcattcaaaacaatgactacagcccgggggaggcaagcacacagaccatcaatcttgacgaccggtcgcactggggcggcgacctgaaaaccatcctgcataccaacatgccaaatgtgaacgagttcatgtttaccaataagtttaaggcgcgggtgatggtgtcgcgcttgcctactaaggacaatcaggtggagctgaaatacgagtgggtggagttcacgctgcccgagggcaactactccgagaccatgaccatagaccttatgaacaacgcgatcgtggagcactacttgaaagtgggcagacagaacggggttctggaaagcgacatcggggtaaagtttgacacccgcaacttcagactggggtttgaccccgtcactggtcttgtcatgcctggggtatatacaaacgaagccttccatccagacatcattttgctgccaggatgcggggtggacttcacccacagccgcctgagcaacttgttgggcatccgcaagcggcaacccttccaggagggctttaggatcacctacgatgatctggagggtggtaacattcccgcactgttggatgtggacgcctaccaggcgagcttgaaagatgacaccgaacagggcgggggtggcgcaggcggcagcaacagcagtggcagcggcgcggaagagaactccaacgcggcagccgcggcaatgcagccggtggaggacatgaacgatcatgccattcgcggcgacacctttgccacacgggctgaggagaagcgcgctgaggccgaagcagcggccgaagctgccgcccccgctgcgcaacccgaggtcgagaagcctcagaagaaaccggtgatcaaacccctgacagaggacagcaagaaacgcagttacaacctaataagcaatgacagcaccttcacccagtaccgcagctggtaccttgcatacaactacggcgaccctcagaccggaatccgctcatggaccctgctttgcactcctgacgtaacctgcggctcggagcaggtctactggtcgttgccagacatgatgcaagaccccgtgaccttccgctccacgcgccagatcagcaactttccggtggtgggcgccgagctgttgcccgtgcactccaagagcttctacaacgaccaggccgtctactcccaactcatccgccagtttacctctctgacccacgtgttcaatcgctttcccgagaaccagattttggcgcgcccgccagcccccaccatcaccaccgtcagtgaaaacgttcctgctctcacagatcacgggacgctaccgctgcgcaacagcatcggaggagtccagcgagtgaccattactgacgccagacgccgcacctgcccctacgtttacaaggccctgggcatagtctcgccgcgcgtcctatcgagccgcactttttgagcaagcatgtccatccttatatcgcccagcaataacacaggctggggcctgcgcttcccaagcaagatgtttggcggggccaagaagcgctccgaccaacacccagtgcgcgtgcgcgggcactaccgcgcgccctggggcgcgcacaaacgcggccgcactgggcgcaccaccgtcgatgacgccatcgacgcggtggtggaggaggcgcgcaactacacgcccacgccgccaccagtgtccacagtggacgcggccattcagaccgtggtgcgcggagcccggcgctatgctaaaatgaagagacggcggaggcgcgtagcacgtcgccaccgccgccgacccggcactgccgcccaacgcgcggcggcggccctgcttaaccgcgcacgtcgcaccggccgacgggcggccatgcgggccgctcgaaggctggccgcgggtattgtcactgtgccccccaggtccaggcgacgagcggccgccgcagcagccgcggccattagtgctatgactcagggtcgcaggggcaacgtgtattgggtgcgcgactcggttagcggcctgcgcgtgcccgtgcgcacccgccccccgcgcaactagattgcaagaaaaaactacttagactcgtactgttgtatgtatccagcggcggcggcgcgcaacgaagctatgtccaagcgcaaaatcaaagaagagatgctccaggtcatcgcgccggagatctatggccccccgaagaaggaagagcaggattacaagccccgaaagctaaagcgggtcaaaaagaaaaagaaagatgatgatgatgaacttgacgacgaggtggaactgctgcacgctaccgcgcccaggcgacgggtacagtggaaaggtcgacgcgtaaaacgtgttttgcgacccggcaccaccgtagtctttacgcccggtgagcgctccacccgcacctacaagcgcgtgtatgatgaggtgtacggcgacgaggacctgcttgagcaggccaacgagcgcctcggggagtttgcctacggaaagcggcataaggacatgctggcgttgccgctggacgagggcaacccaacacctagcctaaagcccgtaacactgcagcaggtgctgcccgcgcttgcaccgtccgaagaaaagcgcggcctaaagcgcgagtctggtgacttggcacccaccgtgcagctgatggtacccaagcgccagcgactggaagatgtcttggaaaaaatgaccgtggaacctgggctggagcccgaggtccgcgtgcggccaatcaagcaggtggcgccgggactgggcgtgcagaccgtggacgttcagatacccactaccagtagcaccagtattgccaccgccacagagggcatggagacacaaacgtccccggttgcctcagcggtggcggatgccgcggtgcaggcggtcgctgcggccgcgtccaagacctctacggaggtgcaaacggacccgtggatgtttcgcgtttcagccccccggcgcccgcgcggttcgaggaagtacggcgccgccagcgcgctactgcccgaatatgccctacatccttccattgcgcctacccccggctatcgtggctacacctaccgccccagaagacgagcaactacccgacgccgaaccaccactggaacccgccgccgccgtcgccgtcgccagcccgtgctggccccgatttccgtgcgcagggtggctcgcgaaggaggcaggaccctggtgctgccaacagcgcgctaccaccccagcatcgtttaaaagccggtctttgtggttcttgcagatatggccctcacctgccgcctccgtttcccggtgccgggattccgaggaagaatgcaccgtaggaggggcatggccggccacggcctgacgggcggcatgcgtcgtgcgcaccaccggcggcggcgcgcgtcgcaccgtcgcatgcgcggcggtatcctgcccctccttattccactgatcgccgcggcgattggcgccgtgcccggaattgcatccgtggccttgcaggcgcagagacactgattaaaaacaagttgcatgtggaaaaatcaaaataaaaagtctggactctcacgctcgcttggtcctgtaactattttgtagaatggaagacatcaactttgcgtctctggccccgcgacacggctcgcgcccgttcatgggaaactggcaagatatcggcaccagcaatatgagcggtggcgccttcagctggggctcgctgtggagcggcattaaaaatttcggttccaccgttaagaactatggcagcaaggcctggaacagcagcacaggccagatgctgagggataagttgaaagagcaaaatttccaacaaaaggtggtagatggcctggcctctggcattagcggggtggtggacctggccaaccaggcagtgcaaaataagattaacagtaagcttgatccccgccctcccgtagaggagcctccaccggccgtggagacagtgtctccagaggggcgtggcgaaaagcgtccgcgccccgacagggaagaaactctggtgacgcaaatagacgagcctccctcgtacgaggaggcactaaagcaaggcctgcccaccacccgtcccatcgcgcccatggctaccggagtgctgggccagcacacacccgtaacgctggacctgcctccccccgccgacacccagcagaaacctgtgctgccaggcccgaccgccgttgttgtaacccgtcctagccgcgcgtccctgcgccgcgccgccagcggtccgcgatcgttgcggcccgtagccagtggcaactggcaaagcacactgaacagcatcgtgggtctgggggtgcaatccctgaagcgccgacgatgcttctgaatagctaacgtgtcgtatgtgtgtcatgtatgcgtccatgtcgccgccagaggagctgctgagccgccgcgcgcccgctttccaagatggctaccccttcgatgatgccgcagtggtcttacatgcacatctcgggccaggacgcctcggagtacctgagccccgggctggtgcagtttgcccgcgccaccgagacgtacttcagcctgaataacaagtttagaaaccccacggtggcgcctacgcacgacgtgaccacagaccggtcccagcgtttgacgctgcggttcatccctgtggaccgtgaggatactgcgtactcgtacaaggcgcggttcaccctagctgtgggtgataaccgtgtgctggacatggcttccacgtactttgacatccgcggcgtgctggacaggggccctacttttaagccctactctggcactgcctacaacgccctggctcccaagggtgccccaaatccttgcgaatgggatgaagctgctactgctcttgaaataaacctagaagaagaggacgatgacaacgaagacgaagtagacgagcaagctgagcagcaaaaaactcacgtatttgggcaggcgccttattctggtataaatattacaaaggagggtattcaaataggtgtcgaaggtcaaacacctaaatatgccgataaaacatttcaacctgaacctcaaataggagaatctcagtggtacgaaactgaaattaatcatgcagctgggagagtccttaaaaagactaccccaatgaaaccatgttacggttcatatgcaaaacccacaaatgaaaatggagggcaaggcattcttgtaaagcaacaaaatggaaagctagaaagtcaagtggaaatgcaatttttctcaactactgaggcgaccgcaggcaatggtgataacttgactcctaaagtggtattgtacagtgaagatgtagatatagaaaccccagacactcatatttcttacatgcccactattaaggaaggtaactcacgagaactaatgggccaacaatctatgcccaacaggcctaattacattgcttttagggacaattttattggtctaatgtattacaacagcacgggtaatatgggtgttctggcgggccaagcatcgcagttgaatgctgttgtagatttgcaagacagaaacacagagctttcataccagcttttgcttgattccattggtgatagaaccaggtacttttctatgtggaatcaggctgttgacagctatgatccagatgttagaattattgaaaatcatggaactgaagatgaacttccaaattactgctttccactgggaggtgtgattaatacagagactcttaccaaggtaaaacctaaaacaggtcaggaaaatggatgggaaaaagatgctacagaattttcagataaaaatgaaataagagttggaaataattttgccatggaaatcaatctaaatgccaacctgtggagaaatttcctgtactccaacatagcgctgtatttgcccgacaagctaaagtacagtccttccaacgtaaaaatttctgataacccaaacacctacgactacatgaacaagcgagtggtggctcccgggttagtggactgctacattaaccttggagcacgctggtcccttgactatatggacaacgtcaacccatttaaccaccaccgcaatgctggcctgcgctaccgctcaatgttgctgggcaatggtcgctatgtgcccttccacatccaggtgcctcagaagttctttgccattaaaaacctccttctcctgccgggctcatacacctacgagtggaacttcaggaaggatgttaacatggttctgcagagctccctaggaaatgacctaagggttgacggagccagcattaagtttgatagcatttgcctttacgccaccttcttccccatggcccacaacaccgcctccacgcttgaggccatgcttagaaacgacaccaacgaccagtcctttaacgactatctctccgccgccaacatgctctaccctatacccgccaacgctaccaacgtgcccatatccatcccctcccgcaactgggcggctttccgcggctgggccttcacgcgccttaagactaaggaaaccccatcactgggctcgggctacgacccttattacacctactctggctctataccctacctagatggaaccttttacctcaaccacacctttaagaaggtggccattacctttgactcttctgtcagctggcctggcaatgaccgcctgcttacccccaacgagtttgaaattaagcgctcagttgacggggagggttacaacgttgcccagtgtaacatgaccaaagactggttcctggtacaaatgctagctaactacaacattggctaccagggcttctatatcccagagagctacaaggaccgcatgtactccttctttagaaacttccagcccatgagccgtcaggtggtggatgatactaaatacaaggactaccaacaggtgggcatcctacaccaacacaacaactctggatttgttggctaccttgcccccaccatgcgcgaaggacaggcctaccctgctaacttcccctatccgcttataggcaagaccgcagttgacagcattacccagaaaaagtttctttgcgatcgcaccctttggcgcatcccattctccagtaactttatgtccatgggcgcactcacagacctgggccaaaaccttctctacgccaactccgcccacgcgctagacatgacttttgaggtggatcccatggacgagcccacccttctttatgttttgtttgaagtctttgacgtggtccgtgtgcaccggccgcaccgcggcgtcatcgaaaccgtgtacctgcgcacgcccttctcggccggcaacgccacaacataaagaagcaagcaacatcaacaacagctgccgccatgggctccagtgagcaggaactgaaagccattgtcaaagatcttggttgtgggccatattttttgggcacctatgacaagcgctttccaggctttgtttctccacacaagctcgcctgcgccatagtcaatacggccggtcgcgagactgggggcgtacactggatggcctttgcctggaacccgcactcaaaaacatgctacctctttgagccctttggcttttctgaccagcgactcaagcaggtttaccagtttgagtacgagtcactcctgcgccgtagcgccattgcttcttcccccgaccgctgtataacgctggaaaagtccacccaaagcgtacaggggcccaactcggccgcctgtggactattctgctgcatgtttctccacgcctttgccaactggccccaaactcccatggatcacaaccccaccatgaaccttattaccggggtacccaactccatgctcaacagtccccaggtacagcccaccctgcgtcgcaaccaggaacagctctacagcttcctggagcgccactcgccctacttccgcagccacagtgcgcagattaggagcgccacttctttttgtcacttgaaaaacatgtaaaaataatgtactagagacactttcaataaaggcaaatgcttttatttgtacactctcgggtgattatttacccccacccttgccgtctgcgccgtttaaaaatcaaaggggttctgccgcgcatcgctatgcgccactggcagggacacgttgcgatactggtgtttagtgctccacttaaactcaggcacaaccatccgcggcagctcggtgaagttttcactccacaggctgcgcaccatcaccaacgcgtttagcaggtcgggcgccgatatcttgaagtcgcagttggggcctccgccctgcgcgcgcgagttgcgatacacagggttgcagcactggaacactatcagcgccgggtggtgcacgctggccagcacgctcttgtcggagatcagatccgcgtccaggtcctccgcgttgctcagggcgaacggagtcaactttggtagctgccttcccaaaaagggcgcgtgcccaggctttgagttgcactcgcaccgtagtggcatcaaaaggtgaccgtgcccggtctgggcgttaggatacagcgcctgcataaaagccttgatctgcttaaaagccacctgagcctttgcgccttcagagaagaacatgccgcaagacttgccggaaaactgattggccggacaggccgcgtcgtgcacgcagcaccttgcgtcggtgttggagatctgcaccacatttcggccccaccggttcttcacgatcttggccttgctagactgctccttcagcgcgcgctgcccgttttcgctcgtcacatccatttcaatcacgtgctccttatttatcataatgcttccgtgtagacacttaagctcgccttcgatctcagcgcagcggtgcagccacaacgcgcagcccgtgggctcgtgatgcttgtaggtcacctctgcaaacgactgcaggtacgcctgcaggaatcgccccatcatcgtcacaaaggtcttgttgctggtgaaggtcagctgcaacccgcggtgctcctcgttcagccaggtcttgcatacggccgccagagcttccacttggtcaggcagtagtttgaagttcgcctttagatcgttatccacgtggtacttgtccatcagcgcgcgcgcagcctccatgcccttctcccacgcagacacgatcggcacactcagcgggttcatcaccgtaatttcactttccgcttcgctgggctcttcctcttcctcttgcgtccgcataccacgcgccactgggtcgtcttcattcagccgccgcactgtgcgcttacctcctttgccatgcttgattagcaccggtgggttgctgaaacccaccatttgtagcgccacatcttctctttcttcctcgctgtccacgattacctctggtgatggcgggcgctcgggcttgggagaagggcgcttctttttcttcttgggcgcaatggccaaatccgccgccgaggtcgatggccgcgggctgggtgtgcgcggcaccagcgcgtcttgtgatgagtcttcctcgtcctcggactcgatacgccgcctcatccgcttttttgggggcgcccggggaggcggcggcgacggggacggggacgacacgtcctccatggttgggggacgtcgcgccgcaccgcgtccgcgctcgggggtggtttcgcgctgctcctcttcccgactggccatttccttctcctataggcagaaaaagatcatggagtcagtcgagaagaaggacagcctaaccgccccctctgagttcgccaccaccgcctccaccgatgccgccaacgcgcctaccaccttccccgtcgaggcacccccgcttgaggaggaggaagtgattatcgagcaggacccaggttttgtaagcgaagacgacgaggaccgctcagtaccaacagaggataaaaagcaagaccaggacaacgcagaggcaaacgaggaacaagtcgggcggggggacgaaaggcatggcgactacctagatgtgggagacgacgtgctgttgaagcatctgcagcgccagtgcgccattatctgcgacgcgttgcaagagcgcagcgatgtgcccctcgccatagcggatgtcagccttgcctacgaacgccacctattctcaccgcgcgtaccccccaaacgccaagaaaacggcacatgcgagcccaacccgcgcctcaacttctaccccgtatttgccgtgccagaggtgcttgccacctatcacatctttttccaaaactgcaagatacccctatcctgccgtgccaaccgcagccgagcggacaagcagctggccttgcggcagggcgctgtcatacctgatatcgcctcgctcaacgaagtgccaaaaatctttgagggtcttggacgcgacgagaagcgcgcggcaaacgctctgcaacaggaaaacagcgaaaatgaaagtcactctggagtgttggtggaactcgagggtgacaacgcgcgcctagccgtactaaaacgcagcatcgaggtcacccactttgcctacccggcacttaacctaccccccaaggtcatgagcacagtcatgagtgagctgatcgtgcgccgtgcgcagcccctggagagggatgcaaatttgcaagaacaaacagaggagggcctacccgcagttggcgacgagcagctagcgcgctggcttcaaacgcgcgagcctgccgacttggaggagcgacgcaaactaatgatggccgcagtgctcgttaccgtggagcttgagtgcatgcagcggttctttgctgacccggagatgcagcgcaagctagaggaaacattgcactacacctttcgacagggctacgtacgccaggcctgcaagatctccaacgtggagctctgcaacctggtctcctaccttggaattttgcacgaaaaccgccttgggcaaaacgtgcttcattccacgctcaagggcgaggcgcgccgcgactacgtccgcgactgcgtttacttatttctatgctacacctggcagacggccatgggcgtttggcagcagtgcttggaggagtgcaacctcaaggagctgcagaaactgctaaagcaaaacttgaaggacctatggacggccttcaacgagcgctccgtggccgcgcacctggcggacatcattttccccgaacgcctgcttaaaaccctgcaacagggtctgccagacttcaccagtcaaagcatgttgcagaactttaggaactttatcctagagcgctcaggaatcttgcccgccacctgctgtgcacttcctagcgactttgtgcccattaagtaccgcgaatgccctccgccgctttggggccactgctaccttctgcagctagccaactaccttgcctaccactctgacataatggaagacgtgagcggtgacggtctactggagtgtcactgtcgctgcaacctatgcaccccgcaccgctccctggtttgcaattcgcagctgcttaacgaaagtcaaattatcggtacctttgagctgcagggtccctcgcctgacgaaaagtccgcggctccggggttgaaactcactccggggctgtggacgtcggcttaccttcgcaaatttgtacctgaggactaccacgcccacgagattaggttctacgaagaccaatcccgcccgccaaatgcggagcttaccgcctgcgtcattacccagggccacattcttggccaattgcaagccatcaacaaagcccgccaagagtttctgctacgaaagggacggggggtttacttggacccccagtccggcgaggagctcaacccaatccccccgccgccgcagccctatcagcagcagccgcgggcccttgcttcccaggatggcacccaaaaagaagctgcagctgccgccgccacccacggacgaggaggaatactgggacagtcaggcagaggaggttttggacgaggaggaggaggacatgatggaagactgggagagcctagacgaggaagcttccgaggtcgaagaggtgtcagacgaaacaccgtcaccctcggtcgcattcccctcgccggcgccccagaaatcggcaaccggttccagcatggctacaacctccgctcctcaggcgccgccggcactgcccgttcgccgacccaaccgtagatgggacaccactggaaccagggccggtaagtccaagcagccgccgccgttagcccaagagcaacaacagcgccaaggctaccgctcatggcgcgggcacaagaacgccatagttgcttgcttgcaagactgtgggggcaacatctccttcgcccgccgctttcttctctaccatcacggcgtggccttcccccgtaacatcctgcattactaccgtcatctctacagcccatactgcaccggcggcagcggcagcggcagcaacagcagcggccacacagaagcaaaggcgaccggatagcaagactctgacaaagcccaagaaatccacagcggcggcagcagcaggaggaggagcgctgcgtctggcgcccaacgaacccgtatcgacccgcgagcttagaaacaggatttttcccactctgtatgctatatttcaacagagcaggggccaagaacaagagctgaaaataaaaaacaggtctctgcgatccctcacccgcagctgcctgtatcacaaaagcgaagatcagcttcggcgcacgctggaagacgcggaggctctcttcagtaaatactgcgcgctgactcttaaggactagtttcgcgccctttctcaaatttaagcgcgaaaactacgtcatctccagcggccacacccggcgccagcacctgtcgtcagcgccattatgagcaaggaaattcccacgccctacatgtggagttaccagccacaaatgggacttgcggctggagctgcccaagactactcaacccgaataaactacatgagcgcgggaccccacatgatatcccgggtcaacggaatccgcgcccaccgaaaccgaattctcttggaacaggcggctattaccaccacacctcgtaataaccttaatccccgtagttggcccgctgccctggtgtaccaggaaagtcccgctcccaccactgtggtacttcccagagacgcccaggccgaagttcagatgactaactcaggggcgcagcttgcgggcggctttcgtcacagggtgcggtcgcccgggcagggtataactcacctgacaatcagagggcgaggtattcagctcaacgacgagtcggtgagctcctcgcttggtctccgtccggacgggacatttcagatcggcggcgccggccgctcttcattcacgcctcgtcaggcaatcctaactctgcagacctcgtcctctgagccgcgctctggaggcattggaactctgcaatttattgaggagtttgtgccatcggtctactttaaccccttctcgggacctcccggccactatccggatcaatttattcctaactttgacgcggtaaaggactcggcggatggctacgactgaatgttaagtggagaggcagagcaactgcgcctgaaacacctggtccactgtcgccgccacaagtgctttgcccgcgactccggtgagttttgctactttgaattgcccgaggatcatatcgagggcccggcgcacggcgtccggcttaccgcccagggagagcttgcccgtagcctgattcgggagtttacccagcgccccctgctagttgagcgggacaggggaccctgtgttctcactgtgatttgcaactgtcctaaccctggattacatcaagatctttgttgccatctctgtgctgagtataataaatacagaaattaaaatatactggggctcctatcgccatcctgtaaacgccaccgtcttcacccgcccaagcaaaccaaggcgaaccttacctggtacttttaacatctctccctctgtgatttacaacagtttcaacccagacggagtgagtctacgagagaacctctccgagctcagctactccatcagaaaaaacaccaccctccttacctgccgggaacgtacgacctagggataacagggtaataagcaattgactctatgtgggatatgctccagcgctacaaccttgaagtcaggcttcctggatgtcagcatctgactttggccagcacctgtcccgcggatttgttccagtccaactacagcgacccaccctaacagagatgaccaacacaaccaacgcggccgccgctaccggacttacatctaccacaaatacaccccaagtttctgcctttgtcaataactgggataacttgggcatgtggtggttctccatagcgcttatgtttgtatgccttattattatgtggctcatctgctgcctaaagcgcaaacgcgcccgaccacccatctatagtcccatcattgtgctacacccaaacaatgatggaatccatagattggacggactgaaacacatgttcttttctcttacagtatgattaaatgagacatgattcctcgagtttttatattactgacccttgttgcgcttttttgtgcgtgctccacattggctgcggtttctcacatcgaagtagactgcattccagccttcacagtctatttgctttacggatttgtcaccctcacgctcatctgcagcctcatcactgtggtcatcgcctttatccagtgcattgactgggtctgtgtgcgctttgcatatctcagacaccatccccagtacagggacaggactatagctgagcttcttagaattctttaattatgaaatttactgtgacttttctgctgattatttgcaccctatctgcgttttgttccccgacctccaagcctcaaagacatatatcatgcagattcactcgtatatggaatattccaagttgctacaatgaaaaaagcgatctttccgaagcctggttatatgcaatcatctctgttatggtgttctgcagtaccatcttagccctagctatatatccctaccttgacattggctggaaacgaatagatgccatgaaccacccaactttccccgcgcccgctatgcttccactgcaacaagttgttgccggcggctttgtcccagccaatcagcctcgccccacttctcccacccccactgaaatcagctactttaatctaacaggaggagatgactgacaccctagatctagaaatggacggaattattacagagcagcgcctgctagaaagacgcagggcagcggccgagcaacagcgcatgaatcaagagctccaagacatggttaacttgcaccagtgcaaaaggggtatcttttgtctggtaaagcaggccaaagtcacctacgacagtaataccaccggacaccgccttagctacaagttgccaaccaagcgtcagaaattggtggtcatggtgggagaaaagcccattaccataactcagcactcggtagaaaccgaaggctgcattcactcaccttgtcaaggacctgaggatctctgcacccttattaagaccctgtgcggtctcaaagatcttattccctttaactaataaaaaaaaataataaagcatcacttacttaaaatcagttagcaaatttctgtccagtttattcagcagcacctccttgccctcctcccagctctggtattgcagcttcctcctggctgcaaactttctccacaatctaaatggaatgtcagtttcctcctgttcctgtccatccgcacccactatcttcatgttgttgcagatgaagcgcgcaagaccgtctgaagataccttcaaccccgtgtatccatatgacacggaaaccggtcctccaactgtgccttttcttactcctccctttgtatcccccaatgggtttcaagagagtccccctggggtactctctttgcgcctatccgaacctctagttacctccaatggcatgcttgcgctcaaaatgggcaacggcctctctctggacgaggccggcaaccttacctcccaaaatgtaaccactgtgagcccacctctcaaaaaaaccaagtcaaacataaacctggaaatatctgcacccctcacagttacctcagaagccctaactgtggctgccgccgcacctctaatggtcgcgggcaacacactcaccatgcaatcacaggccccgctaaccgtgcacgactccaaacttagcattgccacccaaggacccctcacagtgtcagaaggaaagctagccctgcaaacatcaggccccctcaccaccaccgatagcagtacccttactatcactgcctcaccccctctaactactgccactggtagcttgggcattgacttgaaagagcccatttatacacaaaatggaaaactaggactaaagtacggggctcctttgcatgtaacagacgacctaaacactttgaccgtagcaactggtccaggtgtgactattaataatacttccttgcaaactaaagttactggagccttgggttttgattcacaaggcaatatgcaacttaatgtagcaggaggactaaggattgattctcaaaacagacgccttatacttgatgttagttatccgtttgatgctcaaaaccaactaaatctaagactaggacagggccctctttttataaactcagcccacaacttggatattaactacaacaaaggcctttacttgtttacagcttcaaacaattccaaaaagcttgaggttaacctaagcactgccaaggggttgatgtttgacgctacagccatagccattaatgcaggagatgggcttgaatttggttcacctaatgcaccaaacacaaatcccctcaaaacaaaaattggccatggcctagaatttgattcaaacaaggctatggttcctaaactaggaactggccttagttttgacagcacaggtgccattacagtaggaaacaaaaataatgataagctaaccctatggacaggtccaaaaccagaagccaactgcataattgaatacgggaaacaaaacccagatagcaaactaactttaatccttgtaaaaaatggaggaattgttaatggatatgtaacgctaatgggagcctcagactacgttaacaccttatttaaaaacaaaaatgtctccattaatgtagaactatactttgatgccactggtcatatattaccagactcatcttctcttaaaacagatctagaactaaaatacaagcaaaccgctgactttagtgcaagaggttttatgccaagtactacagcgtatccatttgtccttcctaatgcgggaacacataatgaaaattatatttttggtcaatgctactacaaagcaagcgatggtgccctttttccgttggaagttactgttatgcttaataaacgcctgccagatagtcgcacatcctatgttatgacttttttatggtccttgaatgctggtctagctccagaaactactcaggcaaccctcataacctccccatttaccttttcctatattagagaagatgactaataaactctaaagaatcgtttgtgttatgtttcaacgtgtttatttttcaattgcagaaaatttcaagtcatttttcattcagtagtatagccccaccaccacatagcttatacagatcaccgtaccttaatcaaactcacagaaccctagtattcaacctgccacctccctcccaacacacagagtacacagtcctttctccccggctggccttaaaaagcatcatatcatgggtaacagacatattcttaggtgttatattccacacggtttcctgtcgagccaaacgctcatcaagtgatattaataaactccccgggcagctcacttaagttcatgtcgctgtccagctgctgagccacaggctgctgtccaacttgcggttgcttaacgggcggcgaaggagaagtccacgcctacatggggggagagtcataatcgtgcatcaggatagggcggtggtgctgcagcagcgcgcgaataaactgctgccgccgccgctccgtcctgcaggaatacaacatggcagtggtctcctcagcgatgattcgcaccgcccgcagcataaggcgcttgtcctccgggcacagcagcgcaccctgatctcacttaaatcagcacagtaactgcagcacagcaccacaatattgttcaaaatcccacagtgcaaggcgctgtatccaaagctcatggcggggaccacagaacccacgtggccatcataccacaagcgcaggtagattaagtggcgacccctcataaacacgctggacataaacattacctcttttggcatgttgtaattcaccacctcccggtaccatataaacctctgattaaacatggcgccatccaccaccatcctaaaccagctggccaaaacctgccccgccgggntatacactgcagggaaccgggacttggacaatgacaagtgggagagcccaggactcgtaaccatggatcatcatgctcgtcatgatatcaatgttggcacaacacaggcacacgtgcatacacttcctcaggattacaagctcctcccgcgttagaaccatatcccagggaacaacccattcctgaatcagcgtaaatcccacactgcagggaagacctcgcacgtaactcacgttgtgcattgtcaaagtgttacattcgggcagcagcggatgatcctccagtatggtagcgcgggtttctgtctcaaaaggaggtagacgatccctactgtacggagtgcgccgagacaaccgagatcgtgttggtcgtagtgtcatgccaaatggaacgccggacgtagtcatatttcctgaagcaaaaccaggtgcgggcgtgacaaacagatctgcgtctccggtctcgccgcttagatcgctctgtgtagtagttgtagtatatccactctctcaaagcatccaggcgccccctggcttcgggttctatgtaaactccttcatgcgccgctgccctgataacatccaccaccgcagaataagccacacccagccaacctacacattcgttctgcgagtcacacacgggaggagcgggaagagctggaagaaccatgtttttttttttattccaaaagattatccaaaacctcaaaatgaagatctattaagtgaacgcgctcccctccggtggcgtggtcaaactctacagccaaagaacagataatggcatttgtaagatgttgcacaatggcttccaaaaggcaaacggccctcacgtccaagtggacgtaaaggctaaacccttcagggtgaatctcctctataaacattccagcaccttcaaccatgcccaaataattctcatctcgccaccttctcaatatatctctaagcaaatcccgaatatttaagtccgggccattgtaaaaaatttggctccagagcgccctccaccttcagcctcaagcagcgaatcatgattgcaaaaattcaggttcctcacagacctgtataagattcaaaagcggaacattaacaaaaataccgcgatcccgtaggtcccttcgcagggccagctgaacataatcgtgcaggtctgcacggaccagcgcggccacttccccgccaggaaccatgacaaaagaacccacactgattatgacacgcatactcggagctatgctaaccagcgtagccccgatgtaagcttgttgcatgggcggcgatataaaatgcaaggtgctgctcaaaaaatcaggcaaagcctcgcgcaaaaaagaaagcacatcgtagtcatgctcatgcagataaaggcaggtaagctccggaaccaccacagaaaaagacaccatttttctctcaaacatgtctgcgggtttctgcataaacacaaaataaaataacaaaaaaacatttaaacattagaagcctgtcttacaacaggaaaaacaacccttataagcataagacggactacggccatgccggcgtgaccgtaaaaaaactggtcaccgtgattaaaaagcaccaccgacagctcctcggtcagtccggagtcataatgtaagactcggtaaacacatcaggttgattcacatcggtcagtgttaaaaagcgaccgaaatagccngggggaatacaatacccgcaggcgtagagacaacattacagcccccataggaggtataacaaaattaataggagagaaaaacacataaacacctgaaaaaccctcctgcctaggcaaaatagcaccctcccgctccagaacaacatacagcgcttccacagcggcagccataacagtcagccttaccagtaaaaaagaaaacctattaaaaaaacaccactcgacacggcaccagctcaatcagtcacagtgtaaaaaagggccaagtgcagagcgagtatatataggactaaaaaatgacggtaacggttaaagtccacaaaaaacacccagaaaaccgcacgcgaacctacgcccagaaacgaaagccaaaaaacccacaacttcctcaaatcgtcacttccgttttcccacgttacgtcacttcccattttaagaaaactacaattcccaacacatacaagttactccgccctaaaacctacgtcacccgccccgttcccacgccccgcgccacgtcacaaactccaccccctcattatcatattggcttcaatccaaaataaggtatattattgatgatgttaattaacatgcatggatcctcgtctcgacgatgcccttgagagccttcaacccagtcagctccttccggtgggcgcggggcatgactatcgtcgccgcacttatgactgtcttctttatcatgcaactcgtaggacaggtgccggcagcgctctgggtcattttcggcgaggaccgctttcgctggagcgcgacgatgatcggcctgtcgcttgcggtattcggaatcttgcacgccctcgctcaagccttcgtcactggtcccgccaccaaacgtttcggcgagaagcaggccattatcgccggcatggcggccgacgcgctgggctacgtcttgctggcgttcgcgacgcgaggctggatggccttccccattatgattcttctcgcttccggcggcatcgggatgcccgcgttgcaggccatgctgtccaggcaggtagatgacgaccatcagggacagcttcaaggatcgctcgcggctcttaccagcctaacttcgatcactggaccgctgatcgtcacggcgatttatgccgcctcggcgagcacatggaacgggttggcatggattgtaggcgccgccctataccttgtctgcctccccgcgttgcgtcgcggtgcatggagccgggccacctcgacctgaatggaagccggcggcacctcgctaacggattcaccactccaagaattggagccaatcaattcttgcggagaactgtgaatgcgcaaaccaacccttggcagaacatatccatcgcgtccgccatctccagcagccgcacgcggcgcatctcgggcagcgttgggtcctggccacgggtgcgcatgatcgtgctcctgtcgttgaggacccggctaggctggcggggttgccttactggttagcagaatgaatcaccgatacgcgagcgaacgtgaagcgactgctgctgcaaaacgtctgcgacctgagcaacaacatgaatggtcttcggtttccgtgtttcgtaaagtctggaaacgcggaagtcagcgccctgcaccattatgttccggatctgcatcgcaggatgctgctggctaccctgtggaacacctacatctgtattaacgaagcgctggcattgaccctgagtgatttttctctggtcccgccgcatccataccgccagttgtttaccctcacaacgttccagtaaccgggcatgttcatcatcagtaacccgtatcgtgagcatcctctctcgtttcatcggtatcattacccccatgaacagaaattcccccttacacggaggcatcaagtgaccaaacaggaaaaaaccgcccttaacatggcccgctttatcagaagccagacattaacgcttctggagaaactcaacgagctggacgcggatgaacaggcagacatctgtgaatcgcttcacgaccacgctgatgagctttaccgcagctgcctcgcgcgtttcggtgatgacggtgaaaacctctgacacatgcagctcccggagacggtcacagcttgtctgtaagcggatgccgggagcagacaagcccgtcagggcgcgtcagcgggtgttggcgggtgtcggggcgcagccatgacccagtcacgtagcgatagcggagtgtatactggcttaactatgcggcatcagagcagattgtactgagagtgcaccatatgcggtgtgaaataccgcacagatgcgtaaggagaaaataccgcatcaggcgctcttccgcttcctcgctcactgactcgctgcgctcggtcgttcggctgcggcgagcggtatcagctcactcaaaggcggtaatacggttatccacagaatcaggggataacgcaggaaagaacatgtgagcaaaaggccagcaaaaggccaggaaccgtaaaaaggccgcgttgctggcgtttttccataggctccgcccccctgacgagcatcacaaaaatcgacgctcaagtcagaggtggcgaaacccgacaggactataaagataccaggcgtttccccctggaagctccctcgtgcgctctcctgttccgaccctgccgcttaccggatacctgtccgcctttctcccttcgggaagcgtggcgctttctcaatgctcacgctgtaggtatctcagttcggtgtaggtcgttcgctccaagctgggctgtgtgcacgaaccccccgttcagcccgaccgctgcgccttatccggtaactatcgtcttgagtccaacccggtaagacacgacttatcgccactggcagcagccactggtaacaggattagcagagcgaggtatgtaggcggtgctacagagttcttgaagtggtggcctaactacggctacactagaaggacagtatttggtatctgcgctctgctgaagccagttaccttcggaaaaagagttggtagctcttgatccggcaaacaaaccaccgctggtagcggtggtttttttgtttgcaagcagcagattacgcgcagaaaaaaaggatctcaagaagatcctttgatcttttctacggggtctgacgctcagtggaacgaaaactcacgttaagggattttggtcatgagattatcaaaaaggatcttcacctagatccttttaaattaaaaatgaagttttaaatcaatctaaagtatatatgagtaaacttggtctgacagttaccaatgcttaatcagtgaggcacctatctcagcgatctgtctatttcgttcatccatagttgcctgactccccgtcgtgtagataactacgatacgggagggcttaccatctggccccagtgctgcaatgataccgcgagacccacgctcaccggctccagatttatcagcaataaaccagccagccggaagggccgagcgcagaagtggtcctgcaactttatccgcctccatccagtctattaattgttgccgggaagctagagtaagtagttcgccagttaatagtttgcgcaacgttggttgnnnnnnaaaaaggatcttcacctagatccttttcacgtagaaagccagtccgcagaaacggtgctgaccccggatgaatgtcagctactgggctatctggacaagggaaaacgcaagcgcaaagagaaagcaggtagcttgcagtgggcttacatggcgatagctagactgggcggttttatggacagcaagcgaaccggaattgccagctggggcgccctctggtaaggttgggaagccctgcaaagtaaactggatggctttctcgccgccaaggatctgatggcgcaggggatcaagctctgatcaagagacaggatgaggatcgtttcgcatgattgaacaagatggattgcacgcaggttctccggccgcttgggtggagaggctattcggctatgactgggcacaacagacaatcggctgctctgatgccgccgtgttccggctgtcagcgcaggggcgcccggttctttttgtcaagaccgacctgtccggtgccctgaatgaactgcaagacgaggcagcgcggctatcgtggctggccacgacgggcgttccttgcgcagctgtgctcgacgttgtcactgaagcgggaagggactggctgctattgggcgaagtgccggggcaggatctcctgtcatctcaccttgctcctgccgagaaagtatccatcatggctgatgcaatgcggcggctgcatacgcttgatccggctacctgcccattcgaccaccaagcgaaacatcgcatcgagcgagcacgtactcggatggaagccggtcttgtcgatcaggatgatctggacgaagagcatcaggggctcgcgccagccgaactgttcgccaggctcaaggcgagcatgcccgacggcgaggatctcgtcgtgacccatggcgatgcctgcttgccgaatatcatggtggaaaatggccgcttttctggattcatcgactgtggccggctgggtgtggcggaccgctatcaggacatagcgttggctacccgtgatattgctgaagagcttggcggcgaatgggctgaccgcttcctcgtgctttacggtatcgccgctcccgattcgcagcgcatcgccttctatcgccttcttgacgagttcttctgaattttgttaaaatttttgttaaatcagctcattttttaaccaataggccgaaatcggcaacatcccttataaatcaaaagaatagaccgcgatagggttgagtgttgttccagtttggaacaagagtccactattaaagaacgtggactccaacgtcaaagggcgaaaaaccgtctatcagggcgatggcccactacgtgaaccatcacccaaatcaagttttttgcggtcgaggtgccgtaaagctctaaatcggaaccctaaagggagcccccgatttagagcttgacggggaaagccggcgaacgtggcgagaaaggaagggaagaaagcgaaaggagcgggcgctagggcgctggcaagtgtagcggtcacgctgcgcgtaaccaccacacccgcgcgcttaatgcgccgctacagggcgcgtccattcgccattcaggatcgaattaattcttaat

SEQ ID NO: 128 - DNA, 9 bp, Artificial Sequence
  STAT1 binding site (1)
ttccgggaa

SEQ ID NO: 129 - DNA, 9 bp, Artificial Sequence
  STAT1 binding site (2)
ttctcggaa

SEQ ID NO: 130 - protein, 580 aa, Homo sapiens CD44v6
MDKFWWHAAWGLCLVPLSLAQIDLNITCRFAGVFHVEKNGRYSISRTEAADLCKAFNSTLPTMAQMEKALSIGFETCRYGFIEGHVVIPRIHPNSICAANNTGVYILTSNTSQYDTYCFNASAPPEEDCTSVTDLPNAFDGPITITIVNRDGTRYVQKGEYRTNPEDIYPSNPTDDDVSSGSSSERSSTSGGYIFYTFSTVHPIPDEDSPWITDSTDRIPATIQATPSSTTEETATQKEQWFGNRWHEGYRQTPKEDSHSTTGTAAASAHTSHPMQGRTTPSPEDSSWTDFFNPISHPMGRGHQAGRRMDMDSSHSITLQPTANPNTGLVEDLDRTGPLSMTTQQSNSQSFSTSHEGLEEDKDHPTTSTLTSSNRNDVTGGRRDPNHSEGSTTLLEGYTSHYPHTKESRTFIPVTSAKTGSFGVTAVTVGDSNSNVNRSLSGDQDTFHPSGGSHTTHGSESDGHSHGSQEGGANTTSGPIRTPQIPEWLIILASLLALALILAVCIAVNSRRRCGQKKKLVINSGNGAVEDRKPSGLNGEASKSQEMVHLVNKESSETPDQFMTADETRNLQNVDMKIGV

SEQ ID NO: 131 - protein, 436 aa, Artificial Sequence
  HER2(FRP5)-CD28TM,ICD-CD3Z CAR
EVQLQQSGPELKKPGETVKISCKASGYPFTNYGMNWVKQAPGQGLKWMGWINTSTGESTFADDFKGRFDFSLETSANTAYLQINNLKSEDMATYFCARWEVYHGYVPYWGQGTTVTVSSGGGGSGGGGSGGGGSDIQLTQSHKFLSTSVGDRVSITCKASQDVYNAVAWYQQKPGQSPKLLIYSASSRYTGVPSRFTGSGSGPDFTFTISSVQAEDLAVYFCQQHFRTPFTFGSGTKLEIKEPKSCDKTHTCPTRFWVLVVVGGVLACYSLLVTVAFIIFWVRSKRSRLLHSDYMNMTPRRPGPTRKHYQPYAPPRDFAAYRSRVKFSRSADAPAYQQGQNQLYNELNLGRREEYDVLDKRRGRDPEMGGKPQRRKNPQEGLYNELQKDKMAEAYSEIGMKGERRRGKGHDGLYQGLSTATKDTYDALHMQALPPR